European Patent Specification EP 3 766 967 B1, published March 26, 2025. Title: NEW BACTERIOPHAGE AND THERAPEUTIC AGENT FOR BACTERIAL ENDOPHTHALMITIS. Applicant: NATIONAL UNIVERSITY CORPORATION KOCHI UNIVERSITY. The sequence listing filed with the application follows.

SEQUENCE LISTING (3 sequences)

SEQ ID NO: 1 - DNA, 143399 bp, Myoviridae Spounavirinae phiEF7H
gttgttccctcctctcccttagagctactattaatatagtacactgagctgttagcaaacaggtgtgctaaattaatatagagactaaaaatgtagacgggagagtggtaaaaatggataatagcaaacgaattattaaaaaaattatttttattaccatctctgcattagtcatggttactttaagtaagctgttctctaaatatgttattgtagaacaaaatgccccatttcaggcattagttggcggtgcctcatgtgcactgttatctagtattctgtttgactggtatactaataaaaagaaaaaagagaacgtagagaatcaacttaaagaagcaatcagtgacttgcagaagattaaagctatcataaaaagatagcctattaggaggtgggatgggtgtctattaccaataaagacattaaggataaacgtagatatatttttagtcaatctagtaaaacaacaactataaaaagaggggacaaacgcataagtagtgcaacaagaatatgtgcagtttgtggaagaccgctatctaagctcgtattaagaacaggcgtaccaacagtagtagtagaccatattagctgtaagatttcagacattgttagactaaatgtctgtgaggatataaggtcttgttatgcgtattctagtaagaaaggggaaagctagctaatgggtatggcagatagacttaaagataatgcaaaacaaaaaaagttagaaagaacaccagagcaacaactaagagacacatttaatcaagcttcaataaagcttatcaatcaatttatggctaacgttacatcaggtgctatagaagttgatgatattgcagatttaacaaggctatttcagatttatttacaggttaataatataaatgatggaatgcaagaaggtacaggaactctacctgcacttacatctgagcataaagacatcatatctgaaaaggttagcacagaaaagattattaaggacggtgaagaagaggagctaatttctcttgatgagttagccagtcttccagatgaccaacttgaggaagtcttagttaacagagagctacagatgaacagagagaacgaggcgaccttctaatgacgacaaaagcacaacatatagctaaaatggctaaagagatgtatggtacagataaaattacaacggagcagttagcttatataacagatatgctgaccccatcaacgtacctattgagaaatcactctgtgcgtaatcacccaataacttttattatatcaggaagggatgcaacaaaagcacaggcacatagaccataaaccaacaaagctgtggtctttaaactctactaaacgggcatagtaaaataatatacacgtaaacaatatactggtaagagagactaaatcctagtgtataaggacagggttgacctaccgtgctaaatcagttatactataactgtaaaagcctaacgactaaatttctaggtagctaactaaaaggagttagtgagaactagataaaaggcaaataaactatgcaagctcaataaaaataataatatacaggaggtgattaagatagctaaggacagaaaagaaattttcatagaaaagctcaaaagtgtaaaaggaactgactttgaacttataggtgagtttacaaagcaacgagaaaagactctatttcgtcataacgtgtgtgggcatgtttgggaaaccactccggttgtcctacttaactcaaaaaaaggcggagggtgccctcattgtcaatacagaaacaaagcaacttcaccaaaagaatacgaaaaaagagtaacagacacatttaaaggagaatacgttgtactcaatattaatgagtataaaaacaatagtactaaacttaaattcttgcattctaaatgtggtacagaattttatctgcgaccagcaagtttattcattaatgcaactagttgtcctaactgctctaaaaataaccgttgctcaactaagagaactactaatgagtttagagagttgcttcttaaaacaaaaggatactcctatgagctaacggaagatgcagagtacaccggagctaacaaaaaaattaaggttaggcatacaacttgtggttatgtttgggaggctagagctaaccacctgctacagggttcgggttgtcctagatgtaacgaatcaaaaggagagctattagtagctactattcttaagctaagcaacacctcttttttgagagagcacacctttgacgattgtagaagtactagacccttaccttttgactttgcattaattagtaataacaaagtgcgtggtttaattgaatatgatggagaacagcacacgaaaccagtaagttgtttcggaggggaacagaagtttaaaagtacagtaagaaatgataacactaagaatgattattgtactcataaaaaaatacccttactcagagtatcatacactaatagtcctgaacagattgagcacctagttcagcagtttttaaaaagcatagatttgttgtaacgtagagcaacctaaaccaaaaagtaggttgatgatatagtctagtcccctaataaatatcgggaaaccgagggtaaccaaatgggcaaccaaagataataaatgaccaacatagagacaaggcaataattaaatcaagacaattagggttaagattagcccctttataaagcaatttgtaaagaaaactctgttaaacgggcatagctgaataaccaataagctgataagagaacctaagtcctgaaaaggatagaggtaatcccgtgctaaatcagtgcaaagcactgtaaatgcctaacgactaaatttctaggtagctaaccaaatggggttagtgagaactagataagaaaacctcttaagaggaagtaaagcagagcaacctaaaccaaaaattaggttgatgatatagtctagtcccctaataaatatcgggaaaccgagggtataacgtaagtgagatgggtgttggttctatgctacagtttgcagacacgcatagttatgatgctgttaaatgtctttatacattcccaacgaatgagcaaatgactaaatttgtacagacaaggttagaccctgttttacagaatgggtactacagcacaattgtagaccaagaagttaactcattaaaagctaaaaaaataagaaatagttttttgtattttcgttcaagttcaaaaccgggcgctgtggaaggtgtcgatattgactatctatctatggacgagtatgaccgtgtacctgcattagcagaggcttctgcgttggaatccatgtcttcctcaccttataagatagttaacagatggagcactccatcagcacccgatatgggaatacatgggctctttaaagggtcagaccaacattggtatttacataaatgtgagaaatgtaattattacaacgaaatgagttatgatgcatataccccagaggctcctgtagagagtagaggtaacattctttgtgttaacccaaaaggggtcgatgttgttgctaaaacagtagttgacggctcattccagtttgtttgtcaaaagtgcggagaaccgttagacagatggtacaacggtgtatgggtacctaaatatcctgatagaacaaaaaatggtctaggtactagaggatatatgatttcccaaatgaacgcagtatgggtaactgccgaccagttaaagaccaaagaacttcaatcattgtctaaacaagccttttataactatactctgggtgaataacgccccttcaactggaaacagttgtcgaaaactctgttaaacgggcaaagctgaataaccaataagctgataagagaccctaaaccctaaaatagggcagtgggaatcccgtgctaaatcaagcgtaagcttgtaaatgcctaacgactaaatttctaggtagctaaccaaatggggttagtgagaactagataagaaaacctcttagggggaagtaaagcagagcaacctaaaccaaaaattaggttgatgatatagtctagtccgactgccaagagcagtaacaaaatactacgaaagtagcggtagctcgtatccttacgcagacttgaaattaactgttaacgactctgacgttgatagccataagagaaactatttaatagaacctgctaaagacagaggtgattataaatttatatctgttggtattgactggggtaacagacattgggtatctatacatggtgttaaaacaaatggtacggtagatttgataaaacttttttctgtaggtaagtccaacccgctagaccctaatgcaatagatgtagacatacagtctataaaattacagctagctccttacaatccagatataatcgtagctgacgtaggagactcaggggataaagttgctaaacttatgcaaatttatggaaaagaacgagtttttgggtgcgtttacccatcaacccctaaatctacaggtaacttagtacctacttggagcccacaagcaaataaagtatccgctgacaagttaatgcagaataaacgttacattaacaagatgaaagaaggagaaataggttactactcaaaaccagatacagagcttaatttatataaagagcactggaagaatgttgttatacgtgatattgaggacgaaaagacatcgacaggttttagacaaattatcggcagaaaaggtgatgaccactactcacaagcaagcgtttattccatgttagggtatgagtacctaatgaatgtatttacaggagtaaaagagtatggatttgactctgattgggtgtcaactcaattagcacctacgaaacctgatatatttacagaatttgtataggtagattgccttatttagttttagtcaagctgaataaggcattttgtattgtttgatatatatttttgtggtataataaatatagttagggggatagttatggtagacaacaatgtaaaaataagtaaaagtacaattgaaggactaataaataagtctttaagttatgagtacgttataaaaaataacgaattgctgacaaacgaatatcaacatattgtaaaagcgtatgggtttgacaatttttatgacatgtatctatatgcagatagctgtgattctaaagatatgtatttagtaaaaggtggtcaaaaagacttgtctaagctgaaacccgttaaaagaaaagttgttagaaatggtaaaactatgactacaactatttatgaagatacaggcagttcagacagtaataacagtaaccctttagacaaagagagtaaaaagaaaaaagagttagaaccagttaatgctaaggaactacgtaaggtcagcttaggtagtgatgaagaagagaagttagaccctaaaaagatagcaaaattgctagcagacactaaaaaatttggaaataattttgatacgcagtgtactgattatcttattcttgaacaagactctgttacacgaggagtggtagggtttactagagaaggttcttatttaaaaatgtctttctcaatgtcagatgaggctgttgaaggtatgaagatgttagctttttcacagctcacattaaaggcttggaaattgggtctaggggctaagataagcacagataatgcacctgatgtagaggaactaattagcttatatggatacaaaagaaataatacagagtatattgtgtcaatgagctcactgcgtagtcttctaggggagccttagtcataagtgctacgttagtcattatactagtattttcaactattatttttttaatttttaatttactagtaagtaaggtagttaaagaattttataacttaaagatgctagcaaaagagggactaacagataaagtaacagatataacaaatgatataatgcatatattgaaaggagaaataaataatatggaattaattatgaataataagaaactagatgaattaactaataaggtagccactgatgaggactacgatatttttgtagagaagatgggtaagctagttaaagatttgtatgagaactaccagtttttacaacaaaacccaccagaaggagactacacatcaggttattttttagggttccaagtaatcagagcagaatacccagttgagtatgagaatttatttagattagctgtagataaaaatttaaatgaactagagataaacaagagatttgtcgaagctgttaaggatggtaaagttttaccactaggtgaggctatcattgatgaattacaaacagggtgtagctctatactacaggcacaagaagtacgtgtaaatattgtatttggtacaaaagaatatatggctaagcaagaagaagagcgtaaagaacgtcaagctaagttagaagaagaacgagaaagagctatggaagtactaaaaacaaaagatgacgtgcttaacacattaagagtaactgaggctttggctaatgaattaacagatgaagtcgcagaaaaatatgatttaatggagctagttaacagtatgagagaggggctgaaagctcataatggaaattaaaaattctttggggaaagctcttataaaaaatttaagattgcttaaagaaaaaagagatgcaatgcccgataacttagaatatacaagtcaagttatgattcctgtgccctactatctaataaaaaaaggggataatgcagtagaatcattccttatgtgtgcggggatgataaatagggataaagatttaggtctgcctatttctttagagaaaggtaagcaacaagttaagcttaacaatggagaactgacaactattgtagaatgtgttgctacttactcagataaaactgatattgacggtgtagagagattcttagttgaacatctataaaaattaaattaacgagttctattttgtgctatattagatatgcatgaaatagaactcgtttctttttttatgactaactaaggaggtttaatagatggcaggagaagtatttagtagcttgattacaagcgtaaatcctaacccaatgaacgcaggtagccgtaatggtatctctattgaccgtattattctacatcataatgcaacaacaaataaagatgttgctatgaacacgtggctattaggtggtggtgcaggtacgtctgcgcactatgaagtcacaccaacagaaattatagggtgtgttggtgagcagtattcagcattccatgccggaggcacaggtggtatagatgtccctaagattgctaaccctaatcaacgctcaatcggtatcgaaaatgtaaactcgtcaggagcacctaactgggatgtagaccctagaacaattacaaattgtgcccgtttagtggcagatatttgtaaacgttatggtattccatgtgaccgacaacacgtgttaggacataacgaagtaactgcaacagcatgtcccggaggtatggatgtagacgaagttgtacgtcaagctcaacaatttatggtagggggctctaacaacgcagttaaaccagagccaagtaaacctacaccaagcaaaccaagtaacaataaaaataaagaaggagtggcaactatgtattgtttatacgaaagacctattaactcaaaaacaggagtgttagagtggaatggtgatgcatggacagttatgttttgtaatggagtaaattgtcgtagagtatcccacccagatgaaatgaaagtaattgaggatatttacagaaaaaacaacggaaaagacatcccgttctacagccaaaaagagtggaataaaaatgcaccatggtataacagattagagacagtatgtccagtaataggtattactaaaaaatcttaatactagatttaagaccatcttagggtggtcttttttctttctttgtaatattcgtaataatatgtaatggctatgtaaccgcttgttattttggctgtaacaattacatgttatattagttcttgtaagcaacacaaataaagaaaacattgaggagaattttattttgaagaaaactagtattttaggtttaagtttattaagtttaggtttagtagtaggtttaggaaccgaagctaaggcagaagaagtaacagagaatggtaagacatattggaaggtagagtcaggagacacactatcagaaattggagctaagtacaacttagatttcactaatatccacaaagttaataaaggtgttgtagctgaccctaatgttattttcgtaggtgacaaattgttattacctttagatgaaaatggcaagctagtggaacaagtgaataccactgaaccagatattgaagtacaatataacgaaccagtaacacctgaacaacctgtagttgtagaacaagaagttgtagagcaacctgtagttgtagcagaagcccctgcccctgtagtagaggtacctgctgacagtagctcagcaaaagagtggattgcacaacgtgaatctagtggttcttatgatgcaacaaatggtcagtatattggtcgttaccaactatctgcctcttatttaaatggtgactattcacctgccaaccaagaacgagtagctgatgagtatgtagcaggtcgctatggctcatgggagaacgcaaaatctttctggttagcaaatggttggtactaaaattaaatagcaataaagacctctttattaaggggtcttttttttatgctatattaatatatagtaaatagtaatataaaatggttatgattagttatgtggtataatagacttatgttaaaaccatttaaggaggggaaacatgggttatattcaagatgagacatggcagatggttaaaaaagttgctaaaaagaatgggtttgttggtgactggattttaattatccactcatactatgagtatggtggaaatcacgtccagatacatacaacaataaacggagaaagctatagaattttaagattgttagatagcagagagatacttttattagatagaaaaggtaaccctgtaatttatgactatgaaacagttaacgatggtcaaaaaagcttcttttataatgatatggaagagaaagaaatcgaaatacctaatggaagatgcttaaacgataagacaaggataaaaatttatgtataaggtaggtgtaacagttgccaaaatggttagataaagcactgggtatagaaaaatcgtccatagaagaaactaggaatatggaaaattataagatgcatttaagggaaatagacaccaatgtggtcaataacgagccgtacagtatggaaagtattgaaaaaggtatgaatggtaagaccactgcatatatgcaaccaattattggagagatgtcagtaaaccccgggtataaaactaaaccgtctatacgtaactctcaggacttacataagacacttaaaaagtttggtaataacataatattaaatgctattattaatacacggtcaaaccaagtatcgatgtattgtaagcccgcaagaaattctgagacaggtgttggttacgagatacgtttaaaagatattgaagcagaacctacttcacatgacattgctaatattaagcgtattgaaagttttttagaaaacacagcacaatttagagaccctaatagagataattttacaactttttgtaaaaaacttgttcgggcaacatacatgtatgaccaagtaaactttgaaaaggtatttgataaagatggtaactttatcaaatttgatactgtagacccaactacaattttcttagcaacaaatggtgaagggaaactaattaaaaacggtgaaagatttgttcaggttgttgataacagaattgttgctaaatttaatgagagagaactagcattcgcagtacgtaacccaagagcagacatcgaagtaggtcagtatggttacccagagttagaaattgcgttgaagcagtttattgcccatgaaaatacagaggtatttaacgatagattcttctcacatggaggaactaccagaggtatcttacatgtaaaaacagggcaacagcagtctcaacaagcactagacattttccgtagagagtggagaagctcactagcagggataaatggctcatggcaaatacctgtagtttcagcagaagatgtcaaattcgtcaatatgacaccctctgccaatgatatgcaatttgaaaaatggcttaactacttaattaatgttatatctgctttgtatggaattgaccccgcagagataaacttccctaacaatggtggtgcaacaggctctaaaggaggctccctaaatgagggaaactcaaaagagaaaatgcaagcttctcagaataaagggctacaaccccttttaagatttatagaggacaccgttaacacatatattgttgcggaatttggagaaaaataccaattccaatttagagggggagacctaagtgctcaactagataagcttaaaataattgagcaagaaggtaaagtattcagaacagttaacgagataagacatgataaaggtttagaaccgattaaaggcggagacgttatactaaatggtgttcacatacaagctattgggcaagcgttacaagaagaacagctagaataccaaagaagccaagaccgcttaaacagactattagagctatctggtggagatgtagaacaaccagaaccagaagagcctaaagacagtcaaaatgatacagatgtttcatttcaggatgaacaacaaggtttaaacggtaagtctaagaaagttaatggtaaggtagacgacaatgttggcaaggacggtcagttaaaatcggaagaaaacaccaactcaactaagcatggtactgatggtataaaaaaagaataaaagataatggagggggctagctccccctcaactttgtttgtgttactagatagtacatgttctgctatattaaatacagtaaaacgtttaggtggtgaaaagcaaattgtcagaagttagagaaaaatatagtattttcgtaccactggatattgaaaattctatacagaagtctgaatctgtgaatgatggtgaatggtatgttcaaggatatgcaactaccccagatttagatttacaaggagatattattttaccacagggcattgatatttcttattttattgaaaatggttggataaactatgagcataaaaatgatgctgagtttattataggtgccccaactagcaattgttatgttgatgtggacaaagggttattcgtagaggctaagctattaaaggataacaagtacgcacagtctatgtggaagctagctaatacaatccagaaatcaggaatatctcgtcagttaggtttttctattgagggtgcagtagttagtagaaatgcacaagataacagaatcatagaaggtgttaaaatacataatgttgcattaacgacacatccggctaacccaagagctacatgggagacactagttaaatcttggactacaggatatggcacagcaccagatgcacaagtagatgcaggcgcacttagaagagagatgtttaaagaggacatttctaatttgacgtatgcagtaagaactattgcaggactatataataaaaaacctgcagagaaagagtttattttacgtgaagtggctaaggatatagaagtagacacttccgaaaatgaattatctaaatttatgttacaattaagtagagggatttccttgaaagaagcaacaaactttattgaaaaaagaaaggggtaagaaatagtggctaaaacattaaacgatattatagaagattttgatgcacagttaaatgaaaaagtaaaacctactacagatgaggaaattacaaagtctgtagaagaacctactgaaccagaaaaagttgaagaaggtgctgaggttgagccggaagaaaagcctaatgaatctgaggagactacaggcaatgacggagaagaatccggagttactgaaacagttgaagcagaacaggaagaaccagaaactgttgaagaagtagcagttgaggaacctgttgaggaacctgttgaagaatcagcggaaactgttgaaaaatctgataaaactaaagaaaataaagatgaagaagaggaggaagacgaagacaaaaagaaagaaaaagacaaaaaagacaaagataaagaagacaaagaagacatcgagaagtctaccgaagtcgaacaagttatcaaatcttctgaaatcttaggagctatggaagctatctttaaaaatatgttaggtctaagtgaaaagttagacgaaattcatagagagtttaaagaagctaaagaagctaaagaaaaagacgaagcggagtctgttgagaaatctttacttgataaccctgaaattaaaacaggaaaagaggactcagaaggcaaggctgttgggtttgttaataagtctgtagcagttgaggaagaggtggctaccgaagaaccaactgtagaagtagttgttgatggtgaacaagacacagcagaacctgaaaaagaagtaccgttccgtgatagagtacaggctattagaccagactttatggaaacatataaacgtgtgtctgttagcggagtagctcaacgtggtgaattagaatcagttagacacacttggggaactgctagaacaaatgatgacctagctaaaattgaagggtttattaataaatataaataaatttactatatagtgaacgatttttaattgtactgctatattaatagcagaaacaataaaagacctgacattccctcctgaacctccacagggtcaggtcttatattgagaggaatataaagaaaggtgatttatacataatgacagagaaaaagaatacagaacgacaattaacttccgtacaggaagaagtaattaaaggcttcactacaggatatggtattacaccagaatctcaaactgatgccgccgctttaagacgagagtttttagacgaccaaatcacaatgctaacttgggcagacggagacttatcattttaccgtgacatcactaaacgtccggcaacttcaactgtagctaaatatgacgtatatctagcacatggacgtgtaggtcatactcgttttactcgtgaaatcggtgtagcaccaatttcagaccctaacttacgtcaaaaaacagttaacatgaaatacgtttctgatactaaaaatatgagtatcgcaacaggtttagttaacaacattgaagacccaatgcgtatcttgacagacgatgctatctcagttgttgctaaaacaattgaatgggcttctttctacggtgactctgacttatcagaaaacccagatgcaggttcaggtttagagttcgatggtttagctaaactaattgacaaacacaatgtactagatgctaaaggtgctagcttaacagaggctttacttaaccaagcatcagtattagttggtaaaggttatggtacaccaacagatgcttatatgcctatcggtgttcaagcagacttcgttaaccaacaattagaccgccaagttcaagtaattagcgacaacggtcaaaacgctacaatgggattcaacgttaaaggttttaactctgcacgtggtttcattcgtttacatggttcaactgtaatggaattagaacaaattttagatgaaaatagaatgcaacttcctaatgctcctcaaaaagcaactgttaaagctactttagaagcaggaacaaaaggtaaattccgtgatgaagatttaacaatcgacacagaatacaaagttgtagtagtatctgacgatgcagaatctgcaccatctgatgttgcatctgtagtaattgacgacaagaaaaaacaagttaaattagaaatcactattaataacatgtatcaagctcgtccacaatatgttgcaatttaccgtaaaggtttggaaacaggattgttctaccaaatcgctagagtacctgcaagtaaagcagttgaaggagttatcacatttatcgatgtgaacgatgaaattcctgaaacagcggacgtattcgttggagaattaactccatcagtagttcacttgttcgagttactaccaatgatgcgcttaccattagcacaagttaatgcttctgtgacattcgcagtattatggtatggagctttagcattacgtgcacctaagaaatgggctcgcattaagaacgttaaatatatcgcaacaggtaacgtgtttaactaacgctaatctttaaaagactaagcaaaattgaataaaaatggaataggggacggttaatactgttccctatttttattataaaatacatgtatggaggaaataatatgttaaaatcagaaatcttaataaataaaacagtaacaacagcttttggtgaggcaacatttgaccataatggggaaaccacagacctaacagtagaacagcaagaacatttagggactaaagttccatatatacaatatataccagatgcacctaaagctaaagaaaaagaagctactgcagaaaaagcagacgaggcacctaaaaaggctaagaaagcgcctgctaagaaaactacaaaatctaaaaaagaggaagactaaggaggtatttatatgtacccagactacggatacgaggaacaaggggacaatacataccaataccaaccatatgcacatgggaaccctaagcatatagatttagacaaaattgatgatatacagcctgctgattatggttggacacctgctacgctgaaacaatacatgtttggtgtagaagttgttaaccctgaaacaggggagcctttaggagatactttctatgaacatatcatagattcagcaatagctaaagcagagaaacgactagatattgctattatgcctagacttataagaggagaacaccatgattaccaccaatcagatttcaactcttacatgtatactcatgtgtttaaaagacctattattcaagcagaaaagcttcaattagaagttaatggtagagggctatacagatacccgtctaattggtggaaagtgtatgcactagcaggtcatatacaaatgtacccaacatccctcatgcagactggaacacagtttggttatgaaatgacgttctcagggtacccacaattagcaggaatgcctccatcaggaggacaagttgatgctcctcaaatgattcatattgactatgtggcaggaatgctacctaggaaaaatagaggatacaatgaagactgggagtgccctgcggacttagaacagcttgtaataaaatatgcgttaaaagagatattccaacaatggggtagacttataattggtgcaggtattgctagtaagtcactaacagtagatggtattagtgaaagtatacaaacaacacagtctgctatgtatggtggagcttctgcagatattcgacaaattgacgaagacatacaagaattagaaaaatcattggtatcttactttggaatgaacttaggtattatttaaaaaagggggttaacaaatgggtgaaaaaccaattagatttggtggagcaggtgaaacaggtaaccctaacaagcaattaaatactagtagggttgaatttgaaacaaaaggtatggctagcttcattgaaaatagaggtattgacgttttgtgggaaagagcatggctatgtacatgccgtaacccaatgaccctctcacctaagtcggattgccccatctgtaggggaagagggattgcttaccaacctgcagtaaaattaagaatggctatacagagtcaagagaaaggtatctctaatcaagatttaggactactagacacaggaaccgctattggaacgactgagctagattctaagataacctttagggacagaataacagtccccgaagttaaaatatatcaaagctttatttttaatgtaaataaaagaagagtagctaatggactatttttaagctatgatgtgaacagtatagaagatatttatggtaaagacggacgtatcttagttgatggagtcgattttagaatggactatgacacaaatactatttatccaaatgaatctttaatagatactaatatatccataaatatgtctgttacacttagatatattgttatagacctgttaaaagaaagtagataccagtataccacattcggtgttaaacaaacacaatttgaatcactacctaaaaagctcttattgaagcgtgaggacgtgtttattgatagtgaaccattttcattagacatagatacagcaagccgtatggaagagctagagggcaaaaaagatacaagtgaagctatggtagaccctaagcgtaaagctacaaaatcaggaggcttctttggaggtaagttaaatggctagaaaaggacagagacccgtattatttactgattcaaaagcaatacttggcaatctgactcgtgcagtggttgatgaagtactaagtgatgcgcaagatgttgctctacgtaatgggtcttctgtacagagaatgcctagctatttgatagtaacagagtctaggatggcaaaaaatggggttatagatttgaaacctttctttgcacgttctaataaaaagaaatataataaaaaaggggaatggtacctatacatccctattagtatgaaaacacgcaacatgtcaagacgattatacgatgagctgagagcagttccagtaggcacaaaacctgtaactgttaaaatggactatctgtatgatagacggaagcagagcccatcagtgtctagtattaactataaacctaaatctactaatgtaactgttataccacagagttggggtaaaggtacacgtaacacctatgtagctttccgtacagttaacgctaattctcctgcgaatagttggataataaatcgtagaaacgttaatgatgatgatatgagtaagacaatgctaagaaacatagacaggctcatgaagtggaaactaaagaatttaggaggatagtgtatgataccaagtttagacacttacttgtataaagaatttgaagaaaggctaaggataattctatcagagtgctatattatagacgaagctttaaagggaatggacaaagaagctttagaatcttttaaaaacacttattgctctatagatggtaagccacctaagagagaagtagagatgtcctattcattcccacaagaacatctggattcatttgctcgatttgtagtaactctcggtagtagcgaagaagatagcaagtctattggaggaatccaaggaggctacgagtatcgagaaggtaatgtaattagtgaggaagccactattattagagaaggtgacaagctgattataaatacatcaaaaccagtagcggactatctaaacagctcagacataagttttgcagaaagcgaccattttaggattgaagataataaacctgtatttgatttttcatacaatgaggagttagaaggtatatccattaatgtgtcgtatataagcaaaatatcagatgatgatgttgcaggtgtatacaaaggataccaatctaacgataatgttagtataattggaataagttctaatatagatactgctaggtgtttagatgcaattgctagaattatactaatcaccatgagagacagtttagatgaaaaaacagggtatatgttgcaaacactacattttggtgatatgcaagttgtcatagaatcaggtgaaacacttgtgtttggtagaccttgtactgtaaactacagagttactaattctattggatttgatttacaacaaagaatcacagagattattacaaaaaggaggatgaaatcctagtggctaaagaaacagagaaagtagtaaaaaaagaagttaaaaaggagcaacctaaaaaacctaaaggttatgtccatgtcgatacatttttagattatgcaaaagtattatatggactaaataaatatcaggtagcgggtttcagagcactaatggcaggtagagaataccaacacgaggatgctgattttgttccatttttagaaaagtatataggaaaggaagttaaataataaatggctgtagaacaattcccaagaaaaaaagtatcacgtccacatactgagattaccgtagacacaagcggtattggtgggtcatcaagtagctctgacaaaacattaatgttagttggctctgctaaaggcggtaaaccagatactgtttatcgtttccgtaattatcaacaagctaaacaagtactacgtagtggagatttgctagatgctatcgagttagcatggaatgcatctgacgttaataccgcatcagcaggagacattttagcagttcgtgttgaagatgctaaaaacgcaactcttacaaaaggtggtttaacatttgcttcaacaatttatggggtagatgcaaatgaaattcaagtagcattagaagacaacaatttaacacacacaaaaagattaactgttgcattttctaaagatggttataagaaagttttcgataacttaggtaaaattttctctatccaatataaaggtagtgaagctcaagccaactttacaattgcacaagatagcattagtaagaaagcaacaacattaactttaaatgtaggttctgaaccagaaagtacgacagaagtaatgaaatatgagttaggtcaaggggtttactctgagacaaatgttttagttagtgcaatcaatagtttaccagattgggaggctaaattcttccctataggtgacaaaaacttacctactgatgctttagaggcagtaaccaaagtagatgttaagacagaggctgtattcgtaggagctttagcaggagatattgctaaacagctagaatacaatgactatgtaactgtagctgtagatgctacaaaacctgtagaagactttgaattaacaaacctaacaggtggttctgacggaactgctcctgagtcttgggctaataaattcccattactagctaatgaaggtggttactacttagtaccattaacagataaacaagcagttcactctgaggctttagcttttgttaaagaccgtacagacaatggtgacccaatgcgtattatcgttggtggaggcactaatgaaacagtagaggaaagcattactcgtgcaacaaacttacgtgaccctagagcttctttagtaggcttctctggaactcgtaaaatggatgacggacgtttgcttaaattaccgggttacatgatggcttcacaaattgcaggtattgcaagtggtttagaagttggtgaagcaatcactttcaaacacttcaacgtaacatctgtagaccgtgtatttgaaagtagccagttagacatgttaaacgaaagtggagtaatctctatcgagtttgtacgtaaccgtactttaactgcattccgtgtagtacaagacgtaactacttacaatgacaaatctgacccagttaaaaatgaaatgtctgttggtgaagcaaacgacttcttagtttcagaattgaaaattgaactagataacaacttcatcggaactaaagtgattgacacaagcgcaagcttaatcaaaaactttatccaatcattcttagataacaaaaaacgtgctcgtgaaatccaagattacacaccggaagaagtacaagttgtcttagaaggtgacgtggcatcaatcagtatgactgtaatgcctatccgtagcttgaataagattaccgttcagttagtatacaaacaacaaatcttaacagcatagagtgtaggggcagttgcccctcctcttacataatgaataaaatataggagtgatatatacatggctagtgttggaaatcaaacagtccacacaggtaacacagtttacctaatgattggtaataaaattatcggtcgtgcgcaatctgcatcaggtgagcgccaatacggtacacaaggtatctatgaaatcggtagtattatgccacaagaacacgtatacttgaaatatgaaggtacaattactttagaacgtatgcgtatgaaaaaagaagacttagcaagtttaggaattacagcgttaggtgaagacatcttacaacgtgacattattgacatcgtaatgatggataatttaactaaagaaatcgtagtagcttatcgtggttgctctgcaatttcttactcagagtcattcacagctaacgaagttacatcagaaagtacgcagtgagattataaatacaaaatttatatagctgtgctagttcgtaaagagctagtatcgagagttaattgctttgaatccctaaagctcaacgacccaaacagtaactggaaacggtaagctgagaggtgcgaaagcagaaaaaatagttgagatggtataaggttaaatcctaagtactgatacaatgggtctttagcagggacagccctaagtcaattgatacgggacaccttcaacgactatcctctgacggaggagtaaagccacaagccaatggtggaagaaaaattctctaccctaacaagggtacccatatagtctgagctaacatgaaagtgttagaggcaaacgcctacttggaagttgcgttccaaggtaacaaaactgttcacatacctaacttctgcaaaggttaaatagcagacgaactccacccagcttgactgggtggttcttttacggtacaatacttttattattgttagatatttaggagatacaacatgagaaaaaaatggacattacaagaaagaaatattcttataaaaaaatgggcggagactaacaacgtaaatctcttaccagaaacagcaacctttacaggaaataagagcactatatactacgtatggtcagatggggagcttcaaggcttaataggtaaaacgaactttgacagtataatatctggaagtaaacctacagttaacggtctgacagaagagagcaaaaatattagggctaaaaaacgctttttggaatatgggctcgaattactagaggagtatcaaggattcaatacaccacataaggtgagagtgttggatggagtatacgcagggtattatggaaaaacctcattagccacagtcaatcaaaaaagtaccagaggtaaaatagcgcagttaaacataactattcttacagaaagtgagaaaagacgatatttcagagaatatgcagagtctcggggatacacaattattaactaccctgaaaaattagctgttcgaggtaagtgtactttgttatctccccaaggtaatgagtgggagacagtctggtaccattttgcttatcaggagaactgcaattgtccgttagatgttaaacgtagtattggggagcgcatggttagaagtttgcttaaagagaatggtattaactttgaagaacagaaaaagatagttattgatggtagaacattattttttgatttttacttacctgatgacaatacctatattgaatataatgggaaacagcactatgaagacaccggaggttactataagggtaaacttcaagatttacaggaacgtgacaaactaaaggagcagtggtgtaatcaagcaggtgttaatcttgttgttatcccatacactgcaaatagcataaacgaagtagctaatgttttatccgagatagtaccaattaaaaagagactagtttcagttgtttattctgatagtatacctaatgaggatattattgattactataaaacacatacaggtaaggaaacttgtaggaaatatgatttaacacaacgtagactgagcttactttgtaacagagtcggctttaataaaaggaggtacctaaagtgaaatatccatatttagtagaattgtatgcaaaacatgtaattagagatgcagggtacatagaaaatgtaccaccagttatttatgaagacgttgtgaaacgtgttgaagaaataaaaagagaagaaaacttaacaatagattaactagtataagtttaaatagacctaattcagatataggtctattttttttgccactataaatacaaataactagatagtgtggtataataaagatagtgctatattaatttatgagtaaactaggaggaaataataatgacagaaaataatgaaaaggtatttacacctacaccaaatttatcacgtgagcaattaatagaaaagttgcaacgtggagaaaacttgacggatgaagaagtaaatattttgaaatattacaatgatgcagaagaacgtaaacagttagatagaattatcccgggtgttaatgatgtattttctaagcattacaacttaaaagaatatggtttagaatttgatattaaaataaaagcacctaatattatcgaaaatggtaaaattcaggcaagaagagaagcctatttagaaggcatgggaatggcagttagcaactttattttccaaagttaccaaatgttagcaactattcgagtatgtggagtagaggtaccaaaagtattagctgatgatgaaaaaatttataatttatatgtattaggagtaattgcaaaggactatggtgaatggctaaactcctttcgatactagagttaaagaactaggcggaataaaagcccttgttagaaatagctatagtagaaatctatgggcaataatgaaaaaatttaaggtactaccgagtgaccctgcgtggcaaaatctcacaagtgaccaagtagagtggattttatataacatggaaagagacatagaagaacaagaacgactagctaagggaatgcagttagaaagtgagttccaagactatgacgattcatggtatgataaaccacatgatgagttctctccaattcgtgaaggtgacgatgaggaagaaattgctcgtaaacttagtgaaatcacaagtgaggaagacatggctaaacttaaagctcgttgggaggcaagccaagaagttgatgctatccgtgcagaaggtggaacaacaattgaagaagatacgattaacgaacttattgctaacaatgttaaaaaagcaatggaagaggctagacgtattgagaaacatggtggaaacaaatggcaagagaaatcatcaattgagttagaagaggaacgtaagaacctagagtttaactcacagttgaaacaaggagatattcaggaggctatcgatttgtttaacaaagatgtcgagccaacatcattagatgacgaatttcaaatttaagggtagggtattccctgccctttacttgtaaaggaagtgtggaaatgagcaacaattatcgtttttatgttgaggcaatgactggggatgctgttgcaaaacttaatgaaatagacaagttaatggataaaattgattcaaagagtgcaaagggcacccagaattttttccatacaagtcagaaagacattgataaagctgttgaggaaatgcaaaagcttatcaaggcaaaaaaagaactagatagagcttttgataatcagaagataaatgcagaaagcatgggagacatgacagcatataaacgtgctgtatcggatgcagaagaactaactagaagatttaacaaggcacaaaaagaatttcaaaatcatgctagaatgcaagctaaccctaattacataaatgctagtacactaaggcaacaaaaggcatttcgtgatgagttaacagaacaagagagagcaataagaaatatctctagggcacaacaggaactaaacagagtgaactctagggttaaccatcgtgcaaaccaagcaagcgcaacaggaagaatgacttacaatcagtcagagagtatgaagcgtgaccttagacgtactggtgtatttgaaagcctaggttcagaaaataaaagcagacagcaagagctacgagaacgatataaacagagacaagaagagctagcagagactagaagtaatacaaatttagatagacaagttcgtaagaatagggaaactagtattcaggctgagataaaagaaattgagaaagaaattgaagctagaaaacgcctagcagactctattaaagagactgtagagaacttaaaatctaaggaagcttcactaaatgcatctgacataaaagtagatgctgatagaaagagtgctcgtggtgttctagctgagcgtgcaccttctatatcaatggctatgctaggaggtaccgccgccgccataggtggtttatacgcaaaaggagcaactgctaacgcaggtatgcgtgatgcatctatatctttaggacaacgtacaggtactagtgacttccgtgcattaagaaaaagtatgcaagaaatgggtattgagaaacagttaggctataaaggtgctgacatgttacaattccaagaagatgcattgagtaatattggttttacaagtaaagaggacttagcagggagtacaagagccttagcagagggctcaagagcagttccagtagacaatgagactttaagtgacttcatgaatagtcaaatgaagagcggggctattagtggtagagaccaaattaagaatattcaagaaggtttcttaggtgctatccaacgctcagggatggcaggtcgtgagaaagaacagctagaagctcttaaaacattaagtgagcaaagctttactggtcgtaacggaagtaatcaagagcttaaagaacaaatggcaatgttaacaatgctaaaccaaacaggtaagcgtgctgttcaaggtgagcaaggggcacagttaatgtcaagtttatctgcaggtattcaaggtagtgtatggaacaataaggcatctttacttttaggtaaagggacacaattccaagggctagcaggaatgtacgacttaaaagctatgcaagaacaaggagcaacaccagagaacttacagaaaattattggcagtgtccaacaatcagttcccggtgacgaaaagtctcagaagtatgctttcggtagtgctttacacgaactattcggtacagatgctaagaatgaccaaatagatgcaatttgggaggcttatgccaacggtggtttaagtcaggataacgtagacagaataatgaatgaaagccaatctacaggaaaaggcaaatacgataagaacatagaagactatgcaaactctaaagaaggaaccgctaaccgttcagaagctgttacagagaaacaagcttcacagattaatgatatgggggacatcttaagagaaactaactctaaattaggagcacttcctcctgcgttatatgcgttaggagcaggcttaggagctatggctgtttcactagccacatcaggctctattggtggtttatctagtttaatcaaaaaaggaactcgttctacttttagtacaggtggaggggtaactgcagggggcggatttttaaaatcagctaaagaagcattctctgcaggtaaaggctctggcggatggttccaaggtattaaaaatgtaggtagtgtagctaaggactccgcaatgggtgtcggagctaaggctgttgaaggagcaaaaggactaaaaggtgccggaatgggcagtaaggttcttggtggcttaggaaaagcaggtaaattcctaggcaaagttgcaacccctctagcgataggttcctctctactagatattgcaaccgcagatgataaaacaaaggcggtaggggagagtgttggagctattggtggaggtatcggaggagctaagttaggggcaatgattggtacatttattgcacccggtcttggtacaggtatcggaggagctattggtggaggtatcggcgccataggaggtactctagcaggttctaaactaggcggtaaatttgttgatggtgttcgtaaattcttcggaggagaagaagctcatgcggaagaagcagacttaactgcagggcaagatgttgcttctgggcaagagagtaaatcaggagtacaagaagccagagacacggctaacaaacgagtcctatctgagaaaacacgtgcagagaataacgcagaagagtccgccaatctctctatctattctaagttattagatagagcccaacgtatactaaaccaagcaaaaaatcaaaacggtatattcggtaactcaggtagctctaaagattcttctgacggaatgggttcagatgcttctagtaaagactttggaggagactgggagaaagccattagacaagcatctaagaaaatgggagtagatgtttctgacgatgaaatagatacaatacttagattgattcaggcggagtctagtggtgacgagagcgccgttcaacagataattgatgagaacaacttcaatggcaatggtggagctaaaggtttgctacagtatgtccaaagtacttttgatgcatacaaagtagacggtcatgacaacataatgagcgggtatgaccaattgctagctttctttaataatagtaattggaaaaatgacctaaattcttgggatagccgttatcaaaacggtagtacaggatggggtcctactggtaataaaactagagcgatgggtgggcacataactagcccagagtatgcgctactgggagaggtagcaggtcaagatgagtatgttataaatcctagtcagccaacagctccacgtttattagcagaagctactagaaaaacagcccaaaacttccgattaacaggtaatggttctggtcatgattggggagcttcaatttctaaaataaatgcaacaggaggagctcaatcaggttcagctcctacgatgacaaatacaaatgaggtatcagttaatgtcaccatacaaggtggaggaacaagtgatagtatagctagagaaattggtgataagtcagcaggaattatcagcaaaacactcgatgctaccttcacagatttcttcgcaaaagaatacaggagagtgtagaggcttaatgtctctacttttctctaaggaggtttataatgtcagtagagttaagatacccgagatttgatttaactttttttacagagacagacaactaccatatagtttatgatgcaaaagatgggcttactggacgtaataacaataacggtgaagcagagaaggtaagcaataattttatggcagagtctgtaattagtttaactacaaaaaatgctttagaggatgatagtgcagtcttctcattcgtattagcaggggacgtgtattgggatagagtactaaatgctaatgatgcagttattcttaaaatagacccagatacttcctccactaaaaaatcagataaccctgtactactagttggtttaatatctgaggttagactagagggtgactatggggaaaactctaagatgtacaggataacaggacagtctttcgcaaaggcgctaatgcagtttgacttaggtgttattcaggaagtaagtgtagttttgacagatttaggttggttgcctgacgatgcacaagaaggtataaaaatgtctggtagtagtgcaagtcaaatagcagaaagcttaatgaaaagatttttacaatatatgaaatttaattttaatggtcaaggtatagataagttcttagagtgggagctagatagttggacagaggcggagagactaatagatagtaccccttacataaactatgaaggttctttaaagcaacttatagatgatgtaaccgctaaaccgtttaacgaattatatttcgatgcaacaccagagggtaaatgcagaatgattatgcgtagaaccccatttgataaatctgattgggaaaaattacaaacctacacagtaacatctgcagaagtaatatctgaatctgtagcagttaacgatacagaagcttactctatatttaacatatctattaataacttgtatgggactgactctatgatgttaggttctaaaccacaagtattccctgatttagtttctaaatatggttataagaaactagaagtacctaataggtatttagaaggagcaattatagataagagtaacagtggagataaagctaacacaaaacccgaaagtgataatgatagtaaagagagcgatggctcaacagctaaacagatgtttgacagagagtacgctcttgtcttaaactatctaaaagggtatcctgttgatgtgctaagagttaaaaaaagtaatgtaagaacatcaataacacaggtagacagacgtataacagataacgaagcagataaaattatagaccactatattacaaatcaagcattaagtaaagaagacttttctaaatttacaggaataaccgaagaaaatatagaagagggtaacggtaaagtagaacctacatataccgcagttagggacttccttaatgggttagataaaaacctaggagtatctagcataaaagagaaattaatgaactacttcaatttgatacctaaccaagccacatctattgctagtgaatacaaagcacaaggtaacttaggtaaactaaaatatgaagaaataatggagaataacccaagtgatagctcaaccgtcactggttcagataaacgatttgtttctgagttcactaaaagactagcaaattggtactgtgaaaacgctaatttctacagtggggatattgtagttaaaggtgaccctaaatatagattaggtaaccgtttgtttgttcaagatgagcaaaatggtgagttgtgggaatactacatagaatcagtagaacactcgttctcctatacacaagggtatatcactactcttggggtcactagaggtttacaaaatggaggaaacgatagattcactcatttatggggtaaatctgaggacttctccggaggtatgctaggtgagaaaaccttgcaagcactactagacgaacaagcagaagcaaacagtaaaaatgatggaggctctgatagtggaggtagctcaggtaaagagtatacagcaggtgcaggaactcagctagcggtattcccattagacgtaattaatgtaactcagggagaaaatggtggatacagccacatgggagcacttgcaatagacttttcagatggtactcctcataaaccttactatgcaccatttgactgtgaatgtgtgtacactgactcttactcaggggttgcatggcaatctcaaaagcctgttaaatgtgtagatggtagcgttacttacgtaacactattatgtgtacacgacaacaactgggcaagcaacaaagtaggggataagaaagctaaaggggaagtgatagggcactcaggaactgcaggacaagcatcaggagaccatgcccacttcgaggtgtctaaaggtaaatggcaaggttggagcacaagcagtgcgggagtttactttataaaaaacccttctcatttatacgatgtattttctataaaaaataatgtaactggaaaaacaactaaaattatgaatggtggagggtacaattggcgtagtatagactgggacgataaatctggctcaggttctggaaagaaaaagacagttggtgctagagccatggctactccattcggattacgtatgatgcgtagcgctcctgtagaaccagaagaaccaaaagttgttaaacaagtagaaactaaaacagttgttgaaaagaaaccaaaagtagaagttaaaaagctcccaatactttatgggaataacattgccacagaagcaactaaatggggaagagctcactcgaaaacagagtccacattccaatctgccttcaattttggagctaatacagataaagacccatttgaggaagacattatagcaacagacagtgcaggatttgtttggtggtgtttctaccatgcgggcatatcactatctggtggagctagaatggttaccactcgttcactactctatgataaccaattacaaactatctctactagaggtcagaagtctttagagctatttgataagatgaaggtaggagatttagtttggtttaacagagctagtcatgtagggatatattgtggtgagggcaagatggtctcttgtaatggaaaaggtaacatggatgagtccccaaaaacaggtattgttattgtcgacatgtctaaaggttattggtggaacgcttttgacggaaatgtacgtagatataaataaccctattttttagggttattttttttgtataggtagtttttagttattgtgctataatagataatgaggacacatgatgagaggatgaataaattggtaaaacgcagatttcaagcaggtctaggctcagaaattaaaagagtatataaagaaggacaacaaattaacacgctactattagcacaagtaattcaagtaaactataaatataatacagtagacctactagctttacagcataaagaagtatttcaaaattcctatgcaaatgagggacgtttctctgcaagacttcctatggaatttggcggtagaaatatcgttggacagccttatgggcaggttaacccgatagcagtaggaacagtagtattagttggttttattaattccgataaagacatgcctattgtaattagtgtttataataataacgatgtaagcaagcaactttcaagaacacaattttcaaattcagaccctaaagatttagagttaattggggatatgcaccaaaaatttagtttatacccttcattgacatatgatagcgttgatggagaaggaggacgtgtcgttactttttctggtaaatcatttattgcttttgatacaaaagaagtagctaactcctctacaactgatgcaggttatggtactaaatatgaggacttagagacatcatactataataatggtgacctaatagagcctatgaaaggtagagcaccaaatgtactgtttaagcatcaaggggtacttgacgatgatggcaaaccagatttgcacgatttgctaattcatattaacccagatggtacttatagaacttctatgatgaacaaagaagaggattggcgcacactatttgaaatgacaccagatggcagagttaaattaagaaaacaagactctattaatattgatggtggcatagaaataagtgagctaggaatcaacaatgaggggttcgtttatttacgtaatggggatatggatttagaagtacgaaaagacggtatctattcacaagggaaactgtttacagccgatgtagacctatccgatgtatatgacaaactaaatgggttgtctatacagattaaggaaacaaatggtcaattagagattatagctaatggtgtagaagaacaaaatggaaaaatatcagaactttctacagaaataacaattgtagcaggtaaagttgaatcaaaagtaacaaagacagaagttcaggatatgattgacagttcttttgtagatatgtctgatgcgattaaaaaagcacaagaagatgctgacaaagcaaataaagtgattgcagatatgtctagtgataatagactgactccgagtgaaaaaatagatttattaaaagaatgggatattataaaaaatgaatatccaagctatctcgaacaagcagaaacctacgaggttgacagtaaagactacactgctaagtacaattcattagagctatttgttacccctatattggctgacatggagtcaactagctcggtagacggagcaacacttcgcaaaacgtttaattcttactatacagcaagaatagctttactaaactctattagtaaaaaactaaaagacggtatcacagaggctatgaaaaaagcatcccaagcatcactagatgcaacacaagcaatggcagatgcctcacaagctaagattgatgcagataatgctaacaaacttatatctgatatagcaagtgataacaagctaacaccttctgaaaaataccaacttaaaaaggaatgggatgtaattgttaaggaataccctacaacaattgcacaagcagagaagtacgcagtagacacagcagagtatacagctaaatataaagccctagagctgtttgtagagcctttgtttaaagacatggatgaaactagtatagtagacggagaacgccttagagcgacattctcggactattacgcaagtaagattgctttactaaaagaagtaacggactcagctaaaacagagctagatgcctatggtaataaaatatctgtaatggaaacaaacattactcaaacgtcagaagctattactttactagctactagagtacaaactgtagaagacggtgtacaatcaaataaggcacaaatcgaaatacaagctgaacaaattagtcaaaaagtaactgctagtgaggttaaaggaattgtagacgattctattaacaatctaacattaggtggaactaacttatttgttataaagacacagacagcaggtttgctaaacgagaatgatggaactgtaggtactgcagtagacaactcagtagtgtcagactacattaaagttaatcaaaaaacaccatatattgctacactttacggtaacactggcacaaacatgattataacagactggtacgataaaaatagaacatttatttctggggaagctgtggcagactctggggattttagtaaaaagtatgtgtcacctgagaatgcagtctatgctagggtaagttataagaaagcaaactctgtgaatatcaaattcgaggcaggtacaaaggctactgattacagcccttcatgggaagacataaaaggtgaccaaactgctttagaggaatacattaaaaaagtagaagaacaagccaagaaagctcaacaagatgctgaaaatgctaaaaatgatgctgaaaatgcaaataacgcaatagctgatatgtcaaatgacaatatgttagcaccgaatgagaaaaaacaaatactcttacaatgggaacagattaaaacagagtatccaataaacttagaccaagcaactaaatttggggtgtcttctcaacagtatacaacagcgtataacgcactagacgagtacttaaaaccaatactagctgacatgacaacaacttctgtagtagttggttctactttaagaaatacgtttaacaattactatgacaaaagaactactttactaaacagaatatctgacgtagcaaaaaatgtagcagacaaggcacaagaaactgcagatactatcaatgataatttacaaaatattggtgggtacaactatgtagggttctcttccggagacaatatgttgcctagactgatgattaaaaacgttggttactacacattaggttcgtcaaccacagagttcattgacagcatggtagctgtaaaaggtgatgcaacgacccaacctttcgattatactgtaggtacttctgataaagaaattgctggtggcggtttagctgattatcgtatgaaagaaataaaagaaggtcagtggctaacagcttctgcgaatgtgcaggtaataggtggtggctccgctaggttagctatctacactttagaaggggataactgggtaggttctaacagtacacctatacaagtaagtgatggtttgaaacgtgttgtggctcaaagaaaagtaacaggcttaacaaaaggtgtgttaatacgtattgagtcagccgacactaatgttaaagagtttcgatttggtaatgttcaactagaagtgggtatcatcccaactccttggaaaaagtctgatatagatattcaagaggacataaacaatgttgttcagaatatcaaaacatacactgcttgggctaacgatttacagggtcttgattttacaagagaaaaggttgaaggaaaaacttacatgtatgtaggtacctctatgaaagatagtgataactattcagattatacatggaggctaactgatgaacatatagaaggtcagattaatggtaaggaaggcgcatggatttactctccaacagcccctgctaacccatcgcaaggacttatatgggtagacttgtcaaaagtccccaaccaacctaagcgttgggtagattcagaaactgggtgggttgcattaacaccagaagaggttaaagatttgccttggggtgaagatggcacaagcttagccgactgggtgtcacaggcagagcaaagaatatcttctgatagcattataaatactgtactaggttctgaggatttcactagtgtgttcgatacaaaagctaacacttctgacctaggtaacttggctacctatgaagacttagactcaataaaagaggactataaccggctaatcaaagaaggcataaatggtattgattttactccttatgtgactaactccgaactacaacagcttaaagacagctttaacttctctgttcaacaagccggaggggttaacatgcttaaaaactctttaggattctctgggttagacttctggaatggtacagtagggaagaacttactacctaactctacttggaatttaggttttggtagatggggtggtacttcaatcactagttttgaaatattaccaccagaagatgacaagcctacgagtaacatattagcctcaatgccacttcgctcttctactaaagaaataggtaacagacctcacccattaaaagttaactcgggtgaaacgtacacagtaagcttcgactataaagaagaagcattatcttacaacaaggacagacctatccttgttgtaagaaactaccctgataagaacacagaccaatggatggagtactcaatagaaggttgggcagtaatggctaacggaagcactactgacttaactgtttggagacgttttacaaaaacatttacaataggtactagtggctacttagatattttaccgaaaaccataatagaatcgtgggaacacaggtctttttggagagagctaaaaatagagaaagggacacaagccactacttgggtacctaacaaggaagacggggcgtttactggtgatattgttgagactattcaaacagaagaattagccaacctcgggtttggttccggatttattagttctaaaagacctagctcttcattaacacaatctgtagaactacctgaaataggtgctaaccttgagtattcactatctttttatatgaaggtaactacagataaccctgtagctgactttaaatgcggtattcgggtttatgatggaggtactctaacttatacattaggcatagaagatgcaacacagccaataccactagggttccaacaatacaagcttgtgttcactcccacaagtacctctactaaaatagaaatgtttgtagaaaatgggcaagaggcatctgttattatatcaggtattatgtataatatcgggagtatacctcttaaatggcaaccatatccaagtgagatatacaatacgaatgttaagattgatattaatggggtaaccgttaaaaacaatcaaacagatgggtatacaatgattactccccaagagttttcaggatactctcgtattgatggtaacatagaacgtattttcactttaaatggacaggtaacagaagttaaaatgctaaaggctgaaaaacgtataactatggaaccagtatctgtattcgctatgaacacagtaacggatacaaaaagaattagaggttgggcatttgtgccatcatttgaataaataattcaactttttaaccgaaaacctcacttacaagttgttttcggttaatttgtgttatactatatagagaaggacacgaaaggacgatgagactatatggctttaaacggaacaaagtatacagcctttgcccgacatagattagttttagagtggcgcgcaaatcaaaacattgcagggaactactcaacaatcagcgtatggctatatctacaatctatggataaatgggggagacttgatgctcccgctattggtgatgccaaagttaccgtagaaggaactacacagacagaaaaagcttcctctatgttaaatgctttccaaaagaaactattactagctaaagagtggagagttaaccataataatgacggttctaaaagaataactattgggggtagctactttgtaaacgttacttttactgataatggtgtaccaacatattacggtacgataactatacctaacttttcagtagacctgaatagaatacctagaagaagttcattaaaccctgtccctacattaaatttaccggggaacttaccaataacaataaataggcagagctccacattcaaacataatctaactgcttgggtggctaacagagataaccccacattaagtaatgatgcccattggacgtacttgacaaatcttaataatgtagacactagtgggtcatttagttttacagtagcaaataacaaaactatttttactgcattaaacaataggactagttggcaaggcaaggttaaactatggactatagggttagatgatgtagttagtcaggagagaacatacaagattgtccccccaatgaatgcacaagcatcgggaggtaagataaccttaaatgtgggagagaaaatcaatgtatcactaagtaactatcggtctgatgcaaactttacttatgatggggtatttaacattagtgggctcaacatacccattgctacaaattcagcagggaacacaatgtcgtatacactaactcaaacagatgtagacaatatattgaagaaaataccaaatgcggattcctcgtggggtcaagtaactgtaacaagtaagtatagtggagtacaatacaggactccatggacaggacagagaatagatataactatacctaaaaacaagtatgtaccaagcattaatggtacccctacttatgaagatacaagtagtgtctctgtcgggcttacaggtgacaatcaggtagctcttcaaggtaagtctaatatcaaagtgactatccctgctaactttgcaacggctaatggttactctactttgaaaacaattgatgtgtctttaggcggtacatcaaaaacagtcaactattcaaatgcagaaacagttgtagagttaggggctcccgctaaccatacatcagacaccttaatagtcacagtaactgacagtcgtgggtttaagtctaactggacaaagcatgtagacatttacccctacgaaaacccaaatatgtactttacagtcacacgtagaaataactttgagacaactacagatattaatgttaatagtacatggtctcctatcactataggtggtgtaaacaaaaatgctgtccaatcagtaacctacgcaacaaaagtagcaggtgttggtacttatggagcagaaactgctttaaattttacagctaatggtagtatggtaacagtaaaaaatacaccaatagaattagataataccaatacatacgaagttaggttgagtgtaactgataagtttagtacgtttactagaacagctactgttaaaccgggtaaccctatcatgtttattgatgccgataatcgaagtctgtttttaggtaatgcctttgttgacaataacaataatgagctaagaggcttattagagatagaaagagataagtggcaggagaatggtttagtaggaatatccttaaacaacagtgatatatcagcagtcaatggcatatggttctcgacagatacatcaaataacggaggtgaagggctccactttattaaatcaggtaaatcaagaaattcattgacttgggatgactatgattacttttatatgagggacaatggattctatgttaacaatgactctaaccctatatttactgtgactgatggtggggatttaaggttccctaaactggataacttatgggatggggcggcttacatgcacaaagaccagataatagtaccacgtaaaaaactcagtgaatgtagaaatggttgggctttaacgttcagttcttacgataaaagtacaggtaagctgtccttatgggatataattacattctttattcacaagaccgcaccggattctcctttaagtggtacaggtcacaggttcttcttaccagatggtagggatgctacatctcaaaagacaaaatatatatacgtcaatgactatcagttaaggggtcacgaagaaaatgatgacaaaggcggaacagctagcacaaataacagaaataaggttcttatgagggtggatgaatggtaaatatgagaacaatatacgtagaagtaaatgatgaaggttatgtagaaggttggggcagtaacctgtcaggtaataataacattcatagtgtaacaatagaggataacgaccagtttttttataaaaactccttaaattttaagtattcaaatggctctctagtattcgatgaagataaggcactgcacagtgctaaactagccaaaaaagatgaaatgttaactgcatgtaactatgaaaaaaatctacctttgacttttaaactagacaacgaaaattactttgctcaaccgttaactgcggaagaacttaatgaaacaatattgcctctgttgtcaggtttaacagagactgttcctcttgaattagttaaagtaagtgacgatgtacaagtaacattacaagttggatacagtgtaattaaaaatttatatgattatacaaatctaataaatgaatacttaaataaaaagttagaagtagatgtgtttaagatgatagatgaggctactacttttgaagaagttgaggaagtatcatggaaaactacaactagtgatgagttacctaatcaacctaaaatagaagacctccctataaataacaaccaagaaatcgtagataagttaaaacaagagaataaagagctaaaacaaagagtagaatttaacgaactagctttaatggatgcaataaacatgttttctgaaatgaacaagtaagttattattaactaaaggaggtgatatttctatgtacccatacttatcaatgttatatgcatcttatgtaatcaaagaccctgagaactatcctttagagaaggttccggcactaattagagaagatgtggagaaaatcgtggaagagatggcaaaaaagaacgaaaaacaaggatagttaatttagtaattggagtaacaataggtttaatcatagggctactaatttaaactaatataaatgagggtagtttgtgctaccctcttttttatactatattgtactatattaaggaacgaaaggagcggttactatgggacaatcagatggtatgggcggtacattaaaacgtattgcgattcaagtaggtaacgacccgaataaaggttggtatcgatttcaagtaaacccaactcaatataaatataataagccacatcgtgttactatatttaaaactaaatcaaacattataacagaagactttggtaaagatatagaaactatccaattttctggtacaacaggattcagggtagatagcagaggtaaaaatggggcggacagactaaaagaattagaagaaataatagataattacgcaaaacagggcggtaatggtaataggtctagtgtagagatgaaattttataatttcacagacgataaatattttgttgttcatttagcaccagaagggctatccattgaacgttctgcagaacagccattattatttaattacaccttaagtttagtcgtgttaagagaggcaggacagccctctgagagagctcaagtaagccctcagataggtaatgtaagtcctagcattggacggacatacaatgcacaacaggacactagaacacctgctcaaatacttcatgatgaatataggagaagtgttatgctaaatacagcagtaaatcctgcagtaacatcgggagcctataactatggtgtaaatgagttaaaaaaaataatcggatatggagggtagctcatggaaaaagtagaacaatcagcagatttgctaagattttttagatatttaaatgtcgatattaacggtgaagttgtagccaatgttattgacgaccaaccaaactttatatcaaggttctacacccctcatacacgagttaataaaatatctagtacactattagatattgttcgagataatgatataggggaaacaaataaggctttgtctaaagactccttaacttataaatttttaaaaagtggacttaagctttcatctccacgtatttacgagctagcacaaattgtagtactagaatcttttgctcttatatatgctatcgaagaagaaccagagatgtttaaaatgattaacgaatcagatgtaaagcagactagagagaatgttaaatacttaattgattgtttaggaggagcaaaagattatacagacatagtgatggacttacaatctatggatgtcgctctaggatatattcaggagcaagttcctctaatacaaggaggtttaccagtaaatggcacgatataaaaaacatttaattgtatatggggatacaatgcaatccatagcacaaaaagaaacaggctctgtagataattgggtaaaaattgcggagtacaatgacttagtttacccttacatagtagatactatgcaagaaaaaatgagcaacttagaacatctagctacacttggggacaccctttttatacctgatgaaggtaacttattggacattaatacaagctcattaaaccaaagagatatggatttcttattaggcttagctttaggtaaagacttggatatgacaagtgatacagattactacgagaatcatggaacaagtgatgaagtgtttgcaataacacataatgggcatggggacttgaagatagctagtggggcagacaatattaagcaagccactatatcaagattgatgacagctaaggggtctcttatgttgcacccagagtatggtagtgacttgcacttaatgttcggtaaaacaacaattgaacaaatgaagataattagtatagaagtatgcgatacagtacttaaagatacacgagtagcagaatgcgttctagtgaaccattatattgaagaagaccgatatgttggtaactatagagcaaccttaaagtctactagagagcaatttgagtttgttgttcaaaacgataactcaggggctctaattattgtatagaaaggataaggtttaatgagactaaagaaaatttcagagatactaggtagactaattgatgtaactatgataaacacacatgagataaacgatttttcagttggttctactattcgttctatttatgaagctgtttctatggagttagaacagtactatattttaggtagagagaatattttatggggaattgaacaaggagtcctaaatgcttttgactttaggaaaagagaagcaaaaagagcgtatggtatggtaacactagagttccatacggttactcagacccctgtgtatgtgccaacaggaacaacattcgactctagcttgtctggtgcccctagcacgttaacattccaaacgatgcaagactacataattccagaaggtgttataacagcaaaggtagaagtttattgtacaactgtaggtacaaaagggaacatacctaaaggaagaatcaatcgggtaattaacaatatatcaaacttaaaaaccgtgtataatgagtttgattttttaacaggtactgatgaggaaagtatagaatccgttaaaaaaagatttcatgcatttgtggaatcacgtggtagagcaacgataaaagccttagattacggtacacgtcaagtagaggaagttgcaggagtttatatcaaagaagaagtaggctacgttagaatatatgcacatgacttaaacggtgatttaaaacaagaaacactagataaaataaaagtagctattgaggactacagacctgcaggcattaaactggatgtattccctgtaataaaatccaatgtacaagtgagtgcaactgttactataagtgacaaatcgagaataaatagtaaattagaagaaagagtggagcttacaataagaaactacttaaatagtcaagttgtttcacaaccattaatcttagctgacctaattcaggttataatgaatattgacgatgttttaatctatgactgtaaaattaacaacatggaagggaacatggctgttagggacgaagagataattcgtgcaggagaggttattgtagaactgatataaattaggaggaatataatgtgagtaacttttataaaaatatccaccctctgttgagacgtggtaagaaacctaacaagtatgatgatactaactttgcagtgcttaatgcgttgaactatgaattaactcaggcagagcaggagaccattgctagtaagattcattcttcattagaaacagctacaggtgagtacctagatacttggggggactggtttggtgtatatcgtaaagatgattggaatgacgaatattatagaaaaagaattataagagaacttttactaaaaagagccacaattcctgctatcattgatgcgttattggatttccttaacgacaatgatgcagtcatccaaatatatgaaccttggagaaacattttctatacaaataagtcaaaattaaacggtgacgaccatttaatgggttactactaccgttttgcaattatcgatatttcaattgatagaccgtttcctcctgaaattgtagagattattaaggctttcaaacctgcgggagttctattttatctaaggctagacacaagcttaaataagaataaaacaactgtagaaagcccatatgtatacctagacgtgacgaataagacagaattagagttccttaacggtttatactatgacctacgaggtaacattaacctgtctgaccaacgtacacaagtagtagagagtaatatcttccatacgaataactctatgctaaacggggaagatgtgcttgcaggagcatttgaccacggaagaggctacattcacttagcaagtacaacattgcttgattacacaccaaaacctactgactctatgagtgacttaaaaacagctctaggagaatcaggtgctgatatgtataatcaaacaaaagaaaaggacggaagaacagcttctattcaagtacctgcaacaaagaatgttcacaccttgtactcaaacagcattgactttggtggctatgattattcggggaatccgaatgttatgactaagccttatattgctgacaatataaccggcggtacaacaggagtagttgtaacaccaattgatgatggcgcaagactagaaaaaacacgagttgatatatctggaacgtttaacttagcattgggtaatcttttgaataatacagattatataatttcatatgatgtacttgtggaaaatggatatgtaggagatttaaaaacttgtaatgttgcattagaaggacagtttgaaggaaagcctaactattttggtattttttatatgaatagtgtaacatcaacagatgtatggcaaaaggtttctgtaaaattcaatagtggtgccaacatggaaaaattaagtggttttaagtttagagtatatttatctcaacgtgttcaagcagcattaaaaataaaaaatgtgaaaattgaacgtggttcaacagccaccccataccagccaaatttactcgatgcaccatattatctgggtaaggtggctttgggtgagaatattgctaataagtccgttgagtttccaataaaatctagcaattatctcttatataacgctagaatggtagagccttttgttgtaggagaaccttatacaattaccataaaagcaataaaaccagccagtcaaacgtttatggtatataacattggggaaggaactacttattacggaaaactaaatccagttgagggattgacagacgtatggtcactaacattcacaccaagaaatgtttcgtcaactaatcctagcgatttacgtatttttcagtacccatcatcaacattaggcacatgtcaaattgattggttaaaaattgaaaaaggtgacaccagaactcctaacattgattcctacgactacgtaggttctctgatagaagatacagaaacacctacgttagacccgactaagtatacatggacagtaaatggggatataacaaataaaaaggcatatatggtgtttgatattaagacatttatcgaagaaaattatgctatagaatttgaaaaacttattactgacctaggagaagaccaagcattaaataccgtgtttgaaaactttaacatctctacaacacttaaggctctagtaagtccaagttcaccaatcagtttctcggttgaactatacgatttttctacgagtgcatggcacaagttaaacacggatagcttagacttacgtatgcgtacattcaacttagtagcaaaccgtatcacagactatctaaatgattacaagctattatttgttcgttacgtgtttgataacgaaacagataaagatgtaacagttgaactagacatgctaaatgtactattcaagtatcgtttaggtgaggggtacagtataggactacaatcatctgtggaatcactaacggaactcgttcctatagaagggtaatagcaaataatatgttataatataaatagggcacctagttgtgtcctattttttaataaacatgctatattaacaattgaatgataaagaaaagaggtaaataatgtggctattgcaactaacaattcacgagtgtatgcctcactccaattaaaaaataaacaagacagtatgtacctagcaattggtaaaaccactccttggactaatgaagatgccccccctgcaccagaccctactacggctactctaacagaggttatcggttataaaaaggtagcaagagtatctttatgtagagaatatctaccaagtgacgattctaaataccctgtggtgtcctatggttcaagaaaatttacgctaattccagatgaggacggctataaagagcaagcgtggatggtgtatgtagaagcagaaattacaggagatgaactaccaataggaacatttaggcaagtaggtattcatactgacttagtgtctaaggcaagttcagaaaagaaagctttgttacctacagatgtaacagatgcaggtattttgcaattttttgaaaatagacagcaacaaaatagaacaagtgatgtaattttaaaagagaagtttattattacaatggaaaataagaagtcagttaaacaataggaagggtgacatagatggctaaaaatattacaaatgatgatttaggtaaagagccttataacaatagatattaccaaggcaaacgattttcaggtttactatttaaaccagataagccgttacaacaagccgagttaaacgagttacagtcaattattcaaggagatttaggcaatgtggctgaatccatatttagtgacggtgacatccagactggtatggaatatgtactacaagataagaagcttactattaaaaaaggtaaagtattcttaggcggtaaaatgcgtaactttgacgaacagagtatcgatattaccggagagggtacggagtatgtaggtgttaaacttgtacaaaaagttattacagcagaagacgacccatcactgttagaccaaacaagtggtgttcctagccatttctcagaaggggctgaccgattagacgaagatgtagtactagcagttaatgatgattctgcatcaaacatttaccactttgttaacggtgagttatacattaacccagatactcctgagatggataagattaataaaatactagcagaaagaacttatgatgaatctggttcatatcgtgttcgtggttttgatatgtacacagaagttcacccaacagaccctaacaataaaattcagttagttgtcgattcaggtcgggcatatgttttaggttttaaagtagataaacctacaactactcgtattgatattgaaaaatcaagagagttagaaacaatcaataacgaaggtttctactatagcaatgcaactcgtaaaaataaattaggtaattccccagtatcttctgtagaccgtgtaactgcacaagttgaagttgctaaagaacaggtttctcgtggggtcgtaggtggaggtaccgattaccttaaaaacacctctgtaacaaaagttattcgtgtatggactgagggttcaggagcacaggagtacaaacaaggtgaagacttccaattagtaaacggtcaagcaatatcttgggcacctacagggcaagaacctcctgcagggggaacctacttcgttcaatatgtttataataaaacaatgattgaaaatacagattacaaagttgtaattactggtgaaggtgatgctagggaatggtatatcgactttaacgagatgacaggttctaaaccagtcgatgaatcacttgttaacgtagactataaatacttcttagctcgtaaagacctaattgtattagaccataacgggaatttcactgtccataaaggacaacctaacgctttaagactagtagaggcacctaaccatgtagacccattagttttagctattggtacagtagtagtttacccagactcaaatactgctgatgctaaacaatggacaatcacacgtctaacaatggaagagctacagaagttatctgttcgtgtggaaaacatggagtataaccaagcagtgttctacttagaccaaccggcaatggcaggagaaaaccctatctatctacgtggagtattctcggatgcgtttatctcactagataaatatgacgttagtcacccagatgccacaattgcttttgactttgacacagcagaaataacattaccttatgcagaaattaataaaacagttccaacaattatcgaaggttctagtgaagcacatgtgtggggcagactagtaacagcaccgtttaccgaagaagtgggtattagacaaccatttgctacggaagcaatgaacgttaacccatacaacacctttaacaaacagggtgccttaaagctaaacccttctgcagataactggattgaagatgagcgtatcacagttaccaaagaagaaacatctactatgactgttcgtcaatggtggagacatggtggagcatcttggacaaacgatgagatgaacatggtatctaacatcacgcttgaccccggacaatcgtggggaggtgcctctggtacagaagaccaacgtaaacaagggctatccggttctactttaaccagtggtggtcagcaaaccaaagaatcaatgattgagtttatgagacaaattgatgttgaggtttacgcagagaacttgcaacctaatgctaacaacttatacgtaacattcgatggcttgagagtacctgttaccccatcttctggttaccgtaaaggtgccacagaaggcactggtatggcaaatgcagacggaacatttaaaggggtatttaaaatacctgcaggagttcgttgtggtactcgtgaagtatctgttagaaacgatacaaacttagcaagtactacgttcactgcgcaaggtacgctaaaaacaactgaggatattatcataaaaacccatgttactattaacttggttgaccctctggcacaatcattcagttttaacactaacagagttgcaacaagttttgacgtattctttgcatctaaggataacagtacaaatattatttgtcaagtacgtggaatatcagaaggtgggcaacctaataaaactgtgtatgctgaaagagtgttaaaaccttctgaaatcaaagtatcagatgatgcaagtgttcctacgaaaatcagctttgatgacccactaatgtgtaaagcaggtcaagaatactgtttagtattcattactgactctgataaatacacaatgtggattgcaactatgggtcaaaatagagtagacgaaccaacacaaacagtaacatcaaatccttacttggaaggtgtcctatatagttcatctaacgcaagtgcatggtctattcaccaactgtctgatttgaagttcactgtatacacggctaaatttaacgaagaagctgtacttgagttcgatgttatgaagaacgttaatgtagaccgcatagtgttaatgtctacctacctaacacctgcaaacactggttgtagatgggatatgaaactagtccttgataatgagcctgcaggtacaacagtagatgacaaaccttggttacctattgctaactacgtagacttagatgttaaccagttagctcgtgaggctaagcttagagcaacatttaaagctaaccaatacatctcaccaatgctatccttggacgacattatgttcgcaggatttttaacagcattgaaaggtagctatgtatctcgtacaatagatttaacagaggctccatacaacacggttaaaatgtcatatgaacaatttacacctgccggaactgttgtgactgctaaatatagtacagatgaaggtaaaacatggaagacatttacagtacagcctacaacaacacaacgtacacaagactttgttcgtgtagactatgttgaaaagattaatacgggtgggacatttaagtccattaaattccgtcttgatatgacgacccagaattcatttttgcgcccgcgcgtaagacgcttactcactaatatgaccgacaaatagaagatgtaactgtaatgtaacatttctatgcctcctactgtggtatacttactgtatacaaaatagtaggaggttttttaatgggtaaagcattacaattagcaggtactacatttggtaaatggtacgtaaaagagcgagatacttctaagaaaggtagagcatactggatttgtgagtgctcttgtggaagaacagttcaatctattccgagcggtactcttactacaggctcatctgtgatgtgtaaacaatgtgcaaatgagaaatctttagtgggtaagacttttggtaggttgaccgtcattaaggattcaggtgaacgagcaactaatggtagtatcctttgggagtgtaaatgttcctgtgggaaaacaagccttgtcaggggttcagagttgacagggggtcgcacaaagagttgtggttgttactccacggatgtactcaaaaaagtagccactaagcatggattgtctaaagtgaacggaaaacccacaaaattattccgggcatgggcttcgatgaaacaacggtgttacaacaagaaccatgcgagttataaagattacggtggaagaggtataaccatatgttctgaatggcgtgaagactttgaaactttccatgattggtctatagctaacggattttccgatgacttgtctattgatagaattgacaatgacaaaggctattcaccagacaattgtcgatgggtagatgctaaaacccagattcgaaatagacgaaataccattacttacaactggaagggttcagagtacaccttagctgaactgggagaactaacaggtataaacaagatgactataaaatctaggctgaactccggagccactcttgaagaagcactagacccaaaagtgaatacgtcagttttgactatgagttacaagggagaaactaagcctgtcaaacaatggtgtaaagaactgggattgaattacgcaactgtacgtagcagacactataaaggttggactgatgaagaagccttaactggtatacgtaacaaatagcaacagaataagtataatagactctatatgttataatagacatatagagtctattttttttgttaggaggaataaaattgccagaaacacacagacaaacaagctcaggtgcgcttatatttaaaccaactatagctgaacaagagcataaaaatgctatggaatctataaaacaagagagaacagagctagagaaagaactagctaatgttaaagctatcaaagatgagttgtcaaaagagctagcagatattaaacaactgaaagatgaattatcaaaatagtttctaaattgtcttatttaggatttctggttcccttatactattaactaatatatttaaataactatatataaaatatataatatataaataatatataataagactacgaaaaatataaaataggacaaatcaactctgtatacaccttgacaattacctactatgtgatataatgaatatattgattatactaaggtgggtatgtcaaggagcatgtatactaatctaacttaaaggagatttattaataaatgagactagtagtagatattatgcatactcagataaggtatgaagattcggaaaattatcttagaccagaaattcataaggtaatgcattcagaattaggagttaaagcagatggttatcaatttagtcctgcatataaagcaggttactgggatggtattattgattttttcgataaagaaaatgacacgttccccacagggttactacctcatgtagaaacaatactagggaaccttcaatcaactttatcaaagtcaggttacatttttcagtttgagataattgatgatagacctgatgagttcatgtcagtagatgacatggataaggagatagtgcttaatggggataacaatgacaagataacattaagagactatcaatatgaatctgtggagcaagttattaagaacagaataggtattgtaaacgttagtactggtgggggtaaatgcgtagtagcatctacgaacctactgacttacgataaagggtacaaaacatttgaacaactgttcaaggaacacaacattgatttaacacaatcagaggcaactatccctaacacatttggggttacattagtgaatgaaaagggagaaccagaaacgcctagtcatttaactattaatggagttagacatgtaaacaaggtaacaactgagcatggatggactgaaacaattactgacaaccatccattactaactgtatcagaatctggtagctttaaatgggtagaagctaaagacttgaatgtaggtgattggattgttggacgtaaaggtgataatttatttggaacgaatactacatgtaccgtggagagcgcatatagcttaggtttattaacagcagacggctattgtgggcaaccaacccagattacattaaccaataaccaaccggagatactagcggacattcaagatttctttactaaagaagggctgtccactaaggtagaccctaacaaagactctaaagatagtaagatagttaggggtaccgcaggagctagagaactttataataaatatggcttatcacaaggattagccaaggataagtcaatcccagagtgtatcatggaagcaccgaaggaagtacagttagcttatataagtgggtatttagagtgtgaactgagtatggaggtacctaaatgttcaatagaggtaatttctgcctccgagaagttacttcaccaattacaactcttattaggaaacatgggagtttcctcaagattagctaagaaggtagttaaagggtacgaggctaattggtatggtagattaactatcggagtgactgactcagtttacctactaaaacaattaacatttaaaacagcacaacggaacgaaagaagagccttatttattgaaacagcagagtcccgtaatagtaaccaccaaggacaacctgtaccttttggtaaggagttagttaaacgatactgcgataactacctaggggacactaaaggacttagtaaggcattcaaagtaccaagaacaattagcttacatcggcttaaaaatttaattcatgagttccctaatggaaacccgacagattttgctaacctgacaagattaactgatggtagatatgtctattcacaagtaacaagtattgaagatatgggatatgaaccaacttatgatttacacatgcccgaaacacatagttttattgcaaatggtatgataaaccataacactgaaatagcatcaggacttatacagcaaataaccccttacttagagtcaggagaacgtattgcattttttacgaatagttcttctattttttcacagtcaattgaccgtattgagaaaagacttggaataaaagtaggtgcttttggtgcaggtaagaaggacattcagcaagttacttttgtaatgatacctacgattgtatctgcaatatctgcagacccagaggctaagcttaagctgactgctaaagaaagaatgtacaagaaaattgctaaggatatagctccaaaatttgaaagagggtttaaccaaaggagtttgcttgaaggatacctaaataactttcaagttaagacaaaagcagacctgcagttgaaacatgaactagaagaaattttttattcatgtggtacgaacaaacaggttattatgaaaatgaaagggtatcaagcagaataccaaaagattgttgaaaagaaaaatggtaaagttcttaagaagtacaacgaggctatggagtttttagattccatatctgtaatgattgtggatgaggctcaccatacaagttcagatacttggtataaagtgctaacatcttgtaataacgctcagtatagaatggcacttactggttcgattgaccgtacaaatcatgtgctttggcaaagacttcaagctatattcggggagattacgactaaggtgtctaacaacacacttattgagttaggtcactcagccaaacctaaaataacaatattccctattatagctcctgtagatattcaaaccactacgtatatggatgcctatcaaaaaggtatagtagacaatgaatatagaaattctcttattgcaaagttgactaagaagatgtatgataaaggtaatgggattttaattataattaatcgtatagagcacggagaggctattagtaacttactaaaagaagagggagtagctcactactttatcaatggacaacttgaaaatgatttaagggatgaaaaaattcaggacatgcgtgatggagcacttaaagtaatgatttcttctacgattatagatgaaggtgtcgacatttcagggattgacacattaattcttggtgcaggaggtaagtccttaaggcagacactacaacgtgttggtcggggcttacgtaagaaaaaaacaggagaaaacaaagtagaagtattcgatttttatgatttaacaaacaaacatttgaaaaaacattcagagcagagaagaaaaatatatgaagatgagcaatttgaaattgttgatattcctattcctaaataactataataaagaaagggtggcatacaattgcaaagtccatgcctaaatattgaattaaaagaaaaatttaaattaaacaaaggtataacagactttttagagagagttgcagataaatctcagagatggggtgaaacagtagcctcccctatccgtaaaacggatatggcaaaagagactggaaaaaaccctagaacaattacaagatatattaatcaattagaggaactaggtttaataaaaaccgaaacaaaaagaggaatgaatggagggactttagtcgtgtttaacacagatatgcttaattttgagccaaaggaaaaccctatcacgtctgatactaaacaagcaaaggagattagagaacaagttttccctaaagccccaaccaaagtaccaaaacgcagatacagaacaaaagcggagatagctgaggcacgtatacttagtgaaaaacttaaaaaacgtgaagacattttaaatgataaaattgagtttaacgttgttactagaagttttttcgatagttttgacgaaccagaagcgtactttaaaggctatttaatttcaagaatgtataatgcttatgtgacaatcattccttatgaaaaatataatagactgaaaaatttagatgagaaaaaggctaaacaacaactacgagcatacgaaagctcttacaattacgatgtgttgcctagaagatttgttgggacacctcagtacaaaaaatttgtagagctagctaaatattgtgaagagaacaatatcaatcctttagtttatttaacagtgcaatttgatagaacagagtttttgatttctgtaggtaaagcacgagtaggggctacaccctatgtaaatactttgttatgtgcagaggctaaagaggcttacacaaatagaaaactgttctacagaatgttacagaaccaatatggattgtatacgtctatcaattcagaagctacttattatggtgcaacttatccaattatttcaggactattgaatgcttacaatatgccacagaaagacttgtcacagttagatactgtgatttgtgacttagaatataaaaaagatattgacaaaaaagcaggtacgttgtactcttattatacagcaacacttaaatcgttaggtgaatctgacgtatctagtgaagctaaagaaagtattgctaacttcttgaaagaacaagttgcaaacttttctagtaaacgtgggctaacttcaacacagtatgccttagcgttccctattcagataaactctgcacgcagtttattaatgaatgaggaagacgaagaactactttatttattgttaggtaaccagtcacgattatctaatgtaacaaatgatgaagctgaaatgtttattaaacaaggtagaaaattaagtatgtcttggtggggctcacagaacttctcaagaacaatgttcatgttagcggactactatgggtttaaaacaaatatatctaagttaggtatgtacattaaagaatttggtgaggagaaaattcctttagattctgtaggtatgttagatgtaaatagaatctatgatgtcttaatgactgaacaagagattttagagattgacaaaagtaactgggagaaccaaaaagatatgcgtgacgacaaataagaaatataaatgggagagggacggatagtaagatgagtcaaattcaaaaacaagttatttatagagcattaagtgagccattctttgcaaaggaaatcctaagtaaaattccaatggatgagtttaaagattctggatatgagatgattgtttctacaatcaacttatattacagaacacatgatgagagcttagaggaacagagtttattaacactagtagaagataagatgttaaaacaaaacaaaagtttggaagctcaaaacaaagtctttgaggtagttagcgacttatacgaactagagaacgaagatgtagactcagaagttatcagtgagaacattcagaactacgttcgtaaggtactaacacgagaagcaatcatgaaatctgtaacaaatgaaggcacactaggctctgatagtaatattcaacagctaatggatgacttgagagacattcttactatcgagacagcaggcaataattcagaattgctagacttcttcgatgacgtagataaaaagatggagttacttgcaaacttgcaacaaaacaaatacccaactggtttcacagctatcgatgctatttccgatggtgggctagctcgtggagaagtcgggatggttgttgcacctactggtggtggtaaaactacttgggcagttaaccaagctagaaactatgttgtacgtggtttaaatgttctttatgttcctttagaggaaaaagtagaccgtatgattgttcgttttgaacaattattatcacaacaaagtaagaagaacatcttagttgatggtgaattgaataaagacttgtatacccaaatccaacaagcgtatggagcgggtaaagaacagatgaattggggtaacctttggattcgtaaatataaaccacaagagctaacacctagcggtttatctcagttaatctccgatgtaatgattcgtaaaggacagcaaattgatgttgtcattattgactacccagatttaatgaaaaatcctcatgcaagtggaagtaatggtgaatcagatgcaggaggtaaactgtatgaagatattcgtgcgattgcacaagaatatgattttgtttgttggacgttatctcagttgaaccgagcaagctatggtcaagatattaaaaatgcaggagctatcgaaggctctaaacgtaaaatgaacgcagtagagcttatttttacattaaaccaaacatcagaggagtttagtaacggatatttgagagcttacgtagataagttacgtaataatagtgggattgcctatgataaaatgttgtattttaaagtactcccagaaactatgactattagagatgaaacaccagaagaacgagcagaacatgaagcactgttagcagataatgcgatgaatagagcaagtagccactctgatgagaataactacacagcaaacgatgttaataaaaagataagtaatttgaataataccctttcaggaggttggaattaatgaaacatattattaatttttcagattttcatatgcacttttttaaagatttttcaaaaccagacccagagtatggaactgatagggcaaaagagcaaattactatattagacaacttgatgaactatgcacgaaacaaaaatggggatgttttatttaatggagacatgttccataaacgagtatctattgatgttagaatattcaatatgttatttcaagtaattagtagctaccctgatgttgatgttatcatggtcagtggtaatcatgataaggtaactaactctctatattcagatagtgctttagcaccatttagtgctttaccaaatgttacagtttgttctacgttaaacaagattgttaaagatgattatacgttgtatgctgttagttatggggaagaggtcgaagagatgaaagcttggataaaagaacaagctgacaatttagaccatgaaacagttaatattctaagtgcacacattggtgtagatggttcatctactgggaagtactcccatacacttggtggtgcttttaaagtagctgatttataccctgacaagtttgacatagttacattgggtcactatcataaacgacaatttttaggaaacctatctaatgtgttttatgtgggcaataccttacagacttcttttgcggatgaaggtcaagaaaaaggtttttatgatattactatagagggtaagaagtgggaacaaaaatttattaaaactgactatactccgtttgaaacagtaacagctgataacccatcaacaacaggttctatggagaaatcttatatccagtttatcggtaatgtggatgaggttgaggctgtaaagagaataaaagaagagaataacttaagcaatattagaataaaagttcagaaggactaccatgttgagccacgtataaacataacagcaggttcgacacctaatgaagttgtcaatgcatttattagtaaaaagtaccctaacgcaaaaataattaaagaaaaagctctcgactgtttgagagaagcaatggaagtataataattgtttagcctagatatatctaggcttttttgcgttgtactattgactttattagtattttgaagtataatatgtttattgaaataattaatattttgggaggaaaagatgttaaagtttaaacgagttagcgcagagaactatatgtccattggctctgtatctattgatttagacaaccaaggactcgtacttatcgaaggtataaatgatacaaacgaaacatttcagagtaatggctcaggtaaaagtactttactgtctaccgttacttatgcattgtatggagctacccctagtggtttgaaagctgatgctgtaattaataaacaagcaaagaaaaatatgtcagtgattttagaatttgaaaaagatggggtaccatatcgtatcgaacgttatcgtaaacactctaaacataaaaatactactagatttttccaaggaacaaatgatataactcagaaatctgtagcagacactgataaaaagattcaagatgtgttcggtattgattacctgacttatgctaatagtatcatgtatggtcaaggtaacgtagaaatatttgctacagcaactgataagggtaagaaacaaatcttagagaatttagccgatattggtgtttaccgatatgcacaggatgttgctaaagaaagagcacaaaaagcactagctcttgcagaagagctgaacagacagtacattgctaagacatatgaaaaagatgggttaactcaatcttacaatagtgctttacaacaatatgagaatacagaaaagctgattcaacaaaaagagagtgagttagctaatgcagaattagctattaaacaaagtgagaagaatctgtcagagggaagagcgctacgtgaacccgaattagaaaagctaagagagcagatggcacaactaacttcccctgcagacgttcgtgaaattgatgtagaagttgaaacacagtattctaacgttagtagattatctagtgcaaaaacacagaatgatactgctattgagaaattaaaaaaagaactagaagatgttaaaacaaatacaaattgctacctatgtggtgctttattgagcccacagcatagagaacaagaaattcaacgcattcaaagagaaatagcggataaagaagcgtttatcgaaaagcttaatagtgcattagcagtgtattctcctctgttagagcaagcaagagctaaacaagaggaagcaagaaaagctattcaagaacatactaatatttatcataaacttaatggtgaaatgaatgcgttgtatcatgagatagatacattagagaacacattgaacacatctattaataatagggacagcattaaggatatgttagcaagactacaagaaatacctaaacctcaatatgactatgacaaagaccgggaaatagaagatgagctaaataaaattaaccaattaaaattagatgccgaagaagaagctagtcaatataaaactattgcacaagaaattttctctaataaaggcatacgctctgaggtacttgacctagttacacctttcttaaatgaaagagcaaaccattacttatctaccctttcaggttcagatattgaaataaactttagtacccaaacagagaaagcagatggtagtttagctgataagtttgacttagaggtagtgaatggctccggtggaaacacatatcaagcaaactccgagggagagaagaagagaattgatttagcaatatcttttgctattcaagatttagttcagtcaaaagcaaacattgctgttaatttaggtttgtatgatgagtgttttgatggtttagatgcaattggttgtgagaacgttattaaaatattgaaagaacgccaaaagaacattagtagtattttcgtaataactcactcggagaacttgaagccattgtttgagaacgtaatcactatgaaaaaagttcaaggtcgttcttaccttgaagaaagtaaataggtgattacatgaagatttatacattaagtagagagttaaacgaaggtactatatttgtacctacaagtagtagtaatgaagggagactatttagcttcccgctagagacactattcgattggtacccttgttgcccaagatatgagtatcagtacagcacttctcgaaaaaaactatatttgagattgttagactcagacaaaacattagtagctagatacggtgttggggataataaaaagagagttatttcaaaaatagcttgctttaatgagaatgaatggtataatgaagaagtggcaaatgagaatgcagagttgtttaactttgctaaacaatatgacattgttacacctttaaaagaagattacaccttaaaagaagtagataatagtatctctaaagtactggacattcttgatttactttacacaaatcaaaaagttaaagtagaagaagagcttataaataaagtggatactctacaattgagtaaaccagactcggatgaacttaaacaagcgtataaggatatatctgagtatatgaggttagacagagaggaaaaagctacttatgtattaagcaggtcactagactctttaaatagtgtttatgaaaaatttggtaatgtgtatacaatgttaaatattatgaggaaagtagtggcttaaatgtttacagacttgttatctaacgaattaggttcacctaaatatgcagtaagggactacaggtataattgccctttttgcgactacgatactaagtataagttttatgttagggtagaagaaggacacccaaagaataacttatggcattgttttaagtgtggtagttcaggtaacccagtatcttttgtaatgaagtattacaacgtgtcttttaaagaagcgctagagatattagaagaatacggctataggtttaataataaaaattatgtgcctaaatcagataagttaactgatgaggaatacttattacttcttctaggttcgttaggtaagccaaaagaagaaactaaacaagctaaaaaagagttagtagcacccccattgccagatggttttaaactactaagtcagaacctgagagagccagaagcgtaccctttcttattatactgtaataagagggggtttacattgaatgatatttatatgcacaatattggatatgtaaaagattcttgggtacccttagaaaatggtaagtcagttagactcaaagaccacttagtttttttaactcatggaaaagatggtaagtatcaatattggaatactagggctattggggaaagctttattaagtctttgaacgccccaagtaaagagggtgagcattcaaaaaaggatactatatttaatattaatagagctagtcaaacccctcagatagttataacagaaggtgttccagatgcattaacagttggtgagtctggtgtaggtacttttggtaaacaagtgactgacgagcaagttgaacttattttagatagtgtgaatgaagagcaaaaaatatttatctatttagataaagatgctaaaaaagaaattaagaagttagcagagaaactatataagagacataacgagacttatgtagttataagcccaacaactcaagatgcaaatagtctagggagagaagaggcttggaatattataaataactactctgtaaaagcagatggagtagggttaataaaattaatgttatagataggagagggaaaaaaatgaagtatacactagaagatttacatgcaggtatgaaattacgttgcacggacaataaaaactacagtttttggactacgaataaaatctatgaagtaactaaaaaagagtcaggttcactatgtatttttgatgattatggaattgagagcctagatgaggacatcttagtacgtttaaatggtaatacagggaacgcagaatttgaggttgtttctaaggtgatgaaggatgcagattacacagaagaagaccttgaagaagggatgttacttcactgcaaagatgatatgagctttccatggtgggctacaggacaaacctatgaaatctataagggtgaaaaaggaattttatttaccaagtcaggagacggtaaccaatactgtgctaaagaaatagtagctcgattaaatggtagtgcaagcgggtcttttgaattactagaaagaccacataaaacagagttagaaaagaaagtagaagcaagaattaaggaactaaaaggaaagaaactttgtttattctacaagcaacaacaaattaagatagaagaaaacgaaatatctatagaaatcagtaagctaagtgaagcattaaaagcgattgacgtattaagagaatttgaataagaataactataggaggacaacaaacaagatggaaagagtatcagtatactttctaaatagcagaaatattatggatgaggatgagacaaagcgtacttatcatggaacatttaattcaatgaaagaagcagagcagtcagttcgtgactggtggaaagcaaatgactttaagtgtggtacccttagaattattgaaggtactgaggatgggattgttcgttgggactacggaaaccatactgggttctatctatttgtaccagaaggtgctgtagtaaaatacacaatccgtgaaggcgctaagaaaccaaaacgaggaagagaaaatgatgtagcacatgacttgttcacagcagacgatggagtagttattcccgggagattaggttcaaatgttatttctactggaataaaaacatcgtttgaccccaaacaatatggtttattcattaaccctcgaggtggtatgatgaaatacccaatcactttaggaaacacacaaggtgtagtggaaggggaatatcgtggagaggttggtttaccacttaaaaatacgttctctttacaattagatgcaagagctgtttctaagaacgttttaacaatcaatgaagaaggtaaacttattaacatcccagtaacagtagctcggtcaatgtatccaagctttaatgctctttatgaaaaacagctagagaagctaagtgaggagctacagctagtctatggaggagaagttagaatatctaatgctgatgagtatgtggttgcgggaacactatttatcccaaaaggcactcgtttatgtcaagctttcttactaccacgatacgacacacagtttgttgaagtatcagcgttaggtacaactgaacgaggagaaggcgcatatggctcatctggggtggtatagctatgctcatcccagaatttaagccaccattattgtacgttatgggtagcttttctgttatgttagaaaaacaccagtgcagtgtaacttttgatttaagagagccttatttaggtacctcttacgataaaatagtgaagcttattaaaatgacttacccaaactatagcttaacttatgtagggatgacagataataaatataagttcacattaaagaataaggaggactagcatgtacaccaagaaagaggaagtagtgacagttaaacacctagttgataaagagcaaattagagtaggggacatagtaggttacaaaaagactattagagggttcgatgcaaaaagagtaaaagacacactctcagtaacaaatcaaataggtgtagtttctcgtgtatgtgacgagtacattactgttcatgacttttttgataagtgctcacgagaaatatgggcaaagacatttgaaaatttagaagttcgcaaaatagaggatggtaacagcctactacggaggtatgaaaatgaatttcgttgattattttaatcagatgcagaatttagtgattgaagaaaaaacagatgagtatgttttactagagaaagaacatggtcaaaagtatgtgacatatcaagagctagaaggagcgttaagtacagtagcacgcaacactgcatttatggtagaaaattataaccttatgcaagatattaatttaaaaattgtattgaaaaaattaaaagacagtggtacaattacagaagagcttgaaaaagagattcttaaagagttcaaaaatattgaaagtttaatggaggacgaaacatatgagtaaagagagtaaacgcaacaaacgtatcggggagttatcggaagcagacatgagagtgtgggctgagtggttagccacagggcaggttcatgataaaaaccaccaaaaacagttagaacgcttaagtaaacgttcagtatcattatctgatgtaactactattgtcgaatttatgggcaaacggaatgatggttatatttcttctttaattgaacagcaggctgtatttgacaatttattaacaaaactaggtgtaacggaagagaaccgcttagaggctaaagcagagtacgaaaaagagttaagccttattcaagaaaaaatccaaaaagagttagagtctattaaagaaaataaagaaaaataatatgaaagaggttagctgaatgacagactacagcgcagtaggcaagaaaagtcgtaacaaaggcggacgttttgaacgtcaaatggctaaagaactcacagagtggtggggatatgagtttaaccgagtacctgcttctggggggcttcactgggcttctagtaataacgttgccggggacattgtagtccctagcgatgctaacttcccatttgttatagaatgtaaaaatcgtgaagactggacgattgagaacttattcttaaataacaaagaaattaagaactggtgggcacaagttgtgggggatgcaaaagaaacgaaaaatatcccactacttatatttactagaaacagagcaaagaattttgttactatggcatataatgaaaaacttgttaatgagattgaaaaaagaggttaccctttgatggtctctaacataacatatgtagacgactacaaggatactcattgttacaagacatttactacagttttagatgcaataactagctttaagccttatggtagcaaagataaagactactttttattttattttcctagtgactatgactgggaagatagcctagtttatgaaacaaccataatggatgatgctaaacaaatggatgcagaggattcactagatgcactagttaattcttatttaggaggagaatagtatggctaaaacatatcaggaagctctagcaacggtacagtcgtatctcgaatcagatagtgtaatgaaagaaacctcaagtatatctgttagtttctcagctaactggacaggtgagcgggaagactacgttattgatacattgacatacgacattgatttacgagtattcagcttagaaactgcacatgttgtagctatagggaagaaactacctcaagatagcaatgagcatgctgaactccttaaaaaacttaaaaaagaatttaaacaagcttctaaaaaactacgggaggactagagtagatgatagacaacgttaatagtcctagtcattatacgcaaggagaaatagaggtaatagaggttatagaatatattactgctaagtaccctgcggaaattagataccatttaggaaatgttattaagtatatttgtcgagcacctttcaagggaaagctacaagaagaccttaacaaaagttcttggtacttgaaacgagcacaactggttttaacacagtcaccaagtagctatataggtaaatgtaagaaatttttagagaatttcctatttaagaatagccatatcagagatgctcagctaatagaaattccagaagaacctattattgagaaatttttatttcaaacagcacagagttacaataaagaacagcaaaactatattatttcagccttaatggaactaaacagtagttcaggtgatgtgaaaactgttcttgaaaatacagaaaactatttaaaatttattacaacttagtacaatataatgctctttctacgaaaagctatcttttatatttatggtataatagagatagggaaattaaaaagtagaaggagcattttataatgacaaaagcacccagagtgaaaagacttaatatttataacactgaccggtactttaatattaatttaatgaaaaaagaagatatagcaaaaaaaattaaagttaaccgattgaatgaagaagagatagagagggaaatggacgaactagcaagcaacccattgaagacccctataggctacatggatagaacaaatgaaaaatcttatatactttatcaagagaagtatacgaacgacagacttattcagaaattatttaaacatgcagggtctgtgtcttattacacagatacaattgtaccatactacataattgagcaaatatctaagaatttaacaagtgaagtaatctatcctacaaaaaatagctatgagaacagagagattgaaaatgttcaactagctttcactgcttgccctgtaacgattgactgcccagtagtactacctgatgttagcccgtatgatgtgttatttgcactacatcctctaaaaacaaatgtagacaagattcaaatatcgttcccttgtcttacagaagaagagttcgatactagacatgaagaatactatcataaagtaggtagccactatgaggttaaatcagagtacaaatataaattctttaagtatgtacaaacttccttatctatttgggctatgaacatttggctagtgtgtgatagtgatgaggactacaataaaatagacagatatattcagaaagaaaaaattaaacgtaatgctaacagagagcgtgcattaaagagaaagggtaatcaggatgagtaaagataaaacgattaaccgaacagacatagctcgaacaatctctcaccatactggttatcgaatgaaagatatattgaagattttagaagtagaagatgaagtagtagctcaagcagtatcacaaggtatttctgtaaagaatcacaaattatggaaactaaacattaaaaaaaagccagagaaggtagcatgggatggtataaactctaaaagttttatacaacctgaaaaatatgtagttaaatttgtaccattatctaagttgaaagagtcaatagacacttataataaagagagcaaataaagctctcttttttgctctttctatattgacaaataacataatacaaagtatactagtgtcatagagcaacagagaggagaaaagtgtaattgaaaattctattcttacaagagtacattagagaaaatcatgtccataatggaaagaacggacaaacagttgattttaaaagaacagaaatgggtaaaaaacttacaggtctgttaaatacaataggactgacaggtagggactatgctgtagactatgtgtacgacatgattccggaagtacagaaagtcaaccctagaacaggtaaaccaattaagtataagacacctacgttaagacagcgtaaagaaccagaggaacggttactcagacgtttaatgaaatacaaaccagatattatcatcccaatgggggagatgggttgtaaaaatttattaggaagtacttctatcacaaagaatagaggagtaccaactaagaaaacaattacgaatgagaacatactgagaacggctgatgagcaagggcttgaggtagacgaagtagtagactcttttgaaacttgggtactacctatgtttagtatggaatactggacagctaacccaaacattgagaactttatcatggcggatattgatacattgggtaagtttgttcaagaaggggaacaagcatttatccctaaaaaagtagattacgaatttgttgataacattgaacgtgtaagacaaatttttggttttttagacaaaacgaagccagtaactgcatgggacttggagacaaatagtttacgtggtgacttattaggggctaagcctcttgtaatgtctatgagttggctagagggacaaggtgtgactataccgttagaacaccatgaagctaaatggagcccagaagaacttaacgaaatatatgacttatttgagaagtttttagcggacagacagcaaccaaaagtaggacaaaatatccagttcgatattagattcttaatgaacacaaaaggatttacagagtttgaagacaacagagatacaaaaattgcttactatctaattgtttctcagaaagtagacacttcaaaacggctatccgatattgcatatgaattaacagatatgggaggctatgacgaaccgttagagcagtataaaaaacaatataaagaggactatattgctcgtaagaaagcagagattgatgctttcaaagaagctgaaaaagaacgagtagagtgtgagttcaagatagcaatggatagatataagcaagaagttaaagaagctaagcttattggtaaacctactaagtccattattaaaccagtaaaagaaaaagttgtagtacctaagaaatcagatattaaacttattaatgagattgacggtggtaactttaactacgactggattccattagagattatgcacccatatgctagtggagatgtcgattgctgtctacgtatctataacgttctatataaacgaattgaggaacatcctaagatgttggaattatggttgggcttttatcctagactaacagcaacattagcacacatcgaggcttctggtgttctattagactctgaatacgcagaattagtagagaacatctatacagaagaagaacatcggttgcttaatgaaattagaaagctaccagaagtaaaagaagtagaggatgaacatatgatgttctacaaagaggggcttaaagaaatgacaaagcctgtcaaagatagagatgcctctgttgccagactacgagataaatataaaattactgatagtgagaacaaagtacattttaaaccaagttcgtctgaacataaaggtagactgctatttaaagtaatgggacttacactaccttatgataaagaatctattaaaaaagaaacttttgacaatggggtaccagaacatcagctaacatggagagattataaaacagataaacatgcactagcttatattgcagaaaattatccagaggctaaacatgttgctgaacttttgctagagtattctaaagtaaacacactaaaaaataactttgctcaaaagttacctaaattagcatctaacaaggatggcatgattcatggttcatataacagtacaggtacagaatctacacgattgagtgcaaacaacccgaatatgcaacaattaagtagtaaggttggagaccctagacgttttgactataaatatccaattaaacgtttatttagaacaagatttgagggaggtggaatgctacaactagactactccgccctagaaatgcgtattttaggtttgattgcaaaagataaagcaatgacacaagcatttattaatggtgaagatatgcatgaggcaactgcatctcttgtatggaagttacctaaagataatgtaccaaaagatatgcgacaacgtgcgaagagtgtcaacttcggcatcgcttacggtaagcacaattgccgtcttgtagcgtaagctactcgattaaacttacctaaacgggcatagctgaataaccaataagctgataagagaacctaagtcctgaaaaggatagaggcaatcccgtagtaaagacgatttaataaactccactaaaggagtggtattatggaaattggaacaagaacagacaacaaccctttatatagaaaattaagaactgtgcataaagacatgcgcagacgatgtctcaataaaaatgctaaatcatatgagttatacggaggtagaggtgtaactattagtaaggagtgggagaccttaaatgggttcctagcaactgtagatttagtagatggttgggacaaagatacattcctcacaacagggctatccttagataaagacttaaaaggaggagccgagtatagtatagctaactgtacatggatgccacttaatgataacaaaagcctactatcaatgaactacaagaatgtctgtgctattgacccaaatggtcaatattatgttatagacaacattgacaagttttgcagagagcacaaccttaatcattccaatatagttcaagtaattaatggtagatacaagcatcataagctatgggtattctggtatgaaggtgataaacctaagaaagggatacaaccacacatagcgattagcccattgggtgacacctactatttctataaagctcctgacatggaaaagtatgggctaaattctaaatgtgtagctagatgcttaagaggagagagaacaaaacataaagggtggaagtttattaaatctgaaaacctctaacgactatcgaaaagtgagtagctgtcgagaggacacctacaatataactgagtagagtacaccaacaggtggaaatggtaaggctcctagagtaacgactaggagcgtgatatagtctaagcccctaataaatatcgggaaaccgagggtataactggaaagtcctttttcaattgcacctaagttaggtgtaactgtagaagaagcagagcgtatttttgaagagtactttgcaagtaagccaagtattaaacaatttattgaagagacacatcaatttgctcaacgttatggctacgtagaaacactacaaggacatcgtagactattgcgtgactcattctctaaagataagaaagtatttaatggagcaatgcgtaagtcagtaaatacaatcattcaaggaactggtgcctacttaactaacctatcaatggtatacattgacgagtatatcagaaaacacaataagcgttcacgtattgttatcactgtacatgactcacttgttatcgattgcccacgtgatgaagtggacgagatggcaaaagtggctaaatatattatggagaacttgccaattgatttcttaatgattgagtgggaaggtaaagagatgcgttaccctattgtggcagatgtagagattggggagaattacaatgatatggttgattatgatgcagaaattatcaacgagtttgcttcttaccgaggatacgtaaaatacttcaaagaccaagctaagattaaagattactatgataacaaacttatctcagaagagcaaaaagaccaaggtatcaaagttatccaagatgcaatagagtcatataaacaaatgacaatttaataaaaaaatgttaaaaatagcttgactattgacgtatagtatgttattataatatggcagacaagttttctgtattaatacaagaagggggagttagagagtgtgcttaatttacgagtagacgatttagagttcaaaacaattaaaattattgatgataacggagaagttgtgacacatgatttacaaacagagttacaagtcaatgaatttaatgtgagaacagcatttttagagcaacctgctaagtatacttattggacttcgatactagagcgcttgcgcatgtatcaagaaaactatgagttaaaagcagagaagaagaaagcagaactatatgagccttctcgggttgccttaatcaatcaaggagtagctaaacctacaaaagaccagattgaggcacagattatgttagatgaagactattacaaacttagacagagtatagttaacctatcatttaacgtgagacaactgcaatatatagttaaagcttttgaacaaagaaaagatatgcttattcagtatggagcagaccttcgtagggaatatgagtatagccaaaaggttagtatgccagacccaatgaaaaataaggtaaataatggtttctcagactttcaatggaatttagaacagtaaaattagtgataaaaaaaataatataatataaaaaaaatagaaatggagaaatttaaatgaattttcaagaacaattacaacaacaattaaaacaacaaaatattggagaacgtgaagcggtagactacccatcaaatcatttaaaacataaagaattatacttccctaaagcagaaaatggtcagccatcaactctatatgtacgtgtgttacctcctgcagtaccgggagaaaactataatgttagcgctcgtgaggcattcttaacaactcgtaatcgtaatggtaaagatttaaagagcaactttatcttttcagaacaccctaatgcagaagacatcttagaacaagctatgattcgttggaacgcagaaaatcgtgtaccaaacccttatagccgtaatacaaaacctcgtcaacgttactacgttaatgtagtgcagttaattattaaccaacaaacaggggaagttagctatgaaacagattctaatggtcagctaatggttcgtttacttaagttaccacaaacagcttgcatggctattaatgagagcttaagtaacccaatgttacgcccacagttttcacctgatgtaccagaagaagtagcgcaatacagctttatttcttctgcagatgcattccctatttcaattacaaaaccaccacgtagtaacaaacctacttcgtacaatgtacaagtgattagtaatcgtagtttaggtgcattaccacaaggttgggaaaacttattagaagacttgaaataccaagctacaccttctgtagagtacaatcgtgagtttattgagtactttattgatgtagtagacgggaaagaacctgtgcatcaaggagcacaaagtcaaggaacccaagctccacaatttaatcagcaaccagtacagcctcaatttaatcaacagcctgtacaaccacaatttaaccaacaacctgtacaaccaatgcaacaaaatactggttggtcgccacagcaaagccaaccacaacagcctgctacaggttttaatgcaacgaacatgggaacacctccaaacattaatggagggtttagccaacaacctgtacaacaacctgtacaacagcaacaaccgatgggttctttcaatgaacaaccagtgacagacccttctaccatttctgatgcggatatgcctttcaatatgcagtccatgcctgatgtatcaccacaacaaaatgccgtacctgagcaacctgtgactaatacaccagagccagtaagccaaccagttgttaaccaacagccaaataacacacctagtgtagacgacctattagcaggtatggtaggcaacgtttaacaataatgaaacagttaggaggggcatactgccccttttaattctgtgttaactatccaaaatatttagtaggagtgaataatattggcaagaaaaagaaaaagtgaagaaatagattttggaactattgatttgacaaaagaggtaggactaactacatttacggacacaaagttctctaatgtatcagacagactaccaacaatgattccacagcttgattacattttaggtggaggattgccatttggacgtatggtcgaggtctttggtaagaactctagtggtaagtccactttagcagtccatctgacaaaggtagcgcaaatgctagatgtaccaactgtatggattgacgttgaaggtaccgcagacccagaacgcttagcagaactaggggtagactttagtgcaggcggagtattcatggtagagcctaaacagaacaaagacggtagtaaagatacaatcacggtagaacgtgtagcagaagagttacaacgactcttaccagtatttagtaagcttggaaaacctgtattaattatttgggactctgtagcgcaaacagcttctgagaaagagttagaaaaaggtgtaggtaaccaacaaccgggtttgtaataaagctccgttaggtagtaatatctaaaagaaacctatctttatcatgggaaacctctaggaggcaatcatgagtgaagctgtagaaatacagaacatgcaacgactatcgaaaggggagttcttgtcgagaggacatgaatgagaaccgagtagagtacacccaagtgggtggaaatggtagggctcctagagtaacgactaggagtaagatatagtctgtactacatggtgacatgtagcagttcataagagaacgctataagcttaacgaacttataggaacataatagattaaggcaaaagcaatggcacagtttgctcaaatcattgcacctttaatgacaaattcaaaagcattatttattgctattaaccaagcacgtgacgagctaggtagtatgtttggtggagtagactctcccggaggacacgctttacaccactgggctagcttacgattagaagtagttaaagcaagtcagattaagaataaagagctaaatgcattcggtgcagaggaagagacctatgtaggacatatcctgcgtgttaaaacagcaaaatcaaaagtgtcccgtcctaaccaaaaagcggaaatgtacttaatgtccgacacaggactgaacttagaggaaaacatttatcgttcatgttttgcaactaataagcagtatgccttgattagtggaggcacgtggaagtcttatacaacggatgcagggcaagagattaaatttaattcagataaagcttgggtagcttatttacgttcagaagagggaagacctgttcgagacgaactatttgctaaaatgatggtacgctcattcccacatcgttatgctccatttaataatgaggacgtggatgtatgcaaaattccattatatgaatttactaaagaatatatggaaaatcataaggaacaacctaaccaagctactaaagaagaagtccccgaaacaggaacagatgtttcagatttacttaaacaggtagactaatagataagggggcatttagcccctttattagctataaaggagaggaacttattttgcgcaaaggactagcacctaacccattttttgaaatattagaaaaacatcaagactcctctaaacgtactatgactatgaacagcagtggtacacctagttcactacaaccaataagagacatgttcttaaaggcaatgagagaaggtaagaaagtcctaatagagaactctgacttaagtagtgcgaactctgttgttatagagatagaatatgtaggtaatcgttggtgtttaggttatcaacgagtcttattttatggtatggagttaaaaataccacacactatccacttctgtgatgtatatggagcctatgggcacgatgctcagaaggttaagagacaagttaaggtagtgtttgagggggacaacccttttgagtagagatgttcaaaaagaggaaaaagaaatacgtaatggtaatcggtttattacagagactcatggcaaaggagtgtttcctagagatgtagaccgattgtaccataagtatagtaatcttagatataaagtctataacactcataaagactcgttcaatagtgaggcttcacgtaaggagctcaagagctatattgatgagcaatttataaagttaacaaaagagtatgatataaatggagaggtagactttccgggatatattaaaaaagctctgaatttacgagtaaggcacagctatgtaaaaggacggttccgagataccgctagagaacgtctaggcacccaagataacgaagtagagttattgttagggattgacgatagctctcaggcagatattgaggatgcagaacttattgaatcgttattatcaaaagccaatttttcagaaattgaattagcagtatttcagcagttaattcaaggaacagtaagggatgctcgtattattactgaattgtcagaaaactacggggtgtccaagaaagccgtaaaagatgctataaaaaatgttcgtgagtttgtcttaataaatttaacagattagagtaatacctcctttatgtctgctatattagcagtagaaacataaaggaggtattttttagtggaacaaaacaacactggcaagtatgcaccatttattcgtttaattgtgatgggaatctcatttgtggcaactggtttgactacaatatttggttgggaacctttaccattcacagacgaacaaatgaaccaaggtttaatgttagtactatctgtaggtcttgccatctacaactggtacaaaaacaacgctgtaacttcttatggtaaagcaaaagaagaagcaggaaaagaagtagtcggaactagacaagacttcaaaaacagagactaagtacgaggggtgtaacccctccttagttaatacaaaggagcttcgacatgaagatagacgagataagcaaattagaattgcctaatctatttggaaaattccttgtggtagagactatttcggatgggtacactggaaccgtatctggtcactataactacgagatagaccaaaaatctgaggaaacttatatttaccctgtattttggaatgataagcttaacaaatttattaggtcagatgaattagttgtatacactaataaaaataaagtatactatgtttgtaaaacaactatagacccatataatcatgcagtagtagatgagctcacggtagaggaaggcatggacaaagacaagcgtacccttcaagcgtttaaactttttgtaaatgacctattctcatttggtagctacaatatctttctaacaggtaacctatcattagaaaacaaccctgatattgttctagttagcagtgtatcattagacaaacagaccgctaaaatgtacacagaacggacattagaactaactgctacggttttaccagagggagctacaaacaaaaaagttagtttctcagtagataaaccagagcttttagggttaacagtctctgacaataaagcaactgtcacaagtaaagataaggcaggtactgcaattgttaccgtaactactgaggatggagaacacactgataagtgtacagttcagatagaagagtacataaaagttacaggaattaatgttagtggagaatctgctttagaaaaaggtaagacatacaaatttactgctagtattgtacccgataatgcaacgaatcctaaatttacttggtcttctagtagtgataccatagctagtgttaatgcaagcggtgacgttgtagctttagcattaggtgaagcagacattatagcaacaactgaggaaggtagccatgtaggtaaagtacatgttaccgtatcagacccagaaccagtagaaccaactgaataacatagaaaagaggaaagaaaatggctaaagaaatattaaatattgaagacctgttaaaaccagagacactagaagtagcaatagatggtaaataccttattgtaccaacattgtcggatgggtttacaggtacagtagcaggcggatatgcatatgctgttacaaaaaaaggaacagactacacagttaatgaattaatctataatcaaaaggataacacatttaaaccttctgatgaaccaattattataactgatgataatgaaatattcttcattactcgtacattagaagacccatataactaccctgtagttgctacagagaaacttaaaactaaagatgtaaaagaaaaacaagttttacaagcgttcttagcatttgctgatgacagatttaagctaggtgtttacaatgtgttcctagcagatgaaccatttgtatatggggacaaaacagaatagtttcattataagagacccgttaaggtctctttttttttgtatatagtgttgacaatgttgtagtttagttatatactatacttatactgtataaggaggtaaccacatgaacgacaataaggaaaaatgtattaaacaaggaatacgagatacttataaagggtacgatattttattagatgaagagaatggatttttctatgttagcgtacttgacccagatggcaaagaaatcattagtgggtttgtagaggcggataaacctattgaagaatactataaagagctcctaggtaaatgcgaccaagatatatcgtttaaagaccttttagggttcttaaatggacgtagagacactgaacgtacagacatacgttttttaaagagagacagtggggtataattaaatgacaaagataaaacttattacaaaaaagaacacccaaggctatgtcatgaacaccctgctacgtagattttataaaaataatgtagacgtagaatttcttaataaattcaatctacctgatattcataaccacataggggagcatgatgctgttatcatagtagggtttcctttctttgaaagccaacgaggtgcgttagacacggcactgtcatctatggacaacccgtttagcaaggtgtaccatttagcaacatttggggacacctatcgtaatgaaggtagctttcgttcatttgtagacgaggttataagccccgttggtcattttgtagaactaataattgacctaactaagttcactaacacaggtacaaaagaggatgaacaaaatgtagtggctcttgctaaagaggcattagtgtttgccaaagatattatagaagagacagacaactacaatcgttatgaagttacagacagaactatctcttgggttcttcttgtagatttgcttggagagaacctatataaggtgacagagcctagtaaagagctagacaccattttgaaagaacaagaagtacttgtagatgccttgaacataaatatgcaggactatgtgctaagaacaatagggaagatgtctgcaaacgtcattaatggaacagtggtttgtttcggttatgcagaacagcatgtcaacgaagtagcccataaattaattaatttttataagtcacataactatcaaaaagttattgtctttattggtaggcacacaaaaggtgacgacatgtttagtgtaaggagctatggtgtgaatgccggagaggttgtctataaagttcataatggtaaagggaaagacacaacggcaaccgtcttcttaggtaaacctagtgaagctgtaaataacacactgctaagtgtgctttctgaaattttatagtttaactttgtggtataataaagatagataaattttgataggagtgtaaatttttgaaaaacaacgaacctttagagaagttattagacaaattagatgaaccaagaattttacaaacaattattataggtagtttacaacggagctttaatcgagtacacgttggtaaatttaataaactagcacaggagtttgacttagataaggagaacctgtatagcttaaaggcactagttaaggaaattgaagaagataaagagttacacgaactttacgaagctagtatggcaggcaaaattacgctagaggctgttcgtaaagtattgttacaagatgataagtcatcgtttgatgtactgtcttcttacgtagtagaaaatcaagcagtgctagcccgtaaccgagagttcggtaagttacaacgtgagggagcttatcttgaccatctaattagtggtttgaagacatacttattaactgaactaaaagacatgtctagtttaaaatatatcaataaaaatttaaaggcaccgaaagtatcctcagaccgagagcttattctgtgcctatctgattggcatattggtgcttttgttaataacattgacacaggtggatacaactttgaaatctttaaagaacgacttgaaaagttattagaagaagtattccaagtggctatggagcaggatattaagaaaattcatgtttaccatattggggatattattgaacacattaatatgcgtaatgttaaccaagcatttgaagcagagtttcctgctacggagcagattgctaaaggaattagagttcttgctgatacactcaatttactagctaaggcagaatttgaagtgtctttcggtatggttggtggtaaccacgaccgtttccaaggtaacaagaatgataaaattcataatgataatgtggcttatcttgtagtagaccaacttcatttcttacaagaattaggggcattaaacaaagatattaaacttgtagacaacagaagtgacgtttatagttttaaagatacagttgcaggtaaacgtattaaagtaactcatggtgacactgagggcaaaaaagtggatgttaaaatccctaaacatatcaaagatgaagttattgactatttaatcatggggcatatccatacaacacgtattattcaagaagacttttcaagattccatgtgtatgtcggctctcctatgggggcaaacaactactcagcagagaataacttgccaacaacaagtcctgcacagctaattatggtattagaccctgagcgtgatacaccgcagttcatgccagtattcttataggaggtactcgtatggaaggtaatttagtttatattttattggctattgcatatgtaggtgaaggtataactgcctttactaatactaagcgtaaagaaagatacatgattgaagaaggagaggctcctttgccacgtagttcttatgtatttttaggcattaactaccttttaagaatagctatagcaatttctcttatcttcatcataccaactagcttgcaacttaacgtaacaggtattgctttgttcacactaatggtatttgtagttccttttatagcaagaattatcgaagttgttattagaactgcaattgttcgttatgttcaaaaacaatatattaagcagttagaagaacgaaaaggtaaaagagagactaactagtctcttttttgctatattgaataatgaggtgactaagtatgaattttacagaagtaataagccctaatggggagacatcattaatagatgtaaacaacccaccaacattaatcagacgtggggtcttatctattaaaacaaaggttaataatgaagtgaaggaaactcctgtttatattgttgaactagccgaggagctaacaggtactgatgtagtatctgtctataaagtaaaagagattggagattctatccaaaaagactacattgaagaaaaagtgacccctaggttcaaaagcacaacatatctgggtgagttagcacaaaagattaaaggacggtcgataaaggaacaacgaagagttgaaacaaaaccaccattattcctagccccagtagttaatggaatcgatacattcacaggaatcgaaggtaaaggtttctacgaacgtgaagaggacagacatattctattacctgatggaaaaccgggcatagcctatggagataatacaggggtttttatcggtttgagctcgattaagtgggacaaggcatatgtagacgtggagtctataacaaagggttatttgtcacagaaacagatatggtttaacctagatggtcaaagaccacaatttagaagtgagacactataatgacagataaacaattttatgaggcagatattcaagagttaattttaaataagcaaagaatattcggggatataggaaagagcgctattgtttttgagaaagcaatcatgcaaggtaacacaatatgtgattgcctagtcttcacagaaaaacgagggctcattggcatagaaataaaaactgaacgtgactcgacaaaaagattaaataaacaattatctgattatgaaaaggtgtgcgactacgtatatgtattatgccacgataaccatgtacctaaagtagagcaaatacttgctagacataatcataaacacgtaggtatcctagcttacacagagttcatgggagaggcaatgttaggtgagtataaacaacctagccgttcccctaaaaaatcagcttatcatatgttaaatatcttgtggaaagaagatttaataagaatgcttggtacattcagacggtatggtgatagactagaagctaatggagctaaggttatgaaaacaaacagccgttctggtggagtatctggactttatgttaaatctacaactgctagaagaatgactaaacctgaactcattaataatttaataaatagagtaggcggtaccgaagaggctacgagagtgttctgtgatgtgtttatccataataggaatcacccagagaaagcaattaagttaagacattttaaagcaaaagagaataggggtgacctagatggggtttaaaggtgcaaaatatggttcttggaatactgtagttggtaagaactatgtgggtactgggggcagaacaagtggtagtaacacaaaacggctgtccacaaaaggctactaccaagtaggatttgttaaagaatatcagaacttgacagaaaaagatattatgttaaaattagagtatggaaaagacttagtgtctagctacactggtgtacctgcagatatgattaagctacgtaaaaagaaagaggagcaaactctagcatctttagacacagtttattatgttagcattggtaaggaacctgtaggtaagctgtctatacgagctcagagacgttttagagaggtagggttaacatttatatacctagagaagaactacgtacagaggaagcttagaggcggtaatgtacgtagtgtaggatatactaacgcaaccaaatctcagaaacgtaaagcagatagacggaagggcaataagtctaaaacaactagatagatggaggactactatgagtatttatgatgagctaattggtaaaagtgttatagccctagaatatgcggaggatgggtgtgaggcaagccttgtactaaatgatgggtcatgcttaaaagtatcttgtaacccagagccagactgttgtgggtataatgattttgaagttattctcccagatggttttgatttcacagataacattattacaaaagttgaagataatagtgaagaatgttatggcggttcaacagttaggataggcatttttaccaatgatgcacggatagttattgaaggggactacggaagtggttctgggtggaactatggagagtatgtagacgtagaaattgtaaaataatttactattagatggaggtaagctatgcttaaaaaagggaaagaagtaacactaagaaaattttataatattatcacagataaggaatcagtattgctaggggcacgctacacaagctcaataatgactacagatattcctattacaacaacttttgaagatgttgaggtagaccttaagaaagaaacagttgcaggaactatttcattcagaccagtaggagaaagacagattaatgcattaagtttactaaaagaagcaagcacagcttatgggggttacggagagttcctagatgatactattgagaaacctttaatcaatagtgattttgcagtagatgttagcctagcagactctgctttctctaacctacaagagattccatttaacctatatatgtcctccccaaaagttttttatacagaagtatcaattagagggcgtaaacatatgcaatatgtattagaggatgagtcttctagcggtgtaacaagtacattagcactggtattccgtaaaaaattgtatgatggggaaacattgctaggtgtgcatacttacaccgaagcactagcaagagtagagggaattaaagtgttacagtttatcgcaaatggctctgtactagaacaagtaatcggtgcagtgtctgttttagggggtagcacaggaacaaccctgttccctatgtttgacgatatggtgatgcaatttgtgatgattgagtctgttccttgggtgcacatttcttgtgatacaggagcaattgcttttaaggaagaagacatccgcaatgtaaccattaagtcagctagaccgggagaatataaggtgactatctacttgctagacgaaaaagttacattgttaattggataaaattttaaaggaagttgacaatatatgttgacttccttttttgtatgtgctaagataactacagttggataaaaaaaataaatggtatagagggagagatttaacatggactacaaaacaaaggtatatgtaggagcgcttagttggttaggtactttaggagagaaacgatatttagggcaaatgcgtgatgtattagctgtgtacgagctaggtagtcgatacgcaggttactatacagaagatagcgactatgactatatggttgtatacatgccggctccttatgatttaatgcatcctacaacaatttataaacaggaaacagagattgatggaaataaggtagaggtaaaatatatgtctatcgtggaatatgtttaccgtattgaaaatggagatttagaggctttacaaatgttaaatgccacaagctcccaaagtttcttcggagagcctattgaaggtattgacaataagcgtactcgtttagttacgtatatgaaagaactagaatacagaagagaaacatttacttatttagcaccagagaagttgtttagaggaattaatggtcgtattaaagccacaaaaacacgtatggataaggctattgagaatgacgatatggaagtagcggtaaaatgtgctatccttattcgttattttatggacttattagttgtgctagcggacggggaatctattcgtgaaggtctcacgttctctcctattattgcaaatatcattagagagtttaggaaagactgtgagtcagcacaggctaagacacttatcaatactgcacaagtgctattagaggcggatagagaagagattttaaatagtattaaagaccatgggttatcagatggttacgctcaatcagttagacaatatagtttaacaggtcgattgatagatgtactattaggaggatattatgactaagttagaacaaaataaagaaatcttagatatatttaatagaaaaggaaaagtaacagataaagtagaagaatctgccaagattatgctagaattagaccacgattatgactttggtacaggggacattgcttatacagagcgtggcacagataagaagggacgtttctatttagaaagtcgtttgtttattcataaactcatgccctatgggttcattttaaacgctgtagtaagtaaagtacactatggagaccaagaggagaccttagaacgagaggtatcccgtgtatatgagctagagtacaacctaagagataaggtagctgtgctaattaagaacggtaaaccactaaacttctcagaaaataacattagtaacatgttttctgggcacgtagcacagaatattcttgaacaattagatacaatgtctggttcagatatgtatgtatctgtgtatgaacgagttagtcgagttaaggatgaacaaattggtaaagtatctcggttctttgatagattgatgaagtacaacaagattgaattaatttataagagtggcgttcctgaaggctttgctttggcttatgcttatcgagtagttgttgtaggagaaggcaaagtccgtaatgaatggtacgaacctgtaaagagtgtggactatttagataaggaacaaacaaatccggctaaacacctaggtattccaaagtctatctttaagattatttgtgaaggtgggttagagtggacattctaccaaaaaatagctagtcgtttccataaatcattagttaacagaagtactaacaaaactcctaaatcccccactgctatgaagaagatagagaaagagattgctaagttacaacaagcctatgctcgttttggcggggtactgtataacctttatcagtttactaaagagctagatgaacaatatggtatctcccatagtaaggatattatcgaaacagagtgggaatctatatacgaccatattattgcaggagtagttaacgataactataatagtacaactgcttatgatatttctatggttgcaaacctagatttctacagaactgttcgttatctatactatcgagtatatgttgagcaagggcttacttcacaagcagaggctagatacacatacagagactacttgagagcacaccattatatgaatgcggtacctgttaagtaccctaaagctcttaagactgctcatgacattattattatgaattaccgaacaatgaaggataaggtattgaatagtaactttgaaagtagtgtagctaaatataaatatttagaagaagtatcagttagaggtggctatattgttaaggtacctaatagtgtggaagacttaactaaagaaggttctagtttacaccactgtgttgctacttatgctcatcaagtagcagaaggttctactcgtatcctgtttatgcgagataagacagagccagatactagcttagttacttttgaggtaaaaaataataaactagtacaagcaagagggctagttaaccgtgacttgacaaataaggagcaggagttcctagacaaatggttagttaaagcagaaattggtaagtattagtttgcctaaaaaggcggaatatggagtgtgtatagaccaattcacaatgaaaaaagtacactaaacagttgttatttcattattaggtaaaacaacttattttagatagctgatattgaccaacaaatatttcataatgatttagctattaaagttacaaaaaccctactaatacgtggggtttttgcttgtttcaattacatatgaaattttacagatgttctgctatattagttacagaagctaataaaacaaagggtttcgacccttaaaaatgatatttcatataattaaaagttgaaggagtttataactaaaatggctaaaaaagaagtaaacaacagctcagtattactgaatctatacaataataaattgcttgtatctaaggtagacgaggcgttagacgagggtaaaccatacgatttcattattgctttttgtaaagagaagttcgattttgaaattaataaacctgcattatctaggtacaaagagaaacgtagagagtctttagaaacaggagtagacttggaatcactacttgacaaacgtagaaaatcaggtaaaattattgatattaagtctaaagaggtaaccccacttcctaatgaaacatacgataacacatttggacaagtggaacagatatacaatgatgtagaggtgttagatacaatcatacaaaaaggttttaactctctaaaagaggtagactatgttgaagccccacttgctatgaaagcaattgaagtaaaagctaagataacagctaaccagttccaaggtctaagtctaacaggtctaagagagctaagattaagacagtctgctaaagaacaagcaatgactgagattattctacaatttattccagaagaacagcatgaagaagtattcaatgcaattgaatcagcagagaaagagttctatgaaaacttagatttaacagaggaagaccaaagaatcactaaagcgttgcaagcatcaggtatggatataatttaggagggctataatggttgaaaatttgagagaggtaaattataaaacattaaccttagaagaaagtttacatgcattacttgaagggaagacccttattgtaaaagggctagaacaaagacgtaagttagatgtgctagtaaggattttctcagaaggtgttgtacctgttacgcagataagttatgatacaacccctgcggatggttattggagaacaggatattggcagatatacgatttgccaattaatgcccttagcacatacccatgttttatctatgatgatttaaatacggatgaactccctaaatttatgataggggacactgtttactacacaagtaaagaggactctatcaaagattccgccattgtaatcagtgtgtacaaagacgatgttaacaataagtggtactacaagttaagtagagacaacgaaatatatgcagagagtgagattagaagagacaggttataagcctgcctctttttttttaaatttattgttgacaaatatctataactttgttatagtataaatatcaaggatattgataataaattttggaggtgccatgatggcaaatattttagacacattaaagtggttagataaaggggacaaagttactattgaatttgataaagagcggtcgaagtatgcaaaactgactttgcacgattcatcagctaagacaaatattgtccgtaacattgttttttatgatttagacaaaggagtgtatgcttacactggtgaatacacccctgtatgggataacttattagatgatatgcgtaagacacaaggcgcaggacctgaaattaagactacaaaagtaaatcagttagctacctatgaagatgccttaaagtttattgaaacaaatggtacgttttatgtaattggtgaggaagtaattgttaaggttaaagatgcaaaagagctagcattgatgttaatgtactttagagatgctattgaagaactaagaggagaatacgaccctaaaaaacatcatgtagatatgacaattgaattatcaaaagatgttttgaaaaaaatggcagtacctagacatgaattagacttatctttaggtggcttaatgagagctgtatcacataatgttggagaagacctttttgaaactcttgggtttgactacatgaagcaagcttgggaagtcttagttaattgcttgtcactagacactatccatgaggtacctttccgtgtgctagacgaattagagaaagtaacagatagcatgtctactacagaccatattgttaccttgtatgccggtagagaacttaaaaaattctattcagaggaagagtactttgatgtaatcacacacaatttagctgatgtgattatggattggtcaactatttttactacagctgttcttaataatacagaagatgatgaacaccttaaagagttacagcttaactttgagagattcaagctagatgtagcagaggttctattaggtaacgttgcaagacatttactatatgcaggagttaccgatagctttaacgaagttaaccattatgttgtcggagcaggtaacctgattagaacagaaggtttgattagaatagaagagttaactggaacattagacaaccctaaagatgaagatagttctgaaacagataataaagagttactagatgacatctttacaaatacaggtgatgatggtgttgaagactttacaaaagaagtagacgagcttgccatgtttgagaacgaacatgctgaggaacttttggaagtcaataacaaattaaaagacaatcaagagttattacgtaaaactgtggaggcgatgggtatggcttcttactctactattgattcatcatttgaacaagaggaagaaacagatagcaaccacacagagacttgtgaggataccagagctttccaaatgttaagctatgcagtacgttcaggagacaaattacttgaacgtgtagagaaccacccacaaactgaaaaagggttgaaaatggctaaagattctctaaaagagtttgaccatacagtgaaaccagaattagaagcttatttaaaagcagaagagctagcggaagacgttgatagacatgcaattgtaactacaattatccgtatcaaggacactatggaagcagatatggacggctgtaccgacccaatagagcaaggtttattctacgcaggaagcctaaatatgttagaagaaatggaatcattgttacgggctagcaatagaggttatggttgggacgtaacagctatctatcttatcttgtccattgaactagcttatgggacttacgggttgtctgatttagactttacaattaaaaataaagaggaaactcgtaaagaagaacaagatgcaattaatggtattgtaaacttcttagccaatcttttaaatacagtactagaagaagaatcagaatcagaagaaacacctgtagtagtcgaagaggaagaagaggataaggatgacttctcactatctacagaagacactgctaagttattggcagactggtcaaatggtctacctacgtatgtcgttactcgtaaatacggaattagtatgggagctttatactctatcttatatgcaaatggggcagacgttaaatcttctaaagtagcagaacgagtggctcatgtggaaaatgacaaagatatgttaaacgcagttattcgagactacaagaatggtactcgtttagtagatatttatactaaatacaaattatataaaaatggtttgttctatcttttagataaatatcgagtgccacgtagaggacgtacaaagaaataacaatgattaaggtagtggtgctcaactactacctaatcttttattagggaggaacttaattgattctttttatatttagcattattacaatgctatccatgttcttactatatttgtttgggatggcttctgtggctgtaatcaaagtagggtttcttataggtagtcaaaacgatatagctaaaggcatacactctttacttttcacaggtattgcacttactgtagtcaccggaataactagacagtgtttactattattttaaaaaaaattggaggatttagcatgttgttttttattgttttagcagtatttataggcgggcttgctttatggggaatgtatgatagttatgggtacctagactggacttcatggttatttagtattgtggtaggctctgctgtagctacttttttcacactagcggcggttggaattactttcgatgttgtaccaagtcatggggtaacgaaaagtcatgaattacaccctatctatgagaacagtaaagtagttgtagaggctaaaaaagaccagtttgagattaacgtagatggcggtttggtagctattgatgcagaaggtactactatcctatctactaaaggagaggttaagcctaaaattgtgtttacagagaactatataaacaacaactggtggactcgtttcctaggtatagcaggtaaggtaaaagacacttcatcagttctttatttagactcagataccttagtgtacaataagccggaaaagaacagtagcgcaccagatttaaaaattaaataaataatttagaaaaaggggcttgcataaagtctctttttatgttaatgtgtatttatagataggagggctactatggaaggtgaagtagtatacttagatgagtttatgaattttttaactgatagtggaataaatactgatgatattaacgtagtagatgatagacaggagggctagtatgtcttatacaaaagaagcattagaagctagaggctatcagtttgacaatatgtctatgatagataagatggatgccttgttagaactgctagaggaaccagaatttcgagaaaagatgaaagaagagtacgcagagttctctaagaggcacaataacgatgaagaatgaaaagttagagtcttaccttatgaaagagattgcacctattttagatgaaatagagatgagtgaagaattgataaagggaatggagaacaacaacccatccgatacggttacagtctctttttccaaagaagaagtagacatactcttagcaatgttagaccttgaggtacctagattagacagtggttctgaattgtttagccctaatctggtaagggaagctaaactacaattaattaagaacaagctaacttcaaaatgatttctcactagaattaattagtgagaaaaaaattaaataaagctattgacaaataacaaaacatgatgtaaactaagtttataagataaagaagaggagagatacacatgaatgaacaaaagaaagtatatgcaaaattaacagaggacgaggcagtatttgcttgtgaactaggagataaaattaaacaaattagagagagccaagagctatctcgattagaacttgcaaaacgagcaaaagtagaccactcaacattaatcttaattgaacaaggtaaacgactaccaacattgcgtattatgatgaagttgagcaaagcactacaccgagaattagctattagctttacagattaaggaggaggtatcatgagagggagcctagattattacaactatttgtaccaaacaatcgaaaatcgacctacggaggagctagatgtcctttatgacggtctttataaaaaagccggtgacctgtttgcaatagataactttcaaggagttaaagaaggcagactaattttaaaaatattaaaggctattagagaagaaattaatagtagaattgatgaagaaattgacctttacttgtataatatctatgacagtatatcagatgaagacaaacgagtaaattggctatatgaggtgtaggtatgtttagtgttgttaaggctgacagctatgttaaatcagacatagaaatgtatgaatttaagaatgtaaaaagtttggcattgactaagaaagagaaagaactatggacaggcaaaattgctaaatatgttaatgagtttattgtaaatgcttatggagactaccatgggaataaaatacctgaaataaatgttgtaatcaatggtaagctaagaagaaccctaggttcttttgtccaattcactaacacaaacaaacactgtatagagataaatggtaggtttgttaaagaagttattctattacaagaaacacccttagctcaaagagcgcttgatattttaatggatgtagccagacatgaagctatccactatacactttgttatttaaatagtttaagtggaggagacctaccaacgttcaactaccatgacggtggggaggactttgaaaaagatttatgtttgacaggaacttcacctagtggtgctacgaaagaagagtatatttatagttcttttacactaggagccatcagatgccgacaccatagtacttgccctgaatgtgggttggaaacatacatgtatacacgaggacggtactattgctataatgggtgtgtaggggataacggtagaaaaattatatttagaccacaaggtgatattgcaatttatattgatgaaccaaaatctaaagctaaaccaaaagtagaggaagctctaaaagactataaaggagcgttaaagctaccttatacaggtacggaagaaataaaataaaaaaaatagttaaatgtattgacaaataacaaaacatgatgtaaactaagtttataagataaagaagaggagagatttattatggcatacgtaacaaatattgatgtagtagcagatgggttagatttgtataatgggaactatgtggtagaacgaggtcaagtagttacttttaaactacatgtagcgacatggaacaatgagcctacacccgaaaatgcttatgcgattattcgtaataatggggtagattataagagtaaagttgatgaatttggcaatgcagaggttaccttcccagttaatggtcgtcctgaccaagtaacaactagcatctttgcattaacttctggatatgagggggatatgcctcgtgtaatgtcagctatctttagtgacgaaacagaaattaaacaaactgtaatgaacgttacagcatctattaatggggagccagttagtcgtgaaggtgtatttttagaacgagaccaagtagtcactgtagatgttaaagcaacattatctacaggtaagttctgggaaggtgcacaggtaggtgtgtacaataacaacacggaatacttaggtgacctagatgcagatggttatggttcagtaactttccaagtaaaaggaaaacaagggatggacacatcagctatctacgtattcgttaaagaccatgaacgagaagctacactaacagttcctgtgaagtttactaatactactgttactacagaaacttctacagaagaatcgtctactgttgatacgactacaggaacagaggagtcttctactacggatacaaccactgtagaaagctctacaacggattctacgtcctctacagtagattctacagaaagtacagtagaaagctctacagagcaaacagtgaccaatgaggacacttctactgattcaggagtagttgaaactacagaaacttcccaagtagcaggctacacagagtctacttctagttctacagagtctaaagaagttaaggaaactcatactagcactacagaacatgctaaagagttaccatctacaggcacagaggtagactatgggcttgttgggttcggtggtgcaacattaacagttgtggtggcactagtagttaaaaaattgttgaataagtaagaaacacaatattgcgaccctcattaattgggggttgcaaattatattattttttttaaataaacctattgacatttaacaaactataaggtaaactaagttcataagataaaggggggaaacaaatgagtcaagtaagcaaacatggagaaaaacgtgtacgtgaacgtgtaggagtgaataagagctctgtagaccgacaatttgagttagctttagaacgaggatacagacaaaaagagctaacaggtcgtctaaagaaatgggtagtatcaagagtatttaactctaagtaccctcaaacatgtattttatataatggtaaatgcttcattgttagcagtgaaggtacactagttactgtgttaaacatcccaagtaatttactaaaagattttgcaaaattatctaagaaaagaggaaaataaaatggatattatggatattgagtttttagaagaacataaacaattagtaaaagaacatgtagaacaagaattaaaattaatgcaccctcttaagaagttacaagtaatgacagactggttaggagatacagaagacaagctttctcaaggagacttagattacttcaatgacttaacagaaacagagctaatagaggcaatggatgctagtgaaattgtagagtcttattcagatgtcttgttagattttattgactactacaatattgatttaactggtttagaggaacagctaggtgtgtaaccatggataaggctgaaaaggtagataacattgtaagacaggtcacaggggctgttattaagacaactgcaaaagtagcttttattgtttttgttttaacctttgcaggtgttttagtaggttattatagttattcatttttaacaagtgcagggtggtttgccttacctatgatattatcagtagatttgctatatgttgcggtactgttaggcgggctagcctttatatttgcagaggtctacaaagtagttttagaagtgaaaaagatagttaaacgaggagggcaattatgagtaataaaacattagaacaaagagtaatagatgctaacaaagagataaacgataagcttaacgaatcatcaattattcgtaaacaaattgaagaattagaggaacaggaagccatcttactatcagacgtagaggacttacttgattacttagaaaatattggagtagacctataggagggacttattatgaataaaaaagtagaggaaatgacaatggaagaaaaagacaaagcactaattgcaatgggacttattgatgtaacgcaggaggcagactgggtagtattagctacttgtgaagaatgtagagaagagtacgaaggagaggagtacgaagaaggggactgtgcagagtgtgaacattgtggaggagaatactttatgattgagacagctctcgagggtactcgttgtggacgttgtgatgactactttgatatgtgggacgactactttgagtttgagaatgaaggtaacccatataaagataaacatatctgtgaacattgttatgaagaactagtatctatgggaatggaagagaaattttaagatactactaagaaggagacttaatcatgaacgaattagaagaacttaaaaatacactgattagacaaaaactttcaatgttggagagttacgaaatgagagaagcatcattttggataatgtttaatgggatattacgtgtcatcatgtcagtagctgtcatagcctttgtaaactatgctaagcatgtaagaccagataatgtagccacatggtttctagctctgatttgggttattttcctagcagaaggtattaaaggtgcttatgatgctgttgcatttggtattcaccgcaaaaaatttgctaaacatattaaaaatatgcgtgggataatcgcaatcacacaattacttattgaagaagacgaagagaaattaaaaggaggcaagctagatgagtaaagatgagaaattagttgagtggtttgaagttgccttaatggtgattatgtggttgcttatcacgttcagtatcttatacacaatagtttccttacctttcatggtacacgaaggggactggctagggattgtgcgaaacgtactactggacattgtagtattggcaattggggttgtcgctacatggttgcaattaagatttaaaaaaggaatggaggaataattaatgggatatttagagagtgcaattgaagaaattgaacgagtactactaggaaataaaagtcgtgacaccgaagaagtttatttaaacaatgcaattcggtatatcaaaaaagagttaaagaaaaaagaggtagagccaacgtggttaaatgaaccacagacattgttccttaattggtttaacgaattatacgcagtaggtggtttaactcatgtaacagaggcagtaggttttttagaatccacaggaggtagaatgaagtatccagaagcatattctgctttcagtaatttaagtgagaatgaattgcttgaggtttacagtaaattttatacagggttattcttaaaagcacaagggggtgaattagaatgaactttcatggtaaagtatttcatgataaagtatttgacattctttctcgtgattaccctgattggcagaggtatcagacagagaaacgaccacatcccaatgagcttagaaaagactttgccattgatagtacagatagtagatatgaagagtatgttatgggagagtttaatgtagaaacggctagcggagatgttaaagtatacgcagtaggaattagaagagtagttcataaaaaagctgaggaggagtaaatcaagtggagtacacagagaaagacattaaagaaggtatgaagttacgttgcacagataatagtaatgtaggttactgggaagttgataaggtttacgaggtaacacgtaataaagaccttggcttagttatcgcaggggaaggtgaaaggagtcacagaaccgtaaagtatattttaggggtgttaaatggtgacagcaaaattaaatttgaagttgtagaggaaaagcctgtacgatttgctaaggtaacttgtgtataccctcctgatagaggtcttgtagaggttgggcattgttatgaagtgcttaaagagttccctacaggaagtgtgcgtatctaccttaatagtaaactagggaaccatgagttactcccagaccagtttgtctttgtagatgaaccatcaaatgatggagaaaaagacgtagaagagctagatgtagaagctaagatactagccaagattgaacagttaacagcagaagcagaacaactgtttgctaaacgtgaccgtgtaaatgagcaagcacttaacttaaatgcaaaagctcgtaagttagaagaatctttagaggtactaagggagtacatgtagctaagtgtttttatgattacatctattaaggagatgagagaatgatttattatattaattttttagaagatttcgcatcaagttggagtgcagataagcgttatcgtgttcgtagaattatgacaactggtagctacgctattattgacaactatggtcatgtcagattcagcagtgacacagcacgaggtgtccttaagaatatagagcaggagtatgccactcataaggttgagcttacactagcagaagaagaaacaacgaataagcctaggtttaaagtaggggaacgagtgaaagtgtctaatgatttacaggcattcgggatagaatataagactcacataacctctaagatgatgggctgtgcaggtaatgaggctactattacacgtgtttgggggagtaacgtacgctactttattaacatcgatggtatacaccaagattggtgttggacggaggacatgttagataagattgaagaagaacctacactatctattagatgtgttgaggcagttcatcccttttggacaaaaggtaaagcctacgagataaaccttacatctgatggtcgctatcgggtctgggatgacgaggaagatggtagcagtggcaaatccataaaagaactactggacgttatcaatagtggcggtaacaaatttgagctactagatgaaacaccctcagaagcagaacctaggctaaaccatgctatatctgacttagagaaaatagaagctaagattaccgctttatcagaagagtcttttcagctattcaataagagtgaagagttaagtactagagcaattgaactgcaagatgagtcaatagctttagaagaagcattgtatactattaaacaatatttataggaggagatttaaatgcgtaaaaatgtaatttgtagattagaatgtgtttcaaaagacaaagacaacttaggtgaatggactgtagataatatttaccctgtgtttgaatcagaactaggtaaagtatatatcctcgatgatgaaggtaccacttgttccagagatagcgtgtctcttattatctctagtatggctagctttggggtaacatttagggtagcaaaagataaagcagaagaccctatccctagcaatccacaaagcagtacatcattagaaatagttaaagggtatgaacacttagcggagtttatagactcattaagtagcaaccaacgtgtagtgtctcactcagtagaccctaactctcaatggcactatatcatttatgaaactaagtcagctgaattgggcggagtaaccctagaggaattactagacacactagtgtataatgtacatgttgtagtgatggaacgtagtaagagaacatatgagccactagaaaatcacacgtttaagtgggaatatggaacaaagaataccaaggattgggaaaaaattgtacctttattaggttgcaaggtgtttaatactaacctcaatagtaacagagggttccatattactattttgaaataaactgttgacaactactatagtccatgctatagtaggtacatagataaaaaacaaacaatattaggaggtagcatagagtgaaagaaacagaaaagaagtatagcagagagtataaggggctagaatttgaaattattatcacttattaccctgaacaagacatgtattttgtaattgtaaggaacggacagcaccgtacactaactaaggttacagggaaagagtggggaatgagccctcatacagaggaagctgttattgaggtagcacttgatacatgctacacctatattgaaaatcaagaagcgcaaaataactagattaaggagggactatgatggtaggagacttcattttatgggttaaacaagcatggaaagaaacattctgtattcatgactacacggttaaaggtgtatataaaacattagatagtcatgggtacttaaagtgtaaaaagtgtggaagaattaaataggaggacaacaacatgaaccagagacagaagactagacaagaaaataaatggtttgaggagcatgggtatgatacacagcaaccacgagaatgtattgagtgcggggctcctttaagttggaaagatgagttacagaaaagtcatggagtgtgtagtgagtattgttatatgagaagtgttgggctgtcgttatcagattttatttaaggagatgaaacactaatgtttaaaaaagataaaaaagaagaaaagacttatagagaaggagacctccttaaggctgtagggggttactacccagatgctaggttgagtttaggaatcacatatccattgtataaaaccaccaatgagggttggtatattatcaataacgaaggtagtcgggtaaccttaatcgaaatggatgctttaggcattgactacgctgtgatggaagaacccttattagaattaaaagaaggagacccattgctagtcgtgtccgaccttaagagaggtgttcgaggcttagcaggtgcagaagtacagtgtttaaacattaccggtgaaatggcttcactagcaggtacagttgttcattatgataaagatatgagccatattgcaaaggggctgttcactgttaaagagaacgattcttattggtgtgtagcgattgctattccactaaataaagtagctgaccctgattttgcattagagcatttgcttgctacgttaaataaaaaagcctctactaaacgtctggtattgaatgagataaaatatgatttaaaccttcttcacgaagagctagacgaggtgtccaacgaagtagagaagctaacaaaaaacattgaaacaatctataataacagataggaggtacttagatgagtatgccgagtgatttagggaaaacattaaagaaacctattgcaataaataagaatcctgatttttatgaattagcggtaggtggtaaagttatctacaacgaagaagtaatggagattgctaaagctttctctaataagaagaccaagtactacctactaaacacacgaagtaacaaacaagtatgtgtaccagtgtatcatgtaagaccttatgatacccaagtagagggtcttaaactaggtgatgtcctagatgctatgcacattatgacaactgtaacgttaagggcagtgaacaagcacgggtttgttgtcgatgaggatattattgaatgtttagtagatgacatcccagaaaatgcgcttattgttactagtgaggtatcccgtattcagccagaggattttggtaaggtaactattgactattttgtttagatatgttaggatagacttaagataggataggataaacttaggatgcgcttttgtttaggataggcttaggataagataggataaacttaggatagacttaggatagacttaggatgcactttggtttaggataggatgggggatataactatgagttacgttaacgagtttgaaacaattggagattggttagatagagaaatttatgatgtgttactaagagatgagcatgatattgaagaattagataattggggaatggctttgtttgcattaagtgaaggttacgttctaacagatggacttgacaaaccattcctagagttaactagagaagacctagtagcaggctacaaccactttaaagaagagctgaatgggtggttacgaggaggtaaactgctagaagtctctgataatttatctacaattcaggggttcagttttgaccatgacgatgttttattcttagaggataacaacaaagcttatgcaatgctagtaggtattatcattgaagcaagagacacatataaaaatggtttctgtaagggtcactatgtaataccttaccaagattgagttagccttatggctagctttttcttttaccctaagtagcaggctacaaaaatcttctaagtagcaggttgcaaaatcttctaagtagcaggttgcaaaatcttctaagtagcaggctacaaaaatcttctaagtagcaggctacaaaaatcttctaagtagcaggctacaaaaatcttctaagtagcaggttgcaaaatcttctaagtagcaggctacaaaaatcttctaagtagcaggctacaaaaatcttctaagtagcaggctacaaaaatcttctaagtagcaggctacaaaaatcttctaagtagcaggttgcaaaaatcttctaagtagcaggctacaaaaatcttctaagtagcaggttgcaaaatccggatgcgcccggctagcggtggggagtcaagccatgcgggttcaccttaatagctaccgtccccagattgtcggtttttcttactatatatagtaagaaaaataatttaaaaaaaactaaacttttctattgacaaaaaacaaaagctagtataatatagagcgtgtaaggaacaacaataataaaaaaaataaagataaaggggcgctattaaaatgaacaagtataaatttacctatgcagacattaagaatttaccagaggaagaaaaagaaaaagaattaaaaaatcggtgtggtgttttagcggtagagtgcttaagcactaaacagctacaaaagaaaaaacctcgatttatggttttcttaaataccgttatttttgatagtaccgcagaaacaggcggacaatacgcaacggcaaccgttaaaaccgaaccgataggggacggacgttttcgagtgtgtgacggttggggacagctttctaatggaattattgaactgttaaaataatttataaaaaaaatattgacaaataacaaaagataaactacaataaacttgtcagataaagaagggaagttatgaacatgaatgaattagaagcagtgaaagaatggaataataaaattgaggaacaacaagaagtgctaaacaaggttattgttgctttttataaagaaattgacttaaaggttaaaatggtaaaccgtggcttgctagggcagttaccagcttttaacgaactaaaaggaatgctatcaggtatcgagctaacagcaaaggttattgcacccgataacgtgctgcctattacaacccacaactttttagaatatttatttctaggggataacgaacaacgagcatacgcaaaagaatacctagacggctttttaaaatcagtagaataaggggaggaaaattttcctcctttacataaaaaaaagattgacaagttaaaagaaccatgataacatataaatgtagacaagggaggggctttacatgatgaacggactaaaaaaacttgtgaaagctaggcaatacaagaaagaagtaaaaaaaattatcactatgcaaaagaaagcaataaacgaactagaaacattaaacaaaaatttaaaattaattaatcaaaactattgacaaataacaaaagataaactataataggtttataagataaagagaggaagttattgacatgacagaacaacaatttaaaaaagagcatttattagaaccaacagaatggcgtagtgggggctacttagacactagtttaattgaccaatcacaatcttattatattgagtcacgtccgagagtctacggcgggtgttacgtttaccaatatgttacaatgaaagatggcacggtttacgagctttacagcatgacggcaagcactaggggaattgttgcacataactgccacgctagaaacgtattgcaaagagatgtaaaacaatacagagatagcgccattcattattaaggaggggagggctttcctcctttacatagaaaaaaaattgttttatctattgacaaataacaaactatagtgtattataaatttataagataaagagaggaagttttaaatatgaaattatctaatattattctagtggggttgcttgttagcgttgtactactttggggctaccttagcattatgatttgcttacaagtttttagagcgttaggcggttgggatattagaacgttaacggtttgcagtggtttgctatttgcctatgttttcggtttaaaaggaatttgggaacaagggacagggaaaaacaaataaaaaaagtttataaaaaactattgacaaaaaacaaaatatagagtattataggcttataaagataaagagagggagttataaacatgaaattgaacgttattcatttactattttgcttatttcaagaacaagaaagctattctattttaagttacgaatcagtagacgaattttattctaggttaggttatgacttagagagtgagtggctacttagggacttaggtattaatggaacaagtgacttggtagagttgctaacagattacaataatttattagagaatgagataacaaaagcagtcttttctgataaatggttataatttaaataaaactattgacaaaaaacaaattaaggaggaagaataggggaaacggggagggagggacttcctccctttacatagactaggagggcttaaaatgacaacagaggagaaagcactaaacattgcagagaatagaggtataacagattataaggttagggggaacgtattaagctattatactagctacccgatggaaaaatgcacataccttgtaactattgacattgaaacgctagaagaagaaagaaaagaactcaaaaaatattataaaaaaggcttgcaaaatgcttgcttatagactataatataaagaggggtggcggttgttattaataagagaataaaaaaattacaatatgaaagaatcagaaagctagaaaagagaaaaagaggtgaaccacctgaatttattttcaacggtaactattcattggaagaaatagagctatttttacattttagaaaaaaaagtgagggcaaaaaatgagcgtggtggctttgcttggtttacttgtaaaaattacatttatttttaaattgttagcagataaaaaaagttaatcaaaactattgacaaataacaaaagataaactataataagtctatcagataaagagaggaatggtaaacatgacaaaagcagaactacaatataaaaaagcaataggagttgcagtctttgcaacaagtggaaaggataaaaagcaactaggaaacgtggcaccgtttagcatttatgagattttagaaattgacttaaataaaaatcgggtatattatgctttaaattgtggggaacgacatgcagtatgctttactaaactacgcaaagaagaagaaacagggaacgattttattttaatcaataaacaaccatttttcttaaaagatatgcacaaaggtttaagttggtcaaaaagtttataaaaaaactattgacaaataacaataactaatatacaataggtttataaaataaagagaggaagtttttaacatgacaaaagaaaacaacgtatttttaaatgaaaaagagctaatgaaagaagttattgacactttagaaaatggctttgatggttattattgcgacttacatggtgagatttttaatcatggagcaaatgctgacattaaagacttggaagaatatggaatttttaacgcaattggagaaatacaagaatacgaagaagaaaattttggggaggttttgacagacctaggaaacccgacggaggttaccaatacgctttactatattaaaggtcacgagtttttatatggtagattagactttaatgatgttttagcagatgttgcagaggggctaaaattagataaagacttatggaacgaggaagccaccgaggaagtgaacaaggctattattgagtgtttaaaaaaagaagtgccttatttaatagattagaaaaacagggaggagtttcctccctttacatagaaaaaaaatataaaataagggaagtgctaaacatggaaacattagaaaaattcggttatacatggcaaggaatgaaagaagttacaaaagaagaagcagagaaaaacattaagaacggggtcggcacttttctattatatccagataacaacaattgaagcagtgaaagaaagaaagcaatgcaatattagataaagtattgagagcttgcaacttgttaccaactgaaaagaacgtgcaaacagctaaaaactttttagaagaacaaggctttaaagtagaagctagtaaagagttagcgggaaaataccttgtaaaattttcaatttaataataaagaatgaagaggggaagttataaaaatgaaactaacagaaaaggaactaaacacaattttaagagatgatgaaacagggaacgggggaacggctttcttaggtgaaacactagccgacttcttagaagaatcaggtattgactttacaaacctaactattttagaagtaaatgaattactagaaaataatggaattgaaccaattgaggtagtgccatgttaaaaaatatcaaaaaatcagataaactcactagaaaagatatacaaggtttttggggagatgaaacaaaaacattagaagaatggtataagtcaatttcaaaagaatcagacaccgaaaaagtagaaactgctaaaatgattaatacattgaaagaatatgcaaataacaacgaatttcatttcgtaaaaggagagcaaggacaatgacaaacacaaacacaaacaaccaacaatggaatcagaagtttaatgatggtactatgaaccagaacaaccaacaaaaggaagttatcactttacaagtcgcagaaagtttcgtcagtcagattttaacaaaagaatattcggtgattggtttagttattctaatgttttattttatgtttggcatgtttggcattttcgggggtgcaatctatattgctttcactcacacaaaccgtaaaatcggggcatggcaacaagtaagaagcgtatacactattaaggaggaacaagaagaatggaacaattaaaagggctaacaattagagaattgattaagaaactagaagaagtgccagaagaaaataaggacttgcctatttatacttttgaaaatgaaaactctttgcctattaaagatatttcattatatgatgaaaatgctaaacactcacaagaaaacccgttaagttttgatgtaatcagataaggaggggcaaagatgaatagttttatgaataaacaagctaaacaggtaaaaagaagtaaagaaataaaactagtagaagaagtaagaagaaaaaacgtaaagaaacgtttttcagaggaagttagaaagtacctagaaaaagggtatataatcaggttagaaaataaagtttttccatttgctttaatatctattgacctagaaaaaggggaaaaggtcataagtcttattcttgtgaacgaatatgatggaatagcaaactatacagcaatgaaaaaggttaccttaagagaaaaagggaatagagctatcctaaaaagaacgttaacggataaagatataaaagtagtgagtatgtggaaaggaatataaaagaatgagtgtatacagtttaaaattactagcaatcttagggatagtattattcttttcagttatcgggatagtgtacgataataaacaggacgaaaagaaataaacatataaagaggtaaagagataaggaactatagagctatataaatgtgtacacttataggaataagaagaaaaggaactatatacctatacactcatacactcatattcagatagacacataataagtaagggtaaaggagagaggaggagggagagaaagaggaaagaggaaaaaagttgtttacctgagattttaaagaatcgactccatcaaaaacccgacaagggggcgcataagtctatttcaaaataatctgaaataagtatagttattactgtttatagatggttatccttaaatatctgaaaataggggcgtttatctgattatatagttagctatcttatactattaaccatctagcctattactgcattcattgctattatattctatatagggggcgcttatatcgtttatagtgtaattatgaggggaacgactaggaacgcttatacgggcttatagggggctttaaatgcataggctatttatacatatattagaatacacaaggaggaggggcggaaagttagtagattagactgttaaaaacaaacgggggatagatgcacattgttattttactgattgggctaggttaactagctaaaataagaatgctattgtagcaacgtttataagaaataggggtgtacttttcccctagggaggttttaaaagggtataaaattcttttgttatttaataaaaaagtccatcttagctattgacaaataacaacaactttggtattctatatttgtaagataaagaaagggagttatagacatggaatatacattagacgaattgctagaagaggaatatagcacactagacgaattgctagacagtagagaatttaaaaaacaaatggacaaccttaatcacgtcccacaaatgcaaccgcaaagccataacagcaatacgctagcagatacgggacgttatcctgaaaaataaaattgaaaaaaggggttgacaagttcagcccctagtggtattctatatttgtaagataaagaaagggagtttttattatgaatcattataaattatatgtagatatgaaagagggaactcacgattatgtttcggcaactgtctataatatacttgatgaaaaagttttagggttgccagatattaaaaaacctgagaacgtagcttactatactgatgaatggaaaaacgggctatattcttactatgaaaaactcgcaatatcagagttaaacgactacaacgctactttttcacatttataaaaaattaaaaaaaactattgacaaaaaacaacaactagtgtattttattaagtgtaaggaggaacaaacctccttacaccacacaacaggaaggaagtttttactatgacagaatttgctaatatgaataaagaagaggtattggagctacttaatgattggtttggtgttagtgactatgatacagtgatggaagagttaggagagatgaaacaagttacctttacaggtagcacaaaccaacctctattaggtggtaacggtaacttaattagtttacctcaattctttaaaaataacgaagcagaatcagagttcccaacttatggagagctactagaggaactagagaaagatacatggaatctcgaagcagaggacaacacttacaattatagtggctttttagaaagtgaatcagattttaaagttattcaggcagaaaattcagacacgactattgcattctttgcaatccatacgggtatagacataagagcgggctactcaaaagcaatcccagttatttttgaaacttactatgatttttatgaatttctaggtaactacttttgtagtcaaggttactatgcttttaaacacgacaacaaggaatacacaatcagtttagacgtttcggctacctcagaatatgtacgaatttatatagctgatgaaaacaacgaggaactacagcaaggctatgaacaagaaacttgtatggacttagacatagaaagcgtagaaggatacttgaaagaggaaggaattgagtttactgacttaaaacccgcattgtaaccatataaggcactagggagcttatacaatagagctacaagcctcctagtgtaattataaggtaaataactagaaacgcttatacgaaagaatagggggctttaaaatgacaacggatgaattaaaagagttttactatgaaaacgggattgacttgtggaatgataacctatattttgaacaagttgtttctagtggtggatggtactacgacaatgaacgcggtttatggtttaattatgaggattaaaaatttaaacttttctattgacaaaaaacaaaaactttggtattctatacttgtaagataaatagagaggggaactaataaaaatgaaactaaaagactttatcaaactagcagaatccaagggcgctacattagaagcatacaacgagctaggaggttatgaactaactagaggggacacagtagacccgaatccggttttgattgcttacatgcaaggggcttacagcgtagaaataccaaacaaggaactagaaaacaaggagttaacagaactagcgtttgtctataaaaatgtaagtcttatttatccaaatgaaaaagaactattgtcaggactaggactatagcacaacggcatataaagcccgtagcgaggttttagcgggctttatatataaataccttaaggaggaaacaaggtgcttacagtggaaaataagggcgttaggtggctagtgagtaaagaagcatggaaagcaggctttgctatggaggtgctaggcttgccagattgtaaaattagtacagtattaaaatcggtctataaaattattatctaactatttaaactaatctattgacaaataacaaaaactttggtattctatacatgtaagataaataaaacaaaagaaagagagtgacaagaatggaaacgaacaaagcatatgaaagactattgaaagaagtagaaaacttacagaatgatttaatggatatcgaggactattcagaagaagtatatcaagcctttcaaagattaatcgaagaactcgaagaggtaaccgaatagggctagaccagtcctataggtatataccagttgacccgcccccgtggttttttgaccgtactttgggggtggggctatttgcctaccccgaccctggggtataaatttttttgtagctagaaaatttttatatatttataaagtcaacaccccacatataaagtcaacataagggctcaccctagggctcctatataggctcacctaaatactcccatataaaaaagacccctccccgttgataaggataggtcttttttatttagccgtctgccctatgattggttattaggttcaggttccgccatagtctttgcgaagtatgtccagtatttatggaagtctgcaaagtccaagaagtactccccgacaatctctcctgcttgattgcggtaaagtggtactttcgttttctcgtctttatggactccatactctgtgccatttaatgaaatccatacaatatccggagtcacactagttactgttgccttatcacaacctagtatcgggtcacgaagttctggttttgtgaaaactgtatccccaaccttcaatttgtctagtcgctctttgtctattaatgttgtctccatttgttctccctccttatacattataaaaaatatttaacgtctaattactgccctcaaataaagaacattactacccatccaataagcataaataacaatgttgatacagtagcttttgcaaataccatcaaaatagaatcttctgtatttgtagtagtcttagctgtaataaaactaataaatacatctagcccaattgcctgcgcccatgtaagtgttaacaccccaaatgttggggcaattaacccgttccacaagaacatcgtaacataccctccaatagcaagggtcaacaccactagaactaaagtcccaaaaaatttacctaatgcatttgccaattcgtcttttgtattcttatccatcgttttcctccttaataatagctatatttacctcttatttttttgttaattctatttaggcttgcaaaagtaattatgttcaagatatatgcgccaattactgatactgcctgcattgtgcaaaacacgattgttatccagtagcttgtagtagcttccccgctagttagcccccaataaatgctatatgtcaccatgagtgtgtttagcagtatagctacccctcctaccaataatagtaggtaaccagatagtttcatttagttcccctccattgaatgattaagtaagctcttgttcagttcttttaagtaatagtcacacctaacgtgcacaagacccatacgttcccttgtaatagggttataatgtaatcgtgtaggtactgtgtactcattaggtatagataagtctaattgggtagttaaattgactactctatccggagggcacatccatagaggcttattacagtgccaacatgtcccactttgtagtacctcgtattttcgtttaagttgtttctcttcttctattgttaattagtcgtgatagcactgtgtcattgcgtatggctccctccgcttttatatttgttatagtttagtgttaaaccagtcctatatcctctcctagcgtttacaatagttgtttaaggtgataataggtagaatacctatcaccgccctaagaggcatatagggtacttataggactggtgtttagttaactgttttaagtggcataaaaaatatgcgcttaagtcaacattagttcttttactttagatgatgtcaattgcaatataatgatttgttttggatacattagcaatttcataatctaagtatggttctagtacttcgttgttacttcctatctttgttctaactgttatggtagcccctgccgtgggataagtaatgagtacgtccactccgggcttcattaacttaactaaatcttttaacttcatctttatctcctctttaatagcatatgcttaaatctattttatgtcaactgcttaatttttgtgctcgtagttgcacagatattgtatcaacaatgactgcccactgctcctccgtaaaattgaagtcaaactgtgtatagtcttcctcacctgttgtagtaattgcaatgtctccataatcatcaactgagaaatagatagttgcagtcgcattttcctccggattttgaggaagtgtaatagctaactctccttgctctactttcatctattgcccccccttagctctcttccttctcaatcatcttgatacctgtaaaggcatatacagggagttcttctgtgtaagtgtactgattagctttaaaggtaacttcgtagtaactctccatgccacagtgtaacatgtctacatatctaatttccttacaaggcatagcatttttctcactcccacagaagagccagtcttctgtacagtattctactctacctgtgtggatacttctaactgctacgtatggtttttccatctattcttcctcctgtgtaatctcttctaggtcacaagggtgtacatctagtgttcctgtccttagactataacgagagtttcctcgtactgcgtaaacaccatctgggtatactttttcaagatatacagtatccccaattgtaaacccatggtcataacgggtatccccaataaccttaaactgtctttttatcgtatacccatacatgtaagcccgtgctaatacgtattggttaccctcatcaatccattcaactagcttgtcatctggtgtttcatcgtatgggtcaaaatactcattagctaataagctcaacattgaatcgtactttttgattgctcgtgcaacaaaactaggtatctctacttttttagccatctattcttcctcctatttaatcataatacatacaaaatacataaaaaagctaacatcagcaaaacaccaccccatccagctgttacatatgacatatagaaaacgtatataaggtatgttactgctataattgttaataatacaagtatcgtgttaatgagcttttctaaatcaatcattatacaacctcctagtcctcacaagtgcgagtctggttcttattatactcttactcctacttatatccaaagaactttaagtaattttctgcttctttttctaagtgctcgtttagttcatctagggtaacaactttcccacagtcctcacaggtgtaggtctggttcttcttatcttctagcagttcaccatcacatacaaggttgatacaatgggttgtccaactccctacatcatcaggtaagtgccccattatacgtcacctacttttacggcaaatgccatgaatcgttcatccattttgcggatttctttctctgtaaaggtagggatgtcttttaggtagtttgtaaagtcaggagaccctaatcggtcgatatagctatatccccaaccatctttatcttttgcaataatgatgtagtactcgtcttcttcttcctctaccgtatgacctagtacccatgctttggcaagtttctcatggttttctgggttattagctaaccaaaagtacatcttactagggtagcttcctttgtcaatcatgttaataaacgttaagttctcttctttgcacttgtcaatatatttccctactttataaggaataacaactttttcaggttcgtctaaatcatatgctaaggagactgcttttgctatccctgtattgtagcctagagcatgggggttcaatgtaccgtcacaccctacttgagtaaaaacctcgtcacttagtctactaataaattcattcttattcatttagttccctccttaaaaatcaagactgttttcaataagttctgatagtcggagcattacctcatgaggtagctctaattttgtactctcctgtgagtctgcggagctgacttccaaagtatattttacttctgttttctcatttacacgggaagccttcttctcaacacatactttataaagtgctgagttattgactgcgataattttttcttgtgtatttacactagtattgctatcataagtaatttcatagcccattataaaaccctcctatttgtatactggtacagcaaaagcccagtatctttcatcaatttcttttatttcttgttcggtaaatttgctcttacccatgttgggtttatttgagaagtatacttcattattgtgggatgtttcaacccaaagataacaatcttctcctttattaccaagaccagtaaacacgacatggtaaagtggttctttctccacctcatatccatctttcattcgtattaaagtttcaatagggttattcttactttggtctaaccaacaatcgaactctgattcatgtgggtagctgttgccatctaacattctaatttgtgtaaaaatagctaggtctaatgcatgtttattttcctcgtaccattccgcaacaaactttggcacaattacttttttaggttcgtctagctgttttgctaaagagattgcgctaataattgatagatttgacactatacgataaggtgttttactagattcttttagttcttctaattttttaatcaattcttgtttattcatttaatttctttcctttctttcaatagcccactggctgaatgcttgtaagacttgcaactgcgcaatttctgtcatgtatctataatttttataaacagggctattccgataatctgtttttgtagaattggctctcagtctccaaaatagttctataggttcaatatctgttaacgtatatttttcttttaaccaacccaaaacaatttgttgattctcacttagttctacttggtctaccttatcatcagtgtatttgaaccagattttctcatatgttgtttgtccgcctgtgattgttacaaattcggcgcttggttgctcattttgaaatttttctagttgttcttcgtaatgtatatccccaacatcaaattctttaaatttaatcattgtactccccctgttctaaaaaccaatcagtaaatgcttgaataacttgcgcttcctccgttactgataaagagtaatatgcctcttctgttttagggtcttcataggtctccccaatacgttcgagcgcctcaaataaggaatctttactacagtaacctacttttaaccattcaaatacctgtttctgatttttattcagttctggctttttaactgcctctactgcagtcttatacgctatttttaaaaggtctccttcaaaactattagggaaattaatttcaccatttgctttcatatacatatagcaaactctatcaattatttcgttatatctttgtctactcattcactatccctcctcgtcctctacgtcaccccaaccaaagctacagtaggaagagaacacgtctctagctacttcgtctatctcctcattcgtagcattatcgggtacttctactgtctctatttcaccaatacctgcccaagttgtctcaatatatacatttatttttcgcatagtttaatacctaagactacatagtcgtctttctgtgcataatcggtgatataagtaacttctactttaataaactctcctgtatacgaaccacatgtgtactcatttaataaaagaatatctcccacatggtattgtctatcatttttacgtatttcaaatagttttctaccttccttaactgctttaaagtacgtaggtgcaatcttgaggttatgagtaacttctaatttactaactaaatcaaaaatgatagtgtttaatttgttaccctctacctgatgattcaatttttgtaaagttgttgatattacagtatgcctaccttctctatcaataactgagtttcttctgttatacttagtaagtctttccttttctgcttttgcctgtgctagtccatttattgttttagatacttttacttctccatttacaataacttgtactaggtatctgtcgtcctttgttgcaaacttattatccataattagtacctctctttcataatcttaattgaccagttatcgttgttactgaatacccgttctaggtcattcaatgagttggtatttacaatttctttttttagttttctatctgaattaatattaccaaatcgtttaaggaatctttgtttaaagtgggcataacccatatagtcgaaggtaataacgtgttctttaccaaatataccccgctctcttaacttaatctctacactctcataagagctatctactttcataaaattatttagaagagtgtgcaaatcaatacaaatagatgcccctgcactaccgcctataagtatatatttagggcactttatatcggggtaacaaggggcatctaattcataccacatattatttacgtctaccccataccatacactatttacatctactgaggctctttctgtcttaaatggttttatgcaagtatatttcattgtctctcctccaaatcgtctagtacgtcttctaatgttgtgacaaccccctgcaaataaccaagttcatgccacccataccctctcttatcttgctctaacaaattattaattctttttgttttacgtttaatttgccggttatatcttctttttagtccctcttcaaaggtcactaccttttttgcttcctctatatcttttaataattggtctagcccatctccattagtgccatagctatacactagcgctttctcgtccttataggtagttacccctaatgattggtatacatacttcttactggggacaaatacaagagtaatgggtctgtacaattgaggtaaaagacaatcttctgacagcccaccaaaatctgttttagaagataccttctctaccacatacctcatatcttccatacttaacgacttaatacataaaatatatctgttaataaccattttctttagctccccctacacccaaaatagttttcgattctctgttggtttaaaagactccaattctcgtgaagtattactttttccatctgttaaaccttctttcactttatatattaaaaaaaataaatctagctatctacaaatacattgtatcatcagctagattaaaagtcaacactttatatttaattattttatattacaatagttctttatctaaaattattttagggatagcccatattgtagtgtaacgaacccctttatggttacctgtaactaatacgaacgttgccgtgtctagcttagtaccgagtacagatgctagtagttcgtggtcttctttgctaattggtacttcaaaatcaagttctccaagctctaccacaaagttatttgctctaattcccataaagtattcatcattacgttttacatggaatatattcttcgtatgaaaactttgcataacaatatttgcaaaataactgttatccctagctacaataaatctatctacatagatagcctctttactgagtagttcttcaatgcagttactcataacatattctcctcctcttctaatagtagctctgatacgtaaatttccatcattagactttgttcaatcccgtctagtaataaatgcatagcacacaagccacacaacatttcatctaaataaaaatcaccacatgtctcctctaatggtacttgacacattaaacactctatcattgtacagccctccttaatttaagttttctctaacttctgttagcacctctcctaatagattaagtccttcccatttactcatatcacgagagcgtgggtctgattcacgtaaccctattccccatactttatcaaaaggtgatgcctctgcaaacttggttcctttagggatggatagcataaagttacgtaaactatcattttgtgtgaatttataagtatttccagctaaaacgattgatttacgatgctttacccacaagtcttcttcaaaatttttaacttgtctacctaaacgtttagcatcttttgggctctctgtttttaaaattctttttgctgtatcgacatcattaaaaagcattgctttacgtaccatcatgtagtgctctgctgtcgggaaaataatagcttcccctaaacccttaataggtgcactgaactgtgatgggtaccactgtgacaagcactcttttcctagtttattacgtttgcttggggtatgtccccaaaataaaatatatttactcatttaatgttcctcccaatattcatagtagtttcccttatgttcaaaaacaaaatgagggctaggtaactcaccattaacttctatatgctctgggttattataagaatagtagggttcgttaccagtaggactaattgctattactggtttatctttaaaaaatggtggtattttatctccatcatttaagtttaatttataggtacttaatggcacgcttctacgatgccctttcagtgttgtatactcctcaagactaattattctaaggaaacccttagcttttagaggcgctaaactgtctatcgaaacgtcttcttgcttataagtgacaagggcgctataaatggttgaggggtttttgtatgccactgaataattaattgaagtgtgcttatggtttgctaaaaatttctctaattccttagataaaccataaggtgtatcactatcaataacttttactttaatcatgtgttatcctccctatatgcttctctaactgttcctatactttggtctgggtctggtttactaaatggtaagcttgcacgctcttccttactcaatgtttttaagcaagccacatgtactgcaatgacccctgacttagcttccatactatccgggagtgtaagtatatagtcattatacagtttacttaacactagccaataacgattgctactacttttcatattagctaaaatcatcattttttcatagtaatcttgccccatacaagaaagtcctcctattgcagattggaggagctcatcttcaagagctaagatagtatttgcgtaccctttcagctccttgttaagcccctctatagcaatctcaaaacattctctttctggagagcctacagttaaatcattaagtggctcatatgctcttacttctctcccactaggggcttgtcttcgtttacctatacgataagagtctttaaactcatactcggaacgaaaaatttcttcttgactatttcttccagaccttcctccaaaatagcaatcttctactactccaccaagaccattataatgtcctctagttgtccctatgactttagaatgtctaatatgggttagctgacagagctcccctccgttatcagggtcacctacaatagctgtctcacatacaggacagatatatccaaaacacatcactttatctacctccaattaatatacattaagaaaaagttacaattttttcacaaggaatatcatagtatgcctttaaaccataatgttccaacatgtattctttagcataatctacaaggtgctcagggcatttaaatgtgtaagagccactcatcattacaccactattacttaactcttctctcgaagctttagcaaaccacttagcacactctacaggataaccaataacacaccctaaaacttcctcgtcattaaaccctagcttaattgattcattgtatacttctatactcatcttatctgatgttactaggtatatactaccatataacctcgttttatagtaagagcgttccagatggcttagctcttcttcccctaatacgattgctacacgatgacctaaattaaaatctaaaataggctttggaaaaacgtattctgctttctcaacaaactccacttagccaccccttttctcattccctaaattatcttaaatgctgtattagttagaacggtaagtcactattgtgttcttcctcttctgggatatataggatattttcaatcttttcttcaatatgtccaataatctctgtgtgctctttaattttctctttatgattttctctttgcttatttaactttgcatattgctgtaattcatctggtgttagctcttctagtctttttttcatttgttttctccttctaatgtaattttctctacgtcatcaacactaccaaaagatgggggctgtgtcaagttcttatctaaccagttagcgataatgtcatgtaactcgtctatagcctcatcgcttacttcatccgttgggtagtagtcctccgctacttctccatattcactgtatagctgttcccctacagattctaacatacctactacatctacactaataactgctttattgaactgccctactgcaaagcttgttgttcccttttcaggtaatgctccaaatatatcctctacgtgcatccctaagctatctacatatgtttttccttcattaatggacaataatgcaagttttcctgcagacactgcctcttctctcgtagagaacgtctcacacgctttccatacatctgtgtcttcctctagtgctaatacatagtctttatcttccattgtcttgccctctctatccttttaatataatcatatttgtattactgtctagttgccatccatcaaattctaagtagtggtcataagggttaattggttcacctacaactatatagtcctctagtgcgtgaccttggtcttttagctctagtaattcgtctaataaatcttgtgctgtcaaattattcatgccatatagtatcctttctctttagcttcttcccactcatctacagaaaacaaacgctcattccgagacaaagagccataacagtttactgttaagtctaccataaggaagtccttaccgtattgttttgtccaactctctgtatatggtgttactgagtgcacttctttaatatattgctctaacatattcattttatgttaccctttcttggtttaaattttcgtgtttgtgttcggttgtttctacttacttctttgtatctacggattcctaatgccttagattctgggcgagaacgacctatctgtcttacatataagtctagcgcttcttttactttatcatcatacatcttccctaattctcggaaatactcaaactcacctaaatacacataaggcatacgccagtcatctagggtagccgttaccattgttcgtttgtttaaatcataattatagatatatagaaacactatataagcacctgtcatcacagaatagcttgtcctaatttcacttagagttacgctgtctcttaatgatgttaaataaccattccacttttttttacgttcttctgctaaagtttctatgaagtagtttacctctttttcgtccctcaccacttgctacctccttgttgtttatgtctatatattatcatctactttgttatatgtcaacacctttgtaataaaaaagaacctagtaatttacttacttaggctctcttgtttatacgtgtttagtaagttacctttactatcgacaacaacagcattaagctgaccaccatatgcacaggcaccatcaatgaaaatacttctatcacctaagaagacatcgtagctgttctcttttctcaaattaattgtgggtgtgtgacccattacaattgtcttatctgttttattcttctgtaacgctagcggtctcgtccaaatcatttcatctttagtggctgttttccaatcaggctgacgataaacaggtatccctgcgtgtacacataaggtgtctccatgctcatagtatggttctaataaactaattacttcaactacatttgttttttctaataacatctttctagtggtaaacgcatcctgtaggtgttcatctaaatccaatagactacttattgttttatcaccgccattgtacatccacattgcgtacatctcacttaggtcttcgtagtctgcttctcttatcaatggaaatgttaaaaaatctaataacatttggtcatgatttcctaacaaagcagttcctccattaataatatgcttataaacgaaacccagtacttctgcggatttgctacccctatctacgtagtcacctaaaagtattaagtcctcttcatcactattccaatgtttattaagaagcattattagctcatcatagcaaccatgtatatctgatacaataaatactttatctttcaatgaataatagcccctttaactacttctgctagccaataagtagctagtactagtacagtattgacaataaatgttattactataaccagtgctaacttataatttttactcctagcattatagtttatataattttttatgttaactctaatatttttaaacaaagcactcccatatacgttcagtgctatatatagtaaaagcaatacgataaagtagccttgagctagaaacacgtcagactccctgaacgagttattaaaccatatgctaaatatcgcaatcacttggtgaattataagcattgcgccattaccaaaaagaagtatactaaacgctataccgactacgtctctgtactctgaaagtagtctatcatatactattatccctttagtaaaaataaaagcaacaactgccatctgtataagtaaaaatattgttacggctaataagttttctgtatgcatagtcataatttagccactcctttcaaaatgggtaaagaaagaataataggtatatcgttctttttctaccctaccttcatgtataaaggtaaactcaacaaacttaactcttagcggtatatctggtgctttctcccaaggaagtactcttgggaaatcatagaatactcttgtggggtaaacttctttcataagtatcctagggtatcttttctttggtataaatcttttacctattatacttgagtagtcaggtttcattgtaagtcaccatgaatagagtatgctctatttgctttgttaaagtttacttgttttttgtttactaatcttattgcatcttctaataaaagaggttttcctaatttatggttatctaattctggtgagtctacccctacattcagtaagtttggttcgggtctggctaactcatgaatgtgcccatgtagattaattaggttatctctatctcctaaaattagtgggtaatgtgtcatatgcacaaccttatgcattcgttttaaaataataccaacgtcttcccaatgaaccctatcattcagggaagtattgcgtttaatctcttttcgtagaggactattatcgtggttaccctttattagccatatagtgccatttaagcgctctaagacgttagctatactatttaccttggcacccattgcaaagtctcctaggtgatatacaatgtcctctgggcgtactgtagcattccactctctaattaagtattcgttcatctcttccacatctttaaattgtttccgtgtgtccataaaagaggcttccccacaaatgtttctatggaagaagtgcatatcagatattacatattctctccccatacttgctcctccttagtgtgttgcaaaccatacgaatacagctagttgtagatagtgtactgtttggtcgataattagttgtgtctttttattaggtactgtttttaagaaccatgcactttgtgcttttaaatagtccatgataaaatgtggaacccataagcatactacaattagcccaagttttactggtgttcctaagaacaatgtagttgcgacaataatatacgtccagatgtttacatggatgattagtagatataaatcagtctgctttccttttgcgatatagtcactttgtaaggcatagtcccctactgcatgagccattgtaaggataattacatagtataagtaattcaaattaagtcctcctctttgtatgggtaaggacaagtgtcacattcaaatccatattcgttaggtgctccctctaaaatatttccgccacattctgggcaagttgctagtttcattgttctgcctcctttacatgatttcaagatatagccctgcacttggtgttgtagaaatcagcataacttctaggtctaagtgttctccgataccttcgtattgttcaataagtggttttgtttctgataaagtgaatgttacaatttcttcatccgtcatgtgctctactaatgtgactgtgcgaccaaattcaatatgttgtaataaatgtcctagtttaatcattataatttcccccatcaattaataatagtaagataccacctatcacaagtaaccagaatactgctaagattagtaccatttagttgtcctccttgaacagctcatcgtataattcttgaattgcctcacgctttacttttaacattgcaatctgtgctgatatgatattgcttggttttcccaccaaacgtccctctaagtgcccaatatccatattgtattgaataagggtttgttgaaatttttttctaatctctgtgcgttcattaattggttgctctggttcaatctcaaacagttcaaacattgaacgccagcgcccatttacgttattcaataattcactaggtgtgcccccaatatctactgtgtcatacccattgtctttaaagaagtagcccaccgtttcgttgtgataaacaggatattctctcccttctatgaactgtggttctagtgcatctgcttttgtacatttaattccgtatgtcattttattaaacctcccattccttaatgatgtattggcttttatagtttgcatagaaatctgagtcacttgagaagtatatatctagttcttttactttttctagtactccttgaagggatgtaccaactgccatgttagtacctgtccccttatcaattccgagatagagtgtaagtttctttggttctgcaccgagcaattcaaacttagaatgccaatagttatttaattcagctaatagtagctcaggagtggctcctgattctataatgtctccctcatcatctctaaggaagtaacctctagcatcatcatagaatacatcgtactctttaccttctgtgaagatatgctctgttttaagtgtacatctaatttttactgtcattctaattttcctccaattcaatttcttttattgatacaaagccaagtatattgcggaaagtacggtcttcattccagtatataaattgtgttagaagtggtttgtggtcatctgtgtatgttgttttttgtctcgtagtagctttcttcaatttgttcatcaatattttgtaccatttcattataatatgtgactgctttatcatatgaggtgaaagccctcatttttaccgctctatactcaaatttcactaaccatgctgagcttaatttcgtcatttatttcttcctccacttctttgattgacttgattatatatctatggttctctctaaatgcgtggtaagcatcatcaagtgaatatgcgtataatcttgttgtttgcattacagttctatatccgttacgtccaaccattggttcgtcaacttctacttctaactcaaataatagttgttttctaatcattgtttttactccccttttctatgatataatattaccctactattatgattctgtcaacaggcaaaaaaaagaagtagaaaaatctactcctattcatcgtttgacaacttttccataccatatagtaactgtagtagtacatatagtacaatatcaaatccgtcaagtggctttccaagtactataactttaacaattgtcaataccgctaaaaaaataaatagccacccgattattttatttgcatgttttctaattctcataactttctagtacctcttcaatattctttctggtttcgttagctaacttaccagtccgttcaagccaacctctaaccatttctttttctactttgctatgtttattcgcatcctccttgataccttctacattttccatcaagttatctaagtcctccataacatctaataaagtgtttcttagttttaacacatcgatagacaactcatagttccgtttagacaatttttcgttacggataaagttcttttttagttcttgttgtgtttctagtagctgagtagttttaataatatcagcttctaatttactaattccgtctagttcattcatcacatgtcctcctcatattctactacttcctcaataagtttcagtacttcttctgctgtgcccactgtgctatagtccgcaaagttttctgcaggtttcataatagccactgaatagggtttgttctctacataaatatgcccgaatccttttaaagaatgaattacctctactgcccatccattagcgtactcttctcggtatactacttgctcactggttgctcttactggtttattcattgttaaaaccatagaagtttcttacaatgttttctacacgttccatgccctctaagtagctacgtttctcaggggagatatagttcttgtaatgagggacttccttctcttcctctacctcttttgtagtacgttcaatcagtttaataagttttacttcgttctctagttgagactggataatgtctaacagttcatttttcgagcagttgtttagtggtttacttccatagtcaataattgtcatagtagtcctcctattttaatgtgtactctttatatcctttatgtgtatcgtgcccgcactttgtacaaaagcctgcttgttcaatatctattgaagagtaccctgtttgtactgcatacgtctcataagtatggtcacacgtatcttcttctgattcatctattttctctaaacgaatagcctctccttctgccacttcgtggttaaagagcaatactgcagttttaataggctcatatacctctgggtggacggcttcattcatcttaaagctatttccactaaattcattgaaagcatctagccattcctgactgttctcataagatacaattctgtaattcatacgaaagctcctctcgtgttttcttaaataaccagtaccgttcatcaatttcttttatctctgcctctgttaaatagaagtcttttaatttggatagggtatcttgactcaatggctcgtttctaggtagtatacttactgctaactgcccgtccttgcgtaatagtaacccgtagtctctctcctgtttctgaggcattactacatagtacttaggtaaactagcagtgtttgctactgcttgaataaaagtatctgtattagcaaagaaccatttactaaactctgacttggggtactcacatgcgtgtctctgcccttccaagataatttgtaacttatccataagttgttctcgttgtttatcaataaactcttttacctgttttggtacttctacctcattattcatagtttgtctcctttgttatactttgtcaatagtgatatacacatacttgccctctaactgcttaacaatatctagtatgtcatgaccacctagcttaaatgtgtttgtctcaaacccttcgatagtaaaggaagaccaaccgtaccaaccttcttcaaagtccaagacccccatagatttaagtactatatttttagtgatgtcttctaatgaagtacgttctacagcagagaaaatctgaatctctgcgttatcaagatgatacttagaagaaatgcctccatcgtactcctcttctgttgtagtgtcctcagctcctaacgcatacagtgcattacaaataagcatgtttaaggctctgtgctcatggtgatactcaatttcttttactttttcttttattaagtaaggttcgtttgtttctgcaccggggctgttatcaatagttacccaaccttttaatatctgtttacccatgattgctcatccttcctttagtacagcctatcgctgtcaccagtaaatctaaattttcctttgtcagagttactgtttgttcatgtacacagtccggtctaaatacctctactgtacgatttactacagcaatatctacagtatcttccgttgtctggcttaccttgataaactgtttggaaaactccccacggctaacaccttctatcataagctccatttttttatagcctcctctctggaaagtccatgaaagttgtggaaagtacgctcttgtagttcatctactgtatttggtaatgtacgaaattcgtctacccctagtgaaatacttgaggctacctcttcataataacatttaacgtctactcccattttaccataaggtaacaccattacttctatatgaaactcatatggagcattctgtgttaatggttcgtataataaccatgtctcatgatagtttacaggaatatctaatagtaaactgtttaaatcatctagctgttcagataagtatgcaattcttgtcattttacggtcttctgctataggcattgaacaacctaacgtgtcttttatttctttaatttctttggtaagctcagccattaattcaattattttataaaacatttctattccctctcttctatatattccccttcttctaagaaaaagcaagcaggttctccctctccattttcagtatcacctaggtattcatcatctaagaatgcacagtatccagttgagtagagggttacacagtccttatggtacatcgaatcgtccgttaaccgcacaacctcgtccatctcactgaacacttcattacacgccccgcatgatactaactccttactcataggctgcctcctttatctattacgtagtctaccagttctctaataacctctgcctcctctacactagagaggtctgcccaaacttgaagtgtcgcatcgttagccttaccagatattaaattgtgtaagctatctgcaatagttagctttgtacgttcaagatagtgaattagccagactaatacaattagctgtttctcagttagctcagtattagtctttgtgtaaacctcatagttatctaaggttaatgggaatgtttcttcattattaattacttgaaacccgttatttggttcgttttcatattctccataagttactctcttacctatttttagttttacatagatgtctttaccttctttgtgtagtttatctaggtcactattataccactctcttgtttcaattttagtaagttccataaagctaaccctccttactgagttccttgatacgttgtttgatttctgcttctgttttctctagttgtcgcattttgtttttatgtcgagataattcatgttcctttgcagtttctgccattgctaataagttttctaagcttgctgtatttgccattagattgccacctcatagttaaattttccattatgtttatagtttactactttaatttctgatagtggggaatcaaagaagttcctccccttctcccatggtaagataagttctggcacttcttctgatattggtgcattcacctgttgttcaataagttctaaatgtcgttcgtaaatgtgtgcgttatcactcgtccaatataagttacctaactctaaccctacagtatttgccataaccaattgtaatgcatgatactgaataatattaaatggaagtcctaagcaaacatccgaagaccgagccttcacatgtaagtttaatttaccctctacaactgtccagtgagttgtccatacacatggctctaatgacatatcgtataaatcttccacgttccataaagtagtcataattctacgagagtttggtgtgctcttaagttgttcaataactgcctctacctgatttagctttaggtatggttgatgtgttcctgctatcccaccaccttttttaggtacgacttttggaataagtgaacctgctttgcgatttttagctaactcaacatctccactataaacaggaataaaacgttctttgttaaataatgcgtaaccatacgcttttccaatagtgccatcttcttgctcccattcgttccaaatagttacacctcgttcttttaaccacgaaacctcgttagacatttcttgccaaatccactgcaattctgttagcgcccatttaatacctacatgcttactacgtaataaaggagcccccatatctggtgtaattgtaaagtttacaccttcaataaacttagttgttgcaggagttccatcagcatatactgcacgagtaccttctggtagctctgttactccgttcttaataatatccattactaaatctttataaattttatcaaaatccatgttgtgccctcctacatttcttttccctataatagaaatatatcatatctaaatttaaaagtcaacaaaatattataaaaaaaatatgagacatattggtatgtctcatatctactaaattctatactaaactggctagcttgtctaaagcgttatagtccgcatcggttactggttctactttacctaataagtacccattacctacctgagagaagaagtcatggttactagttgttgtagagataccattcattacaatagggtttacgtctgcacttgttgttgggaataaagggttcatccctaagttagctagagctttatttaaattgtactccaaaaatgtattaacatcttttgtccaaccaatctcactatatagttcagcagtatactgtgtttcgttctcccataatttaaatgctaaatcaattacccattgttccatttctttttgttcagtttctggtaactggttaaaccctaactggtatttatagccgatataggttccatgtacagactcgtcacgaataattaatttaataatttcggctgtattaaccatttttgcctcacctaaatagcgtagtggtgtgtaaaaacctgagtaaaataggaagctctccaatagtacggatgcactctttttctgtagtggtgtaccgtttcgataaatatcgttaataatgttagctttatattgtaaacgtttatttgtagctacccattcaaagatattgtcaatctctgtaggtgtattaaatgtgctaaaaattgttgaataacttttagcgtgtactgcttccataaaggctatgttatttaaaacagcttcttcatgctgtgttcttacatcatcaagtagtgagtgtacccccgattctgattgaactgtgtctagtaatgttaacccaccaaacactttatttattaaatcttgctccatatcagagagctttgcccaatcattaacatcgttacctacagggacacgtgtgtccaaccaaaattgctcagtaagctttttccatgtggcttggtcaattacatcatcaatcttattccagttaattccttcatacttttcttgcaaattcatgtgctcatctccttaaattgtacaactttcacactctgaaacccctacttcgcttccgtcttcttcggtgaatgttctaacataataaattgtttttataccttttttccatgcataatgtcttaataaagttaagtcccgagtggatgtagcgccaccctccaccttccaaggataaagattttctggtaactctgagcgcataaacaatgttaaactcataccttggtcaatatgtttttgtgctgttgcgtacacgttgattacgtcaatcatacttgtattgtacgctgacttgtaatatggaattgtcttctcagataaccggggtgcagggtaataagttttacctgttttcccatcttgacgttcttcaatcatagagataattgggtgcaatgaagaagtagtctcattaacataagcaatactaccattcgtttataccgttactttcgtaatactttaacactgctcttagcagtcggactagactataccttatactatcccaaaatagtaccaactattatagtcgttggacgtccctcattttacagaggtttcgatgctgatttcccattgtattacccttagcacctgtaacaaggcttttatttcagcataggctatctaactaattttttctgctttcgcaacattcacgctcaccgtttccagtcacgttgtagtttagttagctttagggggttccagcaatttaagttgtttttgactcatattcacatatgagaaagcccaatattatttaggcgccacagctaaacggttttgatggtatagaccaccttcaataatactgtttcttaatgtttcccaatcttttacattaggtagtaccactccatcaaatacttccgccaccttactagagatttcctgatttagtgttggtacatattcatcaaagtaagaaccgtctgcgtatttagagttctcaaagttatggaatgttgtgccacgctctttagcaatcttattacttgccaccaaagtagcatagttaattaattcaaacagagcatccgtcatttcaatagattcaggtgagccatattctacttggttacttgcgaaccacgcatgtagccccattgcccctaaaccaattgtatgggctttatcattaccattcttgatagtaggtactgcttttatatttgacacatctgtaatatatgttagagctcttaccatcgtctcaattgatgccactacatcattagatgtttctaacaagttaaggatgttaattgaacctaaattacagctaatgtctgtacctaactcttcgtatacttgttcatcatttagcttagatggtgtctgtacctgtaatatttcactgcataaattactcataatgattttgccatcaataggattggctttatttacagtactaacattcataatatatgggtaacctgactcttgttgtaaacggctaatttcttcttctaaatctcgtgcattcattaccttacttctgatatttgggttctgaatcatgttattgtattctgaatcaatgtctacaaatgagaatggtacaccgtattctttagcaacatcatatggagaaaataagtgaattacatccccagactcagctagctcataaaatttatcgggaacaactactcccaaagaaagtgttttgatttgctttgcggattctgcattttcttttctagttgataaaaagtccataatatccgcatggaaaacatttagatagactgcgcctgcaccttgtctttgtcctaactgatttgcgtaccggaaaccatcttctagcattttcataacagggacaaccccgctacctgctccctcaattcccttaatagggtctccaagagctcttaggtttgaaagatttaacaagtagtccatgctttaacatggctcagactatatcttaactaaatttgttacgtttagttctacgcgcttccaaaacaagaatttcacttgtaatgtactctactaggttactcgctaatatcctcccgacaatagctacccgttcgatagtcgttacacttttacaatttttctcctcgaaattttctacacaacttagctttatctccaagtttatcttttcttttaaagtagccggatacgttagctaatgaagtagataggtacctactagcctctgacatatctttaaactcaaaagattcgtttgtttcgatattggttatttttacaggaatagacgtagtatggcaaggttttctccctagtaccctaaaaccatgtttagtgttctctgatatagtacaccattcaaggttctccaaacggttgtcttgtttgtccccatttttatgattcactactggatagttgttagtgttaggtaagaaagtcatagcaaccactctgtggacaagtaggtacttcctaataccttccttgttatacatagctgttttgtagtaaccgtctttatcagtagacaacttgaagtatctgtccttttttctaattctgccgagggttgaaacctcgtaggcagggaaatcagggactgccttccagtattctttttccatataaccacctccttaaataaggagaaaaattgtacttagcacggtattgccatatctttcgacttaggttccaccgttagcctacataaagtagacaccctaggtttctaggttcacgtagtttatagtgagctatattctctaacccactccaccaccaagtttagatagttgaagtgcactgttcaacgttctaccaattgaagacattgaatcttctacttgaattagaaaacagctgacatactcccctcttctaagcctacctgcatttaaaaaagtaggggttgcaggttggtatctacggttaattagctcatctgcaatcttcatagcaagctcttcgtcaccatcacccattgtgagtgcattaaacgctactctatcttcataacgctctaggtatcgttccccatcatctgttttcattgcgtattgtttgtagaaacggtaagcccccataaatgtgtcgaatctgaactttttactatagatgaacttaaataatttttttataaattccattgagtacttgtcagtaatcactgttttatcgatgtacccttctctaataaggtaactaattttctcctctaaagagtagaaaaatactgtgttcttgtttacatgttctaaaaagaatgctctaacagcttctttatctttgtctaactgaatctttccgttattagggatattcaattggttattaagctcaatatatgtgttcatatctacaccccaagttctttttctagttttttaaccaaatcaggtctaacaccattaaatgagaaaccatcatcagcttctacatatggtaatgaagacactcctttttcttttagataagctaaagcttgctcatcatgagagatatttttctcatcaaatgggatattctttccatttaacatattttttaaaaataaacattgaccacacatatcttttgaatatactgttacttttgtcatttactacattctcctaacttttttatcgtatttattaattatacactattttgcattaattgtcaaaaataaagaaccaaaaaaactagagactacaaaagttaattgtagccccttttaataagttacaccttgtcacctaagaaatcttctgattcctgcgatttattcgtaaccttatcaagtagtaaaacagaatagtttttaccagtttcaacctgcaacctattaaacactttctgatattcttctggtgtgtctgtaacttctaataagtattttgcatttaaaaatgatagtaattcaagtagttctgccttactacctgccatttgaactacaacgttaccttcatcgttcgtgtatgttccaattttatttctagtagccaaacaaatcagtccttcgtaaatttaatgtatttgttaactgtatacacatttttaactttttcccaaacgttagggtatacgttcatcaataacttagtatctgcgctagcacgtttgtactctggcattaatttaaatgtgcccccatcaatactaattttagattcccctaactcttccatatcagaaatgatactactttttagctcatcaatctcttctttaatacttttttgcaattcatataatttcttgtaagagcgtaagtccttctctagtagctcctttttttgtaaatctgttgttttcatacatatctctccctctcttatttctataataagattatagcatgtcagatatgtaaagtcaacacttttttatacaaaaagaattgcccattataaaggcaattcttgtccgttgtcttcttcaaaaagaatctctacaggtatattatataatttagcaagttttactctgtttttaacacgaggttcttttataccgttttcccaataagagattgatgaccagtgaactcctatcatattggctaactctcgtagagattcacccctagcctctctcactcttttaaggactttaggttttggtaccttttcttccatgactatccctccttattcttaaaaaataagagcctatcaggtagacaggctcagcatcaggaactatgcgaaagccccgatataagttactttaccattacatttacgtgcaaaagcctctaactctttacgagcacctaaacggtcaggttgcgaagattgaacagtaatttctttaggtaccgttacttcacgtgtacgaatttcagttttaccattttttaatttcttctcatactcctctgtacgagttgttgtcgtagaaatgattccataaaattttttcatattaatagctccttactgttttttttaataaattataatagtggtaatagggttttatgagactcctactcattgtaagccttccttaatagatacttacaactatacgtttatagacctctctcaaaaagtctccgtaacgtcttaccttcatcatttaaaacgtacacagaatttacaaaagttttatacccttctttttcagttctgtactcgtaaggtgaatttggcacacgagtgatttcttcatgtttagagttaagtaatgaaaaagcattctcttgctctaaaagaaactgtaccccatcaattaattcaataaaaggcttaacaataggttcctctgtactgtctttacaatcgtattttcgttctcctaaaatttgtagtatcatgtctatctatctcctctgtttaagtattaatttgtgagtttccactcacaatgctgattgagagagtcgaactcccattcccgggttacaaaaccggagtaatagccattatactaaatcagcgtaacccctcaatagagggagtttcttatactaaattaccatatccgtaggtatttgttttagcttgtttaaacatgatactcttgatagctaagtcattgtacttttcatcgtcttcgtcatcaaggtacacatcaacattaacgttcttacctaaaatatcgattgtttcatctttacctacttgtaagtctttactgttaaatgatacatcaaaatagatgtcgtcttcttttgtacgactaccgaatgatactctatcttcaaataaatttaaacttcgagagttaattacaacaggttgtagcccaccttcaaattgaatagtaactgtataatactgattttcaatattaagaatgttcaaatcagcaatagcttcaccaaatgagatgccaaagcttaattccaacgcaattgctcgtaagcaatcatagtttaacttaattctacggctaaacttaacaacactgtcaatttccccatagtaagctttgtctaacttatcttgcaagtaagtacgaatttcgtctgcatcagggtagtcgaaacgtaaatggtaatggaaacgtcccggacgattaagcataaagtcgtttacacgatttaagttattaacagtaagtgcataaatacgcttgcgttgtgataacccatcgaataagctcaatagtttttcttgtgattcacgaccgtcacggtcattgaatactttttcaaattcatcgaacaagataagagactcttggtcaatactgtcaataaattctgcgatacccggataagcttctgtaattaagataacaggcataccctcttcaatagctcgttgagataagatttgagtaaatagtgatttaccaatccctttatccccacttaaaataacccctaaactacgattgattgttttaaatgtgtgtagtactttctcaattttaactaaacggtcaccataaactttagattctttcaatttaaaatcgtctgtaaccgccaatgagaacccagacattgggttgaatctaactttataagtttgcgcaggcaacttatcataagttttcaggtcgtttgcataaatctcataattactaccataattgattactttcatatattctctccttaatactttttaataaattataaatggagagtgatggagtcgcaccacccgagcctaagcaacagatttacagtctgctccgctactacttacggaataactctccttgaataaccaaccagataggtacctgacacacggacagcacctgtgtctctctgttactggatgattaattgtgtatttcgcatcacctaatatagttatcaaggtaggacttgactatactagatttagctaggttctaactataatttcctatgatagctcctactactaatcatatttatatacagttaaactacacataactaaaccgattaccttggttcgcatgttaagaggcgcaggcaaccaatggacattgcaggtctcgaacctgcgaccgttcggttatgagccgaatgctctgaccaactgagctaaacgtccgtagggtagtagcaacaattacaaatgctactctcctgatgattataaacttatcaaatcggaaagacaggacttgaacctgcgacatcagactcccaaagcctgcactctaccaagctgagctactttccgtgttacctgtttaatttggtcttttaaactactacacacaggtaaagataaaccctctgccaaggggagactatcatcgaaccgtatgtaagttgcgatgggtagtagccatattatattaggttattaggaagttcacctatgcagaaggtgggagtcgaacccacatgtccattacagaccgatgtttctaagacaccgttgtctaccagttccatcacttctgcggttgtactaccaaggttacctctaaaaggctaaactcgtgtctggtagggagccataccttacatggattgcaaggaacctaacctcagtagcaccttttactattaagggtttctgatttaacgttttccctagaccgtaccttaacagtaatactggtgagaggatttgaacccctcttacctacaagcctccgacaagcgctatgggaaacaagcggtgcattaaccataactatgctaaccagtacactactgttttacgcagtcctcatactaataattcatgtggactcaaccccattcagggaagtgttagtctattttttggtgagaactggttaactccatgtacgtcaaacattccctagactactcacttacattgttatttaatgtcacatgacttatgacagccgtactcaaaagtttcaaggacttttacctcactatccaccgacagtatgctcggcaacgtctttctaataataaattacccatcactgttacagtaacagaaccattgaattaacgagcaatatcagtattactaaaagtagtctgtctgtgtggtacaagcactagcagtattacaacctatagtatgtctgtttgtcaatcgttaaattcttttacaggagtacttgttaaacttagggaggtataacaagtatgtgcacataacccgagtgctactccctaaagtagcctatacgggttaacgtagatggagggaatcgaacccccaaccgtccgcttagaaggcggatgctctatccgattgagctacacctacaaattatgggggtaatgagcccccataataactcatagtagtttcatctatcgaggattaaaatgaatatctaacttgaataaagtataacactatttacatagcatgtcaacacttttattaaaataaatttctatacctcactaatgccaatgactatacgtaaggagagaacgttgatggcactggctacttagttggcgctaagttagtgaggtatagaaagagaactacattgaccgaatcgtattatacagccttagtagttgttaacaatgtttggaacttagtagcttactgcaataagctaccccgaagcatcggggtgggactgtggtaagccccaaacccttgggtatgctccatcctgcctccggagaagtcaggctcaattctcattagttaaaggtttactagttaacggttagctgattagtcatactacgtaaactactagtaaaatatagttttccaattaaggctaacaatcggtagaggatttgaacccctattattggttttggagaccaacgtgttaccagttacactaaccgactatgtaaagaaggaaagcgaagaccttctttacagtaattaaaaaaaacaaacaaaaaaaatacaatcatggaatcaaggtgggatgtaaggagatgccatgtgtccacttacagtggaataggtaactacagatttgcactgttttacatcttgtttaatggttacctgttaatagctaacttccagtgataagtcctcttatatggtagttcatgtagtatttgtttgacaatatggtagctagctaaaatgacgacagtaacgggactcgaacccgtgtgttccacgctgacaacgtgttgggacagcctctgccctatactgccattatttatgccgtagtttttttagaaaggaaagtttttttataatatacaacaacagttgaagcgctgatgttactacggcataaatatattttttatgagcttttaataactcaaaacttaatataatagggcttttactcctgcttcatgcacactcactgcattcggtcacacacccagagaggctgaactatcgggagctacccaatagcttctctctgcttttaatgtatggtctagcacggtggctaacaacgttcacctaaacattcagcattaaatagtattgttataagttcttcttatatcatatattttgtaagctgacttaggctacttgtaccaaggtctcttgttaaacccatatttctatggttctcgtcaaagggagtcttttgaggtttctaaggtctgccaagtttctcacgcttccacctaacttagattcttttccacaggaacgtctattatatcccccaagagtcttgtaccttacaatccatgtacactccacataacgcttaactgatactagcttttactagtagttactcttatgtcaccataagacatacctgctacctaaaacactatcgcactctaggctacattcagaatcacgccacgttatcctagcaagctgttcaaactttctgcactaggttctattatattaagttttcaattatcaaaagcagtttttctttactatttaataatagcacaacctctattattttgtcaactacttttttttagagagggtgcccctaattttatataggggcaagagatattaaacatagctgagctatgtaaaagctaatgtaggaattgaacctacttaatgtaagcaacaccagtttagcttataagcattgtttgcaaagtccatgctatgcactcagtaggaatcgaacctattgccgaaggtaccaaactaccctgagtgctcctatagatatattataccacataacgagatattaattttttttggtgatatagtatatctatattttttaaaattttagaaatacctttgatacattccggttatccaacgtatgaatatataatatcatgttattctgattgtgtcaataacttttttacattttttttataattgtgtaatgtcctatttctttttttctgattccttatatttataatatatactatatagtactatatatatatattaattactattagatattatatatagataataagaatctaggaaatttaaaataggacattctaatgctgactcagttacaataaacttatggtggctacctttttacaaaaatgtcctatttcattttttctatctccttatattattatttataatatatagtattaagtattatatattattatatatatagtatataatataagaaagacaaaaatttaaaataggacattttacttaaacaaaaaaaagagagcagttaagccctcttatcttaatgagaaatagttattaattgttcccaatctgacttcctcatcttctggtgtttcatcctctggtttcgtatacaagctagtgattctttctggaacatctactacgttctcagtagctgtctgtatctggaatgcatttacataagttaactcagaatctctatcagctagtttatgaactggaatcattggcaactctgcacctttcattgcaccatttacaattgacattgcatcattagttgttacaccgagtcttctagggaacacagaatatgtcccagatgctaatgaaacctctacaactttctctcttttagggtaattcatgatacttctcctttcaaaatatgttataataatactatatactataataacacattttacaaattacttaaacatgctgaacacgtaagtgacaactgctcctaagacaatcataaaaacgttctctacaatatccctcttgtggtcgaactctttatcgtttactccttccagtgcatctatagtttcttccaacttagtaatctggtaggttaggtgtgcatatttttcttcgtgaacagcaagtcgcttatcaagactattgacaatatctctcaactcactaaccgcactattcagttctacattgtcctgtttaatgcccttctcggttagctctccatgttggagtttatcttccagtcgttgtagtcttaaaacaaggtcatttacttggtaatcgttcatatatgctcctccctgtaagttatgttgctctatattagtcagatgtaaaccacagacagactagtatacctataatagcgcctaccgtgtagactataggtatatagtacccattaaaaaacaagtatagactacctatactaattccatagagcacgaaagtgaacttgtatgatgccaaagggctcagttctgcttgtagtttcttatactgtagtgcacgagtgacatagtaggacatcaagtaaacaaacatttgtagtaacagtacacagaccagtgctgtttcatacattat

SEQ ID NO: 2 - DNA, 143400 bp, Myoviridae Spounavirinae phiEF19G
gttgttccctcctctcccttagagctactattaatatagtacactgagctgttagcaaacaggtgtgctaaattaatatagagactaaaaatgtagacgggagagtggtaaaaatggataatagcaaacgaattattaaaaaaattatttttattaccatctctgcattagtcatggttactttaagtaagctgttctctaaatatgttattgtagaacaaaatgccccatttcaggcattagttggcggtgcctcatgtgcactgttatctagtattctgtttgactggtatactaataaaaagaaaaaagagaacgtagagaatcaacttaaagaagcaatcagtgacttgcagaagattaaagctatcataaaaagatagcctattaggaggtgggatgggtgtctattaccaataaagacattaaggataaacgtagatatatttttagtcaatctagtaaaacaacaactataaaaagaggggacaaacgcataagtagtgcaacaagaatatgtgcagtttgtggaagaccgctatctaagctcgtattaagaacaggcgtaccaacagtagtagtagaccatattagctgtaagatttcagacattgttagactaaatgtctgtgaggatataaggtcttgttatgcgtattctagtaagaaaggggaaagctagctaatgggtatggcagatagacttaaagataatgcaaaacaaaaaaagttagaaagaacaccagagcaacaactaagagacacatttaatcaagcttcaataaagcttatcaatcaatttatggctaacgttacatcaggtgctatagaagttgatgatattgcagatttaacaaggctatttcagatttatttacaggttaataatataaatgatggaatgcaagaaggtacaggaactctacctgcacttacatctgagcataaagacatcatatctgaaaaggttagcacagaaaagattattaaggacggtgaagaagaggagctaatttctcttgatgagttagccagtcttccagatgaccaacttgaggaagtcttagttaacagagagctacagatgaacagagagaacgaggcgaccttctaatgacgacaaaagcacaacatatagctaaaatggctaaagagatgtatggtacagataaaattacaacggagcagttagcttatataacagatatgctgaccccatcaacgtacctattgagaaatcactctgtgcgtaatcacccaataacttttattatatcaggaagggatgcaacaaaagcacaggcacatagaccataaaccaacaaagctgtggtctttaaactctactaaacgggcatagtaaaataatatacacgtaaacaatatactggtaagagagactaaatcctagtgtataaggacagggttgacctaccgtgctaaatcagttatactataactgtaaaagcctaacgactaaatttctaggtagctaactaaaaggagttagtgagaactagataaaaggcaaataaactatgcaagctcaataaaaataataatatacaggaggtgattaagatagctaaggacagaaaagaaattttcatagaaaagctcaaaagtgtaaaaggaactgactttgaacttataggtgagtttacaaagcaacgagaaaagactctatttcgtcataacgtgtgtgggcatgtttgggaaaccactccggttgtcctacttaactcaaaaaaaggcggagggtgccctcattgtcaatacagaaacaaagcaacttcaccaaaagaatacgaaaaaagagtaacagacacatttaaaggagaatacgttgtactcaatattaatgagtataaaaacaatagtactaaacttaaattcttgcattctaaatgtggtacagaattttatctgcgaccagcaagtttattcattaatgcaactagttgtcctaactgctctaaaaataaccgttgctcaactaagagaactactaatgagtttagagagttgcttcttaaaacaaaaggatactcctatgagctaacggaagatgcagagtacaccggagctaacaaaaaaattaaggttaggcatacaacttgtggttatgtttgggaggctagagctaaccacctgctacagggttcgggttgtcctagatgtaacgaatcaaaaggagagctattagtagctactattcttaagctaagcaacacctcttttttgagagagcacacctttgacgattgtagaagtactagacccttaccttttgactttgcattaattagtaataacaaagtgcgtggtttaattgaatatgatggagaacagcacacgaaaccagtaagttgtttcggaggggaacagaagtttaaaagtacagtaagaaatgataacactaagaatgattattgtactcataaaaaaatacccttactcagagtatcatacactaatagtcctgaacagattgagcacctagttcagcagtttttaaaaagcatagatttgttgtaacgtagagcaacctaaaccaaaaagtaggttgatgatatagtctagtcccctaataaatatcgggaaaccgagggtaaccaaatgggcaaccaaagataataaatgaccaacatagagacaaggcaataattaaatcaagacaattagggttaagattagcccctttataaagcaatttgtaaagaaaactctgttaaacgggcatagctgaataaccaataagctgataagagaacctaagtcctgaaaaggatagaggtaatcccgtgctaaatcagtgcaaagcactgtaaatgcctaacgactaaatttctaggtagctaaccaaatggggttagtgagaactagataagaaaacctcttaagaggaagtaaagcagagcaacctaaaccaaaaattaggttgatgatatagtctagtcccctaataaatatcgggaaaccgagggtataacgtaagtgagatgggtgttggttctatgctacagtttgcagacacgcatagttatgatgctgttaaatgtctttatacattcccaacgaatgagcaaatgactaaatttgtacagacaaggttagaccctgttttacagaatgggtactacagcacaattgtagaccaagaagttaactcattaaaagctaaaaaaataagaaatagttttttgtattttcgttcaagttcaaaaccgggcgctgtggaaggtgtcgatattgactatctatctatggacgagtatgaccgtgtacctgcattagcagaggcttctgcgttggaatccatgtcttcctcaccttataagatagttaacagatggagcactccatcagcacccgatatgggaatacatgggctctttaaagggtcagaccaacattggtatttacataaatgtgagaaatgtaattattacaacgaaatgagttatgatgcatataccccagaggctcctgtagagagtagaggtaacattctttgtgttaacccaaaaggggtcgatgttgttgctaaaacagtagttgacggctcattccagtttgtttgtcaaaagtgcggagaaccgttagacagatggtacaacggtgtatgggtacctaaatatcctgatagaacaaaaaatggtctaggtactagaggatatatgatttcccaaatgaacgcagtatgggtaactgccgaccagttaaagaccaaagaacttcaatcattgtctaaacaagccttttataactatactctgggtgaataacgccccttcaactggaaacagttgtcgaaaactctgttaaacgggcaaagctgaataaccaataagctgataagagaccctaaaccctaaaatagggcagtgggaatcccgtgctaaatcaagcgtaagcttgtaaatgcctaacgactaaatttctaggtagctaaccaaatggggttagtgagaactagataagaaaacctcttagggggaagtaaagcagagcaacctaaaccaaaaattaggttgatgatatagtctagtccgactgccaagagcagtaacaaaatactacgaaagtagcggtagctcgtatccttacgcagacttgaaattaactgttaacgactctgacgttgatagccataagagaaactatttaatagaacctgctaaagacagaggtgattataaatttatatctgttggtattgactggggtaacagacattgggtatctatacatggtgttaaaacaaatggtacggtagatttgataaaacttttttctgtaggtaagtccaacccgctagaccctaatgcaatagatgtagacatacagtctataaaattacagctagctccttacaatccagatataatcgtagctgacgtaggagactcaggggataaagttgctaaacttatgcaaatttatggaaaagaacgagtttttgggtgcgtttacccatcaacccctaaatctacaggtaacttagtacctacttggagcccacaagcaaataaagtatccgctgacaagttaatgcagaataaacgttacattaacaagatgaaagaaggagaaataggttactactcaaaaccagatacagagcttaatttatataaagagcactggaagaatgttgttatacgtgatattgaggacgaaaagacatcgacaggttttagacaaattatcggcagaaaaggtgatgaccactactcacaagcaagcgtttattccatgttagggtatgagtacctaatgaatgtatttacaggagtaaaagagtatggatttgactctgattgggtgtcaactcaattagcacctacgaaacctgatatatttacagaatttgtataggtagattgccttatttagttttagtcaagctgaataaggcattttgtattgtttgatatatatttttgtggtataataaatatagttagggggatagttatggtagacaacaatgtaaaaataagtaaaagtacaattgaaggactaataaataagtctttaagttatgagtacgttataaaaaataacgaattgctgacaaacgaatatcaacatattgtaaaagcgtatgggtttgacaatttttatgacatgtatctatatgcagatagctgtgattctaaagatatgtatttagtaaaaggtggtcaaaaagacttgtctaagctgaaacccgttaaaagaaaagttgttagaaatggtaaaactatgactacaactatttatgaagatacaggcagttcagacagtaataacagtaaccctttagacaaagagagtaaaaagaaaaaagagttagaaccagttaatgctaaggaactacgtaaggtcagcttaggtagtgatgaagaagagaagttagaccctaaaaagatagcaaaattgctagcagacactaaaaaatttggaaataattttgatacgcagtgtactgattatcttattcttgaacaagactctgttacacgaggagtggtagggtttactagagaaggttcttatttaaaaatgtctttctcaatgtcagatgaggctgttgaaggtatgaagatgttagctttttcacagctcacattaaaggcttggaaattgggtctaggggctaagataagcacagataatgcacctgatgtagaggaactaattagcttatatggatacaaaagaaataatacagagtatattgtgtcaatgagctcactgcgtagtcttctaggggagccttagtcataagtgctacgttagtcattatactagtattttcaactattatttttttaatttttaatttactagtaagtaaggtagttaaagaattttataacttaaagatgctagcaaaagagggactaacagataaagtaacagatataacaaatgatataatgcatatattgaaaggagaaataaataatatggaattaattatgaataataagaaactagatgaattaactaataaggtagccactgatgaggactacgatatttttgtagagaagatgggtaagctagttaaagatttgtatgagaactaccagtttttacaacaaaacccaccagaaggagactacacatcaggttattttttagggttccaagtaatcagagcagaatacccagttgagtatgagaatttatttagattagctgtagataaaaatttaaatgaactagagataaacaagagatttgtcgaagctgttaaggatggtaaagttttaccactaggtgaggctatcattgatgaattacaaacagggtgtagctctatactacaggcacaagaagtacgtgtaaatattgtatttggtacaaaagaatatatggctaagcaagaagaagagcgtaaagaacgtcaagctaagttagaagaagaacgagaaagagctatggaagtactaaaaacaaaagatgacgtgcttaacacattaagagtaactgaggctttggctaatgaattaacagatgaagtcgcagaaaaatatgatttaatggagctagttaacagtatgagagaggggctgaaagctcataatggaaattaaaaattctttggggaaagctcttataaaaaatttaagattgcttaaagaaaaaagagatgcaatgcccgataacttagaatatacaagtcaagttatgattcctgtgccctactatctaataaaaaaaggggataatgcagtagaatcattccttatgtgtgcggggatgataaatagggataaagatttaggtctgcctatttctttagagaaaggtaagcaacaagttaagcttaacaatggagaactgacaactattgtagaatgtgttgctacttactcagataaaactgatattgacggtgtagagagattcttagttgaacatctataaaaattaaattaacgagttctattttgtgctatattagatatgcatgaaatagaactcgtttctttttttatgactaactaaggaggtttaatagatggcaggagaagtatttagtagcttgattacaagcgtaaatcctaacccaatgaacgcaggtagccgtaatggtatctctattgaccgtattattctacatcataatgcaacaacaaataaagatgttgctatgaacacgtggctattaggtggtggtgcaggtacgtctgcgcactatgaagtcacaccaacagaaattatagggtgtgttggtgagcagtattcagcattccatgccggaggcacaggtggtatagatgtccctaagattgctaaccctaatcaacgctcaatcggtatcgaaaatgtaaactcgtcaggagcacctaactgggatgtagaccctagaacaattacaaattgtgcccgtttagtggcagatatttgtaaacgttatggtattccatgtgaccgacaacacgtgttaggacataacgaagtaactgcaacagcatgtcccggaggtatggatgtagacgaagttgtacgtcaagctcaacaatttatggtagggggctctaacaacgcagttaaaccagagccaagtaaacctacaccaagcaaaccaagtaacaataaaaataaagaaggagtggcaactatgtattgtttatacgaaagacctattaactcaaaaacaggagtgttagagtggaatggtgatgcatggacagttatgttttgtaatggagtaaattgtcgtagagtatcccacccagatgaaatgaaagtaattgaggatatttacagaaaaaacaacggaaaagacatcccgttctacagccaaaaagagtggaataaaaatgcaccatggtataacagattagagacagtatgtccagtaataggtattactaaaaaatcttaatactagatttaagaccatcttagggtggtcttttttctttctttgtaatattcgtaataatatgtaatggctatgtaaccgcttgttattttggctgtaacaattacatgttatattagttcttgtaagcaacacaaataaagaaaacattgaggagaattttattttgaagaaaactagtattttaggtttaagtttattaagtttaggtttagtagtaggtttaggaaccgaagctaaggcagaagaagtaacagagaatggtaagacatattggaaggtagagtcaggagacacactatcagaaattggagctaagtacaacttagatttcactaatatccacaaagttaataaaggtgttgtagctgaccctaatgttattttcgtaggtgacaaattgttattacctttagatgaaaatggcaagctagtggaacaagtgaataccactgaaccagatattgaagtacaatataacgaaccagtaacacctgaacaacctgtagttgtagaacaagaagttgtagagcaacctgtagttgtagcagaagcccctgcccctgtagtagaggtacctgctgacagtagctcagcaaaagagtggattgcacaacgtgaatctagtggttcttatgatgcaacaaatggtcagtatattggtcgttaccaactatctgcctcttatttaaatggtgactattcacctgccaaccaagaacgagtagctgatgagtatgtagcaggtcgctatggctcatgggagaacgcaaaatctttctggttagcaaatggttggtactaaaattaaatagcaataaagacctctttattaaggggtcttttttttatgctatattaatatatagtaaatagtaatataaaatggttatgattagttatgtggtataatagacttatgttaaaaccatttaaggaggggaaacatgggttatattcaagatgagacatggcagatggttaaaaaagttgctaaaaagaatgggtttgttggtgactggattttaattatccactcatactatgagtatggtggaaatcacgtccagatacatacaacaataaacggagaaagctatagaattttaagattgttagatagcagagagatacttttattagatagaaaaggtaaccctgtaatttatgactatgaaacagttaacgatggtcaaaaaagcttcttttataatgatatggaagagaaagaaatcgaaatacctaatggaagatgcttaaacgataagacaaggataaaaatttatgtataaggtaggtgtaacagttgccaaaatggttagataaagcactgggtatagaaaaatcgtccatagaagaaactaggaatatggaaaattataagatgcatttaagggaaatagacaccaatgtggtcaataacgagccgtacagtatggaaagtattgaaaaaggtatgaatggtaagaccactgcatatatgcaaccaattattggagagatgtcagtaaaccccgggtataaaactaaaccgtctatacgtaactctcaggacttacataagacacttaaaaagtttggtaataacataatattaaatgctattattaatacacggtcaaaccaagtatcgatgtattgtaagcccgcaagaaattctgagacaggtgttggttacgagatacgtttaaaagatattgaagcagaacctacttcacatgacattgctaatattaagcgtattgaaagttttttagaaaacacagcacaatttagagaccctaatagagataattttacaactttttgtaaaaaacttgttcgggcaacatacatgtatgaccaagtaaactttgaaaaggtatttgataaagatggtaactttatcaaatttgatactgtagacccaactacaattttcttagcaacaaatggtgaagggaaactaattaaaaacggtgaaagatttgttcaggttgttgataacagaattgttgctaaatttaatgagagagaactagcattcgcagtacgtaacccaagagcagacatcgaagtaggtcagtatggttacccagagttagaaattgcgttgaagcagtttattgcccatgaaaatacagaggtatttaacgatagattcttctcacatggaggaactaccagaggtatcttacatgtaaaaacagggcaacagcagtctcaacaagcactagacattttccgtagagagtggagaagctcactagcagggataaatggctcatggcaaatacctgtagtttcagcagaagatgtcaaattcgtcaatatgacaccctctgccaatgatatgcaatttgaaaaatggcttaactacttaattaatgttatatctgctttgtatggaattgaccccgcagagataaacttccctaacaatggtggtgcaacaggctctaaaggaggctccctaaatgagggaaactcaaaagagaaaatgcaagcttctcagaataaagggctacaaccccttttaagatttatagaggacaccgttaacacatatattgttgcggaatttggagaaaaataccaattccaatttagagggggagacctaagtgctcaactagataagcttaaaataattgagcaagaaggtaaagtattcagaacagttaacgagataagacatgataaaggtttagaaccgattaaaggcggagacgttatactaaatggtgttcacatacaagctattgggcaagcgttacaagaagaacagctagaataccaaagaagccaagaccgcttaaacagactattagagctatctggtggagatgtagaacaaccagaaccagaagagcctaaagacagtcaaaatgatacagatgtttcatttcaggatgaacaacaaggtttaaacggtaagtctaagaaagttaatggtaaggtagacgacaatgttggcaaggacggtcagttaaaatcggaagaaaacaccaactcaactaagcatggtactgatggtataaaaaaagaataaaagataatggagggggctagctccccctcaactttgtttgtgttactagatagtacatgttctgctatattaaatacagtaaaacgtttaggtggtgaaaagcaaattgtcagaagttagagaaaaatatagtattttcgtaccactggatattgaaaattctatacagaagtctgaatctgtgaatgatggtgaatggtatgttcaaggatatgcaactaccccagatttagatttacaaggagatattattttaccacagggcattgatatttcttattttattgaaaatggttggataaactatgagcataaaaatgatgctgagtttattataggtgccccaactagcaattgttatgttgatgtggacaaagggttattcgtagaggctaagctattaaaggataacaagtacgcacagtctatgtggaagctagctaatacaatccagaaatcaggaatatctcgtcagttaggtttttctattgagggtgcagtagttagtagaaatgcacaagataacagaatcatagaaggtgttaaaatacataatgttgcattaacgacacatccggctaacccaagagctacatgggagacactagttaaatcttggactacaggatatggcacagcaccagatgcacaagtagatgcaggcgcacttagaagagagatgtttaaagaggacatttctaatttgacgtatgcagtaagaactattgcaggactatataataaaaaacctgcagagaaagagtttattttacgtgaagtggctaaggatatagaagtagacacttccgaaaatgaattatctaaatttatgttacaattaagtagagggatttccttgaaagaagcaacaaactttattgaaaaaagaaaggggtaagaaatagtggctaaaacattaaacgatattatagaagattttgatgcacagttaaatgaaaaagtaaaacctactacagatgaggaaattacaaagtctgtagaagaacctactgaaccagaaaaagttgaagaaggtgctgaggttgagccggaagaaaagcctaatgaatctgaggagactacaggcaatgacggagaagaatccggagttactgaaacagttgaagcagaacaggaagaaccagaaactgttgaagaagtagcagttgaggaacctgttgaggaacctgttgaagaatcagcggaaactgttgaaaaatctgataaaactaaagaaaataaagatgaagaagaggaggaagacgaagacaaaaagaaagaaaaagacaaaaaagacaaagataaagaagacaaagaagacatcgagaagtctaccgaagtcgaacaagttatcaaatcttctgaaatcttaggagctatggaagctatctttaaaaatatgttaggtctaagtgaaaagttagacgaaattcatagagagtttaaagaagctaaagaagctaaagaaaaagacgaagcggagtctgttgagaaatctttacttgataaccctgaaattaaaacaggaaaagaggactcagaaggcaaggctgttgggtttgttaataagtctgtagcagttgaggaagaggtggctaccgaagaaccaactgtagaagtagttgttgatggtgaacaagacacagcagaacctgaaaaagaagtaccgttccgtgatagagtacaggctattagaccagactttatggaaacatataaacgtgtgtctgttagcggagtagctcaacgtggtgaattagaatcagttagacacacttggggaactgctagaacaaatgatgacctagctaaaattgaagggtttattaataaatataaataaatttactatatagtgaacgatttttaattgtactgctatattaatagcagaaacaataaaagacctgacattccctcctgaacctccacagggtcaggtcttatattgagaggaatataaagaaaggtgatttatacataatgacagagaaaaagaatacagaacgacaattaacttccgtacaggaagaagtaattaaaggcttcactacaggatatggtattacaccagaatctcaaactgatgccgccgctttaagacgagagtttttagacgaccaaatcacaatgctaacttgggcagacggagacttatcattttaccgtgacatcactaaacgtccggcaacttcaactgtagctaaatatgacgtatatctagcacatggacgtgtaggtcatactcgttttactcgtgaaatcggtgtagcaccaatttcagaccctaacttacgtcaaaaaacagttaacatgaaatacgtttctgatactaaaaatatgagtatcgcaacaggtttagttaacaacattgaagacccaatgcgtatcttgacagacgatgctatctcagttgttgctaaaacaattgaatgggcttctttctacggtgactctgacttatcagaaaacccagatgcaggttcaggtttagagttcgatggtttagctaaactaattgacaaacacaatgtactagatgctaaaggtgctagcttaacagaggctttacttaaccaagcatcagtattagttggtaaaggttatggtacaccaacagatgcttatatgcctatcggtgttcaagcagacttcgttaaccaacaattagaccgccaagttcaagtaattagcgacaacggtcaaaacgctacaatgggattcaacgttaaaggttttaactctgcacgtggtttcattcgtttacatggttcaactgtaatggaattagaacaaattttagatgaaaatagaatgcaacttcctaatgctcctcaaaaagcaactgttaaagctactttagaagcaggaacaaaaggtaaattccgtgatgaagatttaacaatcgacacagaatacaaagttgtagtagtatctgacgatgcagaatctgcaccatctgatgttgcatctgtagtaattgacgacaagaaaaaacaagttaaattagaaatcactattaataacatgtatcaagctcgtccacaatatgttgcaatttaccgtaaaggtttggaaacaggattgttctaccaaatcgctagagtacctgcaagtaaagcagttgaaggagttatcacatttatcgatgtgaacgatgaaattcctgaaacagcggacgtattcgttggagaattaactccatcagtagttcacttgttcgagttactaccaatgatgcgcttaccattagcacaagttaatgcttctgtgacattcgcagtattatggtatggagctttagcattacgtgcacctaagaaatgggctcgcattaagaacgttaaatatatcgcaacaggtaacgtgtttaactaacgctaatctttaaaagactaagcaaaattgaataaaaatggaataggggacggttaatactgttccctatttttattataaaatacatgtatggaggaaataatatgttaaaatcagaaatcttaataaataaaacagtaacaacagcttttggtgaggcaacatttgaccataatggggaaaccacagacctaacagtagaacagcaagaacatttagggactaaagttccatatatacaatatataccagatgcacctaaagctaaagaaaaagaagctactgcagaaaaagcagacgaggcacctaaaaaggctaagaaagcgcctgctaagaaaactacaaaatctaaaaaagaggaagactaaggaggtatttatatgtacccagactacggatacgaggaacaaggggacaatacataccaataccaaccatatgcacatgggaaccctaagcatatagatttagacaaaattgatgatatacagcctgctgattatggttggacacctgctacgctgaaacaatacatgtttggtgtagaagttgttaaccctgaaacaggggagcctttaggagatactttctatgaacatatcatagattcagcaatagctaaagcagagaaacgactagatattgctattatgcctagacttataagaggagaacaccatgattaccaccaatcagatttcaactcttacatgtatactcatgtgtttaaaagacctattattcaagcagaaaagcttcaattagaagttaatggtagagggctatacagatacccgtctaattggtggaaagtgtatgcactagcaggtcatatacaaatgtacccaacatccctcatgcagactggaacacagtttggttatgaaatgacgttctcagggtacccacaattagcaggaatgcctccatcaggaggacaagttgatgctcctcaaatgattcatattgactatgtggcaggaatgctacctaggaaaaatagaggatacaatgaagactgggagtgccctgcggacttagaacagcttgtaataaaatatgcgttaaaagagatattccaacaatggggtagacttataattggtgcaggtattgctagtaagtcactaacagtagatggtattagtgaaagtatacaaacaacacagtctgctatgtatggtggagcttctgcagatattcgacaaattgacgaagacatacaagaattagaaaaatcattggtatcttactttggaatgaacttaggtattatttaaaaaagggggttaacaaatgggtgaaaaaccaattagatttggtggagcaggtgaaacaggtaaccctaacaagcaattaaatactagtagggttgaatttgaaacaaaaggtatggctagcttcattgaaaatagaggtattgacgttttgtgggaaagagcatggctatgtacatgccgtaacccaatgaccctctcacctaagtcggattgccccatctgtaggggaagagggattgcttaccaacctgcagtaaaattaagaatggctatacagagtcaagagaaaggtatctctaatcaagatttaggactactagacacaggaaccgctattggaacgactgagctagattctaagataacctttagggacagaataacagtccccgaagttaaaatatatcaaagctttatttttaatgtaaataaaagaagagtagctaatggactatttttaagctatgatgtgaacagtatagaagatatttatggtaaagacggacgtatcttagttgatggagtcgattttagaatggactatgacacaaatactatttatccaaatgaatctttaatagatactaatatatccataaatatgtctgttacacttagatatattgttatagacctgttaaaagaaagtagataccagtataccacattcggtgttaaacaaacacaatttgaatcactacctaaaaagctcttattgaagcgtgaggacgtgtttattgatagtgaaccattttcattagacatagatacagcaagccgtatggaagagctagagggcaaaaaagatacaagtgaagctatggtagaccctaagcgtaaagctacaaaatcaggaggcttctttggaggtaagttaaatggctagaaaaggacagagacccgtattatttactgattcaaaagcaatacttggcaatctgactcgtgcagtggttgatgaagtactaagtgatgcgcaagatgttgctctacgtaatgggtcttctgtacagagaatgcctagctatttgatagtaacagagtctaggatggcaaaaaatggggttatagatttgaaacctttctttgcacgttctaataaaaagaaatataataaaaaaggggaatggtacctatacatccctattagtatgaaaacacgcaacatgtcaagacgattatacgatgagctgagagcagttccagtaggcacaaaacctgtaactgttaaaatggactatctgtatgatagacggaagcagagcccatcagtgtctagtattaactataaacctaaatctactaatgtaactgttataccacagagttggggtaaaggtacacgtaacacctatgtagctttccgtacagttaacgctaattctcctgcgaatagttggataataaatcgtagaaacgttaatgatgatgatatgagtaagacaatgctaagaaacatagacaggctcatgaagtggaaactaaagaatttaggaggatagtgtatgataccaagtttagacacttacttgtataaagaatttgaagaaaggctaaggataattctatcagagtgctatattatagacgaagctttaaagggaatggacaaagaagctttagaatcttttaaaaacacttattgctctatagatggtaagccacctaagagagaagtagagatgtcctattcattcccacaagaacatctggattcatttgctcgatttgtagtaactctcggtagtagcgaagaagatagcaagtctattggaggaatccaaggaggctacgagtatcgagaaggtaatgtaattagtgaggaagccactattattagagaaggtgacaagctgattataaatacatcaaaaccagtagcggactatctaaacagctcagacataagttttgcagaaagcgaccattttaggattgaagataataaacctgtatttgatttttcatacaatgaggagttagaaggtatatccattaatgtgtcgtatataagcaaaatatcagatgatgatgttgcaggtgtatacaaaggataccaatctaacgataatgttagtataattggaataagttctaatatagatactgctaggtgtttagatgcaattgctagaattatactaatcaccatgagagacagtttagatgaaaaaacagggtatatgttgcaaacactacattttggtgatatgcaagttgtcatagaatcaggtgaaacacttgtgtttggtagaccttgtactgtaaactacagagttactaattctattggatttgatttacaacaaagaatcacagagattattacaaaaaggaggatgaaatcctagtggctaaagaaacagagaaagtagtaaaaaaagaagttaaaaaggagcaacctaaaaaacctaaaggttatgtccatgtcgatacatttttagattatgcaaaagtattatatggactaaataaatatcaggtagcgggtttcagagcactaatggcaggtagagaataccaacacgaggatgctgattttgttccatttttagaaaagtatataggaaaggaagttaaataataaatggctgtagaacaattcccaagaaaaaaagtatcacgtccacatactgagattaccgtagacacaagcggtattggtgggtcatcaagtagctctgacaaaacattaatgttagttggctctgctaaaggcggtaaaccagatactgtttatcgtttccgtaattatcaacaagctaaacaagtactacgtagtggagatttgctagatgctatcgagttagcatggaatgcatctgacgttaataccgcatcagcaggagacattttagcagttcgtgttgaagatgctaaaaacgcaactcttacaaaaggtggtttaacatttgcttcaacaatttatggggtagatgcaaatgaaattcaagtagcattagaagacaacaatttaacacacacaaaaagattaactgttgcattttctaaagatggttataagaaagttttcgataacttaggtaaaattttctctatccaatataaaggtagtgaagctcaagccaactttacaattgcacaagatagcattagtaagaaagcaacaacattaactttaaatgtaggttctgaaccagaaagtacgacagaagtaatgaaatatgagttaggtcaaggggtttactctgagacaaatgttttagttagtgcaatcaatagtttaccagattgggaggctaaattcttccctataggtgacaaaaacttacctactgatgctttagaggcagtaaccaaagtagatgttaagacagaggctgtattcgtaggagctttagcaggagatattgctaaacagctagaatacaatgactatgtaactgtagctgtagatgctacaaaacctgtagaagactttgaattaacaaacctaacaggtggttctgacggaactgctcctgagtcttgggctaataaattcccattactagctaatgaaggtggttactacttagtaccattaacagataaacaagcagttcactctgaggctttagcttttgttaaagaccgtacagacaatggtgacccaatgcgtattatcgttggtggaggcactaatgaaacagtagaggaaagcattactcgtgcaacaaacttacgtgaccctagagcttctttagtaggcttctctggaactcgtaaaatggatgacggacgtttgcttaaattaccgggttacatgatggcttcacaaattgcaggtattgcaagtggtttagaagttggtgaagcaatcactttcaaacacttcaacgtaacatctgtagaccgtgtatttgaaagtagccagttagacatgttaaacgaaagtggagtaatctctatcgagtttgtacgtaaccgtactttaactgcattccgtgtagtacaagacgtaactacttacaatgacaaatctgacccagttaaaaatgaaatgtctgttggtgaagcaaacgacttcttagtttcagaattgaaaattgaactagataacaacttcatcggaactaaagtgattgacacaagcgcaagcttaatcaaaaactttatccaatcattcttagataacaaaaaacgtgctcgtgaaatccaagattacacaccggaagaagtacaagttgtcttagaaggtgacgtggcatcaatcagtatgactgtaatgcctatccgtagcttgaataagattaccgttcagttagtatacaaacaacaaatcttaacagcatagagtgtaggggcagttgcccctcctcttacataatgaataaaatataggagtgatatatacatggctagtgttggaaatcaaacagtccacacaggtaacacagtttacctaatgattggtaataaaattatcggtcgtgcgcaatctgcatcaggtgagcgccaatacggtacacaaggtatctatgaaatcggtagtattatgccacaagaacacgtatacttgaaatatgaaggtacaattactttagaacgtatgcgtatgaaaaaagaagacttagcaagtttaggaattacagcgttaggtgaagacatcttacaacgtgacattattgacatcgtaatgatggataatttaactaaagaaatcgtagtagcttatcgtggttgctctgcaatttcttactcagagtcattcacagctaacgaagttacatcagaaagtacgcagtgagattataaatacaaaatttatatagctgtgctagttcgtaaagagctagtatcgagagttaattgctttgaatccctaaagctcaacgacccaaacagtaactggaaacggtaagctgagaggtgcgaaagcagaaaaaatagttgagatggtataaggttaaatcctaagtactgatacaatgggtctttagcagggacagccctaagtcaattgatacgggacaccttcaacgactatcctctgacggaggagtaaagccacaagccaatggtggaagaaaaattctctaccctaacaagggtacccatatagtctgagctaacatgaaagtgttagaggcaaacgcctacttggaagttgcgttccaaggtaacaaaactgttcacatacctaacttctgcaaaggttaaatagcagacgaactccacccagcttgactgggtggttcttttacggtacaatacttttattattgttagatatttaggagatacaacatgagaaaaaaatggacattacaagaaagaaatattcttataaaaaaatgggcggagactaacaacgtaaatctcttaccagaaacagcaacctttacaggaaataagagcactatatactacgtatggtcagatggggagcttcaaggcttaataggtaaaacgaactttgacagtataatatctggaagtaaacctacagttaacggtctgacagaagagagcaaaaatattagggctaaaaaacgctttttggaatatgggctcgaattactagaggagtatcaaggattcaatacaccacataaggtgagagtgttggatggagtatacgcagggtattatggaaaaacctcattagccacagtcaatcaaaaaagtaccagaggtaaaatagcgcagttaaacataactattcttacagaaagtgagaaaagacgatatttcagagaatatgcagagtctcggggatacacaattattaactaccctgaaaaattagctgttcgaggtaagtgtactttgttatctccccaaggtaatgagtgggagacagtctggtaccattttgcttatcaggagaactgcaattgtccgttagatgttaaacgtagtattggggagcgcatggttagaagtttgcttaaagagaatggtattaactttgaagaacagaaaaagatagttattgatggtagaacattattttttgatttttacttacctgatgacaatacctatattgaatataatgggaaacagcactatgaagacaccggaggttactataagggtaaacttcaagatttacaggaacgtgacaaactaaaggagcagtggtgtaatcaagcaggtgttaatcttgttgttatcccatacactgcaaatagcataaacgaagtagctaatgttttatccgagatagtaccaattaaaaagagactagtttcagttgtttattctgatagtatacctaatgaggatattattgattactataaaacacatacaggtaaggaaacttgtaggaaatatgatttaacacaacgtagactgagcttactttgtaacagagtcggctttaataaaaggaggtacctaaagtgaaatatccatatttagtagaattgtatgcaaaacatgtaattagagatgcagggtacatagaaaatgtaccaccagttatttatgaagacgttgtgaaacgtgttgaagaaataaaaagagaagaaaacttaacaatagattaactagtataagtttaaatagacctaattcagatataggtctattttttttgccactataaatacaaataactagatagtgtggtataataaagatagtgctatattaatttatgagtaaactaggaggaaataataatgacagaaaataatgaaaaggtatttacacctacaccaaatttatcacgtgagcaattaatagaaaagttgcaacgtggagaaaacttgacggatgaagaagtaaatattttgaaatattacaatgatgcagaagaacgtaaacagttagatagaattatcccgggtgttaatgatgtattttctaagcattacaacttaaaagaatatggtttagaatttgatattaaaataaaagcacctaatattatcgaaaatggtaaaattcaggcaagaagagaagcctatttagaaggcatgggaatggcagttagcaactttattttccaaagttaccaaatgttagcaactattcgagtatgtggagtagaggtaccaaaagtattagctgatgatgaaaaaatttataatttatatgtattaggagtaattgcaaaggactatggtgaatggctaaactcctttcgatactagagttaaagaactaggcggaataaaagcccttgttagaaatagctatagtagaaatctatgggcaataatgaaaaaatttaaggtactaccgagtgaccctgcgtggcaaaatctcacaagtgaccaagtagagtggattttatataacatggaaagagacatagaagaacaagaacgactagctaagggaatgcagttagaaagtgagttccaagactatgacgattcatggtatgataaaccacatgatgagttctctccaattcgtgaaggtgacgatgaggaagaaattgctcgtaaacttagtgaaatcacaagtgaggaagacatggctaaacttaaagctcgttgggaggcaagccaagaagttgatgctatccgtgcagaaggtggaacaacaattgaagaagatacgattaacgaacttattgctaacaatgttaaaaaagcaatggaagaggctagacgtattgagaaacatggtggaaacaaatggcaagagaaatcatcaattgagttagaagaggaacgtaagaacctagagtttaactcacagttgaaacaaggagatattcaggaggctatcgatttgtttaacaaagatgtcgagccaacatcattagatgacgaatttcaaatttaagggtagggtattccctgccctttacttgtaaaggaagtgtggaaatgagcaacaattatcgtttttatgttgaggcaatgactggggatgctgttgcaaaacttaatgaaatagacaagttaatggataaaattgattcaaagagtgcaaagggcacccagaattttttccatacaagtcagaaagacattgataaagctgttgaggaaatgcaaaagcttatcaaggcaaaaaaagaactagatagagcttttgataatcagaagataaatgcagaaagcatgggagacatgacagcatataaacgtgctgtatcggatgcagaagaactaactagaagatttaacaaggcacaaaaagaatttcaaaatcatgctagaatgcaagctaaccctaattacataaatgctagtacactaaggcaacaaaaggcatttcgtgatgagttaacagaacaagagagagcaataagaaatatctctagggcacaacaggaactaaacagagtgaactctagggttaaccatcgtgcaaaccaagcaagcgcaacaggaagaatgacttacaatcagtcagagagtatgaagcgtgaccttagacgtactggtgtatttgaaagcctaggttcagaaaataaaagcagacagcaagagctacgagaacgatataaacagagacaagaagagctagcagagactagaagtaatacaaatttagatagacaagttcgtaagaatagggaaactagtattcaggctgagataaaagaaattgagaaagaaattgaagctagaaaacgcctagcagactctattaaagagactgtagagaacttaaaatctaaggaagcttcactaaatgcatctgacataaaagtagatgctgatagaaagagtgctcgtggtgttctagctgagcgtgcaccttctatatcaatggctatgctaggaggtaccgccgccgccataggtggtttatacgcaaaaggagcaactgctaacgcaggtatgcgtgatgcatctatatctttaggacaacgtacaggtactagtgacttccgtgcattaagaaaaagtatgcaagaaatgggtattgagaaacagttaggctataaaggtgctgacatgttacaattccaagaagatgcattgagtaatattggttttacaagtaaagaggacttagcagggagtacaagagccttagcagagggctcaagagcagttccagtagacaatgagactttaagtgacttcatgaatagtcaaatgaagagcggggctattagtggtagagaccaaattaagaatattcaagaaggtttcttaggtgctatccaacgctcagggatggcaggtcgtgagaaagaacagctagaagctcttaaaacattaagtgagcaaagctttactggtcgtaacggaagtaatcaagagcttaaagaacaaatggcaatgttaacaatgctaaaccaaacaggtaagcgtgctgttcaaggtgagcaaggggcacagttaatgtcaagtttatctgcaggtattcaaggtagtgtatggaacaataaggcatctttacttttaggtaaagggacacaattccaagggctagcaggaatgtacgacttaaaagctatgcaagaacaaggagcaacaccagagaacttacagaaaattattggcagtgtccaacaatcagttcccggtgacgaaaagtctcagaagtatgctttcggtagtgctttacacgaactattcggtacagatgctaagaatgaccaaatagatgcaatttgggaggcttatgccaacggtggtttaagtcaggataacgtagacagaataatgaatgaaagccaatctacaggaaaaggcaaatacgataagaacatagaagactatgcaaactctaaagaaggaaccgctaaccgttcagaagctgttacagagaaacaagcttcacagattaatgatatgggggacatcttaagagaaactaactctaaattaggagcacttcctcctgcgttatatgcgttaggagcaggcttaggagctatggctgtttcactagccacatcaggctctattggtggtttatctagtttaatcaaaaaaggaactcgttctacttttagtacaggtggaggggtaactgcagggggcggatttttaaaatcagctaaagaagcattctctgcaggtaaaggctctggcggatggttccaaggtattaaaaatgtaggtagtgtagctaaggactccgcaatgggtgtcggagctaaggctgttgaaggagcaaaaggactaaaaggtgccggaatgggcagtaaggttcttggtggcttaggaaaagcaggtaaattcctaggcaaagttgcaacccctctagcgataggttcctctctactagatattgcaaccgcagatgataaaacaaaggcggtaggggagagtgttggagctattggtggaggtatcggaggagctaagttaggggcaatgattggtacatttattgcacccggtcttggtacaggtatcggaggagctattggtggaggtatcggcgccataggaggtactctagcaggttctaaactaggcggtaaatttgttgatggtgttcgtaaattcttcggaggagaagaagctcatgcggaagaagcagacttaactgcagggcaagatgttgcttctgggcaagagagtaaatcaggagtacaagaagccagagacacggctaacaaacgagtcctatctgagaaaacacgtgcagagaataacgcagaagagtccgccaatctctctatctattctaagttattagatagagcccaacgtatactaaaccaagcaaaaaatcaaaacggtatattcggtaactcaggtagctctaaagattcttctgacggaatgggttcagatgcttctagtaaagactttggaggagactgggagaaagccattagacaagcatctaagaaaatgggagtagatgtttctgacgatgaaatagatacaatacttagattgattcaggcggagtctagtggtgacgagagcgccgttcaacagataattgatgagaacaacttcaatggcaatggtggagctaaaggtttgctacagtatgtccaaagtacttttgatgcatacaaagtagacggtcatgacaacataatgagcgggtatgaccaattgctagctttctttaataatagtaattggaaaaatgacctaaattcttgggatagccgttatcaaaacggtagtacaggatggggtcctactggtaataaaactagagcgatgggtgggcacataactagcccagagtatgcgctactgggagaggtagcaggtcaagatgagtatgttataaatcctagtcagccaacagctccacgtttattagcagaagctactagaaaaacagcccaaaacttccgattaacaggtaatggttctggtcatgattggggagcttcaatttctaaaataaatgcaacaggaggagctcaatcaggttcagctcctacgatgacaaatacaaatgaggtatcagttaatgtcaccatacaaggtggaggaacaagtgatagtatagctagagaaattggtgataagtcagcaggaattatcagcaaaacactcgatgctaccttcacagatttcttcgcaaaagaatacaggagagtgtagaggcttaatgtctctacttttctctaaggaggtttataatgtcagtagagttaagatacccgagatttgatttaactttttttacagagacagacaactaccatatagtttatgatgcaaaagatgggcttactggacgtaataacaataacggtgaagcagagaaggtaagcaataattttatggcagagtctgtaattagtttaactacaaaaaatgctttagaggatgatagtgcagtcttctcattcgtattagcaggggacgtgtattgggatagagtactaaatgctaatgatgcagttattcttaaaatagacccagatacttcctccactaaaaaatcagataaccctgtactactagttggtttaatatctgaggttagactagagggtgactatggggaaaactctaagatgtacaggataacaggacagtctttcgcaaaggcgctaatgcagtttgacttaggtgttattcaggaagtaagtgtagttttgacagatttaggttggttgcctgacgatgcacaagaaggtataaaaatgtctggtagtagtgcaagtcaaatagcagaaagcttaatgaaaagatttttacaatatatgaaatttaattttaatggtcaaggtatagataagttcttagagtgggagctagatagttggacagaggcggagagactaatagatagtaccccttacataaactatgaaggttctttaaagcaacttatagatgatgtaaccgctaaaccgtttaacgaattatatttcgatgcaacaccagagggtaaatgcagaatgattatgcgtagaaccccatttgataaatctgattgggaaaaattacaaacctacacagtaacatctgcagaagtaatatctgaatctgtagcagttaacgatacagaagcttactctatatttaacatatctattaataacttgtatgggactgactctatgatgttaggttctaaaccacaagtattccctgatttagtttctaaatatggttataagaaactagaagtacctaataggtatttagaaggagcaattatagataagagtaacagtggagataaagctaacacaaaacccgaaagtgataatgatagtaaagagagcgatggctcaacagctaaacagatgtttgacagagagtacgctcttgtcttaaactatctaaaagggtatcctgttgatgtgctaagagttaaaaaaagtaatgtaagaacatcaataacacaggtagacagacgtataacagataacgaagcagataaaattatagaccactatattacaaatcaagcattaagtaaagaagacttttctaaatttacaggaataaccgaagaaaatatagaagagggtaacggtaaagtagaacctacatataccgcagttagggacttccttaatgggttagataaaaacctaggagtatctagcataaaagagaaattaatgaactacttcaatttgatacctaaccaagccacatctattgctagtgaatacaaagcacaaggtaacttaggtaaactaaaatatgaagaaataatggagaataacccaagtgatagctcaaccgtcactggttcagataaacgatttgtttctgagttcactaaaagactagcaaattggtactgtgaaaacgctaatttctacagtggggatattgtagttaaaggtgaccctaaatatagattaggtaaccgtttgtttgttcaagatgagcaaaatggtgagttgtgggaatactacatagaatcagtagaacactcgttctcctatacacaagggtatatcactactcttggggtcactagaggtttacaaaatggaggaaacgatagattcactcatttatggggtaaatctgaggacttctccggaggtatgctaggtgagaaaaccttgcaagcactactagacgaacaagcagaagcaaacagtaaaaatgatggaggctctgatagtggaggtagctcaggtaaagagtatacagcaggtgcaggaactcagctagcggtattcccattagacgtaattaatgtaactcagggagaaaatggtggatacagccacatgggagcacttgcaatagacttttcagatggtactcctcataaaccttactatgcaccatttgactgtgaatgtgtgtacactgactcttactcaggggttgcatggcaatctcaaaagcctgttaaatgtgtagatggtagcgttacttacgtaacactattatgtgtacacgacaacaactgggcaagcaacaaagtaggggataagaaagctaaaggggaagtgatagggcactcaggaactgcaggacaagcatcaggagaccatgcccacttcgaggtgtctaaaggtaaatggcaaggttggagcacaagcagtgcgggagtttactttataaaaaacccttctcatttatacgatgtattttctataaaaaataatgtaactggaaaaacaactaaaattatgaatggtggagggtacaattggcgtagtatagactgggacgataaatctggctcaggttctggaaagaaaaagacagttggtgctagagccatggctactccattcggattacgtatgatgcgtagcgctcctgtagaaccagaagaaccaaaagttgttaaacaagtagaaactaaaacagttgttgaaaagaaaccaaaagtagaagttaaaaagctcccaatactttatgggaataacattgccacagaagcaactaaatggggaagagctcactcgaaaacagagtccacattccaatctgccttcaattttggagctaatacagataaagacccatttgaggaagacattatagcaacagacagtgcaggatttgtttggtggtgtttctaccatgcgggcatatcactatctggtggagctagaatggttaccactcgttcactactctatgataaccaattacaaactatctctactagaggtcagaagtctttagagctatttgataagatgaaggtaggagatttagtttggtttaacagagctagtcatgtagggatatattgtggtgagggcaagatggtctcttgtaatggaaaaggtaacatggatgagtccccaaaaacaggtattgttattgtcgacatgtctaaaggttattggtggaacgcttttgacggaaatgtacgtagatataaataaccctattttttagggttattttttttgtataggtagtttttagttattgtgctataatagataatgaggacacatgatgagaggatgaataaattggtaaaacgcagatttcaagcaggtctaggctcagaaattaaaagagtatataaagaaggacaacaaattaacacgctactattagcacaagtaattcaagtaaactataaatataatacagtagacctactagctttacagcataaagaagtatttcaaaattcctatgcaaatgagggacgtttctctgcaagacttcctatggaatttggcggtagaaatatcgttggacagccttatgggcaggttaacccgatagcagtaggaacagtagtattagttggttttattaattccgataaagacatgcctattgtaattagtgtttataataataacgatgtaagcaagcaactttcaagaacacaattttcaaattcagaccctaaagatttagagttaattggggatatgcaccaaaaatttagtttatacccttcattgacatatgatagcgttgatggagaaggaggacgtgtcgttactttttctggtaaatcatttattgcttttgatacaaaagaagtagctaactcctctacaactgatgcaggttatggtactaaatatgaggacttagagacatcatactataataatggtgacctaatagagcctatgaaaggtagagcaccaaatgtactgtttaagcatcaaggggtacttgacgatgatggcaaaccagatttgcacgatttgctaattcatattaacccagatggtacttatagaacttctatgatgaacaaagaagaggattggcgcacactatttgaaatgacaccagatggcagagttaaattaagaaaacaagactctattaatattgatggtggcatagaaataagtgagctaggaatcaacaatgaggggttcgtttatttacgtaatggggatatggatttagaagtacgaaaagacggtatctattcacaagggaaactgtttacagccgatgtagacctatccgatgtatatgacaaactaaatgggttgtctatacagattaaggaaacaaatggtcaattagagattatagctaatggtgtagaagaacaaaatggaaaaatatcagaactttctacagaaataacaattgtagcaggtaaagttgaatcaaaagtaacaaagacagaagttcaggatatgattgacagttcttttgtagatatgtctgatgcgattaaaaaagcacaagaagatgctgacaaagcaaataaagtgattgcagatatgtctagtgataatagactgactccgagtgaaaaaatagatttattaaaagaatgggatattataaaaaatgaatatccaagctatctcgaacaagcagaaacctacgaggttgacagtaaagactacactgctaagtacaattcattagagctatttgttacccctatattggctgacatggagtcaactagctcggtagacggagcaacacttcgcaaaacgtttaattcttactatacagcaagaatagctttactaaactctattagtaaaaaactaaaagacggtatcacagaggctatgaaaaaagcatcccaagcatcactagatgcaacacaagcaatggcagatgcctcacaagctaagattgatgcagataatgctaacaaacttatatctgatatagcaagtgataacaagctaacaccttctgaaaaataccaacttaaaaaggaatgggatgtaattgttaaggaataccctacaacaattgcacaagcagagaagtacgcagtagacacagcagagtatacagctaaatataaagccctagagctgtttgtagagcctttgtttaaagacatggatgaaactagtatagtagacggagaacgccttagagcgacattctcggactattacgcaagtaagattgctttactaaaagaagtaacggactcagctaaaacagagctagatgcctatggtaataaaatatctgtaatggaaacaaacattactcaaacgtcagaagctattactttactagctactagagtacaaactgtagaagacggtgtacaatcaaataaggcacaaatcgaaatacaagctgaacaaattagtcaaaaagtaactgctagtgaggttaaaggaattgtagacgattctattaacaatctaacattaggtggaactaacttatttgttataaagacacagacagcaggtttgctaaacgagaatgatggaactgtaggtactgcagtagacaactcagtagtgtcagactacattaaagttaatcaaaaaacaccatatattgctacactttacggtaacactggcacaaacatgattataacagactggtacgataaaaatagaacatttatttctggggaagctgtggcagactctggggattttagtaaaaagtatgtgtcacctgagaatgcagtctatgctagggtaagttataagaaagcaaactctgtgaatatcaaattcgaggcaggtacaaaggctactgattacagcccttcatgggaagacataaaaggtgaccaaactgctttagaggaatacattaaaaaagtagaagaacaagccaagaaagctcaacaagatgctgaaaatgctaaaaatgatgctgaaaatgcaaataacgcaatagctgatatgtcaaatgacaatatgttagcaccgaatgagaaaaaacaaatactcttacaatgggaacagattaaaacagagtatccaataaacttagaccaagcaactaaatttggggtgtcttctcaacagtatacaacagcgtataacgcactagacgagtacttaaaaccaatactagctgacatgacaacaacttctgtagtagttggttctactttaagaaatacgtttaacaattactatgacaaaagaactactttactaaacagaatatctgacgtagcaaaaaatgtagcagacaaggcacaagaaactgcagatactatcaatgataatttacaaaatattggtgggtacaactatgtagggttctcttccggagacaatatgttgcctagactgatgattaaaaacgttggttactacacattaggttcgtcaaccacagagttcattgacagcatggtagctgtaaaaggtgatgcaacgacccaacctttcgattatactgtaggtacttctgataaagaaattgctggtggcggtttagctgattatcgtatgaaagaaataaaagaaggtcagtggctaacagcttctgcgaatgtgcaggtaataggtggtggctccgctaggttagctatctacactttagaaggggataactgggtaggttctaacagtacacctatacaagtaagtgatggtttgaaacgtgttgtggctcaaagaaaagtaacaggcttaacaaaaggtgtgttaatacgtattgagtcagccgacactaatgttaaagagtttcgatttggtaatgttcaactagaagtgggtatcatcccaactccttggaaaaagtctgatatagatattcaagaggacataaacaatgttgttcagaatatcaaaacatacactgcttgggctaacgatttacagggtcttgattttacaagagaaaaggttgaaggaaaaacttacatgtatgtaggtacctctatgaaagatagtgataactattcagattatacatggaggctaactgatgaacatatagaaggtcagattaatggtaaggaaggcgcatggatttactctccaacagcccctgctaacccatcgcaaggacttatatgggtagacttgtcaaaagtccccaaccaacctaagcgttgggtagattcagaaactgggtgggttgcattaacaccagaagaggttaaagatttgccttggggtgaagatggcacaagcttagccgactgggtgtcacaggcagagcaaagaatatcttctgatagcattataaatactgtactaggttctgaggatttcactagtgtgttcgatacaaaagctaacacttctgacctaggtaacttggctacctatgaagacttagactcaataaaagaggactataaccggctaatcaaagaaggcataaatggtattgattttactccttatgtgactaactccgaactacaacagcttaaagacagctttaacttctctgttcaacaagccggaggggttaacatgcttaaaaactctttaggattctctgggttagacttctggaatggtacagtagggaagaacttactacctaactctacttggaatttaggttttggtagatggggtggtacttcaatcactagttttgaaatattaccaccagaagatgacaagcctacgagtaacatattagcctcaatgccacttcgctcttctactaaagaaataggtaacagacctcacccattaaaagttaactcgggtgaaacgtacacagtaagcttcgactataaagaagaagcattatcttacaacaaggacagacctatccttgttgtaagaaactaccctgataagaacacagaccaatggatggagtactcaatagaaggttgggcagtaatggctaacggaagcactactgacttaactgtttggagacgttttacaaaaacatttacaataggtactagtggctacttagatattttaccgaaaaccataatagaatcgtgggaacacaggtctttttggagagagctaaaaatagagaaagggacacaagccactacttgggtacctaacaaggaagacggggcgtttactggtgatattgttgagactattcaaacagaagaattagccaacctcgggtttggttccggatttattagttctaaaagacctagctcttcattaacacaatctgtagaactacctgaaataggtgctaaccttgagtattcactatctttttatatgaaggtaactacagataaccctgtagctgactttaaatgcggtattcgggtttatgatggaggtactctaacttatacattaggcatagaagatgcaacacagccaataccactagggttccaacaatacaagcttgtgttcactcccacaagtacctctactaaaatagaaatgtttgtagaaaatgggcaagaggcatctgttattatatcaggtattatgtataatatcgggagtatacctcttaaatggcaaccatatccaagtgagatatacaatacgaatgttaagattgatattaatggggtaaccgttaaaaacaatcaaacagatgggtatacaatgattactccccaagagttttcaggatactctcgtattgatggtaacatagaacgtattttcactttaaatggacaggtaacagaagttaaaatgctaaaggctgaaaaacgtataactatggaaccagtatctgtattcgctatgaacacagtaacggatacaaaaagaattagaggttgggcatttgtgccatcatttgaataaataattcaactttttaaccgaaaacctcacttacaagttgttttcggttaatttgtgttatactatatagagaaggacacgaaaggacgatgagactatatggctttaaacggaacaaagtatacagcctttgcccgacatagattagttttagagtggcgcgcaaatcaaaacattgcagggaactactcaacaatcagcgtatggctatatctacaatctatggataaatgggggagacttgatgctcccgctattggtgatgccaaagttaccgtagaaggaactacacagacagaaaaagcttcctctatgttaaatgctttccaaaagaaactattactagctaaagagtggagagttaaccataataatgacggttctaaaagaataactattgggggtagctactttgtaaacgttacttttactgataatggtgtaccaacatattacggtacgataactatacctaacttttcagtagacctgaatagaatacctagaagaagttcattaaaccctgtccctacattaaatttaccggggaacttaccaataacaataaataggcagagctccacattcaaacataatctaactgcttgggtggctaacagagataaccccacattaagtaatgatgcccattggacgtacttgacaaatcttaataatgtagacactagtgggtcatttagttttacagtagcaaataacaaaactatttttactgcattaaacaataggactagttggcaaggcaaggttaaactatggactatagggttagatgatgtagttagtcaggagagaacatacaagattgtccccccaatgaatgcacaagcatcgggaggtaagataaccttaaatgtgggagagaaaatcaatgtatcactaagtaactatcggtctgatgcaaactttacttatgatggggtatttaacattagtgggctcaacatacccattgctacaaattcagcagggaacacaatgtcgtatacactaactcaaacagatgtagacaatatattgaagaaaataccaaatgcggattcctcgtggggtcaagtaactgtaacaagtaagtatagtggagtacaatacaggactccatggacaggacagagaatagatataactatacctaaaaacaagtatgtaccaagcattaatggtacccctacttatgaagatacaagtagtgtctctgtcgggcttacaggtgacaatcaggtagctcttcaaggtaagtctaatatcaaagtgactatccctgctaactttgcaacggctaatggttactctactttgaaaacaattgatgtgtctttaggcggtacatcaaaaacagtcaactattcaaatgcagaaacagttgtagagttaggggctcccgctaaccatacatcagacaccttaatagtcacagtaactgacagtcgtgggtttaagtctaactggacaaagcatgtagacatttacccctacgaaaacccaaatatgtactttacagtcacacgtagaaataactttgagacaactacagatattaatgttaatagtacatggtctcctatcactataggtggtgtaaacaaaaatgctgtccaatcagtaacctacgcaacaaaagtagcaggtgttggtacttatggagcagaaactgctttaaattttacagctaatggtagtatggtaacagtaaaaaatacaccaatagaattagataataccaatacatacgaagttaggttgagtgtaactgataagtttagtacgtttactagaacagctactgttaaaccgggtaaccctatcatgtttattgatgccgataatcgaagtctgtttttaggtaatgcctttgttgacaataacaataatgagctaagaggcttattagagatagaaagagataagtggcaggagaatggtttagtaggaatatccttaaacaacagtgatatatcagcagtcaatggcatatggttctcgacagatacatcaaataacggaggtgaagggctccactttattaaatcaggtaaatcaagaaattcattgacttgggatgactatgattacttttatatgagggacaatggattctatgttaacaatgactctaaccctatatttactgtgactgatggtggggatttaaggttccctaaactggataacttatgggatggggcggcttacatgcacaaagaccagataatagtaccacgtaaaaaactcagtgaatgtagaaatggttgggctttaacgttcagttcttacgataaaagtacaggtaagctgtccttatgggatataattacattctttattcacaagaccgcaccggattctcctttaagtggtacaggtcacaggttcttcttaccagatggtagggatgctacatctcaaaagacaaaatatatatacgtcaatgactatcagttaaggggtcacgaagaaaatgatgacaaaggcggaacagctagcacaaataacagaaataaggttcttatgagggtggatgaatggtaaatatgagaacaatatacgtagaagtaaatgatgaaggttatgtagaaggttggggcagtaacctgtcaggtaataataacattcatagtgtaacaatagaggataacgaccagtttttttataaaaactccttaaattttaagtattcaaatggctctctagtattcgatgaagataaggcactgcacagtgctaaactagccaaaaaagatgaaatgttaactgcatgtaactatgaaaaaaatctacctttgacttttaaactagacaacgaaaattactttgctcaaccgttaactgcggaagaacttaatgaaacaatattgcctctgttgtcaggtttaacagagactgttcctcttgaattagttaaagtaagtgacgatgtacaagtaacattacaagttggatacagtgtaattaaaaatttatatgattatacaaatctaataaatgaatacttaaataaaaagttagaagtagatgtgtttaagatgatagatgaggctactacttttgaagaagttgaggaagtatcatggaaaactacaactagtgatgagttacctaatcaacctaaaatagaagacctccctataaataacaaccaagaaatcgtagataagttaaaacaagagaataaagagctaaaacaaagagtagaatttaacgaactagctttaatggatgcaataaacatgttttctgaaatgaacaagtaagttattattaactaaaggaggtgatatttctatgtacccatacttatcaatgttatatgcatcttatgtaatcaaagaccctgagaactatcctttagagaaggttccggcactaattagagaagatgtggagaaaatcgtggaagagatggcaaaaaagaacgaaaaacaaggatagttaatttagtaattggagtaacaataggtttaatcatagggctactaatttaaactaatataaatgagggtagtttgtgctaccctcttttttatactatattgtactatattaaggaacgaaaggagcggttactatgggacaatcagatggtatgggcggtacattaaaacgtattgcgattcaagtaggtaacgacccgaataaaggttggtatcgatttcaagtaaacccaactcaatataaatataataagccacatcgtgttactatatttaaaactaaatcaaacattataacagaagactttggtaaagatatagaaactatccaattttctggtacaacaggattcagggtagatagcagaggtaaaaatggggcggacagactaaaagaattagaagaaataatagataattacgcaaaacagggcggtaatggtaataggtctagtgtagagatgaaattttataatttcacagacgataaatattttgttgttcatttagcaccagaagggctatccattgaacgttctgcagaacagccattattatttaattacaccttaagtttagtcgtgttaagagaggcaggacagccctctgagagagctcaagtaagccctcagataggtaatgtaagtcctagcattggacggacatacaatgcacaacaggacactagaacacctgctcaaatacttcatgatgaatataggagaagtgttatgctaaatacagcagtaaatcctgcagtaacatcgggagcctataactatggtgtaaatgagttaaaaaaaataatcggatatggagggtagctcatggaaaaagtagaacaatcagcagatttgctaagattttttagatatttaaatgtcgatattaacggtgaagttgtagccaatgttattgacgaccaaccaaactttatatcaaggttctacacccctcatacacgagttaataaaatatctagtacactattagatattgttcgagataatgatataggggaaacaaataaggctttgtctaaagactccttaacttataaatttttaaaaagtggacttaagctttcatctccacgtatttacgagctagcacaaattgtagtactagaatcttttgctcttatatatgctatcgaagaagaaccagagatgtttaaaatgattaacgaatcagatgtaaagcagactagagagaatgttaaatacttaattgattgtttaggaggagcaaaagattatacagacatagtgatggacttacaatctatggatgtcgctctaggatatattcaggagcaagttcctctaatacaaggaggtttaccagtaaatggcacgatataaaaaacatttaattgtatatggggatacaatgcaatccatagcacaaaaagaaacaggctctgtagataattgggtaaaaattgcggagtacaatgacttagtttacccttacatagtagatactatgcaagaaaaaatgagcaacttagaacatctagctacacttggggacaccctttttatacctgatgaaggtaacttattggacattaatacaagctcattaaaccaaagagatatggatttcttattaggcttagctttaggtaaagacttggatatgacaagtgatacagattactacgagaatcatggaacaagtgatgaagtgtttgcaataacacataatgggcatggggacttgaagatagctagtggggcagacaatattaagcaagccactatatcaagattgatgacagctaaggggtctcttatgttgcacccagagtatggtagtgacttgcacttaatgttcggtaaaacaacaattgaacaaatgaagataattagtatagaagtatgcgatacagtacttaaagatacacgagtagcagaatgcgttctagtgaaccattatattgaagaagaccgatatgttggtaactatagagcaaccttaaagtctactagagagcaatttgagtttgttgttcaaaacgataactcaggggctctaattattgtatagaaaggataaggtttaatgagactaaagaaaatttcagagatactaggtagactaattgatgtaactatgataaacacacatgagataaacgatttttcagttggttctactattcgttctatttatgaagctgtttctatggagttagaacagtactatattttaggtagagagaatattttatggggaattgaacaaggagtcctaaatgcttttgactttaggaaaagagaagcaaaaagagcgtatggtatggtaacactagagttccatacggttactcagacccctgtgtatgtgccaacaggaacaacattcgactctagcttgtctggtgcccctagcacgttaacattccaaacgatgcaagactacataattccagaaggtgttataacagcaaaggtagaagtttattgtacaactgtaggtacaaaagggaacatacctaaaggaagaatcaatcgggtaattaacaatatatcaaacttaaaaaccgtgtataatgagtttgattttttaacaggtactgatgaggaaagtatagaatccgttaaaaaaagatttcatgcatttgtggaatcacgtggtagagcaacgataaaagccttagattacggtacacgtcaagtagaggaagttgcaggagtttatatcaaagaagaagtaggctacgttagaatatatgcacatgacttaaacggtgatttaaaacaagaaacactagataaaataaaagtagctattgaggactacagacctgcaggcattaaactggatgtattccctgtaataaaatccaatgtacaagtgagtgcaactgttactataagtgacaaatcgagaataaatagtaaattagaagaaagagtggagcttacaataagaaactacttaaatagtcaagttgtttcacaaccattaatcttagctgacctaattcaggttataatgaatattgacgatgttttaatctatgactgtaaaattaacaacatggaagggaacatggctgttagggacgaagagataattcgtgcaggagaggttattgtagaactgatataaattaggaggaatataatgtgagtaacttttataaaaatatccaccctctgttgagacgtggtaagaaacctaacaagtatgatgatactaactttgcagtgcttaatgcgttgaactatgaattaactcaggcagagcaggagaccattgctagtaagattcattcttcattagaaacagctacaggtgagtacctagatacttggggggactggtttggtgtatatcgtaaagatgattggaatgacgaatattatagaaaaagaattataagagaacttttactaaaaagagccacaattcctgctatcattgatgcgttattggatttccttaacgacaatgatgcagtcatccaaatatatgaaccttggagaaacattttctatacaaataagtcaaaattaaacggtgacgaccatttaatgggttactactaccgttttgcaattatcgatatttcaattgatagaccgtttcctcctgaaattgtagagattattaaggctttcaaacctgcgggagttctattttatctaaggctagacacaagcttaaataagaataaaacaactgtagaaagcccatatgtatacctagacgtgacgaataagacagaattagagttccttaacggtttatactatgacctacgaggtaacattaacctgtctgaccaacgtacacaagtagtagagagtaatatcttccatacgaataactctatgctaaacggggaagatgtgcttgcaggagcatttgaccacggaagaggctacattcacttagcaagtacaacattgcttgattacacaccaaaacctactgactctatgagtgacttaaaaacagctctaggagaatcaggtgctgatatgtataatcaaacaaaagaaaaggacggaagaacagcttctattcaagtacctgcaacaaagaatgttcacaccttgtactcaaacagcattgactttggtggctatgattattcggggaatccgaatgttatgactaagccttatattgctgacaatataaccggcggtacaacaggagtagttgtaacaccaattgatgatggcgcaagactagaaaaaacacgagttgatatatctggaacgtttaacttagcattgggtaatcttttgaataatacagattatataatttcatatgatgtacttgtggaaaatggatatgtaggagatttaaaaacttgtaatgttgcattagaaggacagtttgaaggaaagcctaactattttggtattttttatatgaatagtgtaacatcaacagatgtatggcaaaaggtttctgtaaaattcaatagtggtgccaacatggaaaaattaagtggttttaagtttagagtatatttatctcaacgtgttcaagcagcattaaaaataaaaaatgtgaaaattgaacgtggttcaacagccaccccataccagccaaatttactcgatgcaccatattatctgggtaaggtggctttgggtgagaatattgctaataagtccgttgagtttccaataaaatctagcaattatctcttatataacgctagaatggtagagccttttgttgtaggagaaccttatacaattaccataaaagcaataaaaccagccagtcaaacgtttatggtatataacattggggaaggaactacttattacggaaaactaaatccagttgagggattgacagacgtatggtcactaacattcacaccaagaaatgtttcgtcaactaatcctagcgatttacgtatttttcagtacccatcatcaacattaggcacatgtcaaattgattggttaaaaattgaaaaaggtgacaccagaactcctaacattgattcctacgactacgtaggttctctgatagaagatacagaaacacctacgttagacccgactaagtatacatggacagtaaatggggatataacaaataaaaaggcatatatggtgtttgatattaagacatttatcgaagaaaattatgctatagaatttgaaaaacttattactgacctaggagaagaccaagcattaaataccgtgtttgaaaactttaacatctctacaacacttaaggctctagtaagtccaagttcaccaatcagtttctcggttgaactatacgatttttctacgagtgcatggcacaagttaaacacggatagcttagacttacgtatgcgtacattcaacttagtagcaaaccgtatcacagactatctaaatgattacaagctattatttgttcgttacgtgtttgataacgaaacagataaagatgtaacagttgaactagacatgctaaatgtactattcaagtatcgtttaggtgaggggtacagtataggactacaatcatctgtggaatcactaacggaactcgttcctatagaagggtaatagcaaataatatgttataatataaatagggcacctagttgtgtcctattttttaataaacatgctatattaacaattgaatgataaagaaaagaggtaaataatgtggctattgcaactaacaattcacgagtgtatgcctcactccaattaaaaaataaacaagacagtatgtacctagcaattggtaaaaccactccttggactaatgaagatgccccccctgcaccagaccctactacggctactctaacagaggttatcggttataaaaaggtagcaagagtatctttatgtagagaatatctaccaagtgacgattctaaataccctgtggtgtcctatggttcaagaaaatttacgctaattccagatgaggacggctataaagagcaagcgtggatggtgtatgtagaagcagaaattacaggagatgaactaccaataggaacatttaggcaagtaggtattcatactgacttagtgtctaaggcaagttcagaaaagaaagctttgttacctacagatgtaacagatgcaggtattttgcaattttttgaaaatagacagcaacaaaatagaacaagtgatgtaattttaaaagagaagtttattattacaatggaaaataagaagtcagttaaacaataggaagggtgacatagatggctaaaaatattacaaatgatgatttaggtaaagagccttataacaatagatattaccaaggcaaacgattttcaggtttactatttaaaccagataagccgttacaacaagccgagttaaacgagttacagtcaattattcaaggagatttaggcaatgtggctgaatccatatttagtgacggtgacatccagactggtatggaatatgtactacaagataagaagcttactattaaaaaaggtaaagtattcttaggcggtaaaatgcgtaactttgacgaacagagtatcgatattaccggagagggtacggagtatgtaggtgttaaacttgtacaaaaagttattacagcagaagacgacccatcactgttagaccaaacaagtggtgttcctagccatttctcagaaggggctgaccgattagacgaagatgtagtactagcagttaatgatgattctgcatcaaacatttaccactttgttaacggtgagttatacattaacccagatactcctgagatggataagattaataaaatactagcagaaagaacttatgatgaatctggttcatatcgtgttcgtggttttgatatgtacacagaagttcacccaacagaccctaacaataaaattcagttagttgtcgattcaggtcgggcatatgttttaggttttaaagtagataaacctacaactactcgtattgatattgaaaaatcaagagagttagaaacaatcaataacgaaggtttctactatagcaatgcaactcgtaaaaataaattaggtaattccccagtatcttctgtagaccgtgtaactgcacaagttgaagttgctaaagaacaggtttctcgtggggtcgtaggtggaggtaccgattaccttaaaaacacctctgtaacaaaagttattcgtgtatggactgagggttcaggagcacaggagtacaaacaaggtgaagacttccaattagtaaacggtcaagcaatatcttgggcacctacagggcaagaacctcctgcagggggaacctacttcgttcaatatgtttataataaaacaatgattgaaaatacagattacaaagttgtaattactggtgaaggtgatgctagggaatggtatatcgactttaacgagatgacaggttctaaaccagtcgatgaatcacttgttaacgtagactataaatacttcttagctcgtaaagacctaattgtattagaccataacgggaatttcactgtccataaaggacaacctaacgctttaagactagtagaggcacctaaccatgtagacccattagttttagctattggtacagtagtagtttacccagactcaaatactgctgatgctaaacaatggacaatcacacgtctaacaatggaagagctacagaagttatctgttcgtgtggaaaacatggagtataaccaagcagtgttctacttagaccaaccggcaatggcaggagaaaaccctatctatctacgtggagtattctcggatgcgtttatctcactagataaatatgacgttagtcacccagatgccacaattgcttttgactttgacacagcagaaataacattaccttatgcagaaattaataaaacagttccaacaattatcgaaggttctagtgaagcacatgtgtggggcagactagtaacagcaccgtttaccgaagaagtgggtattagacaaccatttgctacggaagcaatgaacgttaacccatacaacacctttaacaaacagggtgccttaaagctaaacccttctgcagataactggattgaagatgagcgtatcacagttaccaaagaagaaacatctactatgactgttcgtcaatggtggagacatggtggagcatcttggacaaacgatgagatgaacatggtatctaacatcacgcttgaccccggacaatcgtggggaggtgcctctggtacagaagaccaacgtaaacaagggctatccggttctactttaaccagtggtggtcagcaaaccaaagaatcaatgattgagtttatgagacaaattgatgttgaggtttacgcagagaacttgcaacctaatgctaacaacttatacgtaacattcgatggcttgagagtacctgttaccccatcttctggttaccgtaaaggtgccacagaaggcactggtatggcaaatgcagacggaacatttaaaggggtatttaaaatacctgcaggagttcgttgtggtactcgtgaagtatctgttagaaacgatacaaacttagcaagtactacgttcactgcgcaaggtacgctaaaaacaactgaggatattatcataaaaacccatgttactattaacttggttgaccctctggcacaatcattcagttttaacactaacagagttgcaacaagttttgacgtattctttgcatctaaggataacagtacaaatattatttgtcaagtacgtggaatatcagaaggtgggcaacctaataaaactgtgtatgctgaaagagtgttaaaaccttctgaaatcaaagtatcagatgatgcaagtgttcctacgaaaatcagctttgatgacccactaatgtgtaaagcaggtcaagaatactgtttagtattcattactgactctgataaatacacaatgtggattgcaactatgggtcaaaatagagtagacgaaccaacacaaacagtaacatcaaatccttacttggaaggtgtcctatatagttcatctaacgcaagtgcatggtctattcaccaactgtctgatttgaagttcactgtatacacggctaaatttaacgaagaagctgtacttgagttcgatgttatgaagaacgttaatgtagaccgcatagtgttaatgtctacctacctaacacctgcaaacactggttgtagatgggatatgaaactagtccttgataatgagcctgcaggtacaacagtagatgacaaaccttggttacctattgctaactacgtagacttagatgttaaccagttagctcgtgaggctaagcttagagcaacatttaaagctaaccaatacatctcaccaatgctatccttggacgacattatgttcgcaggatttttaacagcattgaaaggtagctatgtatctcgtacaatagatttaacagaggctccatacaacacggttaaaatgtcatatgaacaatttacacctgccggaactgttgtgactgctaaatatagtacagatgaaggtaaaacatggaagacatttacagtacagcctacaacaacacaacgtacacaagactttgttcgtgtagactatgttgaaaagattaatacgggtgggacatttaagtccattaaattccgtcttgatatgacgacccagaattcatttttgcgcccgcgcgtaagacgcttactcactaatatgaccgacaaatagaagatgtaactgtaatgtaacatttctatgcctcctactgtggtatacttactgtatacaaaatagtaggaggttttttaatgggtaaagcattacaattagcaggtactacatttggtaaatggtacgtaaaagagcgagatacttctaagaaaggtagagcatactggatttgtgagtgctcttgtggaagaacagttcaatctattccgagcggtactcttactacaggctcatctgtgatgtgtaaacaatgtgcaaatgagaaatctttagtgggtaagacttttggtaggttgaccgtcattaaggattcaggtgaacgagcaactaatggtagtatcctttgggagtgtaaatgttcctgtgggaaaacaagccttgtcaggggttcagagttgacagggggtcgcacaaagagttgtggttgttactccacggatgtactcaaaaaagtagccactaagcatggattgtctaaagtgaacggaaaacccacaaaattattccgggcatgggcttcgatgaaacaacggtgttacaacaagaaccatgcgagttataaagattacggtggaagaggtataaccatatgttctgaatggcgtgaagactttgaaactttccatgattggtctatagctaacggattttccgatgacttgtctattgatagaattgacaatgacaaaggctattcaccagacaattgtcgatgggtagatgctaaaacccagattcgaaatagacgaaataccattacttacaactggaagggttcagagtacaccttagctgaactgggagaactaacaggtataaacaagatgactataaaatctaggctgaactccggagccactcttgaagaagcactagacccaaaagtgaatacgtcagttttgactatgagttacaagggagaaactaagcctgtcaaacaatggtgtaaagaactgggattgaattacgcaactgtacgtagcagacactataaaggttggactgatgaagaagccttaactggtatacgtaacaaatagcaacagaataagtataatagactctatatgttataatagacatatagagtctattttttttgttaggaggaataaaattgccagaaacacacagacaaacaagctcaggtgcgcttatatttaaaccaactatagctgaacaagagcataaaaatgctatggaatctataaaacaagagagaacagagctagagaaagaactagctaatgttaaagctatcaaagatgagttgtcaaaagagctagcagatattaaacaactgaaagatgaattatcaaaatagtttctaaattgtcttatttaggatttctggttcccttatactattaactaatatatttaaataactatatataaaatatataatatataaataatatataataagactacgaaaaatataaaataggacaaatcaactctgtatacaccttgacaattacctactatgtgatataatgaatatattgattatactaaggtgggtatgtcaaggagcatgtatactaatctaacttaaaggagatttattaataaatgagactagtagtagatattatgcatactcagataaggtatgaagattcggaaaattatcttagaccagaaattcataaggtaatgcattcagaattaggagttaaagcagatggttatcaatttagtcctgcatataaagcaggttactgggatggtattattgattttttcgataaagaaaatgacacgttccccacagggttactacctcatgtagaaacaatactagggaaccttcaatcaactttatcaaagtcaggttacatttttcagtttgagataattgatgatagacctgatgagttcatgtcagtagatgacatggataaggagatagtgcttaatggggataacaatgacaagataacattaagagactatcaatatgaatctgtggagcaagttattaagaacagaataggtattgtaaacgttagtactggtgggggtaaatgcgtagtagcatctacgaacctactgacttacgataaagggtacaaaacatttgaacaactgttcaaggaacacaacattgatttaacacaatcagaggcaactatccctaacacatttggggttacattagtgaatgaaaagggagaaccagaaacgcctagtcatttaactattaatggagttagacatgtaaacaaggtaacaactgagcatggatggactgaaacaattactgacaaccatccattactaactgtatcagaatctggtagctttaaatgggtagaagctaaagacttgaatgtaggtgattggattgttggacgtaaaggtgataatttatttggaacgaatactacatgtaccgtggagagcgcatatagcttaggtttattaacagcagacggctattgtgggcaaccaacccagattacattaaccaataaccaaccggagatactagcggacattcaagatttctttactaaagaagggctgtccactaaggtagaccctaacaaagactctaaagatagtaagatagttaggggtaccgcaggagctagagaactttataataaatatggcttatcacaaggattagccaaggataagtcaatcccagagtgtatcatggaagcaccgaaggaagtacagttagcttatataagtgggtatttagagtgtgaactgagtatggaggtacctaaatgttcaatagaggtaatttctgcctccgagaagttacttcaccaattacaactcttattaggaaacatgggagtttcctcaagattagctaagaaggtagttaaagggtacgaggctaattggtatggtagattaactatcggagtgactgactcagtttacctactaaaacaattaacatttaaaacagcacaacggaacgaaagaagagccttatttattgaaacagcagagtcccgtaatagtaaccaccaaggacaacctgtaccttttggtaaggagttagttaaacgatactgcgataactacctaggggacactaaaggacttagtaaggcattcaaagtaccaagaacaattagcttacatcggcttaaaaatttaattcatgagttccctaatggaaacccgacagattttgctaacctgacaagattaactgatggtagatatgtctattcacaagtaacaagtattgaagatatgggatatgaaccaacttatgatttacacatgcccgaaacacatagttttattgcaaatggtatgataaaccataacactgaaatagcatcaggacttatacagcaaataaccccttacttagagtcaggagaacgtattgcattttttacgaatagttcttctattttttcacagtcaattgaccgtattgagaaaagacttggaataaaagtaggtgcttttggtgcaggtaagaaggacattcagcaagttacttttgtaatgatacctacgattgtatctgcaatatctgcagacccagaggctaagcttaagctgactgctaaagaaagaatgtacaagaaaattgctaaggatatagctccaaaatttgaaagagggtttaaccaaaggagtttgcttgaaggatacctaaataactttcaagttaagacaaaagcagacctgcagttgaaacatgaactagaagaaattttttattcatgtggtacgaacaaacaggttattatgaaaatgaaagggtatcaagcagaataccaaaagattgttgaaaagaaaaatggtaaagttcttaagaagtacaacgaggctatggagtttttagattccatatctgtaatgattgtggatgaggctcaccatacaagttcagatacttggtataaagtgctaacatcttgtaataacgctcagtatagaatggcacttactggttcgattgaccgtacaaatcatgtgctttggcaaagacttcaagctatattcggggagattacgactaaggtgtctaacaacacacttattgagttaggtcactcagccaaacctaaaataacaatattccctattatagctcctgtagatattcaaaccactacgtatatggatgcctatcaaaaaggtatagtagacaatgaatatagaaattctcttattgcaaagttgactaagaagatgtatgataaaggtaatgggattttaattataattaatcgtatagagcacggagaggctattagtaacttactaaaagaagagggagtagctcactactttatcaatggacaacttgaaaatgatttaagggatgaaaaaattcaggacatgcgtgatggagcacttaaagtaatgatttcttctacgattatagatgaaggtgtcgacatttcagggattgacacattaattcttggtgcaggaggtaagtccttaaggcagacactacaacgtgttggtcggggcttacgtaagaaaaaaacaggagaaaacaaagtagaagtattcgatttttatgatttaacaaacaaacatttgaaaaaacattcagagcagagaagaaaaatatatgaagatgagcaatttgaaattgttgatattcctattcctaaataactataataaagaaagggtggcatacaattgcaaagtccatgcctaaatattgaattaaaagaaaaatttaaattaaacaaaggtataacagactttttagagagagttgcagataaatctcagagatggggtgaaacagtagcctcccctatccgtaaaacggatatggcaaaagagactggaaaaaaccctagaacaattacaagatatattaatcaattagaggaactaggtttaataaaaaccgaaacaaaaagaggaatgaatggagggactttagtcgtgtttaacacagatatgcttaattttgagccaaaggaaaaccctatcacgtctgatactaaacaagcaaaggagattagagaacaagttttccctaaagccccaaccaaagtaccaaaacgcagatacagaacaaaagcggagatagctgaggcacgtatacttagtgaaaaacttaaaaaacgtgaagacattttaaatgataaaattgagtttaacgttgttactagaagttttttcgatagttttgacgaaccagaagcgtactttaaaggctatttaatttcaagaatgtataatgcttatgtgacaatcattccttatgaaaaatataatagactgaaaaatttagatgagaaaaaggctaaacaacaactacgagcatacgaaagctcttacaattacgatgtgttgcctagaagatttgttgggacacctcagtacaaaaaatttgtagagctagctaaatattgtgaagagaacaatatcaatcctttagtttatttaacagtgcaatttgatagaacagagtttttgatttctgtaggtaaagcacgagtaggggctacaccctatgtaaatactttgttatgtgcagaggctaaagaggcttacacaaatagaaaactgttctacagaatgttacagaaccaatatggattgtatacgtctatcaattcagaagctacttattatggtgcaacttatccaattatttcaggactattgaatgcttacaatatgccacagaaagacttgtcacagttagatactgtgatttgtgacttagaatataaaaaagatattgacaaaaaagcaggtacgttgtactcttattatacagcaacacttaaatcgttaggtgaatctgacgtatctagtgaagctaaagaaagtattgctaacttcttgaaagaacaagttgcaaacttttctagtaaacgtgggctaacttcaacacagtatgccttagcgttccctattcagataaactctgcacgcagtttattaatgaatgaggaagacgaagaactactttatttattgttaggtaaccagtcacgattatctaatgtaacaaatgatgaagctgaaatgtttattaaacaaggtagaaaattaagtatgtcttggtggggctcacagaacttctcaagaacaatgttcatgttagcggactactatgggtttaaaacaaatatatctaagttaggtatgtacattaaagaatttggtgaggagaaaattcctttagattctgtaggtatgttagatgtaaatagaatctatgatgtcttaatgactgaacaagagattttagagattgacaaaagtaactgggagaaccaaaaagatatgcgtgacgacaaataagaaatataaatgggagagggacggatagtaagatgagtcaaattcaaaaacaagttatttatagagcattaagtgagccattctttgcaaaggaaatcctaagtaaaattccaatggatgagtttaaagattctggatatgagatgattgtttctacaatcaacttatattacagaacacatgatgagagcttagaggaacagagtttattaacactagtagaagataagatgttaaaacaaaacaaaagtttggaagctcaaaacaaagtctttgaggtagttagcgacttatacgaactagagaacgaagatgtagactcagaagttatcagtgagaacattcagaactacgttcgtaaggtactaacacgagaagcaatcatgaaatctgtaacaaatgaaggcacactaggctctgatagtaatattcaacagctaatggatgacttgagagacattcttactatcgagacagcaggcaataattcagaattgctagacttcttcgatgacgtagataaaaagatggagttacttgcaaacttgcaacaaaacaaatacccaactggtttcacagctatcgatgctatttccgatggtgggctagctcgtggagaagtcgggatggttgttgcacctactggtggtggtaaaactacttgggcagttaaccaagctagaaactatgttgtacgtggtttaaatgttctttatgttcctttagaggaaaaagtagaccgtatgattgttcgttttgaacaattattatcacaacaaagtaagaagaacatcttagttgatggtgaattgaataaagacttgtatacccaaatccaacaagcgtatggagcgggtaaagaacagatgaattggggtaacctttggattcgtaaatataaaccacaagagctaacacctagcggtttatctcagttaatctccgatgtaatgattcgtaaaggacagcaaattgatgttgtcattattgactacccagatttaatgaaaaatcctcatgcaagtggaagtaatggtgaatcagatgcaggaggtaaactgtatgaagatattcgtgcgattgcacaagaatatgattttgtttgttggacgttatctcagttgaaccgagcaagctatggtcaagatattaaaaatgcaggagctatcgaaggctctaaacgtaaaatgaacgcagtagagcttatttttacattaaaccaaacatcagaggagtttagtaacggatatttgagagcttacgtagataagttacgtaataatagtgggattgcctatgataaaatgttgtattttaaagtactcccagaaactatgactattagagatgaaacaccagaagaacgagcagaacatgaagcactgttagcagataatgcgatgaatagagcaagtagccactctgatgagaataactacacagcaaacgatgttaataaaaagataagtaatttgaataataccctttcaggaggttggaattaatgaaacatattattaatttttcagattttcatatgcacttttttaaagatttttcaaaaccagacccagagtatggaactgatagggcaaaagagcaaattactatattagacaacttgatgaactatgcacgaaacaaaaatggggatgttttatttaatggagacatgttccataaacgagtatctattgatgttagaatattcaatatgttatttcaagtaattagtagctaccctgatgttgatgttatcatggtcagtggtaatcatgataaggtaactaactctctatattcagatagtgctttagcaccatttagtgctttaccaaatgttacagtttgttctacgttaaacaagattgttaaagatgattatacgttgtatgctgttagttatggggaagaggtcgaagagatgaaagcttggataaaagaacaagctgacaatttagaccatgaaacagttaatattctaagtgcacacattggtgtagatggttcatctactgggaagtactcccatacacttggtggtgcttttaaagtagctgatttataccctgacaagtttgacatagttacattgggtcactatcataaacgacaatttttaggaaacctatctaatgtgttttatgtgggcaataccttacagacttcttttgcggatgaaggtcaagaaaaaggtttttatgatattactatagagggtaagaagtgggaacaaaaatttattaaaactgactatactccgtttgaaacagtaacagctgataacccatcaacaacaggttctatggagaaatcttatatccagtttatcggtaatgtggatgaggttgaggctgtaaagagaataaaagaagagaataacttaagcaatattagaataaaagttcagaaggactaccatgttgagccacgtataaacataacagcaggttcgacacctaatgaagttgtcaatgcatttattagtaaaaagtaccctaacgcaaaaataattaaagaaaaagctctcgactgtttgagagaagcaatggaagtataataattgtttagcctagatatatctaggcttttttgcgttgtactattgactttattagtattttgaagtataatatgtttattgaaataattaatattttgggaggaaaagatgttaaagtttaaacgagttagcgcagagaactatatgtccattggctctgtatctattgatttagacaaccaaggactcgtacttatcgaaggtataaatgatacaaacgaaacatttcagagtaatggctcaggtaaaagtactttactgtctaccgttacttatgcattgtatggagctacccctagtggtttgaaagctgatgctgtaattaataaacaagcaaagaaaaatatgtcagtgattttagaatttgaaaaagatggggtaccatatcgtatcgaacgttatcgtaaacactctaaacataaaaatactactagatttttccaaggaacaaatgatataactcagaaatctgtagcagacactgataaaaagattcaagatgtgttcggtattgattacctgacttatgctaatagtatcatgtatggtcaaggtaacgtagaaatatttgctacagcaactgataagggtaagaaacaaatcttagagaatttagccgatattggtgtttaccgatatgcacaggatgttgctaaagaaagagcacaaaaagcactagctcttgcagaagagctgaacagacagtacattgctaagacatatgaaaaagatgggttaactcaatcttacaatagtgctttacaacaatatgagaatacagaaaagctgattcaacaaaaagagagtgagttagctaatgcagaattagctattaaacaaagtgagaagaatctgtcagagggaagagcgctacgtgaacccgaattagaaaagctaagagagcagatggcacaactaacttcccctgcagacgttcgtgaaattgatgtagaagttgaaacacagtattctaacgttagtagattatctagtgcaaaaacacagaatgatactgctattgagaaattaaaaaaagaactagaagatgttaaaacaaatacaaattgctacctatgtggtgctttattgagcccacagcatagagaacaagaaattcaacgcattcaaagagaaatagcggataaagaagcgtttatcgaaaagcttaatagtgcattagcagtgtattctcctctgttagagcaagcaagagctaaacaagaggaagcaagaaaagctattcaagaacatactaatatttatcataaacttaatggtgaaatgaatgcgttgtatcatgagatagatacattagagaacacattgaacacatctattaataatagggacagcattaaggatatgttagcaagactacaagaaatacctaaacctcaatatgactatgacaaagaccgggaaatagaagatgagctaaataaaattaaccaattaaaattagatgccgaagaagaagctagtcaatataaaactattgcacaagaaattttctctaataaaggcatacgctctgaggtacttgacctagttacacctttcttaaatgaaagagcaaaccattacttatctaccctttcaggttcagatattgaaataaactttagtacccaaacagagaaagcagatggtagtttagctgataagtttgacttagaggtagtgaatggctccggtggaaacacatatcaagcaaactccgagggagagaagaagagaattgatttagcaatatcttttgctattcaagatttagttcagtcaaaagcaaacattgctgttaatttaggtttgtatgatgagtgttttgatggtttagatgcaattggttgtgagaacgttattaaaatattgaaagaacgccaaaagaacattagtagtattttcgtaataactcactcggagaacttgaagccattgtttgagaacgtaatcactatgaaaaaagttcaaggtcgttcttaccttgaagaaagtaaataggtgattacatgaagatttatacattaagtagagagttaaacgaaggtactatatttgtacctacaagtagtagtaatgaagggagactatttagcttcccgctagagacactattcgattggtacccttgttgcccaagatatgagtatcagtacagcacttctcgaaaaaaactatatttgagattgttagactcagacaaaacattagtagctagatacggtgttggggataataaaaagagagttatttcaaaaatagcttgctttaatgagaatgaatggtataatgaagaagtggcaaatgagaatgcagagttgtttaactttgctaaacaatatgacattgttacacctttaaaagaagattacaccttaaaagaagtagataatagtatctctaaagtactggacattcttgatttactttacacaaatcaaaaagttaaagtagaagaagagcttataaataaagtggatactctacaattgagtaaaccagactcggatgaacttaaacaagcgtataaggatatatctgagtatatgaggttagacagagaggaaaaagctacttatgtattaagcaggtcactagactctttaaatagtgtttatgaaaaatttggtaatgtgtatacaatgttaaatattatgaggaaagtagtggcttaaatgtttacagacttgttatctaacgaattaggttcacctaaatatgcagtaagggactacaggtataattgccctttttgcgactacgatactaagtataagttttatgttagggtagaagaaggacacccaaagaataacttatggcattgttttaagtgtggtagttcaggtaacccagtatcttttgtaatgaagtattacaacgtgtcttttaaagaagcgctagagatattagaagaatacggctataggtttaataataaaaattatgtgcctaaatcagataagttaactgatgaggaatacttattacttcttctaggttcgttaggtaagccaaaagaagaaactaaacaagctaaaaaagagttagtagcacccccattgccagatggttttaaactactaagtcagaacctgagagagccagaagcgtaccctttcttattatactgtaataagagggggtttacattgaatgatatttatatgcacaatattggatatgtaaaagattcttgggtacccttagaaaatggtaagtcagttagactcaaagaccacttagtttttttaactcatggaaaagatggtaagtatcaatattggaatactagggctattggggaaagctttattaagtctttgaacgccccaagtaaagagggtgagcattcaaaaaaggatactatatttaatattaatagagctagtcaaacccctcagatagttataacagaaggtgttccagatgcattaacagttggtgagtctggtgtaggtacttttggtaaacaagtgactgacgagcaagttgaacttattttagatagtgtgaatgaagagcaaaaaatatttatctatttagataaagatgctaaaaaagaaattaagaagttagcagagaaactatataagagacataacgagacttatgtagttataagcccaacaactcaagatgcaaatagtctagggagagaagaggcttggaatattataaataactactctgtaaaagcagatggagtagggttaataaaattaatgttatagataggagagggaaaaaaatgaagtatacactagaagatttacatgcaggtatgaaattacgttgcacggacaataaaaactacagtttttggactacgaataaaatctatgaagtaactaaaaaagagtcaggttcactatgtatttttgatgattatggaattgagagcctagatgaggacatcttagtacgtttaaatggtaatacagggaacgcagaatttgaggttgtttctaaggtgatgaaggatgcagattacacagaagaagaccttgaagaagggatgttacttcactgcaaagatgatatgagctttccatggtgggctacaggacaaacctatgaaatctataagggtgaaaaaggaattttatttaccaagtcaggagacggtaaccaatactgtgctaaagaaatagtagctcgattaaatggtagtgcaagcgggtcttttgaattactagaaagaccacataaaacagagttagaaaagaaagtagaagcaagaattaaggaactaaaaggaaagaaactttgtttattctacaagcaacaacaaattaagatagaagaaaacgaaatatctatagaaatcagtaagctaagtgaagcattaaaagcgattgacgtattaagagaatttgaataagaataactataggaggacaacaaacaagatggaaagagtatcagtatactttctaaatagcagaaatattatggatgaggatgagacaaagcgtacttatcatggaacatttaattcaatgaaagaagcagagcagtcagttcgtgactggtggaaagcaaatgactttaagtgtggtacccttagaattattgaaggtactgaggatgggattgttcgttgggactacggaaaccatactgggttctatctatttgtaccagaaggtgctgtagtaaaatacacaatccgtgaaggcgctaagaaaccaaaacgaggaagagaaaatgatgtagcacatgacttgttcacagcagacgatggagtagttattcccgggagattaggttcaaatgttatttctactggaataaaaacatcgtttgaccccaaacaatatggtttattcattaaccctcgaggtggtatgatgaaatacccaatcactttaggaaacacacaaggtgtagtggaaggggaatatcgtggagaggttggtttaccacttaaaaatacgttctctttacaattagatgcaagagctgtttctaagaacgttttaacaatcaatgaagaaggtaaacttattaacatcccagtaacagtagctcggtcaatgtatccaagctttaatgctctttatgaaaaacagctagagaagctaagtgaggagctacagctagtctatggaggagaagttagaatatctaatgctgatgagtatgtggttgcgggaacactatttatcccaaaaggcactcgtttatgtcaagctttcttactaccacgatacgacacacagtttgttgaagtatcagcgttaggtacaactgaacgaggagaaggcgcatatggctcatctggggtggtatagctatgctcatcccagaatttaagccaccattattgtacgttatgggtagcttttctgttatgttagaaaaacaccagtgcagtgtaacttttgatttaagagagccttatttaggtacctcttacgataaaatagtgaagcttattaaaatgacttacccaaactatagcttaacttatgtagggatgacagataataaatataagttcacattaaagaataaggaggactagcatgtacaccaagaaagaggaagtagtgacagttaaacacctagttgataaagagcaaattagagtaggggacatagtaggttacaaaaagactattagagggttcgatgcaaaaagagtaaaagacacactctcagtaacaaatcaaataggtgtagtttctcgtgtatgtgacgagtacattactgttcatgacttttttgataagtgctcacgagaaatatgggcaaagacatttgaaaatttagaagttcgcaaaatagaggatggtaacagcctactacggaggtatgaaaatgaatttcgttgattattttaatcagatgcagaatttagtgattgaagaaaaaacagatgagtatgttttactagagaaagaacatggtcaaaagtatgtgacatatcaagagctagaaggagcgttaagtacagtagcacgcaacactgcatttatggtagaaaattataaccttatgcaagatattaatttaaaaattgtattgaaaaaattaaaagacagtggtacaattacagaagagcttgaaaaagagattcttaaagagttcaaaaatattgaaagtttaatggaggacgaaacatatgagtaaagagagtaaacgcaacaaacgtatcggggagttatcggaagcagacatgagagtgtgggctgagtggttagccacagggcaggttcatgataaaaaccaccaaaaacagttagaacgcttaagtaaacgttcagtatcattatctgatgtaactactattgtcgaatttatgggcaaacggaatgatggttatatttcttctttaattgaacagcaggctgtatttgacaatttattaacaaaactaggtgtaacggaagagaaccgcttagaggctaaagcagagtacgaaaaagagttaagccttattcaagaaaaaatccaaaaagagttagagtctattaaagaaaataaagaaaaataatatgaaagaggttagctgaatgacagactacagcgcagtaggcaagaaaagtcgtaacaaaggcggacgttttgaacgtcaaatggctaaagaactcacagagtggtggggatatgagtttaaccgagtacctgcttctggggggcttcactgggcttctagtaataacgttgccggggacattgtagtccctagcgatgctaacttcccatttgttatagaatgtaaaaatcgtgaagactggacgattgagaacttattcttaaataacaaagaaattaagaactggtgggcacaagttgtgggggatgcaaaagaaacgaaaaatatcccactacttatatttactagaaacagagcaaagaattttgttactatggcatataatgaaaaacttgttaatgagattgaaaaaagaggttaccctttgatggtctctaacataacatatgtagacgactacaaggatactcattgttacaagacatttactacagttttagatgcaataactagctttaagccttatggtagcaaagataaagactactttttattttattttcctagtgactatgactgggaagatagcctagtttatgaaacaaccataatggatgatgctaaacaaatggatgcagaggattcactagatgcactagttaattcttatttaggaggagaatagtatggctaaaacatatcaggaagctctagcaacggtacagtcgtatctcgaatcagatagtgtaatgaaagaaacctcaagtatatctgttagtttctcagctaactggacaggtgagcgggaagactacgttattgatacattgacatacgacattgatttacgagtattcagcttagaaactgcacatgttgtagctatagggaagaaactacctcaagatagcaatgagcatgctgaactccttaaaaaacttaaaaaagaatttaaacaagcttctaaaaaactacgggaggactagagtagatgatagacaacgttaatagtcctagtcattatacgcaaggagaaatagaggtaatagaggttatagaatatattactgctaagtaccctgcggaaattagataccatttaggaaatgttattaagtatatttgtcgagcacctttcaagggaaagctacaagaagaccttaacaaaagttcttggtacttgaaacgagcacaactggttttaacacagtcaccaagtagctatataggtaaatgtaagaaatttttagagaatttcctatttaagaatagccatatcagagatgctcagctaatagaaattccagaagaacctattattgagaaatttttatttcaaacagcacagagttacaataaagaacagcaaaactatattatttcagccttaatggaactaaacagtagttcaggtgatgtgaaaactgttcttgaaaatacagaaaactatttaaaatttattacaacttagtacaatataatgctctttctacgaaaagctatcttttatatttatggtataatagagatagggaaattaaaaagtagaaggagcattttataatgacaaaagcacccagagtgaaaagacttaatatttataacactgaccggtactttaatattaatttaatgaaaaaagaagatatagcaaaaaaaattaaagttaaccgattgaatgaagaagagatagagagggaaatggacgaactagcaagcaacccattgaagacccctataggctacatggatagaacaaatgaaaaatcttatatactttatcaagagaagtatacgaacgacagacttattcagaaattatttaaacatgcagggtctgtgtcttattacacagatacaattgtaccatactacataattgagcaaatatctaagaatttaacaagtgaagtaatctatcctacaaaaaatagctatgagaacagagagattgaaaatgttcaactagctttcactgcttgccctgtaacgattgactgcccagtagtactacctgatgttagcccgtatgatgtgttatttgcactacatcctctaaaaacaaatgtagacaagattcaaatatcgttcccttgtcttacagaagaagagttcgatactagacatgaagaatactatcataaagtaggtagccactatgaggttaaatcagagtacaaatataaattctttaagtatgtacaaacttccttatctatttgggctatgaacatttggctagtgtgtgatagtgatgaggactacaataaaatagacagatatattcagaaagaaaaaattaaacgtaatgctaacagagagcgtgcattaaagagaaagggtaatcaggatgagtaaagataaaacgattaaccgaacagacatagctcgaacaatctctcaccatactggttatcgaatgaaagatatattgaagattttagaagtagaagatgaagtagtagctcaagcagtatcacaaggtatttctgtaaagaatcacaaattatggaaactaaacattaaaaaaaagccagagaaggtagcatgggatggtataaactctaaaagttttatacaacctgaaaaatatgtagttaaatttgtaccattatctaagttgaaagagtcaatagacacttataataaagagagcaaataaagctctcttttttgctctttctatattgacaaataacataatacaaagtatactagtgtcatagagcaacagagaggagaaaagtgtaattgaaaattctattcttacaagagtacattagagaaaatcatgtccataatggaaagaacggacaaacagttgattttaaaagaacagaaatgggtaaaaaacttacaggtctgttaaatacaataggactgacaggtagggactatgctgtagactatgtgtacgacatgattccggaagtacagaaagtcaaccctagaacaggtaaaccaattaagtataagacacctacgttaagacagcgtaaagaaccagaggaacggttactcagacgtttaatgaaatacaaaccagatattatcatcccaatgggggagatgggttgtaaaaatttattaggaagtacttctatcacaaagaatagaggagtaccaactaagaaaacaattacgaatgagaacatactgagaacggctgatgagcaagggcttgaggtagacgaagtagtagactcttttgaaacttgggtactacctatgtttagtatggaatactggacagctaacccaaacattgagaactttatcatggcggatattgatacattgggtaagtttgttcaagaaggggaacaagcatttatccctaaaaaagtagattacgaatttgttgataacattgaacgtgtaagacaaatttttggttttttagacaaaacgaagccagtaactgcatgggacttggagacaaatagtttacgtggtgacttattaggggctaagcctcttgtaatgtctatgagttggctagagggacaaggtgtgactataccgttagaacaccatgaagctaaatggagcccagaagaacttaacgaaatatatgacttatttgagaagtttttagcggacagacagcaaccaaaagtaggacaaaatatccagttcgatattagattcttaatgaacacaaaaggatttacagagtttgaagacaacagagatacaaaaattgcttactatctaattgtttctcagaaagtagacacttcaaaacggctatccgatattgcatatgaattaacagatatgggaggctatgacgaaccgttagagcagtataaaaaacaatataaagaggactatattgctcgtaagaaagcagagattgatgctttcaaagaagctgaaaaagaacgagtagagtgtgagttcaagatagcaatggatagatataagcaagaagttaaagaagctaagcttattggtaaacctactaagtccattattaaaccagtaaaagaaaaagttgtagtacctaagaaatcagatattaaacttattaatgagattgacggtggtaactttaactacgactggattccattagagattatgcacccatatgctagtggagatgtcgattgctgtctacgtatctataacgttctatataaacgaattgaggaacatcctaagatgttggaattatggttgggcttttatcctagactaacagcaacattagcacacatcgaggcttctggtgttctattagactctgaatacgcagaattagtagagaacatctatacagaagaagaacatcggttgcttaatgaaattagaaagctaccagaagtaaaagaagtagaggatgaacatatgatgttctacaaagaggggcttaaagaaatgacaaagcctgtcaaagatagagatgcctctgttgccagactacgagataaatataaaattactgatagtgagaacaaagtacattttaaaccaagttcgtctgaacataaaggtagactgctatttaaagtaatgggacttacactaccttatgataaagaatctattaaaaaagaaacttttgacaatggggtaccagaacatcagctaacatggagagattataaaacagataaacatgcactagcttatattgcagaaaattatccagaggctaaacatgttgctgaacttttgctagagtattctaaagtaaacacactaaaaaataactttgctcaaaagttacctaaattagcatctaacaaggatggcatgattcatggttcatataacagtacaggtacagaatctacacgattgagtgcaaacaacccgaatatgcaacaattaagtagtaaggttggagaccctagacgttttgactataaatatccaattaaacgtttatttagaacaagatttgagggaggtggaatgctacaactagactactccgccctagaaatgcgtattttaggtttgattgcaaaagataaagcaatgacacaagcatttattaatggtgaagatatgcatgaggcaactgcatctcttgtatggaagttacctaaagataatgtaccaaaagatatgcgacaacgtgcgaagagtgtcaacttcggcatcgcttacggtaagcacaattgccgtcttgtagcgtaagctactcgattaaacttacctaaacgggcatagctgaataaccaataagctgataagagaacctaagtcctgaaaaggatagaggcaatcccgtagtaaagacgatttaataaactccactaaaggagtggtattatggaaattggaacaagaacagacaacaaccctttatatagaaaattaagaactgtgcataaagacatgcgcagacgatgtctcaataaaaatgctaaatcatatgagttatacggaggtagaggtgtaactattagtaaggagtgggagaccttaaatgggttcctagcaactgtagatttagtagatggttgggacaaagatacattcctcacaacagggctatccttagataaagacttaaaaggaggagccgagtatagtatagctaactgtacatggatgccacttaatgataacaaaagcctactatcaatgaactacaagaatgtctgtgctattgacccaaatggtcaatattatgttatagacaacattgacaagttttgcagagagcacaaccttaatcattccaatatagttcaagtaattaatggtagatacaagcatcataagctatgggtattctggtatgaaggtgataaacctaagaaagggatacaaccacacatagcgattagcccattgggtgacacctactatttctataaagctcctgacatggaaaagtatgggctaaattctaaatgtgtagctagatgcttaagaggagagagaacaaaacataaagggtggaagtttattaaatctgaaaacctctaacgactatcgaaaagtgagtagctgtcgagaggacacctacaatataactgagtagagtacaccaacaggtggaaatggtaaggctcctagagtaacgactaggagcgtgatatagtctaagcccctaataaatatcgggaaaccgagggtataactggaaagtcctttttcaattgcacctaagttaggtgtaactgtagaagaagcagagcgtatttttgaagagtactttgcaagtaagccaagtattaaacaatttattgaagagacacatcaatttgctcaacgttatggctacgtagaaacactacaaggacatcgtagactattgcgtgactcattctctaaagataagaaagtatttaatggagcaatgcgtaagtcagtaaatacaatcattcaaggaactggtgcctacttaactaacctatcaatggtatacattgacgagtatatcagaaaacacaataagcgttcacgtattgttatcactgtacatgactcacttgttatcgattgcccacgtgatgaagtggacgagatggcaaaagtggctaaatatattatggagaacttgccaattgatttcttaatgattgagtgggaaggtaaagagatgcgttaccctattgtggcagatgtagagattggggagaattacaatgatatggttgattatgatgcagaaattatcaacgagtttgcttcttaccgaggatacgtaaaatacttcaaagaccaagctaagattaaagattactatgataacaaacttatctcagaagagcaaaaagaccaaggtatcaaagttatccaagatgcaatagagtcatataaacaaatgacaatttaataaaaaaatgttaaaaatagcttgactattgacgtatagtatgttattataatatggcagacaagttttctgtattaatacaagaagggggagttagagagtgtgcttaatttacgagtagacgatttagagttcaaaacaattaaaattattgatgataacggagaagttgtgacacatgatttacaaacagagttacaagtcaatgaatttaatgtgagaacagcatttttagagcaacctgctaagtatacttattggacttcgatactagagcgcttgcgcatgtatcaagaaaactatgagttaaaagcagagaagaagaaagcagaactatatgagccttctcgggttgccttaatcaatcaaggagtagctaaacctacaaaagaccagattgaggcacagattatgttagatgaagactattacaaacttagacagagtatagttaacctatcatttaacgtgagacaactgcaatatatagttaaagcttttgaacaaagaaaagatatgcttattcagtatggagcagaccttcgtagggaatatgagtatagccaaaaggttagtatgccagacccaatgaaaaataaggtaaataatggtttctcagactttcaatggaatttagaacagtaaaattagtgataaaaaaaataatataatataaaaaaaatagaaatggagaaatttaaatgaattttcaagaacaattacaacaacaattaaaacaacaaaatattggagaacgtgaagcggtagactacccatcaaatcatttaaaacataaagaattatacttccctaaagcagaaaatggtcagccatcaactctatatgtacgtgtgttacctcctgcagtaccgggagaaaactataatgttagcgctcgtgaggcattcttaacaactcgtaatcgtaatggtaaagatttaaagagcaactttatcttttcagaacaccctaatgcagaagacatcttagaacaagctatgattcgttggaacgcagaaaatcgtgtaccaaacccttatagccgtaatacaaaacctcgtcaacgttactacgttaatgtagtgcagttaattattaaccaacaaacaggggaagttagctatgaaacagattctaatggtcagctaatggttcgtttacttaagttaccacaaacagcttgcatggctattaatgagagcttaagtaacccaatgttacgcccacagttttcacctgatgtaccagaagaagtagcgcaatacagctttatttcttctgcagatgcattccctatttcaattacaaaaccaccacgtagtaacaaacctacttcgtacaatgtacaagtgattagtaatcgtagtttaggtgcattaccacaaggttgggaaaacttattagaagacttgaaataccaagctacaccttctgtagagtacaatcgtgagtttattgagtactttattgatgtagtagacgggaaagaacctgtgcatcaaggagcacaaagtcaaggaacccaagctccacaatttaatcagcaaccagtacagcctcaatttaatcaacagcctgtacaaccacaatttaaccaacaacctgtacaaccaatgcaacaaaatactggttggtcgccacagcaaagccaaccacaacagcctgctacaggttttaatgcaacgaacatgggaacacctccaaacattaatggagggtttagccaacaacctgtacaacaacctgtacaacagcaacaaccgatgggttctttcaatgaacaaccagtgacagacccttctaccatttctgatgcggatatgcctttcaatatgcagtccatgcctgatgtatcaccacaacaaaatgccgtacctgagcaacctgtgactaatacaccagagccagtaagccaaccagttgttaaccaacagccaaataacacacctagtgtagacgacctattagcaggtatggtaggcaacgtttaacaataatgaaacagttaggaggggcatactgccccttttaattctgtgttaactatccaaaatatttagtaggagtgaataatattggcaagaaaaagaaaaagtgaagaaatagattttggaactattgatttgacaaaagaggtaggactaactacatttacggacacaaagttctctaatgtatcagacagactaccaacaatgattccacagcttgattacattttaggtggaggattgccatttggacgtatggtcgaggtctttggtaagaactctagtggtaagtccactttagcagtccatctgacaaaggtagcgcaaatgctagatgtaccaactgtatggattgacgttgaaggtaccgcagacccagaacgcttagcagaactaggggtagactttagtgcaggcggagtattcatggtagagcctaaacagaacaaagacggtagtaaagatacaatcacggtagaacgtgtagcagaagagttacaacgactcttaccagtatttagtaagcttggaaaacctgtattaattatttgggactctgtagcgcaaacagcttctgagaaagagttagaaaaaggtgtaggtaaccaacaaccgggtttgtaataaagctccgttaggtagtaatatctaaaagaaacctatctttatcatgggaaacctctaggaggcaatcatgagtgaagctgtagaaatacagaacatgcaacgactatcgaaaggggagttcttgtcgagaggacatgaatgagaaccgagtagagtacacccaagtgggtggaaatggtagggctcctagagtaacgactaggagtaagatatagtctgtactacatggtgacatgtagcagttcataagagaacgctataagcttaacgaacttataggaacataatagattaaggcaaaagcaatggcacagtttgctcaaatcattgcacctttaatgacaaattcaaaagcattatttattgctattaaccaagcacgtgacgagctaggtagtatgtttggtggagtagactctcccggaggacacgctttacaccactgggctagcttacgattagaagtagttaaagcaagtcagattaagaataaagagctaaatgcattcggtgcagaggaagagacctatgtaggacatatcctgcgtgttaaaacagcaaaatcaaaagtgtcccgtcctaaccaaaaagcggaaatgtacttaatgtccgacacaggactgaacttagaggaaaacatttatcgttcatgttttgcaactaataagcagtatgccttgattagtggaggcacgtggaagtcttatacaacggatgcagggcaagagattaaatttaattcagataaagcttgggtagcttatttacgttcagaagagggaagacctgttcgagacgaactatttgctaaaatgatggtacgctcattcccacatcgttatgctccatttaataatgaggacgtggatgtatgcaaaattccattatatgaatttactaaagaatatatggaaaatcataaggaacaacctaaccaagctactaaagaagaagtccccgaaacaggaacagatgtttcagatttacttaaacaggtagactaatagataagggggcatttagcccctttattagctataaaggagaggaacttattttgcgcaaaggactagcacctaacccattttttgaaatattagaaaaacatcaagactcctctaaacgtactatgactatgaacagcagtggtacacctagttcactacaaccaataagagacatgttcttaaaggcaatgagagaaggtaagaaagtcctaatagagaactctgacttaagtagtgcgaactctgttgttatagagatagaatatgtaggtaatcgttggtgtttaggttatcaacgagtcttattttatggtatggagttaaaaataccacacactatccacttctgtgatgtatatggagcctatgggcacgatgctcagaaggttaagagacaagttaaggtagtgtttgagggggacaacccttttgagtagagatgttcaaaaagaggaaaaagaaatacgtaatggtaatcggtttattacagagactcatggcaaaggagtgtttcctagagatgtagaccgattgtaccataagtatagtaatcttagatataaagtctataacactcataaagactcgttcaatagtgaggcttcacgtaaggagctcaagagctatattgatgagcaatttataaagttaacaaaagagtatgatataaatggagaggtagactttccgggatatattaaaaaagctctgaatttacgagtaaggcacagctatgtaaaaggacggttccgagataccgctagagaacgtctaggcacccaagataacgaagtagagttattgttagggattgacgatagctctcaggcagatattgaggatgcagaacttattgaatcgttattatcaaaagccaatttttcagaaattgaattagcagtatttcagcagttaattcaaggaacagtaagggatgctcgtattattactgaattgtcagaaaactacggggtgtccaagaaagccgtaaaagatgctataaaaaatgttcgtgagtttgtcttaataaatttaacagattagagtaatacctcctttatgtctgctatattagcagtagaaacataaaggaggtattttttagtggaacaaaacaacactggcaagtatgcaccatttattcgtttaattgtgatgggaatctcatttgtggcaactggtttgactacaatatttggttgggaacctttaccattcacagacgaacaaatgaaccaaggtttaatgttagtactatctgtaggtcttgccatctacaactggtacaaaaacaacgctgtaacttcttatggtaaagcaaaagaagaagcaggaaaagaagtagtcggaactagacaagacttcaaaaacagagactaagtacgaggggtgtaacccctccttagttaatacaaaggagcttcgacatgaagatagacgagataagcaaattagaattgcctaatctatttggaaaattccttgtggtagagactatttcggatgggtacactggaaccgtatctggtcactataactacgagatagaccaaaaatctgaggaaacttatatttaccctgtattttggaatgataagcttaacaaatttattaggtcagatgaattagttgtatacactaataaaaataaagtatactatgtttgtaaaacaactatagacccatataatcatgcagtagtagatgagctcacggtagaggaaggcatggacaaagacaagcgtacccttcaagcgtttaaactttttgtaaatgacctattctcatttggtagctacaatatctttctaacaggtaacctatcattagaaaacaaccctgatattgttctagttagcagtgtatcattagacaaacagaccgctaaaatgtacacagaacggacattagaactaactgctacggttttaccagagggagctacaaacaaaaaagttagtttctcagtagataaaccagagcttttagggttaacagtctctgacaataaagcaactgtcacaagtaaagataaggcaggtactgcaattgttaccgtaactactgaggatggagaacacactgataagtgtacagttcagatagaagagtacataaaagttacaggaattaatgttagtggagaatctgctttagaaaaaggtaagacatacaaatttactgctagtattgtacccgataatgcaacgaatcctaaatttacttggtcttctagtagtgataccatagctagtgttaatgcaagcggtgacgttgtagctttagcattaggtgaagcagacattatagcaacaactgaggaaggtagccatgtaggtaaagtacatgttaccgtatcagacccagaaccagtagaaccaactgaataacatagaaaagaggaaagaaaatggctaaagaaatattaaatattgaagacctgttaaaaccagagacactagaagtagcaatagatggtaaataccttattgtaccaacattgtcggatgggtttacaggtacagtagcaggcggatatgcatatgctgttacaaaaaaaggaacagactacacagttaatgaattaatctataatcaaaaggataacacatttaaaccttctgatgaaccaattattataactgatgataatgaaatattcttcattactcgtacattagaagacccatataactaccctgtagttgctacagagaaacttaaaactaaagatgtaaaagaaaaacaagttttacaagcgttcttagcatttgctgatgacagatttaagctaggtgtttacaatgtgttcctagcagatgaaccatttgtatatggggacaaaacagaatagtttcattataagagacccgttaaggtctctttttttttgtatatagtgttgacaatgttgtagtttagttatatactatacttatactgtataaggaggtaaccacatgaacgacaataaggaaaaatgtattaaacaaggaatacgagatacttataaagggtacgatattttattagatgaagagaatggatttttctatgttagcgtacttgacccagatggcaaagaaatcattagtgggtttgtagaggcggataaacctattgaagaatactataaagagctcctaggtaaatgcgaccaagatatatcgtttaaagaccttttagggttcttaaatggacgtagagacactgaacgtacagacatacgttttttaaagagagacagtggggtataattaaatgacaaagataaaacttattacaaaaaagaacacccaaggctatgtcatgaacaccctgctacgtagattttataaaaataatgtagacgtagaatttcttaataaattcaatctacctgatattcataaccacataggggagcatgatgctgttatcatagtagggtttcctttctttgaaagccaacgaggtgcgttagacacggcactgtcatctatggacaacccgtttagcaaggtgtaccatttagcaacatttggggacacctatcgtaatgaaggtagctttcgttcatttgtagacgaggttataagccccgttggtcattttgtagaactaataattgacctaactaagttcactaacacaggtacaaaagaggatgaacaaaatgtagtggctcttgctaaagaggcattagtgtttgccaaagatattatagaagagacagacaactacaatcgttatgaagttacagacagaactatctcttgggttcttcttgtagatttgcttggagagaacctatataaggtgacagagcctagtaaagagctagacaccattttgaaagaacaagaagtacttgtagatgccttgaacataaatatgcaggactatgtgctaagaacaatagggaagatgtctgcaaacgtcattaatggaacagtggtttgtttcggttatgcagaacagcatgtcaacgaagtagcccataaattaattaatttttataagtcacataactatcaaaaagttattgtctttattggtaggcacacaaaaggtgacgacatgtttagtgtaaggagctatggtgtgaatgccggagaggttgtctataaagttcataatggtaaagggaaagacacaacggcaaccgtcttcttaggtaaacctagtgaagctgtaaataacacactgctaagtgtgctttctgaaattttatagtttaactttgtggtataataaagatagataaattttgataggagtgtaaatttttgaaaaacaacgaacctttagagaagttattagacaaattagatgaaccaagaattttacaaacaattattataggtagtttacaacggagctttaatcgagtacacgttggtaaatttaataaactagcacaggagtttgacttagataaggagaacctgtatagcttaaaggcactagttaaggaaattgaagaagataaagagttacacgaactttacgaagctagtatggcaggcaaaattacgctagaggctgttcgtaaagtattgttacaagatgataagtcatcgtttgatgtactgtcttcttacgtagtagaaaatcaagcagtgctagcccgtaaccgagagttcggtaagttacaacgtgagggagcttatcttgaccatctaattagtggtttgaagacatacttattaactgaactaaaagacatgtctagtttaaaatatatcaataaaaatttaaaggcaccgaaagtatcctcagaccgagagcttattctgtgcctatctgattggcatattggtgcttttgttaataacattgacacaggtggatacaactttgaaatctttaaagaacgacttgaaaagttattagaagaagtattccaagtggctatggagcaggatattaagaaaattcatgtttaccatattggggatattattgaacacattaatatgcgtaatgttaaccaagcatttgaagcagagtttcctgctacggagcagattgctaaaggaattagagttcttgctgatacactcaatttactagctaaggcagaatttgaagtgtctttcggtatggttggtggtaaccacgaccgtttccaaggtaacaagaatgataaaattcataatgataatgtggcttatcttgtagtagaccaacttcatttcttacaagaattaggggcattaaacaaagatattaaacttgtagacaacagaagtgacgtttatagttttaaagatacagttgcaggtaaacgtattaaagtaactcatggtgacactgagggcaaaaaagtggatgttaaaatccctaaacatatcaaagatgaagttattgactatttaatcatggggcatatccatacaacacgtattattcaagaagacttttcaagattccatgtgtatgtcggctctcctatgggggcaaacaactactcagcagagaataacttgccaacaacaagtcctgcacagctaattatggtattagaccctgagcgtgatacaccgcagttcatgccagtattcttataggaggtactcgtatggaaggtaatttagtttatattttattggctattgcatatgtaggtgaaggtataactgcctttactaatactaagcgtaaagaaagatacatgattgaagaaggagaggctcctttgccacgtagttcttatgtatttttaggcattaactaccttttaagaatagctatagcaatttctcttatcttcatcataccaactagcttgcaacttaacgtaacaggtattgctttgttcacactaatggtatttgtagttccttttatagcaagaattatcgaagttgttattagaactgcaattgttcgttatgttcaaaaacaatatattaagcagttagaagaacgaaaaggtaaaagagagactaactagtctcttttttgctatattgaataatgaggtgactaagtatgaattttacagaagtaataagccctaatggggagacatcattaatagatgtaaacaacccaccaacattaatcagacgtggggtcttatctattaaaacaaaggttaataatgaagtgaaggaaactcctgtttatattgttgaactagccgaggagctaacaggtactgatgtagtatctgtctataaagtaaaagagattggagattctatccaaaaagactacattgaagaaaaagtgacccctaggttcaaaagcacaacatatctgggtgagttagcacaaaagattaaaggacggtcgataaaggaacaacgaagagttgaaacaaaaccaccattattcctagccccagtagttaatggaatcgatacattcacaggaatcgaaggtaaaggtttctacgaacgtgaagaggacagacatattctattacctgatggaaaaccgggcatagcctatggagataatacaggggtttttatcggtttgagctcgattaagtgggacaaggcatatgtagacgtggagtctataacaaagggttatttgtcacagaaacagatatggtttaacctagatggtcaaagaccacaatttagaagtgagacactataatgacagataaacaattttatgaggcagatattcaagagttaattttaaataagcaaagaatattcggggatataggaaagagcgctattgtttttgagaaagcaatcatgcaaggtaacacaatatgtgattgcctagtcttcacagaaaaacgagggctcattggcatagaaataaaaactgaacgtgactcgacaaaaagattaaataaacaattatctgattatgaaaaggtgtgcgactacgtatatgtattatgccacgataaccatgtacctaaagtagagcaaatacttgctagacataatcataaacacgtaggtatcctagcttacacagagttcatgggagaggcaatgttaggtgagtataaacaacctagccgttcccctaaaaaatcagcttatcatatgttaaatatcttgtggaaagaagatttaataagaatgcttggtacattcagacggtatggtgatagactagaagctaatggagctaaggttatgaaaacaaacagccgttctggtggagtatctggactttatgttaaatctacaactgctagaagaatgactaaacctgaactcattaataatttaataaatagagtaggcggtaccgaagaggctacgagagtgttctgtgatgtgtttatccataataggaatcacccagagaaagcaattaagttaagacattttaaagcaaaagagaataggggtgacctagatggggtttaaaggtgcaaaatatggttcttggaatactgtagttggtaagaactatgtgggtactgggggcagaacaagtggtagtaacacaaaacggctgtccacaaaaggctactaccaagtaggatttgttaaagaatatcagaacttgacagaaaaagatattatgttaaaattagagtatggaaaagacttagtgtctagctacactggtgtacctgcagatatgattaagctacgtaaaaagaaagaggagcaaactctagcatctttagacacagtttattatgttagcattggtaaggaacctgtaggtaagctgtctatacgagctcagagacgttttagagaggtagggttaacatttatatacctagagaagaactacgtacagaggaagcttagaggcggtaatgtacgtagtgtaggatatactaacgcaaccaaatctcagaaacgtaaagcagatagacggaagggcaataagtctaaaacaactagatagatggaggactactatgagtatttatgatgagctaattggtaaaagtgttatagccctagaatatgcggaggatgggtgtgaggcaagccttgtactaaatgatgggtcatgcttaaaagtatcttgtaacccagagccagactgttgtgggtataatgattttgaagttattctcccagatggttttgatttcacagataacattattacaaaagttgaagataatagtgaagaatgttatggcggttcaacagttaggataggcatttttaccaatgatgcacggatagttattgaaggggactacggaagtggttctgggtggaactatggagagtatgtagacgtagaaattgtaaaataatttactattagatggaggtaagctatgcttaaaaaagggaaagaagtaacactaagaaaattttataatattatcacagataaggaatcagtattgctaggggcacgctacacaagctcaataatgactacagatattcctattacaacaacttttgaagatgttgaggtagaccttaagaaagaaacagttgcaggaactatttcattcagaccagtaggagaaagacagattaatgcattaagtttactaaaagaagcaagcacagcttatgggggttacggagagttcctagatgatactattgagaaacctttaatcaatagtgattttgcagtagatgttagcctagcagactctgctttctctaacctacaagagattccatttaacctatatatgtcctccccaaaagttttttatacagaagtatcaattagagggcgtaaacatatgcaatatgtattagaggatgagtcttctagcggtgtaacaagtacattagcactggtattccgtaaaaaattgtatgatggggaaacattgctaggtgtgcatacttacaccgaagcactagcaagagtagagggaattaaagtgttacagtttatcgcaaatggctctgtactagaacaagtaatcggtgcagtgtctgttttagggggtagcacaggaacaaccctgttccctatgtttgacgatatggtgatgcaatttgtgatgattgagtctgttccttgggtgcacatttcttgtgatacaggagcaattgcttttaaggaagaagacatccgcaatgtaaccattaagtcagctagaccgggagaatataaggtgactatctacttgctagacgaaaaagttacattgttaattggataaaattttaaaggaagttgacaatatatgttgacttccttttttgtatgtgctaagataactacagttggataaaaaaaataaatggtatagagggagagatttaacatggactacaaaacaaaggtatatgtaggagcgcttagttggttaggtactttaggagagaaacgatatttagggcaaatgcgtgatgtattagctgtgtacgagctaggtagtcgatacgcaggttactatacagaagatagcgactatgactatatggttgtatacatgccggctccttatgatttaatgcatcctacaacaatttataaacaggaaacagagattgatggaaataaggtagaggtaaaatatatgtctatcgtggaatatgtttaccgtattgaaaatggagatttagaggctttacaaatgttaaatgccacaagctcccaaagtttcttcggagagcctattgaaggtattgacaataagcgtactcgtttagttacgtatatgaaagaactagaatacagaagagaaacatttacttatttagcaccagagaagttgtttagaggaattaatggtcgtattaaagccacaaaaacacgtatggataaggctattgagaatgacgatatggaagtagcggtaaaatgtgctatccttattcgttattttatggacttattagttgtgctagcggacggggaatctattcgtgaaggtctcacgttctctcctattattgcaaatatcattagagagtttaggaaagactgtgagtcagcacaggctaagacacttatcaatactgcacaagtgctattagaggcggatagagaagagattttaaatagtattaaagaccatgggttatcagatggttacgctcaatcagttagacaatatagtttaacaggtcgattgatagatgtactattaggaggatattatgactaagttagaacaaaataaagaaatcttagatatatttaatagaaaaggaaaagtaacagataaagtagaagaatctgccaagattatgctagaattagaccacgattatgactttggtacaggggacattgcttatacagagcgtggcacagataagaagggacgtttctatttagaaagtcgtttgtttattcataaactcatgccctatgggttcattttaaacgctgtagtaagtaaagtacactatggagaccaagaggagaccttagaacgagaggtatcccgtgtatatgagctagagtacaacctaagagataaggtagctgtgctaattaagaacggtaaaccactaaacttctcagaaaataacattagtaacatgttttctgggcacgtagcacagaatattcttgaacaattagatacaatgtctggttcagatatgtatgtatctgtgtatgaacgagttagtcgagttaaggatgaacaaattggtaaagtatctcggttctttgatagattgatgaagtacaacaagattgaattaatttataagagtggcgttcctgaaggctttgctttggcttatgcttatcgagtagttgttgtaggagaaggcaaagtccgtaatgaatggtacgaacctgtaaagagtgtggactatttagataaggaacaaacaaatccggctaaacacctaggtattccaaagtctatctttaagattatttgtgaaggtgggttagagtggacattctaccaaaaaatagctagtcgtttccataaatcattagttaacagaagtactaacaaaactcctaaatcccccactgctatgaagaagatagagaaagagattgctaagttacaacaagcctatgctcgttttggcggggtactgtataacctttatcagtttactaaagagctagatgaacaatatggtatctcccatagtaaggatattatcgaaacagagtgggaatctatatacgaccatattattgcaggagtagttaacgataactataatagtacaactgcttatgatatttctatggttgcaaacctagatttctacagaactgttcgttatctatactatcgagtatatgttgagcaagggcttacttcacaagcagaggctagatacacatacagagactacttgagagcacaccattatatgaatgcggtacctgttaagtaccctaaagctcttaagactgctcatgacattattattatgaattaccgaacaatgaaggataaggtattgaatagtaactttgaaagtagtgtagctaaatataaatatttagaagaagtatcagttagaggtggctatattgttaaggtacctaatagtgtggaagacttaactaaagaaggttctagtttacaccactgtgttgctacttatgctcatcaagtagcagaaggttctactcgtatcctgtttatgcgagataagacagagccagatactagcttagttacttttgaggtaaaaaataataaactagtacaagcaagagggctagttaaccgtgacttgacaaataaggagcaggagttcctagacaaatggttagttaaagcagaaattggtaagtattagtttgcctaaaaaggcggaatatggagtgtgtatagaccaattcacaatgaaaaaagtacactaaacagttgttatttcattattaggtaaaacaacttattttagatagctgatattgaccaacaaatatttcataatgatttagctattaaagttacaaaaaccctactaatacgtggggtttttgcttgtttcaattacatatgaaattttacagatgttctgctatattagttacagaagctaataaaacaaagggtttcgacccttaaaaatgatatttcatataattaaaagttgaaggagtttataactaaaatggctaaaaaagaagtaaacaacagctcagtattactgaatctatacaataataaattgcttgtatctaaggtagacgaggcgttagacgagggtaaaccatacgatttcattattgctttttgtaaagagaagttcgattttgaaattaataaacctgcattatctaggtacaaagagaaacgtagagagtctttagaaacaggagtagacttggaatcactacttgacaaacgtagaaaatcaggtaaaattattgatattaagtctaaagaggtaaccccacttcctaatgaaacatacgataacacatttggacaagtggaacagatatacaatgatgtagaggtgttagatacaatcatacaaaaaggttttaactctctaaaagaggtagactatgttgaagccccacttgctatgaaagcaattgaagtaaaagctaagataacagctaaccagttccaaggtctaagtctaacaggtctaagagagctaagattaagacagtctgctaaagaacaagcaatgactgagattattctacaatttattccagaagaacagcatgaagaagtattcaatgcaattgaatcagcagagaaagagttctatgaaaacttagatttaacagaggaagaccaaagaatcactaaagcgttgcaagcatcaggtatggatataatttaggagggctataatggttgaaaatttgagagaggtaaattataaaacattaaccttagaagaaagtttacatgcattacttgaagggaagacccttattgtaaaagggctagaacaaagacgtaagttagatgtgctagtaaggattttctcagaaggtgttgtacctgttacgcagataagttatgatacaacccctgcggatggttattggagaacaggatattggcagatatacgatttgccaattaatgcccttagcacatacccatgttttatctatgatgatttaaatacggatgaactccctaaatttatgataggggacactgtttactacacaagtaaagaggactctatcaaagattccgccattgtaatcagtgtgtacaaagacgatgttaacaataagtggtactacaagttaagtagagacaacgaaatatatgcagagagtgagattagaagagacaggttataagcctgcctctttttttttaaatttattgttgacaaatatctataactttgttatagtataaatatcaaggatattgataataaattttggaggtgccatgatggcaaatattttagacacattaaagtggttagataaaggggacaaagttactattgaatttgataaagagcggtcgaagtatgcaaaactgactttgcacgattcatcagctaagacaaatattgtccgtaacattgttttttatgatttagacaaaggagtgtatgcttacactggtgaatacacccctgtatgggataacttattagatgatatgcgtaagacacaaggcgcaggacctgaaattaagactacaaaagtaaatcagttagctacctatgaagatgccttaaagtttattgaaacaaatggtacgttttatgtaattggtgaggaagtaattgttaaggttaaagatgcaaaagagctagcattgatgttaatgtactttagagatgctattgaagaactaagaggagaatacgaccctaaaaaacatcatgtagatatgacaattgaattatcaaaagatgttttgaaaaaaatggcagtacctagacatgaattagacttatctttaggtggcttaatgagagctgtatcacataatgttggagaagacctttttgaaactcttgggtttgactacatgaagcaagcttgggaagtcttagttaattgcttgtcactagacactatccatgaggtacctttccgtgtgctagacgaattagagaaagtaacagatagcatgtctactacagaccatattgttaccttgtatgccggtagagaacttaaaaaattctattcagaggaagagtactttgatgtaatcacacacaatttagctgatgtgattatggattggtcaactatttttactacagctgttcttaataatacagaagatgatgaacaccttaaagagttacagcttaactttgagagattcaagctagatgtagcagaggttctattaggtaacgttgcaagacatttactatatgcaggagttaccgatagctttaacgaagttaaccattatgttgtcggagcaggtaacctgattagaacagaaggtttgattagaatagaagagttaactggaacattagacaaccctaaagatgaagatagttctgaaacagataataaagagttactagatgacatctttacaaatacaggtgatgatggtgttgaagactttacaaaagaagtagacgagcttgccatgtttgagaacgaacatgctgaggaacttttggaagtcaataacaaattaaaagacaatcaagagttattacgtaaaactgtggaggcgatgggtatggcttcttactctactattgattcatcatttgaacaagaggaagaaacagatagcaaccacacagagacttgtgaggataccagagctttccaaatgttaagctatgcagtacgttcaggagacaaattacttgaacgtgtagagaaccacccacaaactgaaaaagggttgaaaatggctaaagattctctaaaagagtttgaccatacagtgaaaccagaattagaagcttatttaaaagcagaagagctagcggaagacgttgatagacatgcaattgtaactacaattatccgtatcaaggacactatggaagcagatatggacggctgtaccgacccaatagagcaaggtttattctacgcaggaagcctaaatatgttagaagaaatggaatcattgttacgggctagcaatagaggttatggttgggacgtaacagctatctatcttatcttgtccattgaactagcttatgggacttacgggttgtctgatttagactttacaattaaaaataaagaggaaactcgtaaagaagaacaagatgcaattaatggtattgtaaacttcttagccaatcttttaaatacagtactagaagaagaatcagaatcagaagaaacacctgtagtagtcgaagaggaagaagaggataaggatgacttctcactatctacagaagacactgctaagttattggcagactggtcaaatggtctacctacgtatgtcgttactcgtaaatacggaattagtatgggagctttatactctatcttatatgcaaatggggcagacgttaaatcttctaaagtagcagaacgagtggctcatgtggaaaatgacaaagatatgttaaacgcagttattcgagactacaagaatggtactcgtttagtagatatttatactaaatacaaattatataaaaatggtttgttctatcttttagataaatatcgagtgccacgtagaggacgtacaaagaaataacaatgattaaggtagtggtgctcaactactacctaatcttttattagggaggaacttaattgattctttttatatttagcattattacaatgctatccatgttcttactatatttgtttgggatggcttctgtggctgtaatcaaagtagggtttcttataggtagtcaaaacgatatagctaaaggcatacactctttacttttcacaggtattgcacttactgtagtcaccggaataactagacagtgtttactattattttaaaaaaaattggaggatttagcatgttgttttttattgttttagcagtatttataggcgggcttgctttatggggaatgtatgatagttatgggtacctagactggacttcatggttatttagtattgtggtaggctctgctgtagctacttttttcacactagcggcggttggaattactttcgatgttgtaccaagtcatggggtaacgaaaagtcatgaattacaccctatctatgagaacagtaaagtagttgtagaggctaaaaaagaccagtttgagattaacgtagatggcggtttggtagctattgatgcagaaggtactactatcctatctactaaaggagaggttaagcctaaaattgtgtttacagagaactatataaacaacaactggtggactcgtttcctaggtatagcaggtaaggtaaaagacacttcatcagttctttatttagactcagataccttagtgtacaataagccggaaaagaacagtagcgcaccagatttaaaaattaaataaataatttagaaaaaggggcttgcataaagtctctttttatgttaatgtgtatttatagataggagggctactatggaaggtgaagtagtatacttagatgagtttatgaattttttaactgatagtggaataaatactgatgatattaacgtagtagatgatagacaggagggctagtatgtcttatacaaaagaagcattagaagctagaggctatcagtttgacaatatgtctatgatagataagatggatgccttgttagaactgctagaggaaccagaatttcgagaaaagatgaaagaagagtacgcagagttctctaagaggcacaataacgatgaagaatgaaaagttagagtcttaccttatgaaagagattgcacctattttagatgaaatagagatgagtgaagaattgataaagggaatggagaacaacaacccatccgatacggttacagtctctttttccaaagaagaagtagacatactcttagcaatgttagaccttgaggtacctagattagacagtggttctgaattgtttagccctaatctggtaagggaagctaaactacaattaattaagaacaagctaacttcaaaatgatttctcactagaattaattagtgagaaaaaaattaaataaagctattgacaaataacaaaacatgatgtaaactaagtttataagataaagaagaggagagatacacatgaatgaacaaaagaaagtatatgcaaaattaacagaggacgaggcagtatttgcttgtgaactaggagataaaattaaacaaattagagagagccaagagctatctcgattagaacttgcaaaacgagcaaaagtagaccactcaacattaatcttaattgaacaaggtaaacgactaccaacattgcgtattatgatgaagttgagcaaagcactacaccgagaattagctattagctttacagattaaggaggaggtatcatgagagggagcctagattattacaactatttgtaccaaacaatcgaaaatcgacctacggaggagctagatgtcctttatgacggtctttataaaaaagccggtgacctgtttgcaatagataactttcaaggagttaaagaaggcagactaattttaaaaatattaaaggctattagagaagaaattaatagtagaattgatgaagaaattgacctttacttgtataatatctatgacagtatatcagatgaagacaaacgagtaaattggctatatgaggtgtaggtatgtttagtgttgttaaggctgacagctatgttaaatcagacatagaaatgtatgaatttaagaatgtaaaaagtttggcattgactaagaaagagaaagaactatggacaggcaaaattgctaaatatgttaatgagtttattgtaaatgcttatggagactaccatgggaataaaatacctgaaataaatgttgtaatcaatggtaagctaagaagaaccctaggttcttttgtccaattcactaacacaaacaaacactgtatagagataaatggtaggtttgttaaagaagttattctattacaagaaacacccttagctcaaagagcgcttgatattttaatggatgtagccagacatgaagctatccactatacactttgttatttaaatagtttaagtggaggagacctaccaacgttcaactaccatgacggtggggaggactttgaaaaagatttatgtttgacaggaacttcacctagtggtgctacgaaagaagagtatatttatagttcttttacactaggagccatcagatgccgacaccatagtacttgccctgaatgtgggttggaaacatacatgtatacacgaggacggtactattgctataatgggtgtgtaggggataacggtagaaaaattatatttagaccacaaggtgatattgcaatttatattgatgaaccaaaatctaaagctaaaccaaaagtagaggaagctctaaaagactataaaggagcgttaaagctaccttatacaggtacggaagaaataaaataaaaaaaaatagttaaatgtattgacaaataacaaaacatgatgtaaactaagtttataagataaagaagaggagagatttattatggcatacgtaacaaatattgatgtagtagcagatgggttagatttgtataatgggaactatgtggtagaacgaggtcaagtagttacttttaaactacatgtagcgacatggaacaatgagcctacacccgaaaatgcttatgcgattattcgtaataatggggtagattataagagtaaagttgatgaatttggcaatgcagaggttaccttcccagttaatggtcgtcctgaccaagtaacaactagcatctttgcattaacttctggatatgagggggatatgcctcgtgtaatgtcagctatctttagtgacgaaacagaaattaaacaaactgtaatgaacgttacagcatctattaatggggagccagttagtcgtgaaggtgtatttttagaacgagaccaagtagtcactgtagatgttaaagcaacattatctacaggtaagttctgggaaggtgcacaggtaggtgtgtacaataacaacacggaatacttaggtgacctagatgcagatggttatggttcagtaactttccaagtaaaaggaaaacaagggatggacacatcagctatctacgtattcgttaaagaccatgaacgagaagctacactaacagttcctgtgaagtttactaatactactgttactacagaaacttctacagaagaatcgtctactgttgatacgactacaggaacagaggagtcttctactacggatacaaccactgtagaaagctctacaacggattctacgtcctctacagtagattctacagaaagtacagtagaaagctctacagagcaaacagtgaccaatgaggacacttctactgattcaggagtagttgaaactacagaaacttcccaagtagcaggctacacagagtctacttctagttctacagagtctaaagaagttaaggaaactcatactagcactacagaacatgctaaagagttaccatctacaggcacagaggtagactatgggcttgttgggttcggtggtgcaacattaacagttgtggtggcactagtagttaaaaaattgttgaataagtaagaaacacaatattgcgaccctcattaattgggggttgcaaattatattattttttttaaataaacctattgacatttaacaaactataaggtaaactaagttcataagataaaggggggaaacaaatgagtcaagtaagcaaacatggagaaaaacgtgtacgtgaacgtgtaggagtgaataagagctctgtagaccgacaatttgagttagctttagaacgaggatacagacaaaaagagctaacaggtcgtctaaagaaatgggtagtatcaagagtatttaactctaagtaccctcaaacatgtattttatataatggtaaatgcttcattgttagcagtgaaggtacactagttactgtgttaaacatcccaagtaatttactaaaagattttgcaaaattatctaagaaaagaggaaaataaaatggatattatggatattgagtttttagaagaacataaacaattagtaaaagaacatgtagaacaagaattaaaattaatgcaccctcttaagaagttacaagtaatgacagactggttaggagatacagaagacaagctttctcaaggagacttagattacttcaatgacttaacagaaacagagctaatagaggcaatggatgctagtgaaattgtagagtcttattcagatgtcttgttagattttattgactactacaatattgatttaactggtttagaggaacagctaggtgtgtaaccatggataaggctgaaaaggtagataacattgtaagacaggtcacaggggctgttattaagacaactgcaaaagtagcttttattgtttttgttttaacctttgcaggtgttttagtaggttattatagttattcatttttaacaagtgcagggtggtttgccttacctatgatattatcagtagatttgctatatgttgcggtactgttaggcgggctagcctttatatttgcagaggtctacaaagtagttttagaagtgaaaaagatagttaaacgaggagggcaattatgagtaataaaacattagaacaaagagtaatagatgctaacaaagagataaacgataagcttaacgaatcatcaattattcgtaaacaaattgaagaattagaggaacaggaagccatcttactatcagacgtagaggacttacttgattacttagaaaatattggagtagacctataggagggacttattatgaataaaaaagtagaggaaatgacaatggaagaaaaagacaaagcactaattgcaatgggacttattgatgtaacgcaggaggcagactgggtagtattagctacttgtgaagaatgtagagaagagtacgaaggagaggagtacgaagaaggggactgtgcagagtgtgaacattgtggaggagaatactttatgattgagacagctctcgagggtactcgttgtggacgttgtgatgactactttgatatgtgggacgactactttgagtttgagaatgaaggtaacccatataaagataaacatatctgtgaacattgttatgaagaactagtatctatgggaatggaagagaaattttaagatactactaagaaggagacttaatcatgaacgaattagaagaacttaaaaatacactgattagacaaaaactttcaatgttggagagttacgaaatgagagaagcatcattttggataatgtttaatgggatattacgtgtcatcatgtcagtagctgtcatagcctttgtaaactatgctaagcatgtaagaccagataatgtagccacatggtttctagctctgatttgggttattttcctagcagaaggtattaaaggtgcttatgatgctgttgcatttggtattcaccgcaaaaaatttgctaaacatattaaaaatatgcgtgggataatcgcaatcacacaattacttattgaagaagacgaagagaaattaaaaggaggcaagctagatgagtaaagatgagaaattagttgagtggtttgaagttgccttaatggtgattatgtggttgcttatcacgttcagtatcttatacacaatagtttccttacctttcatggtacacgaaggggactggctagggattgtgcgaaacgtactactggacattgtagtattggcaattggggttgtcgctacatggttgcaattaagatttaaaaaaggaatggaggaataattaatgggatatttagagagtgcaattgaagaaattgaacgagtactactaggaaataaaagtcgtgacaccgaagaagtttatttaaacaatgcaattcggtatatcaaaaaagagttaaagaaaaaagaggtagagccaacgtggttaaatgaaccacagacattgttccttaattggtttaacgaattatacgcagtaggtggtttaactcatgtaacagaggcagtaggttttttagaatccacaggaggtagaatgaagtatccagaagcatattctgctttcagtaatttaagtgagaatgaattgcttgaggtttacagtaaattttatacagggttattcttaaaagcacaagggggtgaattagaatgaactttcatggtaaagtatttcatgataaagtatttgacattctttctcgtgattaccctgattggcagaggtatcagacagagaaacgaccacatcccaatgagcttagaaaagactttgccattgatagtacagatagtagatatgaagagtatgttatgggagagtttaatgtagaaacggctagcggagatgttaaagtatacgcagtaggaattagaagagtagttcataaaaaagctgaggaggagtaaatcaagtggagtacacagagaaagacattaaagaaggtatgaagttacgttgcacagataatagtaatgtaggttactgggaagttgataaggtttacgaggtaacacgtaataaagaccttggcttagttatcgcaggggaaggtgaaaggagtcacagaaccgtaaagtatattttaggggtgttaaatggtgacagcaaaattaaatttgaagttgtagaggaaaagcctgtacgatttgctaaggtaacttgtgtataccctcctgatagaggtcttgtagaggttgggcattgttatgaagtgcttaaagagttccctacaggaagtgtgcgtatctaccttaatagtaaactagggaaccatgagttactcccagaccagtttgtctttgtagatgaaccatcaaatgatggagaaaaagacgtagaagagctagatgtagaagctaagatactagccaagattgaacagttaacagcagaagcagaacaactgtttgctaaacgtgaccgtgtaaatgagcaagcacttaacttaaatgcaaaagctcgtaagttagaagaatctttagaggtactaagggagtacatgtagctaagtgtttttatgattacatctattaaggagatgagagaatgatttattatattaattttttagaagatttcgcatcaagttggagtgcagataagcgttatcgtgttcgtagaattatgacaactggtagctacgctattattgacaactatggtcatgtcagattcagcagtgacacagcacgaggtgtccttaagaatatagagcaggagtatgccactcataaggttgagcttacactagcagaagaagaaacaacgaataagcctaggtttaaagtaggggaacgagtgaaagtgtctaatgatttacaggcattcgggatagaatataagactcacataacctctaagatgatgggctgtgcaggtaatgaggctactattacacgtgtttgggggagtaacgtacgctactttattaacatcgatggtatacaccaagattggtgttggacggaggacatgttagataagattgaagaagaacctacactatctattagatgtgttgaggcagttcatcccttttggacaaaaggtaaagcctacgagataaaccttacatctgatggtcgctatcgggtctgggatgacgaggaagatggtagcagtggcaaatccataaaagaactactggacgttatcaatagtggcggtaacaaatttgagctactagatgaaacaccctcagaagcagaacctaggctaaaccatgctatatctgacttagagaaaatagaagctaagattaccgctttatcagaagagtcttttcagctattcaataagagtgaagagttaagtactagagcaattgaactgcaagatgagtcaatagctttagaagaagcattgtatactattaaacaatatttataggaggagatttaaatgcgtaaaaatgtaatttgtagattagaatgtgtttcaaaagacaaagacaacttaggtgaatggactgtagataatatttaccctgtgtttgaatcagaactaggtaaagtatatatcctcgatgatgaaggtaccacttgttccagagatagcgtgtctcttattatctctagtatggctagctttggggtaacatttagggtagcaaaagataaagcagaagaccctatccctagcaatccacaaagcagtacatcattagaaatagttaaagggtatgaacacttagcggagtttatagactcattaagtagcaaccaacgtgtagtgtctcactcagtagaccctaactctcaatggcactatatcatttatgaaactaagtcagctgaattgggcggagtaaccctagaggaattactagacacactagtgtataatgtacatgttgtagtgatggaacgtagtaagagaacatatgagccactagaaaatcacacgtttaagtgggaatatggaacaaagaataccaaggattgggaaaaaattgtacctttattaggttgcaaggtgtttaatactaacctcaatagtaacagagggttccatattactattttgaaataaactgttgacaactactatagtccatgctatagtaggtacatagataaaaaacaaacaatattaggaggtagcatagagtgaaagaaacagaaaagaagtatagcagagagtataaggggctagaatttgaaattattatcacttattaccctgaacaagacatgtattttgtaattgtaaggaacggacagcaccgtacactaactaaggttacagggaaagagtggggaatgagccctcatacagaggaagctgttattgaggtagcacttgatacatgctacacctatattgaaaatcaagaagcgcaaaataactagattaaggagggactatgatggtaggagacttcattttatgggttaaacaagcatggaaagaaacattctgtattcatgactacacggttaaaggtgtatataaaacattagatagtcatgggtacttaaagtgtaaaaagtgtggaagaattaaataggaggacaacaacatgaaccagagacagaagactagacaagaaaataaatggtttgaggagcatgggtatgatacacagcaaccacgagaatgtattgagtgcggggctcctttaagttggaaagatgagttacagaaaagtcatggagtgtgtagtgagtattgttatatgagaagtgttgggctgtcgttatcagattttatttaaggagatgaaacactaatgtttaaaaaagataaaaaagaagaaaagacttatagagaaggagacctccttaaggctgtagggggttactacccagatgctaggttgagtttaggaatcacatatccattgtataaaaccaccaatgagggttggtatattatcaataacgaaggtagtcgggtaaccttaatcgaaatggatgctttaggcattgactacgctgtgatggaagaacccttattagaattaaaagaaggagacccattgctagtcgtgtccgaccttaagagaggtgttcgaggcttagcaggtgcagaagtacagtgtttaaacattaccggtgaaatggcttcactagcaggtacagttgttcattatgataaagatatgagccatattgcaaaggggctgttcactgttaaagagaacgattcttattggtgtgtagcgattgctattccactaaataaagtagctgaccctgattttgcattagagcatttgcttgctacgttaaataaaaaagcctctactaaacgtctggtattgaatgagataaaatatgatttaaaccttcttcacgaagagctagacgaggtgtccaacgaagtagagaagctaacaaaaaacattgaaacaatctataataacagataggaggtacttagatgagtatgccgagtgatttagggaaaacattaaagaaacctattgcaataaataagaatcctgatttttatgaattagcggtaggtggtaaagttatctacaacgaagaagtaatggagattgctaaagctttctctaataagaagaccaagtactacctactaaacacacgaagtaacaaacaagtatgtgtaccagtgtatcatgtaagaccttatgatacccaagtagagggtcttaaactaggtgatgtcctagatgctatgcacattatgacaactgtaacgttaagggcagtgaacaagcacgggtttgttgtcgatgaggatattattgaatgtttagtagatgacatcccagaaaatgcgcttattgttactagtgaggtatcccgtattcagccagaggattttggtaaggtaactattgactattttgtttagatatgttaggatagacttaagataggataggataaacttaggatgcgcttttgtttaggataggcttaggataagataggataaacttaggatagacttaggatagacttaggatgcactttggtttaggataggatgggggatataactatgagttacgttaacgagtttgaaacaattggagattggttagatagagaaatttatgatgtgttactaagagatgagcatgatattgaagaattagataattggggaatggctttgtttgcattaagtgaaggttacgttctaacagatggacttgacaaaccattcctagagttaactagagaagacctagtagcaggctacaaccactttaaagaagagctgaatgggtggttacgaggaggtaaactgctagaagtctctgataatttatctacaattcaggggttcagttttgaccatgacgatgttttattcttagaggataacaacaaagcttatgcaatgctagtaggtattatcattgaagcaagagacacatataaaaatggtttctgtaagggtcactatgtaataccttaccaagattgagttagccttatggctagctttttcttttaccctaagtagcaggctacaaaaatcttctaagtagcaggttgcaaaatcttctaagtagcaggttgcaaaatcttctaagtagcaggctacaaaaatcttctaagtagcaggctacaaaaatcttctaagtagcaggctacaaaaatcttctaagtagcaggttgcaaaatcttctaagtagcaggctacaaaaatcttctaagtagcaggctacaaaaatcttctaagtagcaggctacaaaaatcttctaagtagcaggctacaaaaatcttctaagtagcaggttgcaaaaatcttctaagtagcaggctacaaaaatcttctaagtagcaggttgcaaaatccggatgcgcccggctagcggtggggagtcaagccatgcgggttcaccttaatagctaccgtccccagattgtcggtttttcttactatatatagtaagaaaaataatttaaaaaaaataaacttttctattgacaaaaaacaaaagctagtataatatagagcgtgtaaggaacaacaataataaaaaaaataaagataaaggggcgctattaaaatgaacaagtataaatttacctatgcagacattaagaatttaccagaggaagaaaaagaaaaagaattaaaaaatcggtgtggtgttttagcggtagagtgcttaagcactaaacagctacaaaagaaaaaacctcgatttatggttttcttaaataccgttatttttgatagtaccgcagaaacaggcggacaatacgcaacggcaaccgttaaaaccgaaccgataggggacggacgttttcgagtgtgtgacggttggggacagctttctaatggaattattgaactgttaaaataatttataaaaaaaatattgacaaataacaaaagataaactacaataaacttgtcagataaagaagggaagttatgaacatgaatgaattagaagcagtgaaagaatggaataataaaattgaggaacaacaagaagtgctaaacaaggttattgttgctttttataaagaaattgacttaaaggttaaaatggtaaaccgtggcttgctagggcagttaccagcttttaacgaactaaaaggaatgctatcaggtatcgagctaacagcaaaggttattgcacccgataacgtgctgcctattacaacccacaactttttagaatatttatttctaggggataacgaacaacgagcatacgcaaaagaatacctagacggctttttaaaatcagtagaataaggggaggaaaattttcctcctttacataaaaaaaagattgacaagttaaaagaaccatgataacatataaatgtagacaagggaggggctttacatgatgaacggactaaaaaaacttgtgaaagctaggcaatacaagaaagaagtaaaaaaaattatcactatgcaaaagaaagcaataaacgaactagaaacattaaacaaaaatttaaaattaattaatcaaaactattgacaaataacaaaagataaactataataggtttataagataaagagaggaagttattgacatgacagaacaacaatttaaaaaagagcatttattagaaccaacagaatggcgtagtgggggctacttagacactagtttaattgaccaatcacaatcttattatattgagtcacgtccgagagtctacggcgggtgttacgtttaccaatatgttacaatgaaagatggcacggtttacgagctttacagcatgacggcaagcactaggggaattgttgcacataactgccacgctagaaacgtattgcaaagagatgtaaaacaatacagagatagcgccattcattattaaggaggggagggctttcctcctttacatagaaaaaaaattgttttatctattgacaaataacaaactatagtgtattataaatttataagataaagagaggaagttttaaatatgaaattatctaatattattctagtggggttgcttgttagcgttgtactactttggggctaccttagcattatgatttgcttacaagtttttagagcgttaggcggttgggatattagaacgttaacggtttgcagtggtttgctatttgcctatgttttcggtttaaaaggaatttgggaacaagggacagggaaaaacaaataaaaaaagtttataaaaaactattgacaaaaaacaaaatatagagtattataggcttataaagataaagagagggagttataaacatgaaattgaacgttattcatttactattttgcttatttcaagaacaagaaagctattctattttaagttacgaatcagtagacgaattttattctaggttaggttatgacttagagagtgagtggctacttagggacttaggtattaatggaacaagtgacttggtagagttgctaacagattacaataatttattagagaatgagataacaaaagcagtcttttctgataaatggttataatttaaataaaactattgacaaaaaacaaattaaggaggaagaataggggaaacggggagggagggacttcctccctttacatagactaggagggcttaaaatgacaacagaggagaaagcactaaacattgcagagaatagaggtataacagattataaggttagggggaacgtattaagctattatactagctacccgatggaaaaatgcacataccttgtaactattgacattgaaacgctagaagaagaaagaaaagaactcaaaaaatattataaaaaaggcttgcaaaatgcttgcttatagactataatataaagaggggtggcggttgttattaataagagaataaaaaaattacaatatgaaagaatcagaaagctagaaaagagaaaaagaggtgaaccacctgaatttattttcaacggtaactattcattggaagaaatagagctatttttacattttagaaaaaaaagtgagggcaaaaaatgagcgtggtggctttgcttggtttacttgtaaaaattacatttatttttaaattgttagcagataaaaaaagttaatcaaaactattgacaaataacaaaagataaactataataagtctatcagataaagagaggaatggtaaacatgacaaaagcagaactacaatataaaaaagcaataggagttgcagtctttgcaacaagtggaaaggataaaaagcaactaggaaacgtggcaccgtttagcatttatgagattttagaaattgacttaaataaaaatcgggtatattatgctttaaattgtggggaacgacatgcagtatgctttactaaactacgcaaagaagaagaaacagggaacgattttattttaatcaataaacaaccatttttcttaaaagatatgcacaaaggtttaagttggtcaaaaagtttataaaaaaactattgacaaataacaataactaatatacaataggtttataaaataaagagaggaagtttttaacatgacaaaagaaaacaacgtatttttaaatgaaaaagagctaatgaaagaagttattgacactttagaaaatggctttgatggttattattgcgacttacatggtgagatttttaatcatggagcaaatgctgacattaaagacttggaagaatatggaatttttaacgcaattggagaaatacaagaatacgaagaagaaaattttggggaggttttgacagacctaggaaacccgacggaggttaccaatacgctttactatattaaaggtcacgagtttttatatggtagattagactttaatgatgttttagcagatgttgcagaggggctaaaattagataaagacttatggaacgaggaagccaccgaggaagtgaacaaggctattattgagtgtttaaaaaaagaagtgccttatttaatagattagaaaaacagggaggagtttcctccctttacatagaaaaaaaatataaaataagggaagtgctaaacatggaaacattagaaaaattcggttatacatggcaaggaatgaaagaagttacaaaagaagaagcagagaaaaacattaagaacggggtcggcacttttctattatatccagataacaacaattgaagcagtgaaagaaagaaagcaatgcaatattagataaagtattgagagcttgcaacttgttaccaactgaaaagaacgtgcaaacagctaaaaactttttagaagaacaaggctttaaagtagaagctagtaaagagttagcgggaaaataccttgtaaaattttcaatttaataataaagaatgaagaggggaagttataaaaatgaaactaacagaaaaggaactaaacacaattttaagagatgatgaaacagggaacgggggaacggctttcttaggtgaaacactagccgacttcttagaagaatcaggtattgactttacaaacctaactattttagaagtaaatgaattactagaaaataatggaattgaaccaattgaggtagtgccatgttaaaaaatatcaaaaaatcagataaactcactagaaaagatatacaaggtttttggggagatgaaacaaaaacattagaagaatggtataagtcaatttcaaaagaatcagacaccgaaaaagtagaaactgctaaaatgattaatacattgaaagaatatgcaaataacaacgaatttcatttcgtaaaaggagagcaaggacaatgacaaacacaaacacaaacaaccaacaatggaatcagaagtttaatgatggtactatgaaccagaacaaccaacaaaaggaagttatcactttacaagtcgcagaaagtttcgtcagtcagattttaacaaaagaatattcggtgattggtttagttattctaatgttttattttatgtttggcatgtttggcattttcgggggtgcaatctatattgctttcactcacacaaaccgtaaaatcggggcatggcaacaagtaagaagcgtatacactattaaggaggaacaagaagaatggaacaattaaaagggctaacaattagagaattgattaagaaactagaagaagtgccagaagaaaataaggacttgcctatttatacttttgaaaatgaaaactctttgcctattaaagatatttcattatatgatgaaaatgctaaacactcacaagaaaacccgttaagttttgatgtaatcagataaggaggggcaaagatgaatagttttatgaataaacaagctaaacaggtaaaaagaagtaaagaaataaaactagtagaagaagtaagaagaaaaaacgtaaagaaacgtttttcagaggaagttagaaagtacctagaaaaagggtatataatcaggttagaaaataaagtttttccatttgctttaatatctattgacctagaaaaaggggaaaaggtcataagtcttattcttgtgaacgaatatgatggaatagcaaactatacagcaatgaaaaaggttaccttaagagaaaaagggaatagagctatcctaaaaagaacgttaacggataaagatataaaagtagtgagtatgtggaaaggaatataaaagaatgagtgtatacagtttaaaattactagcaatcttagggatagtattattcttttcagttatcgggatagtgtacgataataaacaggacgaaaagaaataaacatataaagaggtaaagagataaggaactatagagctatataaatgtgtacacttataggaataagaagaaaaggaactatatacctatacactcatacactcatattcagatagacacataataagtaagggtaaaggagagaggaggagggagagaaagaggaaagaggaaaaaagttgtttacctgagattttaaagaatcgactccatcaaaaacccgacaagggggcgcataagtctatttcaaaataatctgaaataagtatagttattactgtttatagatggttatccttaaatatctgaaaataggggcgtttatctgattatatagttagctatcttatactattaaccatctagcctattactgcattcattgctattatattctatatagggggcgcttatatcgtttatagtgtaattatgaggggaacgactaggaacgcttatacgggcttatagggggctttaaatgcataggctatttatacatatattagaatacacaaggaggaggggcggaaagttagtagattagactgttaaaaacaaacgggggatagatgcacattgttattttactgattgggctaggttaactagctaaaataagaatgctattgtagcaacgtttataagaaataggggtgtacttttcccctagggaggttttaaaagggtataaaattcttttgttatttaataaaaaagtccatcttagctattgacaaataacaacaactttggtattctatatttgtaagataaagaaagggagttatagacatggaatatacattagacgaattgctagaagaggaatatagcacactagacgaattgctagacagtagagaatttaaaaaacaaatggacaaccttaatcacgtcccacaaatgcaaccgcaaagccataacagcaatacgctagcagatacgggacgttatcctgaaaaataaaattgaaaaaaggggttgacaagttcagcccctagtggtattctatatttgtaagataaagaaagggagtttttattatgaatcattataaattatatgtagatatgaaagagggaactcacgattatgtttcggcaactgtctataatatacttgatgaaaaagttttagggttgccagatattaaaaaacctgagaacgtagcttactatactgatgaatggaaaaacgggctatattcttactatgaaaaactcgcaatatcagagttaaacgactacaacgctactttttcacatttataaaaaaattaaaaaaaactattgacaaaaaacaacaactagtgtattttattaagtgtaaggaggaacaaacctccttacaccacacaacaggaaggaagtttttactatgacagaatttgctaatatgaataaagaagaggtattggagctacttaatgattggtttggtgttagtgactatgatacagtgatggaagagttaggagagatgaaacaagttacctttacaggtagcacaaaccaacctctattaggtggtaacggtaacttaattagtttacctcaattctttaaaaataacgaagcagaatcagagttcccaacttatggagagctactagaggaactagagaaagatacatggaatctcgaagcagaggacaacacttacaattatagtggctttttagaaagtgaatcagattttaaagttattcaggcagaaaattcagacacgactattgcattctttgcaatccatacgggtatagacataagagcgggctactcaaaagcaatcccagttatttttgaaacttactatgatttttatgaatttctaggtaactacttttgtagtcaaggttactatgcttttaaacacgacaacaaggaatacacaatcagtttagacgtttcggctacctcagaatatgtacgaatttatatagctgatgaaaacaacgaggaactacagcaaggctatgaacaagaaacttgtatggacttagacatagaaagcgtagaaggatacttgaaagaggaaggaattgagtttactgacttaaaacccgcattgtaaccatataaggcactagggagcttatacaatagagctacaagcctcctagtgtaattataaggtaaataactagaaacgcttatacgaaagaatagggggctttaaaatgacaacggatgaattaaaagagttttactatgaaaacgggattgacttgtggaatgataacctatattttgaacaagttgtttctagtggtggatggtactacgacaatgaacgcggtttatggtttaattatgaggattaaaaatttaaacttttctattgacaaaaaacaaaaactttggtattctatacttgtaagataaatagagaggggaactaataaaaatgaaactaaaagactttatcaaactagcagaatccaagggcgctacattagaagcatacaacgagctaggaggttatgaactaactagaggggacacagtagacccgaatccggttttgattgcttacatgcaaggggcttacagcgtagaaataccaaacaaggaactagaaaacaaggagttaacagaactagcgtttgtctataaaaatgtaagtcttatttatccaaatgaaaaagaactattgtcaggactaggactatagcacaacggcatataaagcccgtagcgaggttttagcgggctttatatataaataccttaaggaggaaacaaggtgcttacagtggaaaataagggcgttaggtggctagtgagtaaagaagcatggaaagcaggctttgctatggaggtgctaggcttgccagattgtaaaattagtacagtattaaaatcggtctataaaattattatctaactatttaaactaatctattgacaaataacaaaaactttggtattctatacatgtaagataaataaaacaaaagaaagagagtgacaagaatggaaacgaacaaagcatatgaaagactattgaaagaagtagaaaacttacagaatgatttaatggatatcgaggactattcagaagaagtatatcaagcctttcaaagattaatcgaagaactcgaagaggtaaccgaatagggctagaccagtcctataggtatataccagttgacccgcccccgtggttttttgaccgtactttgggggtggggctatttgcctaccccgaccctggggtataaatttttttgtagctagaaaatttttatatatttataaagtcaacaccccacatataaagtcaacataagggctcaccctagggctcctatataggctcacctaaatactcccatataaaaaagacccctccccgttgataaggataggtcttttttatttagccgtctgccctatgattggttattaggttcaggttccgccatagtctttgcgaagtatgtccagtatttatggaagtctgcaaagtccaagaagtactccccgacaatctctcctgcttgattgcggtaaagtggtactttcgttttctcgtctttatggactccatactctgtgccatttaatgaaatccatacaatatccggagtcacactagttactgttgccttatcacaacctagtatcgggtcacgaagttctggttttgtgaaaactgtatccccaaccttcaatttgtctagtcgctctttgtctattaatgttgtctccatttgttctccctccttatacattataaaaaatatttaacgtctaattactgccctcaaataaagaacattactacccatccaataagcataaataacaatgttgatacagtagcttttgcaaataccatcaaaatagaatcttctgtatttgtagtagtcttagctgtaataaaactaataaatacatctagcccaattgcctgcgcccatgtaagtgttaacaccccaaatgttggggcaattaacccgttccacaagaacatcgtaacataccctccaatagcaagggtcaacaccactagaactaaagtcccaaaaaatttacctaatgcatttgccaattcgtcttttgtattcttatccatcgttttcctccttaataatagctatatttacctcttatttttttgttaattctatttaggcttgcaaaagtaattatgttcaagatatatgcgccaattactgatactgcctgcattgtgcaaaacacgattgttatccagtagcttgtagtagcttccccgctagttagcccccaataaatgctatatgtcaccatgagtgtgtttagcagtatagctacccctcctaccaataatagtaggtaaccagatagtttcatttagttcccctccattgaatgattaagtaagctcttgttcagttcttttaagtaatagtcacacctaacgtgcacaagacccatacgttcccttgtaatagggttataatgtaatcgtgtaggtactgtgtactcattaggtatagataagtctaattgggtagttaaattgactactctatccggagggcacatccatagaggcttattacagtgccaacatgtcccactttgtagtacctcgtattttcgtttaagttgtttctcttcttctattgttaattagtcgtgatagcactgtgtcattgcgtatggctccctccgcttttatatttgttatagtttagtgttaaaccagtcctatatcctctcctagcgtttacaatagttgtttaaggtgataataggtagaatacctatcaccgccctaagaggcatatagggtacttataggactggtgtttagttaactgttttaagtggcataaaaaatatgcgcttaagtcaacattagttcttttactttagatgatgtcaattgcaatataatgatttgttttggatacattagcaatttcataatctaagtatggttctagtacttcgttgttacttcctatctttgttctaactgttatggtagcccctgccgtgggataagtaatgagtacgtccactccgggcttcattaacttaactaaatcttttaacttcatctttatctcctctttaatagcatatgcttaaatctattttatgtcaactgcttaatttttgtgctcgtagttgcacagatattgtatcaacaatgactgcccactgctcctccgtaaaattgaagtcaaactgtgtatagtcttcctcacctgttgtagtaattgcaatgtctccataatcatcaactgagaaatagatagttgcagtcgcattttcctccggattttgaggaagtgtaatagctaactctccttgctctactttcatctattgcccccccttagctctcttccttctcaatcatcttgatacctgtaaaggcatatacagggagttcttctgtgtaagtgtactgattagctttaaaggtaacttcgtagtaactctccatgccacagtgtaacatgtctacatatctaatttccttacaaggcatagcatttttctcactcccacagaagagccagtcttctgtacagtattctactctacctgtgtggatacttctaactgctacgtatggtttttccatctattcttcctcctgtgtaatctcttctaggtcacaagggtgtacatctagtgttcctgtccttagactataacgagagtttcctcgtactgcgtaaacaccatctgggtatactttttcaagatatacagtatccccaattgtaaacccatggtcataacgggtatccccaataaccttaaactgtctttttatcgtatacccatacatgtaagcccgtgctaatacgtattggttaccctcatcaatccattcaactagcttgtcatctggtgtttcatcgtatgggtcaaaatactcattagctaataagctcaacattgaatcgtactttttgattgctcgtgcaacaaaactaggtatctctacttttttagccatctattcttcctcctatttaatcataatacatacaaaatacataaaaaagctaacatcagcaaaacaccaccccatccagctgttacatatgacatatagaaaacgtatataaggtatgttactgctataattgttaataatacaagtatcgtgttaatgagcttttctaaatcaatcattatacaacctcctagtcctcacaagtgcgagtctggttcttattatactcttactcctacttatatccaaagaactttaagtaattttctgcttctttttctaagtgctcgtttagttcatctagggtaacaactttcccacagtcctcacaggtgtaggtctggttcttcttatcttctagcagttcaccatcacatacaaggttgatacaatgggttgtccaactccctacatcatcaggtaagtgccccattatacgtcacctacttttacggcaaatgccatgaatcgttcatccattttgcggatttctttctctgtaaaggtagggatgtcttttaggtagtttgtaaagtcaggagaccctaatcggtcgatatagctatatccccaaccatctttatcttttgcaataatgatgtagtactcgtcttcttcttcctctaccgtatgacctagtacccatgctttggcaagtttctcatggttttctgggttattagctaaccaaaagtacatcttactagggtagcttcctttgtcaatcatgttaataaacgttaagttctcttctttgcacttgtcaatatatttccctactttataaggaataacaactttttcaggttcgtctaaatcatatgctaaggagactgcttttgctatccctgtattgtagcctagagcatgggggttcaatgtaccgtcacaccctacttgagtaaaaacctcgtcacttagtctactaataaattcattcttattcatttagttccctccttaaaaatcaagactgttttcaataagttctgatagtcggagcattacctcatgaggtagctctaattttgtactctcctgtgagtctgcggagctgacttccaaagtatattttacttctgttttctcatttacacgggaagccttcttctcaacacatactttataaagtgctgagttattgactgcgataattttttcttgtgtatttacactagtattgctatcataagtaatttcatagcccattataaaaccctcctatttgtatactggtacagcaaaagcccagtatctttcatcaatttcttttatttcttgttcggtaaatttgctcttacccatgttgggtttatttgagaagtatacttcattattgtgggatgtttcaacccaaagataacaatcttctcctttattaccaagaccagtaaacacgacatggtaaagtggttctttctccacctcatatccatctttcattcgtattaaagtttcaatagggttattcttactttggtctaaccaacaatcgaactctgattcatgtgggtagctgttgccatctaacattctaatttgtgtaaaaatagctaggtctaatgcatgtttattttcctcgtaccattccgcaacaaactttggcacaattacttttttaggttcgtctagctgttttgctaaagagattgcgctaataattgatagatttgacactatacgataaggtgttttactagattcttttagttcttctaattttttaatcaattcttgtttattcatttaatttctttcctttctttcaatagcccactggctgaatgcttgtaagacttgcaactgcgcaatttctgtcatgtatctataatttttataaacagggctattccgataatctgtttttgtagaattggctctcagtctccaaaatagttctataggttcaatatctgttaacgtatatttttcttttaaccaacccaaaacaatttgttgattctcacttagttctacttggtctaccttatcatcagtgtatttgaaccagattttctcatatgttgtttgtccgcctgtgattgttacaaattcggcgcttggttgctcattttgaaatttttctagttgttcttcgtaatgtatatccccaacatcaaattctttaaatttaatcattgtactccccctgttctaaaaaccaatcagtaaatgcttgaataacttgcgcttcctccgttactgataaagagtaatatgcctcttctgttttagggtcttcataggtctccccaatacgttcgagcgcctcaaataaggaatctttactacagtaacctacttttaaccattcaaatacctgtttctgatttttattcagttctggctttttaactgcctctactgcagtcttatacgctatttttaaaaggtctccttcaaaactattagggaaattaatttcaccatttgctttcatatacatatagcaaactctatcaattatttcgttatatctttgtctactcattcactatccctcctcgtcctctacgtcaccccaaccaaagctacagtaggaagagaacacgtctctagctacttcgtctatctcctcattcgtagcattatcgggtacttctactgtctctatttcaccaatacctgcccaagttgtctcaatatatacatttatttttcgcatagtttaatacctaagactacatagtcgtctttctgtgcataatcggtgatataagtaacttctactttaataaactctcctgtatacgaaccacatgtgtactcatttaataaaagaatatctcccacatggtattgtctatcatttttacgtatttcaaatagttttctaccttccttaactgctttaaagtacgtaggtgcaatcttgaggttatgagtaacttctaatttactaactaaatcaaaaatgatagtgtttaatttgttaccctctacctgatgattcaatttttgtaaagttgttgatattacagtatgcctaccttctctatcaataactgagtttcttctgttatacttagtaagtctttccttttctgcttttgcctgtgctagtccatttattgttttagatacttttacttctccatttacaataacttgtactaggtatctgtcgtcctttgttgcaaacttattatccataattagtacctctctttcataatcttaattgaccagttatcgttgttactgaatacccgttctaggtcattcaatgagttggtatttacaatttctttttttagttttctatctgaattaatattaccaaatcgtttaaggaatctttgtttaaagtgggcataacccatatagtcgaaggtaataacgtgttctttaccaaatataccccgctctcttaacttaatctctacactctcataagagctatctactttcataaaattatttagaagagtgtgcaaatcaatacaaatagatgcccctgcactaccgcctataagtatatatttagggcactttatatcggggtaacaaggggcatctaattcataccacatattatttacgtctaccccataccatacactatttacatctactgaggctctttctgtcttaaatggttttatgcaagtatatttcattgtctctcctccaaatcgtctagtacgtcttctaatgttgtgacaaccccctgcaaataaccaagttcatgccacccataccctctcttatcttgctctaacaaattattaattctttttgttttacgtttaatttgccggttatatcttctttttagtccctcttcaaaggtcactaccttttttgcttcctctatatcttttaataattggtctagcccatctccattagtgccatagctatacactagcgctttctcgtccttataggtagttacccctaatgattggtatacatacttcttactggggacaaatacaagagtaatgggtctgtacaattgaggtaaaagacaatcttctgacagcccaccaaaatctgttttagaagataccttctctaccacatacctcatatcttccatacttaacgacttaatacataaaatatatctgttaataaccattttctttagctccccctacacccaaaatagttttcgattctctgttggtttaaaagactccaattctcgtgaagtattactttttccatctgttaaaccttctttcactttatatattaaaaaaaataaatctagctatctacaaatacattgtatcatcagctagattaaaagtcaacactttatatttaattattttatattacaatagttctttatctaaaattattttagggatagcccatattgtagtgtaacgaacccctttatggttacctgtaactaatacgaacgttgccgtgtctagcttagtaccgagtacagatgctagtagttcgtggtcttctttgctaattggtacttcaaaatcaagttctccaagctctaccacaaagttatttgctctaattcccataaagtattcatcattacgttttacatggaatatattcttcgtatgaaaactttgcataacaatatttgcaaaataactgttatccctagctacaataaatctatctacatagatagcctctttactgagtagttcttcaatgcagttactcataacatattctcctcctcttctaatagtagctctgatacgtaaatttccatcattagactttgttcaatcccgtctagtaataaatgcatagcacacaagccacacaacatttcatctaaataaaaatcaccacatgtctcctctaatggtacttgacacattaaacactctatcattgtacagccctccttaatttaagttttctctaacttctgttagcacctctcctaatagattaagtccttcccatttactcatatcacgagagcgtgggtctgattcacgtaaccctattccccatactttatcaaaaggtgatgcctctgcaaacttggttcctttagggatggatagcataaagttacgtaaactatcattttgtgtgaatttataagtatttccagctaaaacgattgatttacgatgctttacccacaagtcttcttcaaaatttttaacttgtctacctaaacgtttagcatcttttgggctctctgtttttaaaattctttttgctgtatcgacatcattaaaaagcattgctttacgtaccatcatgtagtgctctgctgtcgggaaaataatagcttcccctaaacccttaataggtgcactgaactgtgatgggtaccactgtgacaagcactcttttcctagtttattacgtttgcttggggtatgtccccaaaataaaatatatttactcatttaatgttcctcccaatattcatagtagtttcccttatgttcaaaaacaaaatgagggctaggtaactcaccattaacttctatatgctctgggttattataagaatagtagggttcgttaccagtaggactaattgctattactggtttatctttaaaaaatggtggtattttatctccatcatttaagtttaatttataggtacttaatggcacgcttctacgatgccctttcagtgttgtatactcctcaagactaattattctaaggaaacccttagcttttagaggcgctaaactgtctatcgaaacgtcttcttgcttataagtgacaagggcgctataaatggttgaggggtttttgtatgccactgaataattaattgaagtgtgcttatggtttgctaaaaatttctctaattccttagataaaccataaggtgtatcactatcaataacttttactttaatcatgtgttatcctccctatatgcttctctaactgttcctatactttggtctgggtctggtttactaaatggtaagcttgcacgctcttccttactcaatgtttttaagcaagccacatgtactgcaatgacccctgacttagcttccatactatccgggagtgtaagtatatagtcattatacagtttacttaacactagccaataacgattgctactacttttcatattagctaaaatcatcattttttcatagtaatcttgccccatacaagaaagtcctcctattgcagattggaggagctcatcttcaagagctaagatagtatttgcgtaccctttcagctccttgttaagcccctctatagcaatctcaaaacattctctttctggagagcctacagttaaatcattaagtggctcatatgctcttacttctctcccactaggggcttgtcttcgtttacctatacgataagagtctttaaactcatactcggaacgaaaaatttcttcttgactatttcttccagaccttcctccaaaatagcaatcttctactactccaccaagaccattataatgtcctctagttgtccctatgactttagaatgtctaatatgggttagctgacagagctcccctccgttatcagggtcacctacaatagctgtctcacatacaggacagatatatccaaaacacatcactttatctacctccaattaatatacattaagaaaaagttacaattttttcacaaggaatatcatagtatgcctttaaaccataatgttccaacatgtattctttagcataatctacaaggtgctcagggcatttaaatgtgtaagagccactcatcattacaccactattacttaactcttctctcgaagctttagcaaaccacttagcacactctacaggataaccaataacacaccctaaaacttcctcgtcattaaaccctagcttaattgattcattgtatacttctatactcatcttatctgatgttactaggtatatactaccatataacctcgttttatagtaagagcgttccagatggcttagctcttcttcccctaatacgattgctacacgatgacctaaattaaaatctaaaataggctttggaaaaacgtattctgctttctcaacaaactccacttagccaccccttttctcattccctaaattatcttaaatgctgtattagttagaacggtaagtcactattgtgttcttcctcttctgggatatataggatattttcaatcttttcttcaatatgtccaataatctctgtgtgctctttaattttctctttatgattttctctttgcttatttaactttgcatattgctgtaattcatctggtgttagctcttctagtctttttttcatttgttttctccttctaatgtaattttctctacgtcatcaacactaccaaaagatgggggctgtgtcaagttcttatctaaccagttagcgataatgtcatgtaactcgtctatagcctcatcgcttacttcatccgttgggtagtagtcctccgctacttctccatattcactgtatagctgttcccctacagattctaacatacctactacatctacactaataactgctttattgaactgccctactgcaaagcttgttgttcccttttcaggtaatgctccaaatatatcctctacgtgcatccctaagctatctacatatgtttttccttcattaatggacaataatgcaagttttcctgcagacactgcctcttctctcgtagagaacgtctcacacgctttccatacatctgtgtcttcctctagtgctaatacatagtctttatcttccattgtcttgccctctctatccttttaatataatcatatttgtattactgtctagttgccatccatcaaattctaagtagtggtcataagggttaattggttcacctacaactatatagtcctctagtgcgtgaccttggtcttttagctctagtaattcgtctaataaatcttgtgctgtcaaattattcatgccatatagtatcctttctctttagcttcttcccactcatctacagaaaacaaacgctcattccgagacaaagagccataacagtttactgttaagtctaccataaggaagtccttaccgtattgttttgtccaactctctgtatatggtgttactgagtgcacttctttaatatattgctctaacatattcattttatgttaccctttcttggtttaaattttcgtgtttgtgttcggttgtttctacttacttctttgtatctacggattcctaatgccttagattctgggcgagaacgacctatctgtcttacatataagtctagcgcttcttttactttatcatcatacatcttccctaattctcggaaatactcaaactcacctaaatacacataaggcatacgccagtcatctagggtagccgttaccattgttcgtttgtttaaatcataattatagatatatagaaacactatataagcacctgtcatcacagaatagcttgtcctaatttcacttagagttacgctgtctcttaatgatgttaaataaccattccacttttttttacgttcttctgctaaagtttctatgaagtagtttacctctttttcgtccctcaccacttgctacctccttgttgtttatgtctatatattatcatctactttgttatatgtcaacacctttgtaataaaaaagaacctagtaatttacttacttaggctctcttgtttatacgtgtttagtaagttacctttactatcgacaacaacagcattaagctgaccaccatatgcacaggcaccatcaatgaaaatacttctatcacctaagaagacatcgtagctgttctcttttctcaaattaattgtgggtgtgtgacccattacaattgtcttatctgttttattcttctgtaacgctagcggtctcgtccaaatcatttcatctttagtggctgttttccaatcaggctgacgataaacaggtatccctgcgtgtacacataaggtgtctccatgctcatagtatggttctaataaactaattacttcaactacatttgttttttctaataacatctttctagtggtaaacgcatcctgtaggtgttcatctaaatccaatagactacttattgttttatcaccgccattgtacatccacattgcgtacatctcacttaggtcttcgtagtctgcttctcttatcaatggaaatgttaaaaaatctaataacatttggtcatgatttcctaacaaagcagttcctccattaataatatgcttataaacgaaacccagtacttctgcggatttgctacccctatctacgtagtcacctaaaagtattaagtcctcttcatcactattccaatgtttattaagaagcattattagctcatcatagcaaccatgtatatctgatacaataaatactttatctttcaatgaataatagcccctttaactacttctgctagccaataagtagctagtactagtacagtattgacaataaatgttattactataaccagtgctaacttataatttttactcctagcattatagtttatataattttttatgttaactctaatatttttaaacaaagcactcccatatacgttcagtgctatatatagtaaaagcaatacgataaagtagccttgagctagaaacacgtcagactccctgaacgagttattaaaccatatgctaaatatcgcaatcacttggtgaattataagcattgcgccattaccaaaaagaagtatactaaacgctataccgactacgtctctgtactctgaaagtagtctatcatatactattatccctttagtaaaaataaaagcaacaactgccatctgtataagtaaaaatattgttacggctaataagttttctgtatgcatagtcataatttagccactcctttcaaaatgggtaaagaaagaataataggtatatcgttctttttctaccctaccttcatgtataaaggtaaactcaacaaacttaactcttagcggtatatctggtgctttctcccaaggaagtactcttgggaaatcatagaatactcttgtggggtaaacttctttcataagtatcctagggtatcttttctttggtataaatcttttacctattatacttgagtagtcaggtttcattgtaagtcaccatgaatagagtatgctctatttgctttgttaaagtttacttgttttttgtttactaatcttattgcatcttctaataaaagaggttttcctaatttatggttatctaattctggtgagtctacccctacattcagtaagtttggttcgggtctggctaactcatgaatgtgcccatgtagattaattaggttatctctatctcctaaaattagtgggtaatgtgtcatatgcacaaccttatgcattcgttttaaaataataccaacgtcttcccaatgaaccctatcattcagggaagtattgcgtttaatctcttttcgtagaggactattatcgtggttaccctttattagccatatagtgccatttaagcgctctaagacgttagctatactatttaccttggcacccattgcaaagtctcctaggtgatatacaatgtcctctgggcgtactgtagcattccactctctaattaagtattcgttcatctcttccacatctttaaattgtttccgtgtgtccataaaagaggcttccccacaaatgtttctatggaagaagtgcatatcagatattacatattctctccccatacttgctcctccttagtgtgttgcaaaccatacgaatacagctagttgtagatagtgtactgtttggtcgataattagttgtgtctttttattaggtactgtttttaagaaccatgcactttgtgcttttaaatagtccatgataaaatgtggaacccataagcatactacaattagcccaagttttactggtgttcctaagaacaatgtagttgcgacaataatatacgtccagatgtttacatggatgattagtagatataaatcagtctgctttccttttgcgatatagtcactttgtaaggcatagtcccctactgcatgagccattgtaaggataattacatagtataagtaattcaaattaagtcctcctctttgtatgggtaaggacaagtgtcacattcaaatccatattcgttaggtgctccctctaaaatatttccgccacattctgggcaagttgctagtttcattgttctgcctcctttacatgatttcaagatatagccctgcacttggtgttgtagaaatcagcataacttctaggtctaagtgttctccgataccttcgtattgttcaataagtggttttgtttctgataaagtgaatgttacaatttcttcatccgtcatgtgctctactaatgtgactgtgcgaccaaattcaatatgttgtaataaatgtcctagtttaatcattataatttcccccatcaattaataatagtaagataccacctatcacaagtaaccagaatactgctaagattagtaccatttagttgtcctccttgaacagctcatcgtataattcttgaattgcctcacgctttacttttaacattgcaatctgtgctgatatgatattgcttggttttcccaccaaacgtccctctaagtgcccaatatccatattgtattgaataagggtttgttgaaatttttttctaatctctgtgcgttcattaattggttgctctggttcaatctcaaacagttcaaacattgaacgccagcgcccatttacgttattcaataattcactaggtgtgcccccaatatctactgtgtcatacccattgtctttaaagaagtagcccaccgtttcgttgtgataaacaggatattctctcccttctatgaactgtggttctagtgcatctgcttttgtacatttaattccgtatgtcattttattaaacctcccattccttaatgatgtattggcttttatagtttgcatagaaatctgagtcacttgagaagtatatatctagttcttttactttttctagtactccttgaagggatgtaccaactgccatgttagtacctgtccccttatcaattccgagatagagtgtaagtttctttggttctgcaccgagcaattcaaacttagaatgccaatagttatttaattcagctaatagtagctcaggagtggctcctgattctataatgtctccctcatcatctctaaggaagtaacctctagcatcatcatagaatacatcgtactctttaccttctgtgaagatatgctctgttttaagtgtacatctaatttttactgtcattctaattttcctccaattcaatttcttttattgatacaaagccaagtatattgcggaaagtacggtcttcattccagtatataaattgtgttagaagtggtttgtggtcatctgtgtatgttgttttttgtctcgtagtagctttcttcaatttgttcatcaatattttgtaccatttcattataatatgtgactgctttatcatatgaggtgaaagccctcatttttaccgctctatactcaaatttcactaaccatgctgagcttaatttcgtcatttatttcttcctccacttctttgattgacttgattatatatctatggttctctctaaatgcgtggtaagcatcatcaagtgaatatgcgtataatcttgttgtttgcattacagttctatatccgttacgtccaaccattggttcgtcaacttctacttctaactcaaataatagttgttttctaatcattgtttttactccccttttctatgatataatattaccctactattatgattctgtcaacaggcaaaaaaaagaagtagaaaaatctactcctattcatcgtttgacaacttttccataccatatagtaactgtagtagtacatatagtacaatatcaaatccgtcaagtggctttccaagtactataactttaacaattgtcaataccgctaaaaaaataaatagccacccgattattttatttgcatgttttctaattctcataactttctagtacctcttcaatattctttctggtttcgttagctaacttaccagtccgttcaagccaacctctaaccatttctttttctactttgctatgtttattcgcatcctccttgataccttctacattttccatcaagttatctaagtcctccataacatctaataaagtgtttcttagttttaacacatcgatagacaactcatagttccgtttagacaatttttcgttacggataaagttcttttttagttcttgttgtgtttctagtagctgagtagttttaataatatcagcttctaatttactaattccgtctagttcattcatcacatgtcctcctcatattctactacttcctcaataagtttcagtacttcttctgctgtgcccactgtgctatagtccgcaaagttttctgcaggtttcataatagccactgaatagggtttgttctctacataaatatgcccgaatccttttaaagaatgaattacctctactgcccatccattagcgtactcttctcggtatactacttgctcactggttgctcttactggtttattcattgttaaaaccatagaagtttcttacaatgttttctacacgttccatgccctctaagtagctacgtttctcaggggagatatagttcttgtaatgagggacttccttctcttcctctacctcttttgtagtacgttcaatcagtttaataagttttacttcgttctctagttgagactggataatgtctaacagttcatttttcgagcagttgtttagtggtttacttccatagtcaataattgtcatagtagtcctcctattttaatgtgtactctttatatcctttatgtgtatcgtgcccgcactttgtacaaaagcctgcttgttcaatatctattgaagagtaccctgtttgtactgcatacgtctcataagtatggtcacacgtatcttcttctgattcatctattttctctaaacgaatagcctctccttctgccacttcgtggttaaagagcaatactgcagttttaataggctcatatacctctgggtggacggcttcattcatcttaaagctatttccactaaattcattgaaagcatctagccattcctgactgttctcataagatacaattctgtaattcatacgaaagctcctctcgtgttttcttaaataaccagtaccgttcatcaatttcttttatctctgcctctgttaaatagaagtcttttaatttggatagggtatcttgactcaatggctcgtttctaggtagtatacttactgctaactgcccgtccttgcgtaatagtaacccgtagtctctctcctgtttctgaggcattactacatagtacttaggtaaactagcagtgtttgctactgcttgaataaaagtatctgtattagcaaagaaccatttactaaactctgacttggggtactcacatgcgtgtctctgcccttccaagataatttgtaacttatccataagttgttctcgttgtttatcaataaactcttttacctgttttggtacttctacctcattattcatagtttgtctcctttgttatactttgtcaatagtgatatacacatacttgccctctaactgcttaacaatatctagtatgtcatgaccacctagcttaaatgtgtttgtctcaaacccttcgatagtaaaggaagaccaaccgtaccaaccttcttcaaagtccaagacccccatagatttaagtactatatttttagtgatgtcttctaatgaagtacgttctacagcagagaaaatctgaatctctgcgttatcaagatgatacttagaagaaatgcctccatcgtactcctcttctgttgtagtgtcctcagctcctaacgcatacagtgcattacaaataagcatgtttaaggctctgtgctcatggtgatactcaatttcttttactttttcttttattaagtaaggttcgtttgtttctgcaccggggctgttatcaatagttacccaaccttttaatatctgtttacccatgattgctcatccttcctttagtacagcctatcgctgtcaccagtaaatctaaattttcctttgtcagagttactgtttgttcatgtacacagtccggtctaaatacctctactgtacgatttactacagcaatatctacagtatcttccgttgtctggcttaccttgataaactgtttggaaaactccccacggctaacaccttctatcataagctccatttttttatagcctcctctctggaaagtccatgaaagttgtggaaagtacgctcttgtagttcatctactgtatttggtaatgtacgaaattcgtctacccctagtgaaatacttgaggctacctcttcataataacatttaacgtctactcccattttaccataaggtaacaccattacttctatatgaaactcatatggagcattctgtgttaatggttcgtataataaccatgtctcatgatagtttacaggaatatctaatagtaaactgtttaaatcatctagctgttcagataagtatgcaattcttgtcattttacggtcttctgctataggcattgaacaacctaacgtgtcttttatttctttaatttctttggtaagctcagccattaattcaattattttataaaacatttctattccctctcttctatatattccccttcttctaagaaaaagcaagcaggttctccctctccattttcagtatcacctaggtattcatcatctaagaatgcacagtatccagttgagtagagggttacacagtccttatggtacatcgaatcgtccgttaaccgcacaacctcgtccatctcactgaacacttcattacacgccccgcatgatactaactccttactcataggctgcctcctttatctattacgtagtctaccagttctctaataacctctgcctcctctacactagagaggtctgcccaaacttgaagtgtcgcatcgttagccttaccagatattaaattgtgtaagctatctgcaatagttagctttgtacgttcaagatagtgaattagccagactaatacaattagctgtttctcagttagctcagtattagtctttgtgtaaacctcatagttatctaaggttaatgggaatgtttcttcattattaattacttgaaacccgttatttggttcgttttcatattctccataagttactctcttacctatttttagttttacatagatgtctttaccttctttgtgtagtttatctaggtcactattataccactctcttgtttcaattttagtaagttccataaagctaaccctccttactgagttccttgatacgttgtttgatttctgcttctgttttctctagttgtcgcattttgtttttatgtcgagataattcatgttcctttgcagtttctgccattgctaataagttttctaagcttgctgtatttgccattagattgccacctcatagttaaattttccattatgtttatagtttactactttaatttctgatagtggggaatcaaagaagttcctccccttctcccatggtaagataagttctggcacttcttctgatattggtgcattcacctgttgttcaataagttctaaatgtcgttcgtaaatgtgtgcgttatcactcgtccaatataagttacctaactctaaccctacagtatttgccataaccaattgtaatgcatgatactgaataatattaaatggaagtcctaagcaaacatccgaagaccgagccttcacatgtaagtttaatttaccctctacaactgtccagtgagttgtccatacacatggctctaatgacatatcgtataaatcttccacgttccataaagtagtcataattctacgagagtttggtgtgctcttaagttgttcaataactgcctctacctgatttagctttaggtatggttgatgtgttcctgctatcccaccaccttttttaggtacgacttttggaataagtgaacctgctttgcgatttttagctaactcaacatctccactataaacaggaataaaacgttctttgttaaataatgcgtaaccatacgcttttccaatagtgccatcttcttgctcccattcgttccaaatagttacacctcgttcttttaaccacgaaacctcgttagacatttcttgccaaatccactgcaattctgttagcgcccatttaatacctacatgcttactacgtaataaaggagcccccatatctggtgtaattgtaaagtttacaccttcaataaacttagttgttgcaggagttccatcagcatatactgcacgagtaccttctggtagctctgttactccgttcttaataatatccattactaaatctttataaattttatcaaaatccatgttgtgccctcctacatttcttttccctataatagaaatatatcatatctaaatttaaaagtcaacaaaatattataaaaaaaatatgagacatattggtatgtctcatatctactaaattctatactaaactggctagcttgtctaaagcgttatagtccgcatcggttactggttctactttacctaataagtacccattacctacctgagagaagaagtcatggttactagttgttgtagagataccattcattacaatagggtttacgtctgcacttgttgttgggaataaagggttcatccctaagttagctagagctttatttaaattgtactccaaaaatgtattaacatcttttgtccaaccaatctcactatatagttcagcagtatactgtgtttcgttctcccataatttaaatgctaaatcaattacccattgttccatttctttttgttcagtttctggtaactggttaaaccctaactggtatttatagccgatataggttccatgtacagactcgtcacgaataattaatttaataatttcggctgtattaaccatttttgcctcacctaaatagcgtagtggtgtgtaaaaacctgagtaaaataggaagctctccaatagtacggatgcactctttttctgtagtggtgtaccgtttcgataaatatcgttaataatgttagctttatattgtaaacgtttatttgtagctacccattcaaagatattgtcaatctctgtaggtgtattaaatgtgctaaaaattgttgaataacttttagcgtgtactgcttccataaaggctatgttatttaaaacagcttcttcatgctgtgttcttacatcatcaagtagtgagtgtacccccgattctgattgaactgtgtctagtaatgttaacccaccaaacactttatttattaaatcttgctccatatcagagagctttgcccaatcattaacatcgttacctacagggacacgtgtgtccaaccaaaattgctcagtaagctttttccatgtggcttggtcaattacatcatcaatcttattccagttaattccttcatacttttcttgcaaattcatgtgctcatctccttaaattgtacaactttcacactctgaaacccctacttcgcttccgtcttcttcggtgaatgttctaacataataaattgtttttataccttttttccatgcataatgtcttaataaagttaagtcccgagtggatgtagcgccaccctccaccttccaaggataaagattttctggtaactctgagcgcataaacaatgttaaactcataccttggtcaatatgtttttgtgctgttgcgtacacgttgattacgtcaatcatacttgtattgtacgctgacttgtaatatggaattgtcttctcagataaccggggtgcagggtaataagttttacctgttttcccatcttgacgttcttcaatcatagagataattgggtgcaatgaagaagtagtctcattaacataagcaatactaccattcgtttataccgttactttcgtaatactttaacactgctcttagcagtcggactagactataccttatactatcccaaaatagtaccaactattatagtcgttggacgtccctcattttacagaggtttcgatgctgatttcccattgtattacccttagcacctgtaacaaggcttttatttcagcataggctatctaactaattttttctgctttcgcaacattcacgctcaccgtttccagtcacgttgtagtttagttagctttagggggttccagcaatttaagttgtttttgactcatattcacatatgagaaagcccaatattatttaggcgccacagctaaacggttttgatggtatagaccaccttcaataatactgtttcttaatgtttcccaatcttttacattaggtagtaccactccatcaaatacttccgccaccttactagagatttcctgatttagtgttggtacatattcatcaaagtaagaaccgtctgcgtatttagagttctcaaagttatggaatgttgtgccacgctctttagcaatcttattacttgccaccaaagtagcatagttaattaattcaaacagagcatccgtcatttcaatagattcaggtgagccatattctacttggttacttgcgaaccacgcatgtagccccattgcccctaaaccaattgtatgggctttatcattaccattcttgatagtaggtactgcttttatatttgacacatctgtaatatatgttagagctcttaccatcgtctcaattgatgccactacatcattagatgtttctaacaagttaaggatgttaattgaacctaaattacagctaatgtctgtacctaactcttcgtatacttgttcatcatttagcttagatggtgtctgtacctgtaatatttcactgcataaattactcataatgattttgccatcaataggattggctttatttacagtactaacattcataatatatgggtaacctgactcttgttgtaaacggctaatttcttcttctaaatctcgtgcattcattaccttacttctgatatttgggttctgaatcatgttattgtattctgaatcaatgtctacaaatgagaatggtacaccgtattctttagcaacatcatatggagaaaataagtgaattacatccccagactcagctagctcataaaatttatcgggaacaactactcccaaagaaagtgttttgatttgctttgcggattctgcattttcttttctagttgataaaaagtccataatatccgcatggaaaacatttagatagactgcgcctgcaccttgtctttgtcctaactgatttgcgtaccggaaaccatcttctagcattttcataacagggacaaccccgctacctgctccctcaattcccttaatagggtctccaagagctcttaggtttgaaagatttaacaagtagtccatgctttaacatggctcagactatatcttaactaaatttgttacgtttagttctacgcgcttccaaaacaagaatttcacttgtaatgtactctactaggttactcgctaatatcctcccgacaatagctacccgttcgatagtcgttacacttttacaatttttctcctcgaaattttctacacaacttagctttatctccaagtttatcttttcttttaaagtagccggatacgttagctaatgaagtagataggtacctactagcctctgacatatctttaaactcaaaagattcgtttgtttcgatattggttatttttacaggaatagacgtagtatggcaaggttttctccctagtaccctaaaaccatgtttagtgttctctgatatagtacaccattcaaggttctccaaacggttgtcttgtttgtccccatttttatgattcactactggatagttgttagtgttaggtaagaaagtcatagcaaccactctgtggacaagtaggtacttcctaataccttccttgttatacatagctgttttgtagtaaccgtctttatcagtagacaacttgaagtatctgtccttttttctaattctgccgagggttgaaacctcgtaggcagggaaatcagggactgccttccagtattctttttccatataaccacctccttaaataaggagaaaaattgtacttagcacggtattgccatatctttcgacttaggttccaccgttagcctacataaagtagacaccctaggtttctaggttcacgtagtttatagtgagctatattctctaacccactccaccaccaagtttagatagttgaagtgcactgttcaacgttctaccaattgaagacattgaatcttctacttgaattagaaaacagctgacatactcccctcttctaagcctacctgcatttaaaaaagtaggggttgcaggttggtatctacggttaattagctcatctgcaatcttcatagcaagctcttcgtcaccatcacccattgtgagtgcattaaacgctactctatcttcataacgctctaggtatcgttccccatcatctgttttcattgcgtattgtttgtagaaacggtaagcccccataaatgtgtcgaatctgaactttttactatagatgaacttaaataatttttttataaattccattgagtacttgtcagtaatcactgttttatcgatgtacccttctctaataaggtaactaattttctcctctaaagagtagaaaaatactgtgttcttgtttacatgttctaaaaagaatgctctaacagcttctttatctttgtctaactgaatctttccgttattagggatattcaattggttattaagctcaatatatgtgttcatatctacaccccaagttctttttctagttttttaaccaaatcaggtctaacaccattaaatgagaaaccatcatcagcttctacatatggtaatgaagacactcctttttcttttagataagctaaagcttgctcatcatgagagatatttttctcatcaaatgggatattctttccatttaacatattttttaaaaataaacattgaccacacatatcttttgaatatactgttacttttgtcatttactacattctcctaacttttttatcgtatttattaattatacactattttgcattaattgtcaaaaataaagaaccaaaaaaactagagactacaaaagttaattgtagccccttttaataagttacaccttgtcacctaagaaatcttctgattcctgcgatttattcgtaaccttatcaagtagtaaaacagaatagtttttaccagtttcaacctgcaacctattaaacactttctgatattcttctggtgtgtctgtaacttctaataagtattttgcatttaaaaatgatagtaattcaagtagttctgccttactacctgccatttgaactacaacgttaccttcatcgttcgtgtatgttccaattttatttctagtagccaaacaaatcagtccttcgtaaatttaatgtatttgttaactgtatacacatttttaactttttcccaaacgttagggtatacgttcatcaataacttagtatctgcgctagcacgtttgtactctggcattaatttaaatgtgcccccatcaatactaattttagattcccctaactcttccatatcagaaatgatactactttttagctcatcaatctcttctttaatacttttttgcaattcatataatttcttgtaagagcgtaagtccttctctagtagctcctttttttgtaaatctgttgttttcatacatatctctccctctcttatttctataataagattatagcatgtcagatatgtaaagtcaacacttttttatacaaaaagaattgcccattataaaggcaattcttgtccgttgtcttcttcaaaaagaatctctacaggtatattatataatttagcaagttttactctgtttttaacacgaggttcttttataccgttttcccaataagagattgatgaccagtgaactcctatcatattggctaactctcgtagagattcacccctagcctctctcactcttttaaggactttaggttttggtaccttttcttccatgactatccctccttattcttaaaaaataagagcctatcaggtagacaggctcagcatcaggaactatgcgaaagccccgatataagttactttaccattacatttacgtgcaaaagcctctaactctttacgagcacctaaacggtcaggttgcgaagattgaacagtaatttctttaggtaccgttacttcacgtgtacgaatttcagttttaccattttttaatttcttctcatactcctctgtacgagttgttgtcgtagaaatgattccataaaattttttcatattaatagctccttactgttttttttaataaattataatagtggtaatagggttttatgagactcctactcattgtaagccttccttaatagatacttacaactatacgtttatagacctctctcaaaaagtctccgtaacgtcttaccttcatcatttaaaacgtacacagaatttacaaaagttttatacccttctttttcagttctgtactcgtaaggtgaatttggcacacgagtgatttcttcatgtttagagttaagtaatgaaaaagcattctcttgctctaaaagaaactgtaccccatcaattaattcaataaaaggcttaacaataggttcctctgtactgtctttacaatcgtattttcgttctcctaaaatttgtagtatcatgtctatctatctcctctgtttaagtattaatttgtgagtttccactcacaatgctgattgagagagtcgaactcccattcccgggttacaaaaccggagtaatagccattatactaaatcagcgtaacccctcaatagagggagtttcttatactaaattaccatatccgtaggtatttgttttagcttgtttaaacatgatactcttgatagctaagtcattgtacttttcatcgtcttcgtcatcaaggtacacatcaacattaacgttcttacctaaaatatcgattgtttcatctttacctacttgtaagtctttactgttaaatgatacatcaaaatagatgtcgtcttcttttgtacgactaccgaatgatactctatcttcaaataaatttaaacttcgagagttaattacaacaggttgtagcccaccttcaaattgaatagtaactgtataatactgattttcaatattaagaatgttcaaatcagcaatagcttcaccaaatgagatgccaaagcttaattccaacgcaattgctcgtaagcaatcatagtttaacttaattctacggctaaacttaacaacactgtcaatttccccatagtaagctttgtctaacttatcttgcaagtaagtacgaatttcgtctgcatcagggtagtcgaaacgtaaatggtaatggaaacgtcccggacgattaagcataaagtcgtttacacgatttaagttattaacagtaagtgcataaatacgcttgcgttgtgataacccatcgaataagctcaatagtttttcttgtgattcacgaccgtcacggtcattgaatactttttcaaattcatcgaacaagataagagactcttggtcaatactgtcaataaattctgcgatacccggataagcttctgtaattaagataacaggcataccctcttcaatagctcgttgagataagatttgagtaaatagtgatttaccaatccctttatccccacttaaaataacccctaaactacgattgattgttttaaatgtgtgtagtactttctcaattttaactaaacggtcaccataaactttagattctttcaatttaaaatcgtctgtaaccgccaatgagaacccagacattgggttgaatctaactttataagtttgcgcaggcaacttatcataagttttcaggtcgtttgcataaatctcataattactaccataattgattactttcatatattctctccttaatactttttaataaattataaatggagagtgatggagtcgcaccacccgagcctaagcaacagatttacagtctgctccgctactacttacggaataactctccttgaataaccaaccagataggtacctgacacacggacagcacctgtgtctctctgttactggatgattaattgtgtatttcgcatcacctaatatagttatcaaggtaggacttgactatactagatttagctaggttctaactataatttcctatgatagctcctactactaatcatatttatatacagttaaactacacataactaaaccgattaccttggttcgcatgttaagaggcgcaggcaaccaatggacattgcaggtctcgaacctgcgaccgttcggttatgagccgaatgctctgaccaactgagctaaacgtccgtagggtagtagcaacaattacaaatgctactctcctgatgattataaacttatcaaatcggaaagacaggacttgaacctgcgacatcagactcccaaagcctgcactctaccaagctgagctactttccgtgttacctgtttaatttggtcttttaaactactacacacaggtaaagataaaccctctgccaaggggagactatcatcgaaccgtatgtaagttgcgatgggtagtagccatattatattaggttattaggaagttcacctatgcagaaggtgggagtcgaacccacatgtccattacagaccgatgtttctaagacaccgttgtctaccagttccatcacttctgcggttgtactaccaaggttacctctaaaaggctaaactcgtgtctggtagggagccataccttacatggattgcaaggaacctaacctcagtagcaccttttactattaagggtttctgatttaacgttttccctagaccgtaccttaacagtaatactggtgagaggatttgaacccctcttacctacaagcctccgacaagcgctatgggaaacaagcggtgcattaaccataactatgctaaccagtacactactgttttacgcagtcctcatactaataattcatgtggactcaaccccattcagggaagtgttagtctattttttggtgagaactggttaactccatgtacgtcaaacattccctagactactcacttacattgttatttaatgtcacatgacttatgacagccgtactcaaaagtttcaaggacttttacctcactatccaccgacagtatgctcggcaacgtctttctaataataaattacccatcactgttacagtaacagaaccattgaattaacgagcaatatcagtattactaaaagtagtctgtctgtgtggtacaagcactagcagtattacaacctatagtatgtctgtttgtcaatcgttaaattcttttacaggagtacttgttaaacttagggaggtataacaagtatgtgcacataacccgagtgctactccctaaagtagcctatacgggttaacgtagatggagggaatcgaacccccaaccgtccgcttagaaggcggatgctctatccgattgagctacacctacaaattatgggggtaatgagcccccataataactcatagtagtttcatctatcgaggattaaaatgaatatctaacttgaataaagtataacactatttacatagcatgtcaacacttttattaaaataaatttctatacctcactaatgccaatgactatacgtaaggagagaacgttgatggcactggctacttagttggcgctaagttagtgaggtatagaaagagaactacattgaccgaatcgtattatacagccttagtagttgttaacaatgtttggaacttagtagcttactgcaataagctaccccgaagcatcggggtgggactgtggtaagccccaaacccttgggtatgctccatcctgcctccggagaagtcaggctcaattctcattagttaaaggtttactagttaacggttagctgattagtcatactacgtaaactactagtaaaatatagttttccaattaaggctaacaatcggtagaggatttgaacccctattattggttttggagaccaacgtgttaccagttacactaaccgactatgtaaagaaggaaagcgaagaccttctttacagtaattaaaaaaaacaaacaaaaaaaatacaatcatggaatcaaggtgggatgtaaggagatgccatgtgtccacttacagtggaataggtaactacagatttgcactgttttacatcttgtttaatggttacctgttaatagctaacttccagtgataagtcctcttatatggtagttcatgtagtatttgtttgacaatatggtagctagctaaaatgacgacagtaacgggactcgaacccgtgtgttccacgctgacaacgtgttgggacagcctctgccctatactgccattatttatgccgtagtttttttagaaaggaaagtttttttataatatacaacaacagttgaagcgctgatgttactacggcataaatatattttttatgagcttttaataactcaaaacttaatataatagggcttttactcctgcttcatgcacactcactgcattcggtcacacacccagagaggctgaactatcgggagctacccaatagcttctctctgcttttaatgtatggtctagcacggtggctaacaacgttcacctaaacattcagcattaaatagtattgttataagttcttcttatatcatatattttgtaagctgacttaggctacttgtaccaaggtctcttgttaaacccatatttctatggttctcgtcaaagggagtcttttgaggtttctaaggtctgccaagtttctcacgcttccacctaacttagattcttttccacaggaacgtctattatatcccccaagagtcttgtaccttacaatccatgtacactccacataacgcttaactgatactagcttttactagtagttactcttatgtcaccataagacatacctgctacctaaaacactatcgcactctaggctacattcagaatcacgccacgttatcctagcaagctgttcaaactttctgcactaggttctattatattaagttttcaattatcaaaagcagtttttctttactatttaataatagcacaacctctattattttgtcaactacttttttttagagagggtgcccctaattttatataggggcaagagatattaaacatagctgagctatgtaaaagctaatgtaggaattgaacctacttaatgtaagcaacaccagtttagcttataagcattgtttgcaaagtccatgctatgcactcagtaggaatcgaacctattgccgaaggtaccaaactaccctgagtgctcctatagatatattataccacataacgagatattaattttttttggtgatatagtatatctatattttttaaaattttagaaatacctttgatacattccggttatccaacgtatgaatatataatatcatgttattctgattgtgtcaataacttttttacatttttttataattgtgtaatgtcctatttctttttttctgattccttatatttataatatatactatatagtactatatatatatattaattactattagatattatatatagataataagaatctaggaaatttaaaataggacattctaatgctgactcagttacaataaacttatggtggctacctttttacaaaaatgtcctatttcattttttctatctccttatattattatttataatatatagtattaagtattatatattattatatatatagtatataatataagaaagacaaaaatttaaaataggacattttacttaaacaaaaaaaaagagagcagttaagccctcttatcttaatgagaaatagttattaattgttcccaatctgacttcctcatcttctggtgtttcatcctctggtttcgtatacaagctagtgattctttctggaacatctactacgttctcagtagctgtctgtatctggaatgcatttacataagttaactcagaatctctatcagctagtttatgaactggaatcattggcaactctgcacctttcattgcaccatttacaattgacattgcatcattagttgttacaccgagtcttctagggaacacagaatatgtcccagatgctaatgaaacctctacaactttctctcttttagggtaattcatgatacttctcctttcaaaatatgttataataatactatatactataataacacattttacaaattacttaaacatgctgaacacgtaagtgacaactgctcctaagacaatcataaaaacgttctctacaatatccctcttgtggtcgaactctttatcgtttactccttccagtgcatctatagtttcttccaacttagtaatctggtaggttaggtgtgcatatttttcttcgtgaacagcaagtcgcttatcaagactattgacaatatctctcaactcactaaccgcactattcagttctacattgtcctgtttaatgcccttctcggttagctctccatgttggagtttatcttccagtcgttgtagtcttaaaacaaggtcatttacttggtaatcgttcatatatgctcctccctgtaagttatgttgctctatattagtcagatgtaaaccacagacagactagtatacctataatagcgcctaccgtgtagactataggtatatagtacccattaaaaaacaagtatagactacctatactaattccatagagcacgaaagtgaacttgtatgatgccaaagggctcagttctgcttgtagtttcttatactgtagtgcacgagtgacatagtaggacatcaagtaaacaaacatttgtagtaacagtacacagaccagtgctgtttcatacattat

SEQ ID NO: 3 - DNA, 143280 bp, Myoviridae Spounavirinae phiEF14H1
gttgttccctcctctcccttagagctactattaatatagtacactgagctgttagcaaacaggtgtgctaaattaatatagagactaaaaatgtagacgggagagtggtaaaaatggataatagcaaacgaattattaaaaaaattatttttattaccatctctgcattagtcatggttactttaagtaagctgttctctaaatatgttattgtagaacaaaatgccccatttcaggcattagttggcggtgcctcatgtgcactgttatctagtattctgtttgactggtatactaataaaaagaaaaaagagaacgtagagaatcaacttaaagaagcaatcagtgacttgcagaagattaaagctatcataaaaagatagcctattaggaggtgggatgggtgtctattaccaataaagacattaaggataaacgtagatatatttttagtcaatctagtaaaacaacaactataaaaagaggggacaaacgcataagtagtgcaacaagaatatgtgcagtttgtggaagaccgctatctaagctcgtattaagaacaggcgtaccaacagtagtagtagaccatattagctgtaagatttcagacattgttagactaaatgtctgtgaggatataaggtcttgttatgcgtattctagtaagaaaggggaaagctagctaatgggtatggcagatagacttaaagataatgcaaaacaaaaaaagttagaaagaacaccagagcaacaactaagagacacatttaatcaagcttcaataaagcttatcaatcaatttatggctaacgttacatcaggtgctatagaagttgatgatattgcagatttaacaaggctatttcagatttatttacaggttaataatataaatgatggaatgcaagaaggtacaggaactctacctgcacttacatctgagcataaagacatcatatctgaaaaggttagcacagaaaagattattaaggacggtgaagaagaggagctaatttctcttgatgagttagccagtcttccagatgaccaacttgaggaagtcttagttaacagagagctacagatgaacagagagaacgaggcgaccttctaatgacgacaaaagcacaacatatagctaaaatggctaaagagatgtatggtacagataaaattacaacggagcagttagcttatataacagatatgctgaccccatcaacgtacctattgagaaatcactctgtgcgtaatcacccaataacttttattatatcaggaagggatgcaacaaaagcacaggcacatagaccataaaccaacaaagctgtggtctttaaactctactaaacgggcatagtaaaataatatacacgtaaacaatatactggtaagagagactaaatcctagtgtataaggacagggttgacctaccgtgctaaatcagttatactataactgtaaaagcctaacgactaaatttctaggtagctaactaaaaggagttagtgagaactagataaaaggcaaataaactatgcaagctcaataaaaataataatatacaggaggtgattaagatagctaaggacagaaaagaaattttcatagaaaagctcaaaagtgtaaaaggaactgactttgaacttataggtgagtttacaaagcaacgagaaaagactctatttcgtcataacgtgtgtgggcatgtttgggaaaccactccggttgtcctacttaactcaaaaaaaggcggagggtgccctcattgtcaatacagaaacaaagcaacttcaccaaaagaatacgaaaaaagagtaacagacacatttaaaggagaatacgttgtactcaatattaatgagtataaaaacaatagtactaaacttaaattcttgcattctaaatgtggtacagaattttatctgcgaccagcaagtttattcattaatgcaactagttgtcctaactgctctaaaaataaccgttgctcaactaagagaactactaatgagtttagagagttgcttcttaaaacaaaaggatactcctatgagctaacggaagatgcagagtacaccggagctaacaaaaaaattaaggttaggcatacaacttgtggttatgtttgggaggctagagctaaccacctgctacagggttcgggttgtcctagatgtaacgaatcaaaaggagagctattagtagctactattcttaagctaagcaacacctcttttttgagagagcacacctttgacgattgtagaagtactagacccttaccttttgactttgcattaattagtaataacaaagtgcgtggtttaattgaatatgatggagaacagcacacgaaaccagtaagttgtttcggaggggaacagaagtttaaaagtacagtaagaaatgataacactaagaatgattattgtactcataaaaaaatacccttactcagagtatcatacactaatagtcctgaacagattgagcacctagttcagcagtttttaaaaagcatagatttgttgtaacgtagagcaacctaaaccaaaaagtaggttgatgatatagtctagtcccctaataaatatcgggaaaccgagggtaaccaaatgggcaaccaaagataataaatgaccaacatagagacaaggcaataattaaatcaagacaattagggttaagattagcccctttataaagcaatttgtaaagaaaactctgttaaacgggcatagctgaataaccaataagctgataagagaacctaagtcctgaaaaggatagaggtaatcccgtgctaaatcagtgcaaagcactgtaaatgcctaacgactaaatttctaggtagctaaccaaatggggttagtgagaactagataagaaaacctcttaagaggaagtaaagcagagcaacctaaaccaaaaattaggttgatgatatagtctagtcccctaataaatatcgggaaaccgagggtataacgtaagtgagatgggtgttggttctatgctacagtttgcagacacgcatagttatgatgctgttaaatgtctttatacattcccaacgaatgagcaaatgactaaatttgtacagacaaggttagaccctgttttacagaatgggtactacagcacaattgtagaccaagaagttaactcattaaaagctaaaaaaataagaaatagttttttgtattttcgttcaagttcaaaaccgggcgctgtggaaggtgtcgatattgactatctatctatggacgagtatgaccgtgtacctgcattagcagaggcttctgcgttggaatccatgtcttcctcaccttataagatagttaacagatggagcactccatcagcacccgatatgggaatacatgggctctttaaagggtcagaccaacattggtatttacataaatgtgagaaatgtaattattacaacgaaatgagttatgatgcatataccccagaggctcctgtagagagtagaggtaacattctttgtgttaacccaaaaggggtcgatgttgttgctaaaacagtagttgacggctcattccagtttgtttgtcaaaagtgcggagaaccgttagacagatggtacaacggtgtatgggtacctaaatatcctgatagaacaaaaaatggtctaggtactagaggatatatgatttcccaaatgaacgcagtatgggtaactgccgaccagttaaagaccaaagaacttcaatcattgtctaaacaagccttttataactatactctgggtgaataacgccccttcaactggaaacagttgtcgaaaactctgttaaacgggcaaagctgaataaccaataagctgataagagaccctaagtcctgaaaaggatagaggtaatcccgtgctaaatcagtgcaaagcattgtaaatgcctaacgactaaatttctaggtagctaaccaaatggggttagtgagaactagataagaaaacctcttagggggaagtaaagcagagcaacctaaaccaaaaattaggttgatgatatagtctagtccgactgccaagagcagtaacaaaatactacgaaagtagcggtagctcgtatccttacgcagacttgaaattaactgttaacgactctgacgttgatagccataagagaaactatttaatagaacctgctaaagacagaggtgattataaatttatatctgttggtattgactggggtaacagacattgggtatctatacatggtgttaaaacaaatggtacggtagatttgataaaacttttttctgtaggtaagtccaacccgctagaccctaatgcaatagatgtagacatacagtctataaaattacagctagctccttacaatccagatataatcgtagctgacgtaggagactcaggggataaagttgctaaacttatgcaaatttatggaaaagaacgagtttttgggtgcgtttacccatcaacccctaaatctacaggtaacttagtacctacttggagcccacaagcaaataaagtatccgctgacaagttaatgcagaataaacgttacattaacaagatgaaagaaggagaaataggttactactcaaaaccagatacagagcttaatttatataaagagcactggaagaatgttgttatacgtgatattgaggacgaaaagacatcgacaggttttagacaaattatcggcagaaaaggtgatgaccactactcacaagcaagcgtttattccatgttagggtatgagtacctaatgaatgtatttacaggagtaaaagagtatggatttgactctgattgggtgtcaactcaattagcacctacgaaacctgatatatttacagaatttgtataggtagattgccttatttagttttagtcaagctgaataaggcattttgtattgtttgatatatatttttgtggtataataaatatagttagggggatagttatggtagacaacaatgtaaaaataagtaaaagtacaattgaaggactaataaataagtctttaagttatgagtacgttataaaaaataacgaattgctgacaaacgaatatcaacatattgtaaaagcgtatgggtttgacaatttttatgacatgtatctatatgcagatagctgtgattctaaagatatgtatttagtaaaaggtggtcaaaaagacttgtctaagctgaaacccgttaaaagaaaagttgttagaaatggtaaaactatgactacaactatttatgaagatacaggcagttcagacagtaataacagtaaccctttagacaaagagagtaaaaagaaaaaagagttagaaccagttaatgctaaggaactacgtaaggtcagcttaggtagtgatgaagaagagaagttagaccctaaaaagatagcaaaattgctagcagacactaaaaaatttggaaataattttgatacgcagtgtactgattatcttattcttgaacaagactctgttacacgaggagtggtagggtttactagagaaggttcttatttaaaaatgtctttctcaatgtcagatgaggctgttgaaggtatgaagatgttagctttttcacagctcacattaaaggcttggaaattgggtctaggggctaagataagcacagataatgcacctgatgtagaggaactaattagcttatatggatacaaaagaaataatacagagtatattgtgtcaatgagctcactgcgtagtcttctaggggagccttagtcataagtgctacgttagtcattatactagtattttcaactattatttttttaatttttaatttactagtaagtaaggtagttaaagaattttataacttaaagatgctagcaaaagagggactaacagataaagtaacagatataacaaatgatataatgcatatattgaaaggagaaataaataatatggaattaattatgaataataagaaactagatgaattaactaataaggtagccactgatgaggactacgatatttttgtagagaagatgggtaagctagttaaagatttgtatgagaactaccagtttttacaacaaaacccaccagaaggagactacacatcaggttattttttagggttccaagtaatcagagcagaatacccagttgagtatgagaatttatttagattagctgtagataaaaatttaaatgaactagagataaacaagagatttgtcgaagctgttaaggatggtaaagttttaccactaggtgaggctatcattgatgaattacaaacagggtgtagctctatactacaggcacaagaagtacgtgtaaatattgtatttggtacaaaagaatatatggctaagcaagaagaagagcgtaaagaacgtcaagctaagttagaagaagaacgagaaagagctatggaagtactaaaaacaaaagatgacgtgcttaacacattaagagtaactgaggctttggctaatgaattaacagatgaagtcgcagaaaaatatgatttaatggagctagttaacagtatgagagaggggctgaaagctcataatggaaattaaaaattctttggggaaagctcttataaaaaatttaagattgcttaaagaaaaaagagatgcaatgcccgataacttagaatatacaagtcaagttatgattcctgtgccctactatctaataaaaaaaggggataatgcagtagaatcattccttatgtgtgcggggatgataaatagggataaagatttaggtctgcctatttctttagagaaaggtaagcaacaagttaagcttaacaatggagaactgacaactattgtagaatgtgttgctacttactcagataaaactgatattgacggtgtagagagattcttagttgaacatctataaaaattaaattaacgagttctattttgtgctatattagatatgcatgaaatagaactcgtttctttttttatgactaactaaggaggtttaatagatggcaggagaagtatttagtagcttgattacaagcgtaaatcctaacccaatgaacgcaggtagccgtaatggtatctctattgaccgtattattctacatcataatgcaacaacaaataaagatgttgctatgaacacgtggctattaggtggtggtgcaggtacgtctgcgcactatgaagtcacaccaacagaaattatagggtgtgttggtgagcagtattcagcattccatgccggaggcacaggtggtatagatgtccctaagattgctaaccctaatcaacgctcaatcggtatcgaaaatgtaaactcgtcaggagcacctaactgggatgtagaccctagaacaattacaaattgtgcccgtttagtggcagatatttgtaaacgttatggtattccatgtgaccgacaacacgtgttaggacataacgaagtaactgcaacagcatgtcccggaggtatggatgtagacgaagttgtacgtcaagctcaacaatttatggtagggggctctaacaacgcagttaaaccagagccaagtaaacctacaccaagcaaaccaagtaacaataaaaataaagaaggagtggcaactatgtattgtttatacgaaagacctattaactcaaaaacaggagtgttagagtggaatggtgatgcatggacagttatgttttgtaatggagtaaattgtcgtagagtatcccacccagatgaaatgaaagtaattgaggatatttacagaaaaaacaacggaaaagacatcccgttctacagccaaaaagagtggaataaaaatgcaccatggtataacagattagagacagtatgtccagtaataggtattactaaaaaatcttaatactagatttaagaccatcttagggtggtcttttttctttctttgtaatattcgtaataatatgtaatggctatgtaaccgcttgttattttggctgtaacaattacatgttatattagttcttgtaagcaacacaaataaagaaaacattgaggagaattttattttgaagaaaactagtattttaggtttaagtttattaagtttaggtttagtagtaggtttaggaaccgaagctaaggcagaagaagtaacagagaatggtaagacatattggaaggtagagtcaggagacacactatcagaaattggagctaagtacaacttagatttcactaatatccacaaagttaataaaggtgttgtagctgaccctaatgttattttcgtaggtgacaaattgttattacctttagatgaaaatggcaagctagtggaacaagtgaataccactgaaccagatattgaagtacaatataacgaaccagtaacacctgaacaacctgtagttgtagaacaagaagttgtagagcaacctgtagttgtagcagaagcccctgcccctgtagtagaggtacctgctgacagtagctcagcaaaagagtggattgcacaacgtgaatctagtggttcttatgatgcaacaaatggtcagtatattggtcgttaccaactatctgcctcttatttaaatggtgactattcacctgccaaccaagaacgagtagctgatgagtatgtagcaggtcgctatggctcatgggagaacgcaaaatctttctggttagcaaatggttggtactaaaattaaatagcaataaagacctctttattaaggggtcttttttttatgctatattaatatatagtaaatagtaatataaaatggttatgattagttatgtggtataatagacttatgttaaaaccatttaaggaggggaaacatgggttatattcaagatgagacatggcagatggttaaaaaagttgctaaaaagaatgggtttgttggtgactggattttaattatccactcatactatgagtatggtggaaatcacgtccagatacatacaacaataaacggagaaagctatagaattttaagattgttagatagcagagagatacttttattagatagaaaaggtaaccctgtaatttatgactatgaaacagttaacgatggtcaaaaaagcttcttttataatgatatggaagagaaagaaatcgaaatacctaatggaagatgcttaaacgataagacaaggataaaaatttatgtataaggtaggtgtaacagttgccaaaatggttagataaagcactgggtatagaaaaatcgtccatagaagaaactaggaatatggaaaattataagatgcatttaagggaaatagacaccaatgtggtcaataacgagccgtacagtatggaaagtattgaaaaaggtatgaatggtaagaccactgcatatatgcaaccaattattggagagatgtcagtaaaccccgggtataaaactaaaccgtctatacgtaactctcaggacttacataagacacttaaaaagtttggtaataacataatattaaatgctattattaatacacggtcaaaccaagtatcgatgtattgtaagcccgcaagaaattctgagacaggtgttggttacgagatacgtttaaaagatattgaagcagaacctacttcacatgacattgctaatattaagcgtattgaaagttttttagaaaacacagcacaatttagagaccctaatagagataattttacaactttttgtaaaaaacttgttcgggcaacatacatgtatgaccaagtaaactttgaaaaggtatttgataaagatggtaactttatcaaatttgatactgtagacccaactacaattttcttagcaacaaatggtgaagggaaactaattaaaaacggtgaaagatttgttcaggttgttgataacagaattgttgctaaatttaatgagagagaactagcattcgcagtacgtaacccaagagcagacatcgaagtaggtcagtatggttacccagagttagaaattgcgttgaagcagtttattgcccatgaaaatacagaggtatttaacgatagattcttctcacatggaggaactaccagaggtatcttacatgtaaaaacagggcaacagcagtctcaacaagcactagacattttccgtagagagtggagaagctcactagcagggataaatggctcatggcaaatacctgtagtttcagcagaagatgtcaaattcgtcaatatgacaccctctgccaatgatatgcaatttgaaaaatggcttaactacttaattaatgttatatctgctttgtatggaattgaccccgcagagataaacttccctaacaatggtggtgcaacaggctctaaaggaggctccctaaatgagggaaactcaaaagagaaaatgcaagcttctcagaataaagggctacaaccccttttaagatttatagaggacaccgttaacacatatattgttgcggaatttggagaaaaataccaattccaatttagagggggagacctaagtgctcaactagataagcttaaaataattgagcaagaaggtaaagtattcagaacagttaacgagataagacatgataaaggtttagaaccgattaaaggcggagacgttatactaaatggtgttcacatacaagctattgggcaagcgttacaagaagaacagctagaataccaaagaagccaagaccgcttaaacagactattagagctatctggtggagatgtagaacaaccagaaccagaagagcctaaagacagtcaaaatgatacagatgtttcatttcaggatgaacaacaaggtttaaacggtaagtctaagaaagttaatggtaaggtagacgacaatgttggcaaggacggtcagttaaaatcggaagaaaacaccaactcaactaagcatggtactgatggtataaaaaaagaataaaagataatggagggggctagctccccctcaactttgtttgtgttactagatagtacatgttctgctatattaaatacagtaaaacgtttaggtggtgaaaagcaaattgtcagaagttagagaaaaatatagtattttcgtaccactggatattgaaaattctatacagaagtctgaatctgtgaatgatggtgaatggtatgttcaaggatatgcaactaccccagatttagatttacaaggagatattattttaccacagggcattgatatttcttattttattgaaaatggttggataaactatgagcataaaaatgatgctgagtttattataggtgccccaactagcaattgttatgttgatgtggacaaagggttattcgtagaggctaagctattaaaggataacaagtacgcacagtctatgtggaagctagctaatacaatccagaaatcaggaatatctcgtcagttaggtttttctattgagggtgcagtagttagtagaaatgcacaagataacagaatcatagaaggtgttaaaatacataatgttgcattaacgacacatccggctaacccaagagctacatgggagacactagttaaatcttggactacaggatatggcacagcaccagatgcacaagtagatgcaggcgcacttagaagagagatgtttaaagaggacatttctaatttgacgtatgcagtaagaactattgcaggactatataataaaaaacctgcagagaaagagtttattttacgtgaagtggctaaggatatagaagtagacacttccgaaaatgaattatctaaatttatgttacaattaagtagagggatttccttgaaagaagcaacaaactttattgaaaaaagaaaggggtaagaaatagtggctaaaacattaaacgatattatagaagattttgatgcacagttaaatgaaaaagtaaaacctactacagatgaggaaattacaaagtctgtagaagaacctactgaaccagaaaaagttgaagaaggtgctgaggttgagccggaagaaaagcctaatgaatctgaggagactacaggcaatgacggagaagaatccggagttactgaaacagttgaagcagaacaggaagaaccagaaactgttgaagaagtagcagttgaggaacctgttgaggaacctgttgaagaatcagcggaaactgttgaaaaatctgataaaactaaagaaaataaagatgaagaagaggaggaagacgaagacaaaaagaaagaaaaagacaaaaaagacaaagataaagaagacaaagaagacatcgagaagtctaccgaagtcgaacaagttatcaaatcttctgaaatcttaggagctatggaagctatctttaaaaatatgttaggtctaagtgaaaagttagacgaaattcatagagagtttaaagaagctaaagaagctaaagaaaaagacgaagcggagtctgttgagaaatctttacttgataaccctgaaattaaaacaggaaaagaggactcagaaggcaaggctgttgggtttgttaataagtctgtagcagttgaggaagaggtggctaccgaagaaccaactgtagaagtagttgttgatggtgaacaagacacagcagaacctgaaaaagaagtaccgttccgtgatagagtacaggctattagaccagactttatggaaacatataaacgtgtgtctgttagcggagtagctcaacgtggtgaattagaatcagttagacacacttggggaactgctagaacaaatgatgacctagctaaaattgaagggtttattaataaatataaataaatttactatatagtgaacgatttttaattgtactgctatattaatagcagaaacaataaaagacctgacattccctcctgaacctccacagggtcaggtcttatattgagaggaatataaagaaaggtgatttatacataatgacagagaaaaagaatacagaacgacaattaacttccgtacaggaagaagtaattaaaggcttcactacaggatatggtattacaccagaatctcaaactgatgccgccgctttaagacgagagtttttagacgaccaaatcacaatgctaacttgggcagacggagacttatcattttaccgtgacatcactaaacgtccggcaacttcaactgtagctaaatatgacgtatatctagcacatggacgtgtaggtcatactcgttttactcgtgaaatcggtgtagcaccaatttcagaccctaacttacgtcaaaaaacagttaacatgaaatacgtttctgatactaaaaatatgagtatcgcaacaggtttagttaacaacattgaagacccaatgcgtatcttgacagacgatgctatctcagttgttgctaaaacaattgaatgggcttctttctacggtgactctgacttatcagaaaacccagatgcaggttcaggtttagagttcgatggtttagctaaactaattgacaaacacaatgtactagatgctaaaggtgctagcttaacagaggctttacttaaccaagcatcagtattagttggtaaaggttatggtacaccaacagatgcttatatgcctatcggtgttcaagcagacttcgttaaccaacaattagaccgccaagttcaagtaattagcgacaacggtcaaaacgctacaatgggattcaacgttaaaggttttaactctgcacgtggtttcattcgtttacatggttcaactgtaatggaattagaacaaattttagatgaaaatagaatgcaacttcctaatgctcctcaaaaagcaactgttaaagctactttagaagcaggaacaaaaggtaaattccgtgatgaagatttaacaatcgacacagaatacaaagttgtagtagtatctgacgatgcagaatctgcaccatctgatgttgcatctgtagtaattgacgacaagaaaaaacaagttaaattagaaatcactattaataacatgtatcaagctcgtccacaatatgttgcaatttaccgtaaaggtttggaaacaggattgttctaccaaatcgctagagtacctgcaagtaaagcagttgaaggagttatcacatttatcgatgtgaacgatgaaattcctgaaacagcggacgtattcgttggagaattaactccatcagtagttcacttgttcgagttactaccaatgatgcgcttaccattagcacaagttaatgcttctgtgacattcgcagtattatggtatggagctttagcattacgtgcacctaagaaatgggctcgcattaagaacgttaaatatatcgcaacaggtaacgtgtttaactaacgctaatctttaaaagactaagcaaaattgaataaaaatggaataggggacggttaatactgttccctatttttattataaaatacatgtatggaggaaataatatgttaaaatcagaaatcttaataaataaaacagtaacaacagcttttggtgaggcaacatttgaccataatggggaaaccacagacctaacagtagaacagcaagaacatttagggactaaagttccatatatacaatatataccagatgcacctaaagctaaagaaaaagaagctactgcagaaaaagcagacgaggcacctaaaaaggctaagaaagcgcctgctaagaaaactacaaaatctaaaaaagaggaagactaaggaggtatttatatgtacccagactacggatacgaggaacaaggggacaatacataccaataccaaccatatgcacatgggaaccctaagcatatagatttagacaaaattgatgatatacagcctgctgattatggttggacacctgctacgctgaaacaatacatgtttggtgtagaagttgttaaccctgaaacaggggagcctttaggagatactttctatgaacatatcatagattcagcaatagctaaagcagagaaacgactagatattgctattatgcctagacttataagaggagaacaccatgattaccaccaatcagatttcaactcttacatgtatactcatgtgtttaaaagacctattattcaagcagaaaagcttcaattagaagttaatggtagagggctatacagatacccgtctaattggtggaaagtgtatgcactagcaggtcatatacaaatgtacccaacatccctcatgcagactggaacacagtttggttatgaaatgacgttctcagggtacccacaattagcaggaatgcctccatcaggaggacaagttgatgctcctcaaatgattcatattgactatgtggcaggaatgctacctaggaaaaatagaggatacaatgaagactgggagtgccctgcggacttagaacagcttgtaataaaatatgcgttaaaagagatattccaacaatggggtagacttataattggtgcaggtattgctagtaagtcactaacagtagatggtattagtgaaagtatacaaacaacacagtctgctatgtatggtggagcttctgcagatattcgacaaattgacgaagacatacaagaattagaaaaatcattggtatcttactttggaatgaacttaggtattatttaaaaaagggggttaacaaatgggtgaaaaaccaattagatttggtggagcaggtgaaacaggtaaccctaacaagcaattaaatactagtagggttgaatttgaaacaaaaggtatggctagcttcattgaaaatagaggtattgacgttttgtgggaaagagcatggctatgtacatgccgtaacccaatgaccctctcacctaagtcggattgccccatctgtaggggaagagggattgcttaccaacctgcagtaaaattaagaatggctatacagagtcaagagaaaggtatctctaatcaagatttaggactactagacacaggaaccgctattggaacgactgagctagattctaagataacctttagggacagaataacagtccccgaagttaaaatatatcaaagctttatttttaatgtaaataaaagaagagtagctaatggactatttttaagctatgatgtgaacagtatagaagatatttatggtaaagacggacgtatcttagttgatggagtcgattttagaatggactatgacacaaatactatttatccaaatgaatctttaatagatactaatatatccataaatatgtctgttacacttagatatattgttatagacctgttaaaagaaagtagataccagtataccacattcggtgttaaacaaacacaatttgaatcactacctaaaaagctcttattgaagcgtgaggacgtgtttattgatagtgaaccattttcattagacatagatacagcaagccgtatggaagagctagagggcaaaaaagatacaagtgaagctatggtagaccctaagcgtaaagctacaaaatcaggaggcttctttggaggtaagttaaatggctagaaaaggacagagacccgtattatttactgattcaaaagcaatacttggcaatctgactcgtgcagtggttgatgaagtactaagtgatgcgcaagatgttgctctacgtaatgggtcttctgtacagagaatgcctagctatttgatagtaacagagtctaggatggcaaaaaatggggttatagatttgaaacctttctttgcacgttctaataaaaagaaatataataaaaaaggggaatggtacctatacatccctattagtatgaaaacacgcaacatgtcaagacgattatacgatgagctgagagcagttccagtaggcacaaaacctgtaactgttaaaatggactatctgtatgatagacggaagcagagcccatcagtgtctagtattaactataaacctaaatctactaatgtaactgttataccacagagttggggtaaaggtacacgtaacacctatgtagctttccgtacagttaacgctaattctcctgcgaatagttggataataaatcgtagaaacgttaatgatgatgatatgagtaagacaatgctaagaaacatagacaggctcatgaagtggaaactaaagaatttaggaggatagtgtatgataccaagtttagacacttacttgtataaagaatttgaagaaaggctaaggataattctatcagagtgctatattatagacgaagctttaaagggaatggacaaagaagctttagaatcttttaaaaacacttattgctctatagatggtaagccacctaagagagaagtagagatgtcctattcattcccacaagaacatctggattcatttgctcgatttgtagtaactctcggtagtagcgaagaagatagcaagtctattggaggaatccaaggaggctacgagtatcgagaaggtaatgtaattagtgaggaagccactattattagagaaggtgacaagctgattataaatacatcaaaaccagtagcggactatctaaacagctcagacataagttttgcagaaagcgaccattttaggattgaagataataaacctgtatttgatttttcatacaatgaggagttagaaggtatatccattaatgtgtcgtatataagcaaaatatcagatgatgatgttgcaggtgtatacaaaggataccaatctaacgataatgttagtataattggaataagttctaatatagatactgctaggtgtttagatgcaattgctagaattatactaatcaccatgagagacagtttagatgaaaaaacagggtatatgttgcaaacactacattttggtgatatgcaagttgtcatagaatcaggtgaaacacttgtgtttggtagaccttgtactgtaaactacagagttactaattctattggatttgatttacaacaaagaatcacagagattattacaaaaaggaggatgaaatcctagtggctaaagaaacagagaaagtagtaaaaaaagaagttaaaaaggagcaacctaaaaaacctaaaggttatgtccatgtcgatacatttttagattatgcaaaagtattatatggactaaataaatatcaggtagcgggtttcagagcactaatggcaggtagagaataccaacacgaggatgctgattttgttccatttttagaaaagtatataggaaaggaagttaaataataaatggctgtagaacaattcccaagaaaaaaagtatcacgtccacatactgagattaccgtagacacaagcggtattggtgggtcatcaagtagctctgacaaaacattaatgttagttggctctgctaaaggcggtaaaccagatactgtttatcgtttccgtaattatcaacaagctaaacaagtactacgtagtggagatttgctagatgctatcgagttagcatggaatgcatctgacgttaataccgcatcagcaggagacattttagcagttcgtgttgaagatgctaaaaacgcaactcttacaaaaggtggtttaacatttgcttcaacaatttatggggtagatgcaaatgaaattcaagtagcattagaagacaacaatttaacacacacaaaaagattaactgttgcattttctaaagatggttataagaaagttttcgataacttaggtaaaattttctctatccaatataaaggtagtgaagctcaagccaactttacaattgcacaagatagcattagtaagaaagcaacaacattaactttaaatgtaggttctgaaccagaaagtacgacagaagtaatgaaatatgagttaggtcaaggggtttactctgagacaaatgttttagttagtgcaatcaatagtttaccagattgggaggctaaattcttccctataggtgacaaaaacttacctactgatgctttagaggcagtaaccaaagtagatgttaagacagaggctgtattcgtaggagctttagcaggagatattgctaaacagctagaatacaatgactatgtaactgtagctgtagatgctacaaaacctgtagaagactttgaattaacaaacctaacaggtggttctgacggaactgctcctgagtcttgggctaataaattcccattactagctaatgaaggtggttactacttagtaccattaacagataaacaagcagttcactctgaggctttagcttttgttaaagaccgtacagacaatggtgacccaatgcgtattatcgttggtggaggcactaatgaaacagtagaggaaagcattactcgtgcaacaaacttacgtgaccctagagcttctttagtaggcttctctggaactcgtaaaatggatgacggacgtttgcttaaattaccgggttacatgatggcttcacaaattgcaggtattgcaagtggtttagaagttggtgaagcaatcactttcaaacacttcaacgtaacatctgtagaccgtgtatttgaaagtagccagttagacatgttaaacgaaagtggagtaatctctatcgagtttgtacgtaaccgtactttaactgcattccgtgtagtacaagacgtaactacttacaatgacaaatctgacccagttaaaaatgaaatgtctgttggtgaagcaaacgacttcttagtttcagaattgaaaattgaactagataacaacttcatcggaactaaagtgattgacacaagcgcaagcttaatcaaaaactttatccaatcattcttagataacaaaaaacgtgctcgtgaaatccaagattacacaccggaagaagtacaagttgtcttagaaggtgacgtggcatcaatcagtatgactgtaatgcctatccgtagcttgaataagattaccgttcagttagtatacaaacaacaaatcttaacagcatagagtgtaggggcagttgcccctcctcttacataatgaataaaatataggagtgatatatacatggctagtgttggaaatcaaacagtccacacaggtaacacagtttacctaatgattggtaataaaattatcggtcgtgcgcaatctgcatcaggtgagcgccaatacggtacacaaggtatctatgaaatcggtagtattatgccacaagaacacgtatacttgaaatatgaaggtacaattactttagaacgtatgcgtatgaaaaaagaagacttagcaagtttaggaattacagcgttaggtgaagacatcttacaacgtgacattattgacatcgtaatgatggataatttaactaaagaaatcgtagtagcttatcgtggttgctctgcaatttcttactcagagtcattcacagctaacgaagttacatcagaaagtacgcagtgagattataaatacaaaatttatatagctgtgctagttcgtaaagagctagtatcgagagttaattgctttgaatccctaaagctcaacgacccaaacagtaactggaaacggtaagctgagaggtgcgaaagcagaaaaaatagttgagatggtataaggttaaatcctaagtactgatacaatgggtctttagcagggacagccctaagtcaattgatacgggacaccttcaacgactatcctctgacggaggagtaaagccacaagccaatggtggaagaaaaattctctaccctaacaagggtacccatatagtctgagctaacatgaaagtgttagaggcaaacgcctacttggaagttgcgttccaaggtaacaaaactgttcacatacctaacttctgcaaaggttaaatagcagacgaactccacccagcttgactgggtggttcttttacggtacaatacttttattattgttagatatttaggagatacaacatgagaaaaaaatggacattacaagaaagaaatattcttataaaaaaatgggcggagactaacaacgtaaatctcttaccagaaacagcaacctttacaggaaataagagcactatatactacgtatggtcagatggggagcttcaaggcttaataggtaaaacgaactttgacagtataatatctggaagtaaacctacagttaacggtctgacagaagagagcaaaaatattagggctaaaaaacgctttttggaatatgggctcgaattactagaggagtatcaaggattcaatacaccacataaggtgagagtgttggatggagtatacgcagggtattatggaaaaacctcattagccacagtcaatcaaaaaagtaccagaggtaaaatagcgcagttaaacataactattcttacagaaagtgagaaaagacgatatttcagagaatatgcagagtctcggggatacacaattattaactaccctgaaaaattagctgttcgaggtaagtgtactttgttatctccccaaggtaatgagtgggagacagtctggtaccattttgcttatcaggagaactgcaattgtccgttagatgttaaacgtagtattggggagcgcatggttagaagtttgcttaaagagaatggtattaactttgaagaacagaaaaagatagttattgatggtagaacattattttttgatttttacttacctgatgacaatacctatattgaatataatgggaaacagcactatgaagacaccggaggttactataagggtaaacttcaagatttacaggaacgtgacaaactaaaggagcagtggtgtaatcaagcaggtgttaatcttgttgttatcccatacactgcaaatagcataaacgaagtagctaatgttttatccgagatagtaccaattaaaaagagactagtttcagttgtttattctgatagtatacctaatgaggatattattgattactataaaacacatacaggtaaggaaacttgtaggaaatatgatttaacacaacgtagactgagcttactttgtaacagagtcggctttaataaaaggaggtacctaaagtgaaatatccatatttagtagaattgtatgcaaaacatgtaattagagatgcagggtacatagaaaatgtaccaccagttatttatgaagacgttgtgaaacgtgttgaagaaataaaaagagaagaaaacttaacaatagattaactagtataagtttaaatagacctaattcagatataggtctattttttttgccactataaatacaaataactagatagtgtggtataataaagatagtgctatattaatttatgagtaaactaggaggaaataataatgacagaaaataatgaaaaggtatttacacctacaccaaatttatcacgtgagcaattaatagaaaagttgcaacgtggagaaaacttgacggatgaagaagtaaatattttgaaatattacaatgatgcagaagaacgtaaacagttagatagaattatcccgggtgttaatgatgtattttctaagcattacaacttaaaagaatatggtttagaatttgatattaaaataaaagcacctaatattatcgaaaatggtaaaattcaggcaagaagagaagcctatttagaaggcatgggaatggcagttagcaactttattttccaaagttaccaaatgttagcaactattcgagtatgtggagtagaggtaccaaaagtattagctgatgatgaaaaaatttataatttatatgtattaggagtaattgcaaaggactatggtgaatggctaaactcctttcgatactagagttaaagaactaggcggaataaaagcccttgttagaaatagctatagtagaaatctatgggcaataatgaaaaaatttaaggtactaccgagtgaccctgcgtggcaaaatctcacaagtgaccaagtagagtggattttatataacatggaaagagacatagaagaacaagaacgactagctaagggaatgcagttagaaagtgagttccaagactatgacgattcatggtatgataaaccacatgatgagttctctccaattcgtgaaggtgacgatgaggaagaaattgctcgtaaacttagtgaaatcacaagtgaggaagacatggctaaacttaaagctcgttgggaggcaagccaagaagttgatgctatccgtgcagaaggtggaacaacaattgaagaagatacgattaacgaacttattgctaacaatgttaaaaaagcaatggaagaggctagacgtattgagaaacatggtggaaacaaatggcaagagaaatcatcaattgagttagaagaggaacgtaagaacctagagtttaactcacagttgaaacaaggagatattcaggaggctatcgatttgtttaacaaagatgtcgagccaacatcattagatgacgaatttcaaatttaagggtagggtattccctgccctttacttgtaaaggaagtgtggaaatgagcaacaattatcgtttttatgttgaggcaatgactggggatgctgttgcaaaacttaatgaaatagacaagttaatggataaaattgattcaaagagtgcaaagggcacccagaattttttccatacaagtcagaaagacattgataaagctgttgaggaaatgcaaaagcttatcaaggcaaaaaaagaactagatagagcttttgataatcagaagataaatgcagaaagcatgggagacatgacagcatataaacgtgctgtatcggatgcagaagaactaactagaagatttaacaaggcacaaaaagaatttcaaaatcatgctagaatgcaagctaaccctaattacataaatgctagtacactaaggcaacaaaaggcatttcgtgatgagttaacagaacaagagagagcaataagaaatatctctagggcacaacaggaactaaacagagtgaactctagggttaaccatcgtgcaaaccaagcaagcgcaacaggaagaatgacttacaatcagtcagagagtatgaagcgtgaccttagacgtactggtgtatttgaaagcctaggttcagaaaataaaagcagacagcaagagctacgagaacgatataaacagagacaagaagagctagcagagactagaagtaatacaaatttagatagacaagttcgtaagaatagggaaactagtattcaggctgagataaaagaaattgagaaagaaattgaagctagaaaacgcctagcagactctattaaagagactgtagagaacttaaaatctaaggaagcttcactaaatgcatctgacataaaagtagatgctgatagaaagagtgctcgtggtgttctagctgagcgtgcaccttctatatcaatggctatgctaggaggtaccgccgccgccataggtggtttatacgcaaaaggagcaactgctaacgcaggtatgcgtgatgcatctatatctttaggacaacgtacaggtactagtgacttccgtgcattaagaaaaagtatgcaagaaatgggtattgagaaacagttaggctataaaggtgctgacatgttacaattccaagaagatgcattgagtaatattggttttacaagtaaagaggacttagcagggagtacaagagccttagcagagggctcaagagcagttccagtagacaatgagactttaagtgacttcatgaatagtcaaatgaagagcggggctattagtggtagagaccaaattaagaatattcaagaaggtttcttaggtgctatccaacgctcagggatggcaggtcgtgagaaagaacagctagaagctcttaaaacattaagtgagcaaagctttactggtcgtaacggaagtaatcaagagcttaaagaacaaatggcaatgttaacaatgctaaaccaaacaggtaagcgtgctgttcaaggtgagcaaggggcacagttaatgtcaagtttatctgcaggtattcaaggtagtgtatggaacaataaggcatctttacttttaggtaaagggacacaattccaagggctagcaggaatgtacgacttaaaagctatgcaagaacaaggagcaacaccagagaacttacagaaaattattggcagtgtccaacaatcagttcccggtgacgaaaagtctcagaagtatgctttcggtagtgctttacacgaactattcggtacagatgctaagaatgaccaaatagatgcaatttgggaggcttatgccaacggtggtttaagtcaggataacgtagacagaataatgaatgaaagccaatctacaggaaaaggcaaatacgataagaacatagaagactatgcaaactctaaagaaggaaccgctaaccgttcagaagctgttacagagaaacaagcttcacagattaatgatatgggggacatcttaagagaaactaactctaaattaggagcacttcctcctgcgttatatgcgttaggagcaggcttaggagctatggctgtttcactagccacatcaggctctattggtggtttatctagtttaatcaaaaaaggaactcgttctacttttagtacaggtggaggggtaactgcagggggcggatttttaaaatcagctaaagaagcattctctgcaggtaaaggctctggcggatggttccaaggtattaaaaatgtaggtagtgtagctaaggactccgcaatgggtgtcggagctaaggctgttgaaggagcaaaaggactaaaaggtgccggaatgggcagtaaggttcttggtggcttaggaaaagcaggtaaattcctaggcaaagttgcaacccctctagcgataggttcctctctactagatattgcaaccgcagatgataaaacaaaggcggtaggggagagtgttggagctattggtggaggtatcggaggagctaagttaggggcaatgattggtacatttattgcacccggtcttggtacaggtatcggaggagctattggtggaggtatcggcgccataggaggtactctagcaggttctaaactaggcggtaaatttgttgatggtgttcgtaaattcttcggaggagaagaagctcatgcggaagaagcagacttaactgcagggcaagatgttgcttctgggcaagagagtaaatcaggagtacaagaagccagagacacggctaacaaacgagtcctatctgagaaaacacgtgcagagaataacgcagaagagtccgccaatctctctatctattctaagttattagatagagcccaacgtatactaaaccaagcaaaaaatcaaaacggtatattcggtaactcaggtagctctaaagattcttctgacggaatgggttcagatgcttctagtaaagactttggaggagactgggagaaagccattagacaagcatctaagaaaatgggagtagatgtttctgacgatgaaatagatacaatacttagattgattcaggcggagtctagtggtgacgagagcgccgttcaacagataattgatgagaacaacttcaatggcaatggtggagctaaaggtttgctacagtatgtccaaagtacttttgatgcatacaaagtagacggtcatgacaacataatgagcgggtatgaccaattgctagctttctttaataatagtaattggaaaaatgacctaaattcttgggatagccgttatcaaaacggtagtacaggatggggtcctactggtaataaaactagagcgatgggtgggcacataactagcccagagtatgcgctactgggagaggtagcaggtcaagatgagtatgttataaatcctagtcagccaacagctccacgtttattagcagaagctactagaaaaacagcccaaaacttccgattaacaggtaatggttctggtcatgattggggagcttcaatttctaaaataaatgcaacaggaggagctcaatcaggttcagctcctacgatgacaaatacaaatgaggtatcagttaatgtcaccatacaaggtggaggaacaagtgatagtatagctagagaaattggtgataagtcagcaggaattatcagcaaaacactcgatgctaccttcacagatttcttcgcaaaagaatacaggagagtgtagaggcttaatgtctctacttttctctaaggaggtttataatgtcagtagagttaagatacccgagatttgatttaactttttttacagagacagacaactaccatatagtttatgatgcaaaagatgggcttactggacgtaataacaataacggtgaagcagagaaggtaagcaataattttatggcagagtctgtaattagtttaactacaaaaaatgctttagaggatgatagtgcagtcttctcattcgtattagcaggggacgtgtattgggatagagtactaaatgctaatgatgcagttattcttaaaatagacccagatacttcctccactaaaaaatcagataaccctgtactactagttggtttaatatctgaggttagactagagggtgactatggggaaaactctaagatgtacaggataacaggacagtctttcgcaaaggcgctaatgcagtttgacttaggtgttattcaggaagtaagtgtagttttgacagatttaggttggttgcctgacgatgcacaagaaggtataaaaatgtctggtagtagtgcaagtcaaatagcagaaagcttaatgaaaagatttttacaatatatgaaatttaattttaatggtcaaggtatagataagttcttagagtgggagctagatagttggacagaggcggagagactaatagatagtaccccttacataaactatgaaggttctttaaagcaacttatagatgatgtaaccgctaaaccgtttaacgaattatatttcgatgcaacaccagagggtaaatgcagaatgattatgcgtagaaccccatttgataaatctgattgggaaaaattacaaacctacacagtaacatctgcagaagtaatatctgaatctgtagcagttaacgatacagaagcttactctatatttaacatatctattaataacttgtatgggactgactctatgatgttaggttctaaaccacaagtattccctgatttagtttctaaatatggttataagaaactagaagtacctaataggtatttagaaggagcaattatagataagagtaacagtggagataaagctaacacaaaacccgaaagtgataatgatagtaaagagagcgatggctcaacagctaaacagatgtttgacagagagtacgctcttgtcttaaactatctaaaagggtatcctgttgatgtgctaagagttaaaaaaagtaatgtaagaacatcaataacacaggtagacagacgtataacagataacgaagcagataaaattatagaccactatattacaaatcaagcattaagtaaagaagacttttctaaatttacaggaataaccgaagaaaatatagaagagggtaacggtaaagtagaacctacatataccgcagttagggacttccttaatgggttagataaaaacctaggagtatctagcataaaagagaaattaatgaactacttcaatttgatacctaaccaagccacatctattgctagtgaatacaaagcacaaggtaacttaggtaaactaaaatatgaagaaataatggagaataacccaagtgatagctcaaccgtcactggttcagataaacgatttgtttctgagttcactaaaagactagcaaattggtactgtgaaaacgctaatttctacagtggggatattgtagttaaaggtgaccctaaatatagattaggtaaccgtttgtttgttcaagatgagcaaaatggtgagttgtgggaatactacatagaatcagtagaacactcgttctcctatacacaagggtatatcactactcttggggtcactagaggtttacaaaatggaggaaacgatagattcactcatttatggggtaaatctgaggacttctccggaggtatgctaggtgagaaaaccttgcaagcactactagacgaacaagcagaagcaaacagtaaaaatgatggaggctctgatagtggaggtagctcaggtaaagagtatacagcaggtgcaggaactcagctagcggtattcccattagacgtaattaatgtaactcagggagaaaatggtggatacagccacatgggagcacttgcaatagacttttcagatggtactcctcataaaccttactatgcaccatttgactgtgaatgtgtgtacactgactcttactcaggggttgcatggcaatctcaaaagcctgttaaatgtgtagatggtagcgttacttacgtaacactattatgtgtacacgacaacaactgggcaagcaacaaagtaggggataagaaagctaaaggggaagtgatagggcactcaggaactgcaggacaagcatcaggagaccatgcccacttcgaggtgtctaaaggtaaatggcaaggttggagcacaagcagtgcgggagtttactttataaaaaacccttctcatttatacgatgtattttctataaaaaataatgtaactggaaaaacaactaaaattatgaatggtggagggtacaattggcgtagtatagactgggacgataaatctggctcaggttctggaaagaaaaagacagttggtgctagagccatggctactccattcggattacgtatgatgcgtagcgctcctgtagaaccagaagaaccaaaagttgttaaacaagtagaaactaaaacagttgttgaaaagaaaccaaaagtagaagttaaaaagctcccaatactttatgggaataacattgccacagaagcaactaaatggggaagagctcactcgaaaacagagtccacattccaatctgccttcaattttggagctaatacagataaagacccatttgaggaagacattatagcaacagacagtgcaggatttgtttggtggtgtttctaccatgcgggcatatcactatctggtggagctagaatggttaccactcgttcactactctatgataaccaattacaaactatctctactagaggtcagaagtctttagagctatttgataagatgaaggtaggagatttagtttggtttaacagagctagtcatgtagggatatattgtggtgagggcaagatggtctcttgtaatggaaaaggtaacatggatgagtccccaaaaacaggtattgttattgtcgacatgtctaaaggttattggtggaacgcttttgacggaaatgtacgtagatataaataaccctattttttagggttatttttttttgtataggtagtttttagttattgtgctataatagataatgaggacacatgatgagaggatgaataaattggtaaaacgcagatttcaagcaggtctaggctcagaaattaaaagagtatataaagaaggacaacaaattaacacgctactattagcacaagtaattcaagtaaactataaatataatacagtagacctactagctttacagcataaagaagtatttcaaaattcctatgcaaatgagggacgtttctctgcaagacttcctatggaatttggcggtagaaatatcgttggacagccttatgggcaggttaacccgatagcagtaggaacagtagtattagttggttttattaattccgataaagacatgcctattgtaattagtgtttataataataacgatgtaagcaagcaactttcaagaacacaattttcaaattcagaccctaaagatttagagttaattggggatatgcaccaaaaatttagtttatacccttcattgacatatgatagcgttgatggagaaggaggacgtgtcgttactttttctggtaaatcatttattgcttttgatacaaaagaagtagctaactcctctacaactgatgcaggttatggtactaaatatgaggacttagagacatcatactataataatggtgacctaatagagcctatgaaaggtagagcaccaaatgtactgtttaagcatcaaggggtacttgacgatgatggcaaaccagatttgcacgatttgctaattcatattaacccagatggtacttatagaacttctatgatgaacaaagaagaggattggcgcacactatttgaaatgacaccagatggcagagttaaattaagaaaacaagactctattaatattgatggtggcatagaaataagtgagctaggaatcaacaatgaggggttcgtttatttacgtaatggggatatggatttagaagtacgaaaagacggtatctattcacaagggaaactgtttacagccgatgtagacctatccgatgtatatgacaaactaaatgggttgtctatacagattaaggaaacaaatggtcaattagagattatagctaatggtgtagaagaacaaaatggaaaaatatcagaactttctacagaaataacaattgtagcaggtaaagttgaatcaaaagtaacaaagacagaagttcaggatatgattgacagttcttttgtagatatgtctgatgcgattaaaaaagcacaagaagatgctgacaaagcaaataaagtgattgcagatatgtctagtgataatagactgactccgagtgaaaaaatagatttattaaaagaatgggatattataaaaaatgaatatccaagctatctcgaacaagcagaaacctacgaggttgacagtaaagactacactgctaagtacaattcattagagctatttgttacccctatattggctgacatggagtcaactagctcggtagacggagcaacacttcgcaaaacgtttaattcttactatacagcaagaatagctttactaaactctattagtaaaaaactaaaagacggtatcacagaggctatgaaaaaagcatcccaagcatcactagatgcaacacaagcaatggcagatgcctcacaagctaagattgatgcagataatgctaacaaacttatatctgatatagcaagtgataacaagctaacaccttctgaaaaataccaacttaaaaaggaatgggatgtaattgttaaggaataccctacaacaattgcacaagcagagaagtacgcagtagacacagcagagtatacagctaaatataaagccctagagctgtttgtagagcctttgtttaaagacatggatgaaactagtatagtagacggagaacgccttagagcgacattctcggactattacgcaagtaagattgctttactaaaagaagtaacggactcagctaaaacagagctagatgcctatggtaataaaatatctgtaatggaaacaaacattactcaaacgtcagaagctattactttactagctactagagtacaaactgtagaagacggtgtacaatcaaataaggcacaaatcgaaatacaagctgaacaaattagtcaaaaagtaactgctagtgaggttaaaggaattgtagacgattctattaacaatctaacattaggtggaactaacttatttgttataaagacacagacagcaggtttgctaaacgagaatgatggaactgtaggtactgcagtagacaactcagtagtgtcagactacattaaagttaatcaaaaaacaccatatattgctacactttacggtaacactggcacaaacatgattataacagactggtacgataaaaatagaacatttatttctggggaagctgtggcagactctggggattttagtaaaaagtatgtgtcacctgagaatgcagtctatgctagggtaagttataagaaagcaaactctgtgaatatcaaattcgaggcaggtacaaaggctactgattacagcccttcatgggaagacataaaaggtgaccaaactgctttagaggaatacattaaaaaagtagaagaacaagccaagaaagctcaacaagatgctgaaaatgctaaaaatgatgctgaaaatgcaaataacgcaatagctgatatgtcaaatgacaatatgttagcaccgaatgagaaaaaacaaatactcttacaatgggaacagattaaaacagagtatccaataaacttagaccaagcaactaaatttggggtgtcttctcaacagtatacaacagcgtataacgcactagacgagtacttaaaaccaatactagctgacatgacaacaacttctgtagtagttggttctactttaagaaatacgtttaacaattactatgacaaaagaactactttactaaacagaatatctgacgtagcaaaaaatgtagcagacaaggcacaagaaactgcagatactatcaatgataatttacaaaatattggtgggtacaactatgtagggttctcttccggagacaatatgttgcctagactgatgattaaaaacgttggttactacacattaggttcgtcaaccacagagttcattgacagcatggtagctgtaaaaggtgatgcaacgacccaacctttcgattatactgtaggtacttctgataaagaaattgctggtggcggtttagctgattatcgtatgaaagaaataaaagaaggtcagtggctaacagcttctgcgaatgtgcaggtaataggtggtggctccgctaggttagctatctacactttagaaggggataactgggtaggttctaacagtacacctatacaagtaagtgatggtttgaaacgtgttgtggctcaaagaaaagtaacaggcttaacaaaaggtgtgttaatacgtattgagtcagccgacactaatgttaaagagtttcgatttggtaatgttcaactagaagtgggtatcatcccaactccttggaaaaagtctgatatagatattcaagaggacataaacaatgttgttcagaatatcaaaacatacactgcttgggctaacgatttacagggtcttgattttacaagagaaaaggttgaaggaaaaacttacatgtatgtaggtacctctatgaaagatagtgataactattcagattatacatggaggctaactgatgaacatatagaaggtcagattaatggtaaggaaggcgcatggatttactctccaacagcccctgctaacccatcgcaaggacttatatgggtagacttgtcaaaagtccccaaccaacctaagcgttgggtagattcagaaactgggtgggttgcattaacaccagaagaggttaaagatttgccttggggtgaagatggcacaagcttagccgactgggtgtcacaggcagagcaaagaatatcttctgatagcattataaatactgtactaggttctgaggatttcactagtgtgttcgatacaaaagctaacacttctgacctaggtaacttggctacctatgaagacttagactcaataaaagaggactataaccggctaatcaaagaaggcataaatggtattgattttactccttatgtgactaactccgaactacaacagcttaaagacagctttaacttctctgttcaacaagccggaggggttaacatgcttaaaaactctttaggattctctgggttagacttctggaatggtacagtagggaagaacttactacctaactctacttggaatttaggttttggtagatggggtggtacttcaatcactagttttgaaatattaccaccagaagatgacaagcctacgagtaacatattagcctcaatgccacttcgctcttctactaaagaaataggtaacagacctcacccattaaaagttaactcgggtgaaacgtacacagtaagcttcgactataaagaagaagcattatcttacaacaaggacagacctatccttgttgtaagaaactaccctgataagaacacagaccaatggatggagtactcaatagaaggttgggcagtaatggctaacggaagcactactgacttaactgtttggagacgttttacaaaaacatttacaataggtactagtggctacttagatattttaccgaaaaccataatagaatcgtgggaacacaggtctttttggagagagctaaaaatagagaaagggacacaagccactacttgggtacctaacaaggaagacggggcgtttactggtgatattgttgagactattcaaacagaagaattagccaacctcgggtttggttccggatttattagttctaaaagacctagctcttcattaacacaatctgtagaactacctgaaataggtgctaaccttgagtattcactatctttttatatgaaggtaactacagataaccctgtagctgactttaaatgcggtattcgggtttatgatggaggtactctaacttatacattaggcatagaagatgcaacacagccaataccactagggttccaacaatacaagcttgtgttcactcccacaagtacctctactaaaatagaaatgtttgtagaaaatgggcaagaggcatctgttattatatcaggtattatgtataatatcgggagtatacctcttaaatggcaaccatatccaagtgagatatacaatacgaatgttaagattgatattaatggggtaaccgttaaaaacaatcaaacagatgggtatacaatgattactccccaagagttttcaggatactctcgtattgatggtaacatagaacgtattttcactttaaatggacaggtaacagaagttaaaatgctaaaggctgaaaaacgtataactatggaaccagtatctgtattcgctatgaacacagtaacggatacaaaaagaattagaggttgggcatttgtgccatcatttgaataaataattcaactttttaaccgaaaacctcacttacaagttgttttcggttaatttgtgttatactatatagagaaggacacgaaaggacgatgagactatatggctttaaacggaacaaagtatacagcctttgcccgacatagattagttttagagtggcgcgcaaatcaaaacattgcagggaactactcaacaatcagcgtatggctatatctacaatctatggataaatgggggagacttgatgctcccgctattggtgatgccaaagttaccgtagaaggaactacacagacagaaaaagcttcctctatgttaaatgctttccaaaagaaactattactagctaaagagtggagagttaaccataataatgacggttctaaaagaataactattgggggtagctactttgtaaacgttacttttactgataatggtgtaccaacatattacggtacgataactatacctaacttttcagtagacctgaatagaatacctagaagaagttcattaaaccctgtccctacattaaatttaccggggaacttaccaataacaataaataggcagagctccacattcaaacataatctaactgcttgggtggctaacagagataaccccacattaagtaatgatgcccattggacgtacttgacaaatcttaataatgtagacactagtgggtcatttagttttacagtagcaaataacaaaactatttttactgcattaaacaataggactagttggcaaggcaaggttaaactatggactatagggttagatgatgtagttagtcaggagagaacatacaagattgtccccccaatgaatgcacaagcatcgggaggtaagataaccttaaatgtgggagagaaaatcaatgtatcactaagtaactatcggtctgatgcaaactttacttatgatggggtatttaacattagtgggctcaacatacccattgctacaaattcagcagggaacacaatgtcgtatacactaactcaaacagatgtagacaatatattgaagaaaataccaaatgcggattcctcgtggggtcaagtaactgtaacaagtaagtatagtggagtacaatacaggactccatggacaggacagagaatagatataactatacctaaaaacaagtatgtaccaagcattaatggtacccctacttatgaagatacaagtagtgtctctgtcgggcttacaggtgacaatcaggtagctcttcaaggtaagtctaatatcaaagtgactatccctgctaactttgcaacggctaatggttactctactttgaaaacaattgatgtgtctttaggcggtacatcaaaaacagtcaactattcaaatgcagaaacagttgtagagttaggggctcccgctaaccatacatcagacaccttaatagtcacagtaactgacagtcgtgggtttaagtctaactggacaaagcatgtagacatttacccctacgaaaacccaaatatgtactttacagtcacacgtagaaataactttgagacaactacagatattaatgttaatagtacatggtctcctatcactataggtggtgtaaacaaaaatgctgtccaatcagtaacctacgcaacaaaagtagcaggtgttggtacttatggagcagaaactgctttaaattttacagctaatggtagtatggtaacagtaaaaaatacaccaatagaattagataataccaatacatacgaagttaggttgagtgtaactgataagtttagtacgtttactagaacagctactgttaaaccgggtaaccctatcatgtttattgatgccgataatcgaagtctgtttttaggtaatgcctttgttgacaataacaataatgagctaagaggcttattagagatagaaagagataagtggcaggagaatggtttagtaggaatatccttaaacaacagtgatatatcagcagtcaatggcatatggttctcgacagatacatcaaataacggaggtgaagggctccactttattaaatcaggtaaatcaagaaattcattgacttgggatgactatgattacttttatatgagggacaatggattctatgttaacaatgactctaaccctatatttactgtgactgatggtggggatttaaggttccctaaactggataacttatgggatggggcggcttacatgcacaaagaccagataatagtaccacgtaaaaaactcagtgaatgtagaaatggttgggctttaacgttcagttcttacgataaaagtacaggtaagctgtccttatgggatataattacattctttattcacaagaccgcaccggattctcctttaagtggtacaggtcacaggttcttcttaccagatggtagggatgctacatctcaaaagacaaaatatatatacgtcaatgactatcagttaaggggtcacgaagaaaatgatgacaaaggcggaacagctagcacaaataacagaaataaggttcttatgagggtggatgaatggtaaatatgagaacaatatacgtagaagtaaatgatgaaggttatgtagaaggttggggcagtaacctgtcaggtaataataacattcatagtgtaacaatagaggataacgaccagtttttttataaaaactccttaaattttaagtattcaaatggctctctagtattcgatgaagataaggcactgcacagtgctaaactagccaaaaaagatgaaatgttaactgcatgtaactatgaaaaaaatctacctttgacttttaaactagacaacgaaaattactttgctcaaccgttaactgcggaagaacttaatgaaacaatattgcctctgttgtcaggtttaacagagactgttcctcttgaattagttaaagtaagtgacgatgtacaagtaacattacaagttggatacagtgtaattaaaaatttatatgattatacaaatctaataaatgaatacttaaataaaaagttagaagtagatgtgtttaagatgatagatgaggctactacttttgaagaagttgaggaagtatcatggaaaactacaactagtgatgagttacctaatcaacctaaaatagaagacctccctataaataacaaccaagaaatcgtagataagttaaaacaagagaataaagagctaaaacaaagagtagaatttaacgaactagctttaatggatgcaataaacatgttttctgaaatgaacaagtaagttattattaactaaaggaggtgatatttctatgtacccatacttatcaatgttatatgcatcttatgtaatcaaagaccctgagaactatcctttagagaaggttccggcactaattagagaagatgtggagaaaatcgtggaagagatggcaaaaaagaacgaaaaacaaggatagttaatttagtaattggagtaacaataggtttaatcatagggctactaatttaaactaatataaatgagggtagtttgtgctaccctcttttttatactatattgtactatattaaggaacgaaaggagcggttactatgggacaatcagatggtatgggcggtacattaaaacgtattgcgattcaagtaggtaacgacccgaataaaggttggtatcgatttcaagtaaacccaactcaatataaatataataagccacatcgtgttactatatttaaaactaaatcaaacattataacagaagactttggtaaagatatagaaactatccaattttctggtacaacaggattcagggtagatagcagaggtaaaaatggggcggacagactaaaagaattagaagaaataatagataattacgcaaaacagggcggtaatggtaataggtctagtgtagagatgaaattttataatttcacagacgataaatattttgttgttcatttagcaccagaagggctatccattgaacgttctgcagaacagccattattatttaattacaccttaagtttagtcgtgttaagagaggcaggacagccctctgagagagctcaagtaagccctcagataggtaatgtaagtcctagcattggacggacatacaatgcacaacaggacactagaacacctgctcaaatacttcatgatgaatataggagaagtgttatgctaaatacagcagtaaatcctgcagtaacatcgggagcctataactatggtgtaaatgagttaaaaaaaataatcggatatggagggtagctcatggaaaaagtagaacaatcagcagatttgctaagattttttagatatttaaatgtcgatattaacggtgaagttgtagccaatgttattgacgaccaaccaaactttatatcaaggttctacacccctcatacacgagttaataaaatatctagtacactattagatattgttcgagataatgatataggggaaacaaataaggctttgtctaaagactccttaacttataaatttttaaaaagtggacttaagctttcatctccacgtatttacgagctagcacaaattgtagtactagaatcttttgctcttatatatgctatcgaagaagaaccagagatgtttaaaatgattaacgaatcagatgtaaagcagactagagagaatgttaaatacttaattgattgtttaggaggagcaaaagattatacagacatagtgatggacttacaatctatggatgtcgctctaggatatattcaggagcaagttcctctaatacaaggaggtttaccagtaaatggcacgatataaaaaacatttaattgtatatggggatacaatgcaatccatagcacaaaaagaaacaggctctgtagataattgggtaaaaattgcggagtacaatgacttagtttacccttacatagtagatactatgcaagaaaaaatgagcaacttagaacatctagctacacttggggacaccctttttatacctgatgaaggtaacttattggacattaatacaagctcattaaaccaaagagatatggatttcttattaggcttagctttaggtaaagacttggatatgacaagtgatacagattactacgagaatcatggaacaagtgatgaagtgtttgcaataacacataatgggcatggggacttgaagatagctagtggggcagacaatattaagcaagccactatatcaagattgatgacagctaaggggtctcttatgttgcacccagagtatggtagtgacttgcacttaatgttcggtaaaacaacaattgaacaaatgaagataattagtatagaagtatgcgatacagtacttaaagatacacgagtagcagaatgcgttctagtgaaccattatattgaagaagaccgatatgttggtaactatagagcaaccttaaagtctactagagagcaatttgagtttgttgttcaaaacgataactcaggggctctaattattgtatagaaaggataaggtttaatgagactaaagaaaatttcagagatactaggtagactaattgatgtaactatgataaacacacatgagataaacgatttttcagttggttctactattcgttctatttatgaagctgtttctatggagttagaacagtactatattttaggtagagagaatattttatggggaattgaacaaggagtcctaaatgcttttgactttaggaaaagagaagcaaaaagagcgtatggtatggtaacactagagttccatacggttactcagacccctgtgtatgtgccaacaggaacaacattcgactctagcttgtctggtgcccctagcacgttaacattccaaacgatgcaagactacataattccagaaggtgttataacagcaaaggtagaagtttattgtacaactgtaggtacaaaagggaacatacctaaaggaagaatcaatcgggtaattaacaatatatcaaacttaaaaaccgtgtataatgagtttgattttttaacaggtactgatgaggaaagtatagaatccgttaaaaaaagatttcatgcatttgtggaatcacgtggtagagcaacgataaaagccttagattacggtacacgtcaagtagaggaagttgcaggagtttatatcaaagaagaagtaggctacgttagaatatatgcacatgacttaaacggtgatttaaaacaagaaacactagataaaataaaagtagctattgaggactacagacctgcaggcattaaactggatgtattccctgtaataaaatccaatgtacaagtgagtgcaactgttactataagtgacaaatcgagaataaatagtaaattagaagaaagagtggagcttacaataagaaactacttaaatagtcaagttgtttcacaaccattaatcttagctgacctaattcaggttataatgaatattgacgatgttttaatctatgactgtaaaattaacaacatggaagggaacatggctgttagggacgaagagataattcgtgcaggagaggttattgtagaactgatataaattaggaggaatataatgtgagtaacttttataaaaatatccaccctctgttgagacgtggtaagaaacctaacaagtatgatgatactaactttgcagtgcttaatgcgttgaactatgaattaactcaggcagagcaggagaccattgctagtaagattcattcttcattagaaacagctacaggtgagtacctagatacttggggggactggtttggtgtatatcgtaaagatgattggaatgacgaatattatagaaaaagaattataagagaacttttactaaaaagagccacaattcctgctatcattgatgcgttattggatttccttaacgacaatgatgcagtcatccaaatatatgaaccttggagaaacattttctatacaaataagtcaaaattaaacggtgacgaccatttaatgggttactactaccgttttgcaattatcgatatttcaattgatagaccgtttcctcctgaaattgtagagattattaaggctttcaaacctgcgggagttctattttatctaaggctagacacaagcttaaataagaataaaacaactgtagaaagcccatatgtatacctagacgtgacgaataagacagaattagagttccttaacggtttatactatgacctacgaggtaacattaacctgtctgaccaacgtacacaagtagtagagagtaatatcttccatacgaataactctatgctaaacggggaagatgtgcttgcaggagcatttgaccacggaagaggctacattcacttagcaagtacaacattgcttgattacacaccaaaacctactgactctatgagtgacttaaaaacagctctaggagaatcaggtgctgatatgtataatcaaacaaaagaaaaggacggaagaacagcttctattcaagtacctgcaacaaagaatgttcacaccttgtactcaaacagcattgactttggtggctatgattattcggggaatccgaatgttatgactaagccttatattgctgacaatataaccggcggtacaacaggagtagttgtaacaccaattgatgatggcgcaagactagaaaaaacacgagttgatatatctggaacgtttaacttagcattgggtaatcttttgaataatacagattatataatttcatatgatgtacttgtggaaaatggatatgtaggagatttaaaaacttgtaatgttgcattagaaggacagtttgaaggaaagcctaactattttggtattttttatatgaatagtgtaacatcaacagatgtatggcaaaaggtttctgtaaaattcaatagtggtgccaacatggaaaaattaagtggttttaagtttagagtatatttatctcaacgtgttcaagcagcattaaaaataaaaaatgtgaaaattgaacgtggttcaacagccaccccataccagccaaatttactcgatgcaccatattatctgggtaaggtggctttgggtgagaatattgctaataagtccgttgagtttccaataaaatctagcaattatctcttatataacgctagaatggtagagccttttgttgtaggagaaccttatacaattaccataaaagcaataaaaccagccagtcaaacgtttatggtatataacattggggaaggaactacttattacggaaaactaaatccagttgagggattgacagacgtatggtcactaacattcacaccaagaaatgtttcgtcaactaatcctagcgatttacgtatttttcagtacccatcatcaacattaggcacatgtcaaattgattggttaaaaattgaaaaaggtgacaccagaactcctaacattgattcctacgactacgtaggttctctgatagaagatacagaaacacctacgttagacccgactaagtatacatggacagtaaatggggatataacaaataaaaaggcatatatggtgtttgatattaagacatttatcgaagaaaattatgctatagaatttgaaaaacttattactgacctaggagaagaccaagcattaaataccgtgtttgaaaactttaacatctctacaacacttaaggctctagtaagtccaagttcaccaatcagtttctcggttgaactatacgatttttctacgagtgcatggcacaagttaaacacggatagcttagacttacgtatgcgtacattcaacttagtagcaaaccgtatcacagactatctaaatgattacaagctattatttgttcgttacgtgtttgataacgaaacagataaagatgtaacagttgaactagacatgctaaatgtactattcaagtatcgtttaggtgaggggtacagtataggactacaatcatctgtggaatcactaacggaactcgttcctatagaagggtaatagcaaataatatgttataatataaatagggcacctagttgtgtcctattttttaataaacatgctatattaacaattgaatgataaagaaaagaggtaaataatgtggctattgcaactaacaattcacgagtgtatgcctcactccaattaaaaaataaacaagacagtatgtacctagcaattggtaaaaccactccttggactaatgaagatgccccccctgcaccagaccctactacggctactctaacagaggttatcggttataaaaaggtagcaagagtatctttatgtagagaatatctaccaagtgacgattctaaataccctgtggtgtcctatggttcaagaaaatttacgctaattccagatgaggacggctataaagagcaagcgtggatggtgtatgtagaagcagaaattacaggagatgaactaccaataggaacatttaggcaagtaggtattcatactgacttagtgtctaaggcaagttcagaaaagaaagctttgttacctacagatgtaacagatgcaggtattttgcaattttttgaaaatagacagcaacaaaatagaacaagtgatgtaattttaaaagagaagtttattattacaatggaaaataagaagtcagttaaacaataggaagggtgacatagatggctaaaaatattacaaatgatgatttaggtaaagagccttataacaatagatattaccaaggcaaacgattttcaggtttactatttaaaccagataagccgttacaacaagccgagttaaacgagttacagtcaattattcaaggagatttaggcaatgtggctgaatccatatttagtgacggtgacatccagactggtatggaatatgtactacaagataagaagcttactattaaaaaaggtaaagtattcttaggcggtaaaatgcgtaactttgacgaacagagtatcgatattaccggagagggtacggagtatgtaggtgttaaacttgtacaaaaagttattacagcagaagacgacccatcactgttagaccaaacaagtggtgttcctagccatttctcagaaggggctgaccgattagacgaagatgtagtactagcagttaatgatgattctgcatcaaacatttaccactttgttaacggtgagttatacattaacccagatactcctgagatggataagattaataaaatactagcagaaagaacttatgatgaatctggttcatatcgtgttcgtggttttgatatgtacacagaagttcacccaacagaccctaacaataaaattcagttagttgtcgattcaggtcgggcatatgttttaggttttaaagtagataaacctacaactactcgtattgatattgaaaaatcaagagagttagaaacaatcaataacgaaggtttctactatagcaatgcaactcgtaaaaataaattaggtaattccccagtatcttctgtagaccgtgtaactgcacaagttgaagttgctaaagaacaggtttctcgtggggtcgtaggtggaggtaccgattaccttaaaaacacctctgtaacaaaagttattcgtgtatggactgagggttcaggagcacaggagtacaaacaaggtgaagacttccaattagtaaacggtcaagcaatatcttgggcacctacagggcaagaacctcctgcagggggaacctacttcgttcaatatgtttataataaaacaatgattgaaaatacagattacaaagttgtaattactggtgaaggtgatgctagggaatggtatatcgactttaacgagatgacaggttctaaaccagtcgatgaatcacttgttaacgtagactataaatacttcttagctcgtaaagacctaattgtattagaccataacgggaatttcactgtccataaaggacaacctaacgctttaagactagtagaggcacctaaccatgtagacccattagttttagctattggtacagtagtagtttacccagactcaaatactgctgatgctaaacaatggacaatcacacgtctaacaatggaagagctacagaagttatctgttcgtgtggaaaacatggagtataaccaagcagtgttctacttagaccaaccggcaatggcaggagaaaaccctatctatctacgtggagtattctcggatgcgtttatctcactagataaatatgacgttagtcacccagatgccacaattgcttttgactttgacacagcagaaataacattaccttatgcagaaattaataaaacagttccaacaattatcgaaggttctagtgaagcacatgtgtggggcagactagtaacagcaccgtttaccgaagaagtgggtattagacaaccatttgctacggaagcaatgaacgttaacccatacaacacctttaacaaacagggtgccttaaagctaaacccttctgcagataactggattgaagatgagcgtatcacagttaccaaagaagaaacatctactatgactgttcgtcaatggtggagacatggtggagcatcttggacaaacgatgagatgaacatggtatctaacatcacgcttgaccccggacaatcgtggggaggtgcctctggtacagaagaccaacgtaaacaagggctatccggttctactttaaccagtggtggtcagcaaaccaaagaatcaatgattgagtttatgagacaaattgatgttgaggtttacgcagagaacttgcaacctaatgctaacaacttatacgtaacattcgatggcttgagagtacctgttaccccatcttctggttaccgtaaaggtgccacagaaggcactggtatggcaaatgcagacggaacatttaaaggggtatttaaaatacctgcaggagttcgttgtggtactcgtgaagtatctgttagaaacgatacaaacttagcaagtactacgttcactgcgcaaggtacgctaaaaacaactgaggatattatcataaaaacccatgttactattaacttggttgaccctctggcacaatcattcagttttaacactaacagagttgcaacaagttttgacgtattctttgcatctaaggataacagtacaaatattatttgtcaagtacgtggaatatcagaaggtgggcaacctaataaaactgtgtatgctgaaagagtgttaaaaccttctgaaatcaaagtatcagatgatgcaagtgttcctacgaaaatcagctttgatgacccactaatgtgtaaagcaggtcaagaatactgtttagtattcattactgactctgataaatacacaatgtggattgcaactatgggtcaaaatagagtagacgaaccaacacaaacagtaacatcaaatccttacttggaaggtgtcctatatagttcatctaacgcaagtgcatggtctattcaccaactgtctgatttgaagttcactgtatacacggctaaatttaacgaagaagctgtacttgagttcgatgttatgaagaacgttaatgtagaccgcatagtgttaatgtctacctacctaacacctgcaaacactggttgtagatgggatatgaaactagtccttgataatgagcctgcaggtacaacagtagatgacaaaccttggttacctattgctaactacgtagacttagatgttaaccagttagctcgtgaggctaagcttagagcaacatttaaagctaaccaatacatctcaccaatgctatccttggacgacattatgttcgcaggatttttaacagcattgaaaggtagctatgtatctcgtacaatagatttaacagaggctccatacaacacggttaaaatgtcatatgaacaatttacacctgccggaactgttgtgactgctaaatatagtacagatgaaggtaaaacatggaagacatttacagtacagcctacaacaacacaacgtacacaagactttgttcgtgtagactatgttgaaaagattaatacgggtgggacatttaagtccattaaattccgtcttgatatgacgacccagaattcatttttgcgcccgcgcgtaagacgcttactcactaatatgaccgacaaatagaagatgtaactgtaatgtaacatttctatgcctcctactgtggtatacttactgtatacaaaatagtaggaggttttttaatgggtaaagcattacaattagcaggtactacatttggtaaatggtacgtaaaagagcgagatacttctaagaaaggtagagcatactggatttgtgagtgctcttgtggaagaacagttcaatctattccgagcggtactcttactacaggctcatctgtgatgtgtaaacaatgtgcaaatgagaaatctttagtgggtaagacttttggtaggttgaccgtcattaaggattcaggtgaacgagcaactaatggtagtatcctttgggagtgtaaatgttcctgtgggaaaacaagccttgtcaggggttcagagttgacagggggtcgcacaaagagttgtggttgttactccacggatgtactcaaaaaagtagccactaagcatggattgtctaaagtgaacggaaaacccacaaaattattccgggcatgggcttcgatgaaacaacggtgttacaacaagaaccatgcgagttataaagattacggtggaagaggtataaccatatgttctgaatggcgtgaagactttgaaactttccatgattggtctatagctaacggattttccgatgacttgtctattgatagaattgacaatgacaaaggctattcaccagacaattgtcgatgggtagatgctaaaacccagattcgaaatagacgaaataccattacttacaactggaagggttcagagtacaccttagctgaactgggagaactaacaggtataaacaagatgactataaaatctaggctgaactccggagccactcttgaagaagcactagacccaaaagtgaatacgtcagttttgactatgagttacaagggagaaactaagcctgtcaaacaatggtgtaaagaactgggattgaattacgcaactgtacgtagcagacactataaaggttggactgatgaagaagccttaactggtatacgtaacaaatagcaacagaataagtataatagactctatatgttataatagacatatagagtctattttttttgttaggaggaataaaattgccagaaacacacagacaaacaagctcaggtgcgcttatatttaaaccaactatagctgaacaagagcataaaaatgctatggaatctataaaacaagagagaacagagctagagaaagaactagctaatgttaaagctatcaaagatgagttgtcaaaagagctagcagatattaaacaactgaaagatgaattatcaaaatagtttctaaattgtcttatttaggatttctggttcccttatactattaactaatatatttaaataactatatataaaatatataatatataaataatatataataagactacgaaaaatataaaataggacaaatcaactctgtatacaccttgacaattacctactatgtgatataatgaatatattgattatactaaggtgggtatgtcaaggagcatgtatactaatctaacttaaaggagatttattaataaatgagactagtagtagatattatgcatactcagataaggtatgaagattcggaaaattatcttagaccagaaattcataaggtaatgcattcagaattaggagttaaagcagatggttatcaatttagtcctgcatataaagcaggttactgggatggtattattgattttttcgataaagaaaatgacacgttccccacagggttactacctcatgtagaaacaatactagggaaccttcaatcaactttatcaaagtcaggttacatttttcagtttgagataattgatgatagacctgatgagttcatgtcagtagatgacatggataaggagatagtgcttaatggggataacaatgacaagataacattaagagactatcaatatgaatctgtggagcaagttattaagaacagaataggtattgtaaacgttagtactggtgggggtaaatgcgtagtagcatctacgaacctactgacttacgataaagggtacaaaacatttgaacaactgttcaaggaacacaacattgatttaacacaatcagaggcaactatccctaacacatttggggttacattagtgaatgaaaagggagaaccagaaacgcctagtcatttaactattaatggagttagacatgtaaacaaggtaacaactgagcatggatggactgaaacaattactgacaaccatccattactaactgtatcagaatctggtagctttaaatgggtagaagctaaagacttgaatgtaggtgattggattgttggacgtaaaggtgataatttatttggaacgaatactacatgtaccgtggagagcgcatatagcttaggtttattaacagcagacggctattgtgggcaaccaacccagattacattaaccaataaccaaccggagatactagcggacattcaagatttctttactaaagaagggctgtccactaaggtagaccctaacaaagactctaaagatagtaagatagttaggggtaccgcaggagctagagaactttataataaatatggcttatcacaaggattagccaaggataagtcaatcccagagtgtatcatggaagcaccgaaggaagtacagttagcttatataagtgggtatttagagtgtgaactgagtatggaggtacctaaatgttcaatagaggtaatttctgcctccgagaagttacttcaccaattacaactcttattaggaaacatgggagtttcctcaagattagctaagaaggtagttaaagggtacgaggctaattggtatggtagattaactatcggagtgactgactcagtttacctactaaaacaattaacatttaaaacagcacaacggaacgaaagaagagccttatttattgaaacagcagagtcccgtaatagtaaccaccaaggacaacctgtaccttttggtaaggagttagttaaacgatactgcgataactacctaggggacactaaaggacttagtaaggcattcaaagtaccaagaacaattagcttacatcggcttaaaaatttaattcatgagttccctaatggaaacccgacagattttgctaacctgacaagattaactgatggtagatatgtctattcacaagtaacaagtattgaagatatgggatatgaaccaacttatgatttacacatgcccgaaacacatagttttattgcaaatggtatgataaaccataacactgaaatagcatcaggacttatacagcaaataaccccttacttagagtcaggagaacgtattgcattttttacgaatagttcttctattttttcacagtcaattgaccgtattgagaaaagacttggaataaaagtaggtgcttttggtgcaggtaagaaggacattcagcaagttacttttgtaatgatacctacgattgtatctgcaatatctgcagacccagaggctaagcttaagctgactgctaaagaaagaatgtacaagaaaattgctaaggatatagctccaaaatttgaaagagggtttaaccaaaggagtttgcttgaaggatacctaaataactttcaagttaagacaaaagcagacctgcagttgaaacatgaactagaagaaattttttattcatgtggtacgaacaaacaggttattatgaaaatgaaagggtatcaagcagaataccaaaagattgttgaaaagaaaaatggtaaagttcttaagaagtacaacgaggctatggagtttttagattccatatctgtaatgattgtggatgaggctcaccatacaagttcagatacttggtataaagtgctaacatcttgtaataacgctcagtatagaatggcacttactggttcgattgaccgtacaaatcatgtgctttggcaaagacttcaagctatattcggggagattacgactaaggtgtctaacaacacacttattgagttaggtcactcagccaaacctaaaataacaatattccctattatagctcctgtagatattcaaaccactacgtatatggatgcctatcaaaaaggtatagtagacaatgaatatagaaattctcttattgcaaagttgactaagaagatgtatgataaaggtaatgggattttaattataattaatcgtatagagcacggagaggctattagtaacttactaaaagaagagggagtagctcactactttatcaatggacaacttgaaaatgatttaagggatgaaaaaattcaggacatgcgtgatggagcacttaaagtaatgatttcttctacgattatagatgaaggtgtcgacatttcagggattgacacattaattcttggtgcaggaggtaagtccttaaggcagacactacaacgtgttggtcggggcttacgtaagaaaaaaacaggagaaaacaaagtagaagtattcgatttttatgatttaacaaacaaacatttgaaaaaacattcagagcagagaagaaaaatatatgaagatgagcaatttgaaattgttgatattcctattcctaaataactataataaagaaagggtggcatacaattgcaaagtccatgcctaaatattgaattaaaagaaaaatttaaattaaacaaaggtataacagactttttagagagagttgcagataaatctcagagatggggtgaaacagtagcctcccctatccgtaaaacggatatggcaaaagagactggaaaaaaccctagaacaattacaagatatattaatcaattagaggaactaggtttaataaaaaccgaaacaaaaagaggaatgaatggagggactttagtcgtgtttaacacagatatgcttaattttgagccaaaggaaaaccctatcacgtctgatactaaacaagcaaaggagattagagaacaagttttccctaaagccccaaccaaagtaccaaaacgcagatacagaacaaaagcggagatagctgaggcacgtatacttagtgaaaaacttaaaaaacgtgaagacattttaaatgataaaattgagtttaacgttgttactagaagttttttcgatagttttgacgaaccagaagcgtactttaaaggctatttaatttcaagaatgtataatgcttatgtgacaatcattccttatgaaaaatataatagactgaaaaatttagatgagaaaaaggctaaacaacaactacgagcatacgaaagctcttacaattacgatgtgttgcctagaagatttgttgggacacctcagtacaaaaaatttgtagagctagctaaatattgtgaagagaacaatatcaatcctttagtttatttaacagtgcaatttgatagaacagagtttttgatttctgtaggtaaagcacgagtaggggctacaccctatgtaaatactttgttatgtgcagaggctaaagaggcttacacaaatagaaaactgttctacagaatgttacagaaccaatatggattgtatacgtctatcaattcagaagctacttattatggtgcaacttatccaattatttcaggactattgaatgcttacaatatgccacagaaagacttgtcacagttagatactgtgatttgtgacttagaatataaaaaagatattgacaaaaaagcaggtacgttgtactcttattatacagcaacacttaaatcgttaggtgaatctgacgtatctagtgaagctaaagaaagtattgctaacttcttgaaagaacaagttgcaaacttttctagtaaacgtgggctaacttcaacacagtatgccttagcgttccctattcagataaactctgcacgcagtttattaatgaatgaggaagacgaagaactactttatttattgttaggtaaccagtcacgattatctaatgtaacaaatgatgaagctgaaatgtttattaaacaaggtagaaaattaagtatgtcttggtggggctcacagaacttctcaagaacaatgttcatgttagcggactactatgggtttaaaacaaatatatctaagttaggtatgtacattaaagaatttggtgaggagaaaattcctttagattctgtaggtatgttagatgtaaatagaatctatgatgtcttaatgactgaacaagagattttagagattgacaaaagtaactgggagaaccaaaaagatatgcgtgacgacaaataagaaatataaatgggagagggacggatagtaagatgagtcaaattcaaaaacaagttatttatagagcattaagtgagccattctttgcaaaggaaatcctaagtaaaattccaatggatgagtttaaagattctggatatgagatgattgtttctacaatcaacttatattacagaacacatgatgagagcttagaggaacagagtttattaacactagtagaagataagatgttaaaacaaaacaaaagtttggaagctcaaaacaaagtctttgaggtagttagcgacttatacgaactagagaacgaagatgtagactcagaagttatcagtgagaacattcagaactacgttcgtaaggtactaacacgagaagcaatcatgaaatctgtaacaaatgaaggcacactaggctctgatagtaatattcaacagctaatggatgacttgagagacattcttactatcgagacagcaggcaataattcagaattgctagacttcttcgatgacgtagataaaaagatggagttacttgcaaacttgcaacaaaacaaatacccaactggtttcacagctatcgatgctatttccgatggtgggctagctcgtggagaagtcgggatggttgttgcacctactggtggtggtaaaactacttgggcagttaaccaagctagaaactatgttgtacgtggtttaaatgttctttatgttcctttagaggaaaaagtagaccgtatgattgttcgttttgaacaattattatcacaacaaagtaagaagaacatcttagttgatggtgaattgaataaagacttgtatacccaaatccaacaagcgtatggagcgggtaaagaacagatgaattggggtaacctttggattcgtaaatataaaccacaagagctaacacctagcggtttatctcagttaatctccgatgtaatgattcgtaaaggacagcaaattgatgttgtcattattgactacccagatttaatgaaaaatcctcatgcaagtggaagtaatggtgaatcagatgcaggaggtaaactgtatgaagatattcgtgcgattgcacaagaatatgattttgtttgttggacgttatctcagttgaaccgagcaagctatggtcaagatattaaaaatgcaggagctatcgaaggctctaaacgtaaaatgaacgcagtagagcttatttttacattaaaccaaacatcagaggagtttagtaacggatatttgagagcttacgtagataagttacgtaataatagtgggattgcctatgataaaatgttgtattttaaagtactcccagaaactatgactattagagatgaaacaccagaagaacgagcagaacatgaagcactgttagcagataatgcgatgaatagagcaagtagccactctgatgagaataactacacagcaaacgatgttaataaaaagataagtaatttgaataataccctttcaggaggttggaattaatgaaacatattattaatttttcagattttcatatgcacttttttaaagatttttcaaaaccagacccagagtatggaactgatagggcaaaagagcaaattactatattagacaacttgatgaactatgcacgaaacaaaaatggggatgttttatttaatggagacatgttccataaacgagtatctattgatgttagaatattcaatatgttatttcaagtaattagtagctaccctgatgttgatgttatcatggtcagtggtaatcatgataaggtaactaactctctatattcagatagtgctttagcaccatttagtgctttaccaaatgttacagtttgttctacgttaaacaagattgttaaagatgattatacgttgtatgctgttagttatggggaagaggtcgaagagatgaaagcttggataaaagaacaagctgacaatttagaccatgaaacagttaatattctaagtgcacacattggtgtagatggttcatctactgggaagtactcccatacacttggtggtgcttttaaagtagctgatttataccctgacaagtttgacatagttacattgggtcactatcataaacgacaatttttaggaaacctatctaatgtgttttatgtgggcaataccttacagacttcttttgcggatgaaggtcaagaaaaaggtttttatgatattactatagagggtaagaagtgggaacaaaaatttattaaaactgactatactccgtttgaaacagtaacagctgataacccatcaacaacaggttctatggagaaatcttatatccagtttatcggtaatgtggatgaggttgaggctgtaaagagaataaaagaagagaataacttaagcaatattagaataaaagttcagaaggactaccatgttgagccacgtataaacataacagcaggttcgacacctaatgaagttgtcaatgcatttattagtaaaaagtaccctaacgcaaaaataattaaagaaaaagctctcgactgtttgagagaagcaatggaagtataataattgtttagcctagatatatctaggcttttttgcgttgtactattgactttattagtattttgaagtataatatgtttattgaaataattaatattttgggaggaaaagatgttaaagtttaaacgagttagcgcagagaactatatgtccattggctctgtatctattgatttagacaaccaaggactcgtacttatcgaaggtataaatgatacaaacgaaacatttcagagtaatggctcaggtaaaagtactttactgtctaccgttacttatgcattgtatggagctacccctagtggtttgaaagctgatgctgtaattaataaacaagcaaagaaaaatatgtcagtgattttagaatttgaaaaagatggggtaccatatcgtatcgaacgttatcgtaaacactctaaacataaaaatactactagatttttccaaggaacaaatgatataactcagaaatctgtagcagacactgataaaaagattcaagatgtgttcggtattgattacctgacttatgctaatagtatcatgtatggtcaaggtaacgtagaaatatttgctacagcaactgataagggtaagaaacaaatcttagagaatttagccgatattggtgtttaccgatatgcacaggatgttgctaaagaaagagcacaaaaagcactagctcttgcagaagagctgaacagacagtacattgctaagacatatgaaaaagatgggttaactcaatcttacaatagtgctttacaacaatatgagaatacagaaaagctgattcaacaaaaagagagtgagttagctaatgcagaattagctattaaacaaagtgagaagaatctgtcagagggaagagcgctacgtgaacccgaattagaaaagctaagagagcagatggcacaactaacttcccctgcagacgttcgtgaaattgatgtagaagttgaaacacagtattctaacgttagtagattatctagtgcaaaaacacagaatgatactgctattgagaaattaaaaaaagaactagaagatgttaaaacaaatacaaattgctacctatgtggtgctttattgagcccacagcatagagaacaagaaattcaacgcattcaaagagaaatagcggataaagaagcgtttatcgaaaagcttaatagtgcattagcagtgtattctcctctgttagagcaagcaagagctaaacaagaggaagcaagaaaagctattcaagaacatactaatatttatcataaacttaatggtgaaatgaatgcgttgtatcatgagatagatacattagagaacacattgaacacatctattaataatagggacagcattaaggatatgttagcaagactacaagaaatacctaaacctcaatatgactatgacaaagaccgggaaatagaagatgagctaaataaaattaaccaattaaaattagatgccgaagaagaagctagtcaatataaaactattgcacaagaaattttctctaataaaggcatacgctctgaggtacttgacctagttacacctttcttaaatgaaagagcaaaccattacttatctaccctttcaggttcagatattgaaataaactttagtacccaaacagagaaagcagatggtagtttagctgataagtttgacttagaggtagtgaatggctccggtggaaacacatatcaagcaaactccgagggagagaagaagagaattgatttagcaatatcttttgctattcaagatttagttcagtcaaaagcaaacattgctgttaatttaggtttgtatgatgagtgttttgatggtttagatgcaattggttgtgagaacgttattaaaatattgaaagaacgccaaaagaacattagtagtattttcgtaataactcactcggagaacttgaagccattgtttgagaacgtaatcactatgaaaaaagttcaaggtcgttcttaccttgaagaaagtaaataggtgattacatgaagatttatacattaagtagagagttaaacgaaggtactatatttgtacctacaagtagtagtaatgaagggagactatttagcttcccgctagagacactattcgattggtacccttgttgcccaagatatgagtatcagtacagcacttctcgaaaaaaactatatttgagattgttagactcagacaaaacattagtagctagatacggtgttggggataataaaaagagagttatttcaaaaatagcttgctttaatgagaatgaatggtataatgaagaagtggcaaatgagaatgcagagttgtttaactttgctaaacaatatgacattgttacacctttaaaagaagattacaccttaaaagaagtagataatagtatctctaaagtactggacattcttgatttactttacacaaatcaaaaagttaaagtagaagaagagcttataaataaagtggatactctacaattgagtaaaccagactcggatgaacttaaacaagcgtataaggatatatctgagtatatgaggttagacagagaggaaaaagctacttatgtattaagcaggtcactagactctttaaatagtgtttatgaaaaatttggtaatgtgtatacaatgttaaatattatgaggaaagtagtggcttaaatgtttacagacttgttatctaacgaattaggttcacctaaatatgcagtaagggactacaggtataattgccctttttgcgactacgatactaagtataagttttatgttagggtagaagaaggacacccaaagaataacttatggcattgttttaagtgtggtagttcaggtaacccagtatcttttgtaatgaagtattacaacgtgtcttttaaagaagcgctagagatattagaagaatacggctataggtttaataataaaaattatgtgcctaaatcagataagttaactgatgaggaatacttattacttcttctaggttcgttaggtaagccaaaagaagaaactaaacaagctaaaaaagagttagtagcacccccattgccagatggttttaaactactaagtcagaacctgagagagccagaagcgtaccctttcttattatactgtaataagagggggtttacattgaatgatatttatatgcacaatattggatatgtaaaagattcttgggtacccttagaaaatggtaagtcagttagactcaaagaccacttagtttttttaactcatggaaaagatggtaagtatcaatattggaatactagggctattggggaaagctttattaagtctttgaacgccccaagtaaagagggtgagcattcaaaaaaggatactatatttaatattaatagagctagtcaaacccctcagatagttataacagaaggtgttccagatgcattaacagttggtgagtctggtgtaggtacttttggtaaacaagtgactgacgagcaagttgaacttattttagatagtgtgaatgaagagcaaaaaatatttatctatttagataaagatgctaaaaaagaaattaagaagttagcagagaaactatataagagacataacgagacttatgtagttataagcccaacaactcaagatgcaaatagtctagggagagaagaggcttggaatattataaataactactctgtaaaagcagatggagtagggttaataaaattaatgttatagataggagagggaaaaaaatgaagtatacactagaagatttacatgcaggtatgaaattacgttgcacggacaataaaaactacagtttttggactacgaataaaatctatgaagtaactaaaaaagagtcaggttcactatgtatttttgatgattatggaattgagagcctagatgaggacatcttagtacgtttaaatggtaatacagggaacgcagaatttgaggttgtttctaaggtgatgaaggatgcagattacacagaagaagaccttgaagaagggatgttacttcactgcaaagatgatatgagctttccatggtgggctacaggacaaacctatgaaatctataagggtgaaaaaggaattttatttaccaagtcaggagacggtaaccaatactgtgctaaagaaatagtagctcgattaaatggtagtgcaagcgggtcttttgaattactagaaagaccacataaaacagagttagaaaagaaagtagaagcaagaattaaggaactaaaaggaaagaaactttgtttattctacaagcaacaacaaattaagatagaagaaaacgaaatatctatagaaatcagtaagctaagtgaagcattaaaagcgattgacgtattaagagaatttgaataagaataactataggaggacaacaaacaagatggaaagagtatcagtatactttctaaatagcagaaatattatggatgaggatgagacaaagcgtacttatcatggaacatttaattcaatgaaagaagcagagcagtcagttcgtgactggtggaaagcaaatgactttaagtgtggtacccttagaattattgaaggtactgaggatgggattgttcgttgggactacggaaaccatactgggttctatctatttgtaccagaaggtgctgtagtaaaatacacaatccgtgaaggcgctaagaaaccaaaacgaggaagagaaaatgatgtagcacatgacttgttcacagcagacgatggagtagttattcccgggagattaggttcaaatgttatttctactggaataaaaacatcgtttgaccccaaacaatatggtttattcattaaccctcgaggtggtatgatgaaatacccaatcactttaggaaacacacaaggtgtagtggaaggggaatatcgtggagaggttggtttaccacttaaaaatacgttctctttacaattagatgcaagagctgtttctaagaacgttttaacaatcaatgaagaaggtaaacttattaacatcccagtaacagtagctcggtcaatgtatccaagctttaatgctctttatgaaaaacagctagagaagctaagtgaggagctacagctagtctatggaggagaagttagaatatctaatgctgatgagtatgtggttgcgggaacactatttatcccaaaaggcactcgtttatgtcaagctttcttactaccacgatacgacacacagtttgttgaagtatcagcgttaggtacaactgaacgaggagaaggcgcatatggctcatctggggtggtatagctatgctcatcccagaatttaagccaccattattgtacgttatgggtagcttttctgttatgttagaaaaacaccagtgcagtgtaacttttgatttaagagagccttatttaggtacctcttacgataaaatagtgaagcttattaaaatgacttacccaaactatagcttaacttatgtagggatgacagataataaatataagttcacattaaagaataaggaggactagcatgtacaccaagaaagaggaagtagtgacagttaaacacctagttgataaagagcaaattagagtaggggacatagtaggttacaaaaagactattagagggttcgatgcaaaaagagtaaaagacacactctcagtaacaaatcaaataggtgtagtttctcgtgtatgtgacgagtacattactgttcatgacttttttgataagtgctcacgagaaatatgggcaaagacatttgaaaatttagaagttcgcaaaatagaggatggtaacagcctactacggaggtatgaaaatgaatttcgttgattattttaatcagatgcagaatttagtgattgaagaaaaaacagatgagtatgttttactagagaaagaacatggtcaaaagtatgtgacatatcaagagctagaaggagcgttaagtacagtagcacgcaacactgcatttatggtagaaaattataaccttatgcaagatattaatttaaaaattgtattgaaaaaattaaaagacagtggtacaattacagaagagcttgaaaaagagattcttaaagagttcaaaaatattgaaagtttaatggaggacgaaacatatgagtaaagagagtaaacgcaacaaacgtatcggggagttatcggaagcagacatgagagtgtgggctgagtggttagccacagggcaggttcatgataaaaaccaccaaaaacagttagaacgcttaagtaaacgttcagtatcattatctgatgtaactactattgtcgaatttatgggcaaacggaatgatggttatatttcttctttaattgaacagcaggctgtatttgacaatttattaacaaaactaggtgtaacggaagagaaccgcttagaggctaaagcagagtacgaaaaagagttaagccttattcaagaaaaaatccaaaaagagttagagtctattaaagaaaataaagaaaaataatatgaaagaggttagctgaatgacagactacagcgcagtaggcaagaaaagtcgtaacaaaggcggacgttttgaacgtcaaatggctaaagaactcacagagtggtggggatatgagtttaaccgagtacctgcttctggggggcttcactgggcttctagtaataacgttgccggggacattgtagtccctagcgatgctaacttcccatttgttatagaatgtaaaaatcgtgaagactggacgattgagaacttattcttaaataacaaagaaattaagaactggtgggcacaagttgtgggggatgcaaaagaaacgaaaaatatcccactacttatatttactagaaacagagcaaagaattttgttactatggcatataatgaaaaacttgttaatgagattgaaaaaagaggttaccctttgatggtctctaacataacatatgtagacgactacaaggatactcattgttacaagacatttactacagttttagatgcaataactagctttaagccttatggtagcaaagataaagactactttttattttattttcctagtgactatgactgggaagatagcctagtttatgaaacaaccataatggatgatgctaaacaaatggatgcagaggattcactagatgcactagttaattcttatttaggaggagaatagtatggctaaaacatatcaggaagctctagcaacggtacagtcgtatctcgaatcagatagtgtaatgaaagaaacctcaagtatatctgttagtttctcagctaactggacaggtgagcgggaagactacgttattgatacattgacatacgacattgatttacgagtattcagcttagaaactgcacatgttgtagctatagggaagaaactacctcaagatagcaatgagcatgctgaactccttaaaaaacttaaaaaagaatttaaacaagcttctaaaaaactacgggaggactagagtagatgatagacaacgttaatagtcctagtcattatacgcaaggagaaatagaggtaatagaggttatagaatatattactgctaagtaccctgcggaaattagataccatttaggaaatgttattaagtatatttgtcgagcacctttcaagggaaagctacaagaagaccttaacaaaagttcttggtacttgaaacgagcacaactggttttaacacagtcaccaagtagctatataggtaaatgtaagaaatttttagagaatttcctatttaagaatagccatatcagagatgctcagctaatagaaattccagaagaacctattattgagaaatttttatttcaaacagcacagagttacaataaagaacagcaaaactatattatttcagccttaatggaactaaacagtagttcaggtgatgtgaaaactgttcttgaaaatacagaaaactatttaaaatttattacaacttagtacaatataatgctctttctacgaaaagctatcttttatatttatggtataatagagatagggaaattaaaaagtagaaggagcattttataatgacaaaagcacccagagtgaaaagacttaatatttataacactgaccggtactttaatattaatttaatgaaaaaagaagatatagcaaaaaaaattaaagttaaccgattgaatgaagaagagatagagagggaaatggacgaactagcaagcaacccattgaagacccctataggctacatggatagaacaaatgaaaaatcttatatactttatcaagagaagtatacgaacgacagacttattcagaaattatttaaacatgcagggtctgtgtcttattacacagatacaattgtaccatactacataattgagcaaatatctaagaatttaacaagtgaagtaatctatcctacaaaaaatagctatgagaacagagagattgaaaatgttcaactagctttcactgcttgccctgtaacgattgactgcccagtagtactacctgatgttagcccgtatgatgtgttatttgcactacatcctctaaaaacaaatgtagacaagattcaaatatcgttcccttgtcttacagaagaagagttcgatactagacatgaagaatactatcataaagtaggtagccactatgaggttaaatcagagtacaaatataaattctttaagtatgtacaaacttccttatctatttgggctatgaacatttggctagtgtgtgatagtgatgaggactacaataaaatagacagatatattcagaaagaaaaaattaaacgtaatgctaacagagagcgtgcattaaagagaaagggtaatcaggatgagtaaagataaaacgattaaccgaacagacatagctcgaacaatctctcaccatactggttatcgaatgaaagatatattgaagattttagaagtagaagatgaagtagtagctcaagcagtatcacaaggtatttctgtaaagaatcacaaattatggaaactaaacattaaaaaaaagccagagaaggtagcatgggatggtataaactctaaaagttttatacaacctgaaaaatatgtagttaaatttgtaccattatctaagttgaaagagtcaatagacacttataataaagagagcaaataaagctctcttttttgctctttctatattgacaaataacataatacaaagtatactagtgtcatagagcaacagagaggagaaaagtgtaattgaaaattctattcttacaagagtacattagagaaaatcatgtccataatggaaagaacggacaaacagttgattttaaaagaacagaaatgggtaaaaaacttacaggtctgttaaatacaataggactgacaggtagggactatgctgtagactatgtgtacgacatgattccggaagtacagaaagtcaaccctagaacaggtaaaccaattaagtataagacacctacgttaagacagcgtaaagaaccagaggaacggttactcagacgtttaatgaaatacaaaccagatattatcatcccaatgggggagatgggttgtaaaaatttattaggaagtacttctatcacaaagaatagaggagtaccaactaagaaaacaattacgaatgagaacatactgagaacggctgatgagcaagggcttgaggtagacgaagtagtagactcttttgaaacttgggtactacctatgtttagtatggaatactggacagctaacccaaacattgagaactttatcatggcggatattgatacattgggtaagtttgttcaagaaggggaacaagcatttatccctaaaaaagtagattacgaatttgttgataacattgaacgtgtaagacaaatttttggttttttagacaaaacgaagccagtaactgcatgggacttggagacaaatagtttacgtggtgacttattaggggctaagcctcttgtaatgtctatgagttggctagagggacaaggtgtgactataccgttagaacaccatgaagctaaatggagcccagaagaacttaacgaaatatatgacttatttgagaagtttttagcggacagacagcaaccaaaagtaggacaaaatatccagttcgatattagattcttaatgaacacaaaaggatttacagagtttgaagacaacagagatacaaaaattgcttactatctaattgtttctcagaaagtagacacttcaaaacggctatccgatattgcatatgaattaacagatatgggaggctatgacgaaccgttagagcagtataaaaaacaatataaagaggactatattgctcgtaagaaagcagagattgatgctttcaaagaagctgaaaaagaacgagtagagtgtgagttcaagatagcaatggatagatataagcaagaagttaaagaagctaagcttattggtaaacctactaagtccattattaaaccagtaaaagaaaaagttgtagtacctaagaaatcagatattaaacttattaatgagattgacggtggtaactttaactacgactggattccattagagattatgcacccatatgctagtggagatgtcgattgctgtctacgtatctataacgttctatataaacgaattgaggaacatcctaagatgttggaattatggttgggcttttatcctagactaacagcaacattagcacacatcgaggcttctggtgttctattagactctgaatacgcagaattagtagagaacatctatacagaagaagaacatcggttgcttaatgaaattagaaagctaccagaagtaaaagaagtagaggatgaacatatgatgttctacaaagaggggcttaaagaaatgacaaagcctgtcaaagatagagatgcctctgttgccagactacgagataaatataaaattactgatagtgagaacaaagtacattttaaaccaagttcgtctgaacataaaggtagactgctatttaaagtaatgggacttacactaccttatgataaagaatctattaaaaaagaaacttttgacaatggggtaccagaacatcagctaacatggagagattataaaacagataaacatgcactagcttatattgcagaaaattatccagaggctaaacatgttgctgaacttttgctagagtattctaaagtaaacacactaaaaaataactttgctcaaaagttacctaaattagcatctaacaaggatggcatgattcatggttcatataacagtacaggtacagaatctacacgattgagtgcaaacaacccgaatatgcaacaattaagtagtaaggttggagaccctagacgttttgactataaatatccaattaaacgtttatttagaacaagatttgagggaggtggaatgctacaactagactactccgccctagaaatgcgtattttaggtttgattgcaaaagataaagcaatgacacaagcatttattaatggtgaagatatgcatgaggcaactgcatctcttgtatggaagttacctaaagataatgtaccaaaagatatgcgacaacgtgcgaagagtgtcaacttcggcatcgcttacggtaagcacaattgccgtcttgtagcgtaagctactcgattaaacttacctaaacgggcatagctgaataaccaataagctgataagagaacctaagtcctgaaaaggatagaggcaatcccgtagtaaagacgatttaataaactccactaaaggagtggtattatggaaattggaacaagaacagacaacaaccctttatatagaaaattaagaactgtgcataaagacatgcgcagacgatgtctcaataaaaatgctaaatcatatgagttatacggaggtagaggtgtaactattagtaaggagtgggagaccttaaatgggttcctagcaactgtagatttagtagatggttgggacaaagatacattcctcacaacagggctatccttagataaagacttaaaaggaggagccgagtatagtatagctaactgtacatggatgccacttaatgataacaaaagcctactatcaatgaactacaagaatgtctgtgctattgacccaaatggtcaatattatgttatagacaacattgacaagttttgcagagagcacaaccttaatcattccaatatagttcaagtaattaatggtagatacaagcatcataagctatgggtattctggtatgaaggtgataaacctaagaaagggatacaaccacacatagcgattagcccattgggtgacacctactatttctataaagctcctgacatggaaaagtatgggctaaattctaaatgtgtagctagatgcttaagaggagagagaacaaaacataaagggtggaagtttattaaatctgaaaacctctaacgactatcgaaaagtgagtagctgtcgagaggacacctacaatataactgagtagagtacaccaacaggtggaaatggtaaggctcctagagtaacgactaggagcgtgatatagtctaagcccctaataaatatcgggaaaccgagggtataactggaaagtcctttttcaattgcacctaagttaggtgtaactgtagaagaagcagagcgtatttttgaagagtactttgcaagtaagccaagtattaaacaatttattgaagagacacatcaatttgctcaacgttatggctacgtagaaacactacaaggacatcgtagactattgcgtgactcattctctaaagataagaaagtatttaatggagcaatgcgtaagtcagtaaatacaatcattcaaggaactggtgcctacttaactaacctatcaatggtatacattgacgagtatatcagaaaacacaataagcgttcacgtattgttatcactgtacatgactcacttgttatcgattgcccacgtgatgaagtggacgagatggcaaaagtggctaaatatattatggagaacttgccaattgatttcttaatgattgagtgggaaggtaaagagatgcgttaccctattgtggcagatgtagagattggggagaattacaatgatatggttgattatgatgcagaaattatcaacgagtttgcttcttaccgaggatacgtaaaatacttcaaagaccaagctaagattaaagattactatgataacaaacttatctcagaagagcaaaaagaccaaggtatcaaagttatccaagatgcaatagagtcatataaacaaatgacaatttaataaaaaaatgttaaaaatagcttgactattgacgtatagtatgttattataatatggcagacaagttttctgtattaatacaagaagggggagttagagagtgtgcttaatttacgagtagacgatttagagttcaaaacaattaaaattattgatgataacggagaagttgtgacacatgatttacaaacagagttacaagtcaatgaatttaatgtgagaacagcatttttagagcaacctgctaagtatacttattggacttcgatactagagcgcttgcgcatgtatcaagaaaactatgagttaaaagcagagaagaagaaagcagaactatatgagccttctcgggttgccttaatcaatcaaggagtagctaaacctacaaaagaccagattgaggcacagattatgttagatgaagactattacaaacttagacagagtatagttaacctatcatttaacgtgagacaactgcaatatatagttaaagcttttgaacaaagaaaagatatgcttattcagtatggagcagaccttcgtagggaatatgagtatagccaaaaggttagtatgccagacccaatgaaaaataaggtaaataatggtttctcagactttcaatggaatttagaacagtaaaattagtgataaaaaaaataatataatataaaaaaaatagaaatggagaaatttaaatgaattttcaagaacaattacaacaacaattaaaacaacaaaatattggagaacgtgaagcggtagactacccatcaaatcatttaaaacataaagaattatacttccctaaagcagaaaatggtcagccatcaactctatatgtacgtgtgttacctcctgcagtaccgggagaaaactataatgttagcgctcgtgaggcattcttaacaactcgtaatcgtaatggtaaagatttaaagagcaactttatcttttcagaacaccctaatgcagaagacatcttagaacaagctatgattcgttggaacgcagaaaatcgtgtaccaaacccttatagccgtaatacaaaacctcgtcaacgttactacgttaatgtagtgcagttaattattaaccaacaaacaggggaagttagctatgaaacagattctaatggtcagctaatggttcgtttacttaagttaccacaaacagcttgcatggctattaatgagagcttaagtaacccaatgttacgcccacagttttcacctgatgtaccagaagaagtagcgcaatacagctttatttcttctgcagatgcattccctatttcaattacaaaaccaccacgtagtaacaaacctacttcgtacaatgtacaagtgattagtaatcgtagtttaggtgcattaccacaaggttgggaaaacttattagaagacttgaaataccaagctacaccttctgtagagtacaatcgtgagtttattgagtactttattgatgtagtagacgggaaagaacctgtgcatcaaggagcacaaagtcaaggaacccaagctccacaatttaatcagcaaccagtacagcctcaatttaatcaacagcctgtacaaccacaatttaaccaacaacctgtacaaccaatgcaacaaaatactggttggtcgccacagcaaagccaaccacaacagcctgctacaggttttaatgcaacgaacatgggaacacctccaaacattaatggagggtttagccaacaacctgtacaacaacctgtacaacagcaacaaccgatgggttctttcaatgaacaaccagtgacagacccttctaccatttctgatgcggatatgcctttcaatatgcagtccatgcctgatgtatcaccacaacaaaatgccgtacctgagcaacctgtgactaatacaccagagccagtaagccaaccagttgttaaccaacagccaaataacacacctagtgtagacgacctattagcaggtatggtaggcaacgtttaacaataatgaaacagttaggaggggcatactgccccttttaattctgtgttaactatccaaaatatttagtaggagtgaataatattggcaagaaaaagaaaaagtgaagaaatagattttggaactattgatttgacaaaagaggtaggactaactacatttacggacacaaagttctctaatgtatcagacagactaccaacaatgattccacagcttgattacattttaggtggaggattgccatttggacgtatggtcgaggtctttggtaagaactctagtggtaagtccactttagcagtccatctgacaaaggtagcgcaaatgctagatgtaccaactgtatggattgacgttgaaggtaccgcagacccagaacgcttagcagaactaggggtagactttagtgcaggcggagtattcatggtagagcctaaacagaacaaagacggtagtaaagatacaatcacggtagaacgtgtagcagaagagttacaacgactcttaccagtatttagtaagcttggaaaacctgtattaattatttgggactctgtagcgcaaacagcttctgagaaagagttagaaaaaggtgtaggtaaccaacaaccgggtttgtaataaagctccgttaggtagtaatatctaaaagaaacctatctttatcatgggaaacctctaggaggcaatcatgagtgaagctgtagaaatacagaacatgcaacgactatcgaaaggggagttcttgtcgagaggacatgaatgagaaccgagtagagtacacccaagtgggtggaaatggtagggctcctagagtaacgactaggagtaagatatagtctgtactacatggtgacatgtagcagttcataagagaacgctataagcttaacgaacttataggaacataatagattaaggcaaaagcaatggcacagtttgctcaaatcattgcacctttaatgacaaattcaaaagcattatttattgctattaaccaagcacgtgacgagctaggtagtatgtttggtggagtagactctcccggaggacacgctttacaccactgggctagcttacgattagaagtagttaaagcaagtcagattaagaataaagagctaaatgcattcggtgcagaggaagagacctatgtaggacatatcctgcgtgttaaaacagcaaaatcaaaagtgtcccgtcctaaccaaaaagcggaaatgtacttaatgtccgacacaggactgaacttagaggaaaacatttatcgttcatgttttgcaactaataagcagtatgccttgattagtggaggcacgtggaagtcttatacaacggatgcagggcaagagattaaatttaattcagataaagcttgggtagcttatttacgttcagaagagggaagacctgttcgagacgaactatttgctaaaatgatggtacgctcattcccacatcgttatgctccatttaataatgaggacgtggatgtatgcaaaattccattatatgaatttactaaagaatatatggaaaatcataaggaacaacctaaccaagctactaaagaagaagtccccgaaacaggaacagatgtttcagatttacttaaacaggtagactaatagataagggggcatttagcccctttattagctataaaggagaggaacttattttgcgcaaaggactagcacctaacccattttttgaaatattagaaaaacatcaagactcctctaaacgtactatgactatgaacagcagtggtacacctagttcactacaaccaataagagacatgttcttaaaggcaatgagagaaggtaagaaagtcctaatagagaactctgacttaagtagtgcgaactctgttgttatagagatagaatatgtaggtaatcgttggtgtttaggttatcaacgagtcttattttatggtatggagttaaaaataccacacactatccacttctgtgatgtatatggagcctatgggcacgatgctcagaaggttaagagacaagttaaggtagtgtttgagggggacaacccttttgagtagagatgttcaaaaagaggaaaaagaaatacgtaatggtaatcggtttattacagagactcatggcaaaggagtgtttcctagagatgtagaccgattgtaccataagtatagtaatcttagatataaagtctataacactcataaagactcgttcaatagtgaggcttcacgtaaggagctcaagagctatattgatgagcaatttataaagttaacaaaagagtatgatataaatggagaggtagactttccgggatatattaaaaaagctctgaatttacgagtaaggcacagctatgtaaaaggacggttccgagataccgctagagaacgtctaggcacccaagataacgaagtagagttattgttagggattgacgatagctctcaggcagatattgaggatgcagaacttattgaatcgttattatcaaaagccaatttttcagaaattgaattagcagtatttcagcagttaattcaaggaacagtaagggatgctcgtattattactgaattgtcagaaaactacggggtgtccaagaaagccgtaaaagatgctataaaaaatgttcgtgagtttgtcttaataaatttaacagattagagtaatacctcctttatgtctgctatattagcagtagaaacataaaggaggtattttttagtggaacaaaacaacactggcaagtatgcaccatttattcgtttaattgtgatgggaatctcatttgtggcaactggtttgactacaatatttggttgggaacctttaccattcacagacgaacaaatgaaccaaggtttaatgttagtactatctgtaggtcttgccatctacaactggtacaaaaacaacgctgtaacttcttatggtaaagcaaaagaagaagcaggaaaagaagtagtcggaactagacaagacttcaaaaacagagactaagtacgaggggtgtaacccctccttagttaatacaaaggagcttcgacatgaagatagacgagataagcaaattagaattgcctaatctatttggaaaattccttgtggtagagactatttcggatgggtacactggaaccgtatctggtcactataactacgagatagaccaaaaatctgaggaaacttatatttaccctgtattttggaatgataagcttaacaaatttattaggtcagatgaattagttgtatacactaataaaaataaagtatactatgtttgtaaaacaactatagacccatataatcatgcagtagtagatgagctcacggtagaggaaggcatggacaaagacaagcgtacccttcaagcgtttaaactttttgtaaatgacctattctcatttggtagctacaatatctttctaacaggtaacctatcattagaaaacaaccctgatattgttctagttagcagtgtatcattagacaaacagaccgctaaaatgtacacagaacggacattagaactaactgctacggttttaccagagggagctacaaacaaaaaagttagtttctcagtagataaaccagagcttttagggttaacagtctctgacaataaagcaactgtcacaagtaaagataaggcaggtactgcaattgttaccgtaactactgaggatggagaacacactgataagtgtacagttcagatagaagagtacataaaagttacaggaattaatgttagtggagaatctgctttagaaaaaggtaagacatacaaatttactgctagtattgtacccgataatgcaacgaatcctaaatttacttggtcttctagtagtgataccatagctagtgttaatgcaagcggtgacgttgtagctttagcattaggtgaagcagacattatagcaacaactgaggaaggtagccatgtaggtaaagtacatgttaccgtatcagacccagaaccagtagaaccaactgaataacatagaaaagaggaaagaaaatggctaaagaaatattaaatattgaagacctgttaaaaccagagacactagaagtagcaatagatggtaaataccttattgtaccaacattgtcggatgggtttacaggtacagtagcaggcggatatgcatatgctgttacaaaaaaaggaacagactacacagttaatgaattaatctataatcaaaaggataacacatttaaaccttctgatgaaccaattattataactgatgataatgaaatattcttcattactcgtacattagaagacccatataactaccctgtagttgctacagagaaacttaaaactaaagatgtaaaagaaaaacaagttttacaagcgttcttagcatttgctgatgacagatttaagctaggtgtttacaatgtgttcctagcagatgaaccatttgtatatggggacaaaacagaatagtttcattataagagacccgttaaggtctctttttttttgtatatagtgttgacaatgttgtagtttagttatatactatacttatactgtataaggaggtaaccacatgaacgacaataaggaaaaatgtattaaacaaggaatacgagatacttataaagggtacgatattttattagatgaagagaatggatttttctatgttagcgtacttgacccagatggcaaagaaatcattagtgggtttgtagaggcggataaacctattgaagaatactataaagagctcctaggtaaatgcgaccaagatatatcgtttaaagaccttttagggttcttaaatggacgtagagacactgaacgtacagacatacgttttttaaagagagacagtggggtataattaaatgacaaagataaaacttattacaaaaaagaacacccaaggctatgtcatgaacaccctgctacgtagattttataaaaataatgtagacgtagaatttcttaataaattcaatctacctgatattcataaccacataggggagcatgatgctgttatcatagtagggtttcctttctttgaaagccaacgaggtgcgttagacacggcactgtcatctatggacaacccgtttagcaaggtgtaccatttagcaacatttggggacacctatcgtaatgaaggtagctttcgttcatttgtagacgaggttataagccccgttggtcattttgtagaactaataattgacctaactaagttcactaacacaggtacaaaagaggatgaacaaaatgtagtggctcttgctaaagaggcattagtgtttgccaaagatattatagaagagacagacaactacaatcgttatgaagttacagacagaactatctcttgggttcttcttgtagatttgcttggagagaacctatataaggtgacagagcctagtaaagagctagacaccattttgaaagaacaagaagtacttgtagatgccttgaacataaatatgcaggactatgtgctaagaacaatagggaagatgtctgcaaacgtcattaatggaacagtggtttgtttcggttatgcagaacagcatgtcaacgaagtagcccataaattaattaatttttataagtcacataactatcaaaaagttattgtctttattggtaggcacacaaaaggtgacgacatgtttagtgtaaggagctatggtgtgaatgccggagaggttgtctataaagttcataatggtaaagggaaagacacaacggcaaccgtcttcttaggtaaacctagtgaagctgtaaataacacactgctaagtgtgctttctgaaattttatagtttaactttgtggtataataaagatagataaattttgataggagtgtaaatttttgaaaaacaacgaacctttagagaagttattagacaaattagatgaaccaagaattttacaaacaattattataggtagtttacaacggagctttaatcgagtacacgttggtaaatttaataaactagcacaggagtttgacttagataaggagaacctgtatagcttaaaggcactagttaaggaaattgaagaagataaagagttacacgaactttacgaagctagtatggcaggcaaaattacgctagaggctgttcgtaaagtattgttacaagatgataagtcatcgtttgatgtactgtcttcttacgtagtagaaaatcaagcagtgctagcccgtaaccgagagttcggtaagttacaacgtgagggagcttatcttgaccatctaattagtggtttgaagacatacttattaactgaactaaaagacatgtctagtttaaaatatatcaataaaaatttaaaggcaccgaaagtatcctcagaccgagagcttattctgtgcctatctgattggcatattggtgcttttgttaataacattgacacaggtggatacaactttgaaatctttaaagaacgacttgaaaagttattagaagaagtattccaagtggctatggagcaggatattaagaaaattcatgtttaccatattggggatattattgaacacattaatatgcgtaatgttaaccaagcatttgaagcagagtttcctgctacggagcagattgctaaaggaattagagttcttgctgatacactcaatttactagctaaggcagaatttgaagtgtctttcggtatggttggtggtaaccacgaccgtttccaaggtaacaagaatgataaaattcataatgataatgtggcttatcttgtagtagaccaacttcatttcttacaagaattaggggcattaaacaaagatattaaacttgtagacaacagaagtgacgtttatagttttaaagatacagttgcaggtaaacgtattaaagtaactcatggtgacactgagggcaaaaaagtggatgttaaaatccctaaacatatcaaagatgaagttattgactatttaatcatggggcatatccatacaacacgtattattcaagaagacttttcaagattccatgtgtatgtcggctctcctatgggggcaaacaactactcagcagagaataacttgccaacaacaagtcctgcacagctaattatggtattagaccctgagcgtgatacaccgcagttcatgccagtattcttataggaggtactcgtatggaaggtaatttagtttatattttattggctattgcatatgtaggtgaaggtataactgcctttactaatactaagcgtaaagaaagatacatgattgaagaaggagaggctcctttgccacgtagttcttatgtatttttaggcattaactaccttttaagaatagctatagcaatttctcttatcttcatcataccaactagcttgcaacttaacgtaacaggtattgctttgttcacactaatggtatttgtagttccttttatagcaagaattatcgaagttgttattagaactgcaattgttcgttatgttcaaaaacaatatattaagcagttagaagaacgaaaaggtaaaagagagactaactagtctcttttttgctatattgaataatgaggtgactaagtatgaattttacagaagtaataagccctaatggggagacatcattaatagatgtaaacaacccaccaacattaatcagacgtggggtcttatctattaaaacaaaggttaataatgaagtgaaggaaactcctgtttatattgttgaactagccgaggagctaacaggtactgatgtagtatctgtctataaagtaaaagagattggagattctatccaaaaagactacattgaagaaaaagtgacccctaggttcaaaagcacaacatatctgggtgagttagcacaaaagattaaaggacggtcgataaaggaacaacgaagagttgaaacaaaaccaccattattcctagccccagtagttaatggaatcgatacattcacaggaatcgaaggtaaaggtttctacgaacgtgaagaggacagacatattctattacctgatggaaaaccgggcatagcctatggagataatacaggggtttttatcggtttgagctcgattaagtgggacaaggcatatgtagacgtggagtctataacaaagggttatttgtcacagaaacagatatggtttaacctagatggtcaaagaccacaatttagaagtgagacactataatgacagataaacaattttatgaggcagatattcaagagttaattttaaataagcaaagaatattcggggatataggaaagagcgctattgtttttgagaaagcaatcatgcaaggtaacacaatatgtgattgcctagtcttcacagaaaaacgagggctcattggcatagaaataaaaactgaacgtgactcgacaaaaagattaaataaacaattatctgattatgaaaaggtgtgcgactacgtatatgtattatgccacgataaccatgtacctaaagtagagcaaatacttgctagacataatcataaacacgtaggtatcctagcttacacagagttcatgggagaggcaatgttaggtgagtataaacaacctagccgttcccctaaaaaatcagcttatcatatgttaaatatcttgtggaaagaagatttaataagaatgcttggtacattcagacggtatggtgatagactagaagctaatggagctaaggttatgaaaacaaacagccgttctggtggagtatctggactttatgttaaatctacaactgctagaagaatgactaaacctgaactcattaataatttaataaatagagtaggcggtaccgaagaggctacgagagtgttctgtgatgtgtttatccataataggaatcacccagagaaagcaattaagttaagacattttaaagcaaaagagaataggggtgacctagatggggtttaaaggtgcaaaatatggttcttggaatactgtagttggtaagaactatgtgggtactgggggcagaacaagtggtagtaacacaaaacggctgtccacaaaaggctactaccaagtaggatttgttaaagaatatcagaacttgacagaaaaagatattatgttaaaattagagtatggaaaagacttagtgtctagctacactggtgtacctgcagatatgattaagctacgtaaaaagaaagaggagcaaactctagcatctttagacacagtttattatgttagcattggtaaggaacctgtaggtaagctgtctatacgagctcagagacgttttagagaggtagggttaacatttatatacctagagaagaactacgtacagaggaagcttagaggcggtaatgtacgtagtgtaggatatactaacgcaaccaaatctcagaaacgtaaagcagatagacggaagggcaataagtctaaaacaactagatagatggaggactactatgagtatttatgatgagctaattggtaaaagtgttatagccctagaatatgcggaggatgggtgtgaggcaagccttgtactaaatgatgggtcatgcttaaaagtatcttgtaacccagagccagactgttgtgggtataatgattttgaagttattctcccagatggttttgatttcacagataacattattacaaaagttgaagataatagtgaagaatgttatggcggttcaacagttaggataggcatttttaccaatgatgcacggatagttattgaaggggactacggaagtggttctgggtggaactatggagagtatgtagacgtagaaattgtaaaataatttactattagatggaggtaagctatgcttaaaaaagggaaagaagtaacactaagaaaattttataatattatcacagataaggaatcagtattgctaggggcacgctacacaagctcaataatgactacagatattcctattacaacaacttttgaagatgttgaggtagaccttaagaaagaaacagttgcaggaactatttcattcagaccagtaggagaaagacagattaatgcattaagtttactaaaagaagcaagcacagcttatgggggttacggagagttcctagatgatactattgagaaacctttaatcaatagtgattttgcagtagatgttagcctagcagactctgctttctctaacctacaagagattccatttaacctatatatgtcctccccaaaagttttttatacagaagtatcaattagagggcgtaaacatatgcaatatgtattagaggatgagtcttctagcggtgtaacaagtacattagcactggtattccgtaaaaaattgtatgatggggaaacattgctaggtgtgcatacttacaccgaagcactagcaagagtagagggaattaaagtgttacagtttatcgcaaatggctctgtactagaacaagtaatcggtgcagtgtctgttttagggggtagcacaggaacaaccctgttccctatgtttgacgatatggtgatgcaatttgtgatgattgagtctgttccttgggtgcacatttcttgtgatacaggagcaattgcttttaaggaagaagacatccgcaatgtaaccattaagtcagctagaccgggagaatataaggtgactatctacttgctagacgaaaaagttacattgttaattggataaaattttaaaggaagttgacaatatatgttgacttccttttttgtatgtgctaagataactacagttggataaaaaaaaataaatggtatagagggagagatttaacatggactacaaaacaaaggtatatgtaggagcgcttagttggttaggtactttaggagagaaacgatatttagggcaaatgcgtgatgtattagctgtgtacgagctaggtagtcgatacgcaggttactatacagaagatagcgactatgactatatggttgtatacatgccggctccttatgatttaatgcatcctacaacaatttataaacaggaaacagagattgatggaaataaggtagaggtaaaatatatgtctatcgtggaatatgtttaccgtattgaaaatggagatttagaggctttacaaatgttaaatgccacaagctcccaaagtttcttcggagagcctattgaaggtattgacaataagcgtactcgtttagttacgtatatgaaagaactagaatacagaagagaaacatttacttatttagcaccagagaagttgtttagaggaattaatggtcgtattaaagccacaaaaacacgtatggataaggctattgagaatgacgatatggaagtagcggtaaaatgtgctatccttattcgttattttatggacttattagttgtgctagcggacggggaatctattcgtgaaggtctcacgttctctcctattattgcaaatatcattagagagtttaggaaagactgtgagtcagcacaggctaagacacttatcaatactgcacaagtgctattagaggcggatagagaagagattttaaatagtattaaagaccatgggttatcagatggttacgctcaatcagttagacaatatagtttaacaggtcgattgatagatgtactattaggaggatattatgactaagttagaacaaaataaagaaatcttagatatatttaatagaaaaggaaaagtaacagataaagtagaagaatctgccaagattatgctagaattagaccacgattatgactttggtacaggggacattgcttatacagagcgtggcacagataagaagggacgtttctatttagaaagtcgtttgtttattcataaactcatgccctatgggttcattttaaacgctgtagtaagtaaagtacactatggagaccaagaggagaccttagaacgagaggtatcccgtgtatatgagctagagtacaacctaagagataaggtagctgtgctaattaagaacggtaaaccactaaacttctcagaaaataacattagtaacatgttttctgggcacgtagcacagaatattcttgaacaattagatacaatgtctggttcagatatgtatgtatctgtgtatgaacgagttagtcgagttaaggatgaacaaattggtaaagtatctcggttctttgatagattgatgaagtacaacaagattgaattaatttataagagtggcgttcctgaaggctttgctttggcttatgcttatcgagtagttgttgtaggagaaggcaaagtccgtaatgaatggtacgaacctgtaaagagtgtggactatttagataaggaacaaacaaatccggctaaacacctaggtattccaaagtctatctttaagattatttgtgaaggtgggttagagtggacattctaccaaaaaatagctagtcgtttccataaatcattagttaacagaagtactaacaaaactcctaaatcccccactgctatgaagaagatagagaaagagattgctaagttacaacaagcctatgctcgttttggcggggtactgtataacctttatcagtttactaaagagctagatgaacaatatggtatctcccatagtaaggatattatcgaaacagagtgggaatctatatacgaccatattattgcaggagtagttaacgataactataatagtacaactgcttatgatatttctatggttgcaaacctagatttctacagaactgttcgttatctatactatcgagtatatgttgagcaagggcttacttcacaagcagaggctagatacacatacagagactacttgagagcacaccattatatgaatgcggtacctgttaagtaccctaaagctcttaagactgctcatgacattattattatgaattaccgaacaatgaaggataaggtattgaatagtaactttgaaagtagtgtagctaaatataaatatttagaagaagtatcagttagaggtggctatattgttaaggtacctaatagtgtggaagacttaactaaagaaggttctagtttacaccactgtgttgctacttatgctcatcaagtagcagaaggttctactcgtatcctgtttatgcgagataagacagagccagatactagcttagttacttttgaggtaaaaaataataaactagtacaagcaagagggctagttaaccgtgacttgacaaataaggagcaggagttcctagacaaatggttagttaaagcagaaattggtaagtattagtttgcctaaaaaggcggaatatggagtgtgtatagaccaattcacaatgaaaaaagtacactaaacagttgttatttcattattaggtaaaacaacttattttagatagctgatattgaccaacaaatatttcataatgatttagctattaaagttacaaaaaccctactaatacgtggggtttttgcttgtttcaattacatatgaaattttacagatgttctgctatattagttacagaagctaataaaacaaagggtttcgacccttaaaaatgatatttcatataattaaaagttgaaggagtttataactaaaatggctaaaaaagaagtaaacaacagctcagtattactgaatctatacaataataaattgcttgtatctaaggtagacgaggcgttagacgagggtaaaccatacgatttcattattgctttttgtaaagagaagttcgattttgaaattaataaacctgcattatctaggtacaaagagaaacgtagagagtctttagaaacaggagtagacttggaatcactacttgacaaacgtagaaaatcaggtaaaattattgatattaagtctaaagaggtaaccccacttcctaatgaaacatacgataacacatttggacaagtggaacagatatacaatgatgtagaggtgttagatacaatcatacaaaaaggttttaactctctaaaagaggtagactatgttgaagccccacttgctatgaaagcaattgaagtaaaagctaagataacagctaaccagttccaaggtctaagtctaacaggtctaagagagctaagattaagacagtctgctaaagaacaagcaatgactgagattattctacaatttattccagaagaacagcatgaagaagtattcaatgcaattgaatcagcagagaaagagttctatgaaaacttagatttaacagaggaagaccaaagaatcactaaagcgttgcaagcatcaggtatggatataatttaggagggctataatggttgaaaatttgagagaggtaaattataaaacattaaccttagaagaaagtttacatgcattacttgaagggaagacccttattgtaaaagggctagaacaaagacgtaagttagatgtgctagtaaggattttctcagaaggtgttgtacctgttacgcagataagttatgatacaacccctgcggatggttattggagaacaggatattggcagatatacgatttgccaattaatgcccttagcacatacccatgttttatctatgatgatttaaatacggatgaactccctaaatttatgataggggacactgtttactacacaagtaaagaggactctatcaaagattccgccattgtaatcagtgtgtacaaagacgatgttaacaataagtggtactacaagttaagtagagacaacgaaatatatgcagagagtgagattagaagagacaggttataagcctgcctcttttttttttaaatttattgttgacaaatatctataactttgttatagtataaatatcaaggatattgataataaattttggaggtgccatgatggcaaatattttagacacattaaagtggttagataaaggggacaaagttactattgaatttgataaagagcggtcgaagtatgcaaaactgactttgcacgattcatcagctaagacaaatattgtccgtaacattgttttttatgatttagacaaaggagtgtatgcttacactggtgaatacacccctgtatgggataacttattagatgatatgcgtaagacacaaggcgcaggacctgaaattaagactacaaaagtaaatcagttagctacctatgaagatgccttaaagtttattgaaacaaatggtacgttttatgtaattggtgaggaagtaattgttaaggttaaagatgcaaaagagctagcattgatgttaatgtactttagagatgctattgaagaactaagaggagaatacgaccctaaaaaacatcatgtagatatgacaattgaattatcaaaagatgttttgaaaaaaatggcagtacctagacatgaattagacttatctttaggtggcttaatgagagctgtatcacataatgttggagaagacctttttgaaactcttgggtttgactacatgaagcaagcttgggaagtcttagttaattgcttgtcactagacactatccatgaggtacctttccgtgtgctagacgaattagagaaagtaacagatagcatgtctactacagaccatattgttaccttgtatgccggtagagaacttaaaaaattctattcagaggaagagtactttgatgtaatcacacacaatttagctgatgtgattatggattggtcaactatttttactacagctgttcttaataatacagaagatgatgaacaccttaaagagttacagcttaactttgagagattcaagctagatgtagcagaggttctattaggtaacgttgcaagacatttactatatgcaggagttaccgatagctttaacgaagttaaccattatgttgtcggagcaggtaacctgattagaacagaaggtttgattagaatagaagagttaactggaacattagacaaccctaaagatgaagatagttctgaaacagataataaagagttactagatgacatctttacaaatacaggtgatgatggtgttgaagactttacaaaagaagtagacgagcttgccatgtttgagaacgaacatgctgaggaacttttggaagtcaataacaaattaaaagacaatcaagagttattacgtaaaactgtggaggcgatgggtatggcttcttactctactattgattcatcatttgaacaagaggaagaaacagatagcaaccacacagagacttgtgaggataccagagctttccaaatgttaagctatgcagtacgttcaggagacaaattacttgaacgtgtagagaaccacccacaaactgaaaaagggttgaaaatggctaaagattctctaaaagagtttgaccatacagtgaaaccagaattagaagcttatttaaaagcagaagagctagcggaagacgttgatagacatgcaattgtaactacaattatccgtatcaaggacactatggaagcagatatggacggctgtaccgacccaatagagcaaggtttattctacgcaggaagcctaaatatgttagaagaaatggaatcattgttacgggctagcaatagaggttatggttgggacgtaacagctatctatcttatcttgtccattgaactagcttatgggacttacgggttgtctgatttagactttacaattaaaaataaagaggaaactcgtaaagaagaacaagatgcaattaatggtattgtaaacttcttagccaatcttttaaatacagtactagaagaagaatcagaatcagaagaaacacctgtagtagtcgaagaggaagaagaggataaggatgacttctcactatctacagaagacactgctaagttattggcagactggtcaaatggtctacctacgtatgtcgttactcgtaaatacggaattagtatgggagctttatactctatcttatatgcaaatggggcagacgttaaatcttctaaagtagcagaacgagtggctcatgtggaaaatgacaaagatatgttaaacgcagttattcgagactacaagaatggtactcgtttagtagatatttatactaaatacaaattatataaaaatggtttgttctatcttttagataaatatcgagtgccacgtagaggacgtacaaagaaataacaatgattaaggtagtggtgctcaactactacctaatcttttattagggaggaacttaattgattctttttatatttagcattattacaatgctatccatgttcttactatatttgtttgggatggcttctgtggctgtaatcaaagtagggtttcttataggtagtcaaaacgatatagctaaaggcatacactctttacttttcacaggtattgcacttactgtagtcaccggaataactagacagtgtttactattattttaaaaaaaattggaggatttagcatgttgttttttattgttttagcagtatttataggcgggcttgctttatggggaatgtatgatagttatgggtacctagactggacttcatggttatttagtattgtggtaggctctgctgtagctacttttttcacactagcggcggttggaattactttcgatgttgtaccaagtcatggggtaacgaaaagtcatgaattacaccctatctatgagaacagtaaagtagttgtagaggctaaaaaagaccagtttgagattaacgtagatggcggtttggtagctattgatgcagaaggtactactatcctatctactaaaggagaggttaagcctaaaattgtgtttacagagaactatataaacaacaactggtggactcgtttcctaggtatagcaggtaaggtaaaagacacttcatcagttctttatttagactcagataccttagtgtacaataagccggaaaagaacagtagcgcaccagatttaaaaattaaataaataatttagaaaaaggggcttgcataaagtctctttttatgttaatgtgtatttatagataggagggctactatggaaggtgaagtagtatacttagatgagtttatgaattttttaactgatagtggaataaatactgatgatattaacgtagtagatgatagacaggagggctagtatgtcttatacaaaagaagcattagaagctagaggctatcagtttgacaatatgtctatgatagataagatggatgccttgttagaactgctagaggaaccagaatttcgagaaaagatgaaagaagagtacgcagagttctctaagaggcacaataacgatgaagaatgaaaagttagagtcttaccttatgaaagagattgcacctattttagatgaaatagagatgagtgaagaattgataaagggaatggagaacaacaacccatccgatacggttacagtctctttttccaaagaagaagtagacatactcttagcaatgttagaccttgaggtacctagattagacagtggttctgaattgtttagccctaatctggtaagggaagctaaactacaattaattaagaacaagctaacttcaaaatgatttctcactagaattaattagtgagaaaaaaattaaataaagctattgacaaataacaaaacatgatgtaaactaagtttataagataaagaagaggagagatacacatgaatgaacaaaagaaagtatatgcaaaattaacagaggacgaggcagtatttgcttgtgaactaggagataaaattaaacaaattagagagagccaagagctatctcgattagaacttgcaaaacgagcaaaagtagaccactcaacattaatcttaattgaacaaggtaaacgactaccaacattgcgtattatgatgaagttgagcaaagcactacaccgagaattagctattagctttacagattaaggaggaggtatcatgagagggagcctagattattacaactatttgtaccaaacaatcgaaaatcgacctacggaggagctagatgtcctttatgacggtctttataaaaaagccggtgacctgtttgcaatagataactttcaaggagttaaagaaggcagactaattttaaaaatattaaaggctattagagaagaaattaatagtagaattgatgaagaaattgacctttacttgtataatatctatgacagtatatcagatgaagacaaacgagtaaattggctatatgaggtgtaggtatgtttagtgttgttaaggctgacagctatgttaaatcagacatagaaatgtatgaatttaagaatgtaaaaagtttggcattgactaagaaagagaaagaactatggacaggcaaaattgctaaatatgttaatgagtttattgtaaatgcttatggagactaccatgggaataaaatacctgaaataaatgttgtaatcaatggtaagctaagaagaaccctaggttcttttgtccaattcactaacacaaacaaacactgtatagagataaatggtaggtttgttaaagaagttattctattacaagaaacacccttagctcaaagagcgcttgatattttaatggatgtagccagacatgaagctatccactatacactttgttatttaaatagtttaagtggaggagacctaccaacgttcaactaccatgacggtggggaggactttgaaaaagatttatgtttgacaggaacttcacctagtggtgctacgaaagaagagtatatttatagttcttttacactaggagccatcagatgccgacaccatagtacttgccctgaatgtgggttggaaacatacatgtatacacgaggacggtactattgctataatgggtgtgtaggggataacggtagaaaaattatatttagaccacaaggtgatattgcaatttatattgatgaaccaaaatctaaagctaaaccaaaagtagaggaagctctaaaagactataaaggagcgttaaagctaccttatacaggtacggaagaaataaaataaaaaaaaatagttaaatgtattgacaaataacaaaacatgatgtaaactaagtttataagataaagaagaggagagatttattatggcatacgtaacaaatattgatgtagtagcagatgggttagatttgtataatgggaactatgtggtagaacgaggtcaagtagttacttttaaactacatgtagcgacatggaacaatgagcctacacccgaaaatgcttatgcgattattcgtaataatggggtagattataagagtaaagttgatgaatttggcaatgcagaggttaccttcccagttaatggtcgtcctgaccaagtaacaactagcatctttgcattaacttctggatatgagggggatatgcctcgtgtaatgtcagctatctttagtgacgaaacagaaattaaacaaactgtaatgaacgttacagcatctattaatggggagccagttagtcgtgaaggtgtatttttagaacgagaccaagtagtcactgtagatgttaaagcaacattatctacaggtaagttctgggaaggtgcacaggtaggtgtgtacaataacaacacggaatacttaggtgacctagatgcagatggttatggttcagtaactttccaagtaaaaggaaaacaagggatggacacatcagctatctacgtattcgttaaagaccatgaacgagaagctacactaacagttcctgtgaagtttactaatactactgttactacagaaacttctacagaagaatcgtctactgttgatacgactacaggaacagaggagtcttctactacggatacaaccactgtagaaagctctacaacggattctacgtcctctacagtagattctacagaaagtacagtagaaagctctacagagcaaacagtgaccaatgaggacacttctactgattcaggagtagttgaaactacagaaacttcccaagtagcaggctacacagagtctacttctagttctacagagtctaaagaagttaaggaaactcatactagcactacagaacatgctaaagagttaccatctacaggcacagaggtagactatgggcttgttgggttcggtggtgcaacattaacagttgtggtggcactagtagttaaaaaattgttgaataagtaagaaacacaatattgcgaccctcattaattgggggttgcaaattatattattttttttaaataaacctattgacatttaacaaactataaggtaaactaagttcataagataaaggggggaaacaaatgagtcaagtaagcaaacatggagaaaaacgtgtacgtgaacgtgtaggagtgaataagagctctgtagaccgacaatttgagttagctttagaacgaggatacagacaaaaagagctaacaggtcgtctaaagaaatgggtagtatcaagagtatttaactctaagtaccctcaaacatgtattttatataatggtaaatgcttcattgttagcagtgaaggtacactagttactgtgttaaacatcccaagtaatttactaaaagattttgcaaaattatctaagaaaagaggaaaataaaatggatattatggatattgagtttttagaagaacataaacaattagtaaaagaacatgtagaacaagaattaaaattaatgcaccctcttaagaagttacaagtaatgacagactggttaggagatacagaagacaagctttctcaaggagacttagattacttcaatgacttaacagaaacagagctaatagaggcaatggatgctagtgaaattgtagagtcttattcagatgtcttgttagattttattgactactacaatattgatttaactggtttagaggaacagctaggtgtgtaaccatggataaggctgaaaaggtagataacattgtaagacaggtcacaggggctgttattaagacaactgcaaaagtagcttttattgtttttgttttaacctttgcaggtgttttagtaggttattatagttattcatttttaacaagtgcagggtggtttgccttacctatgatattatcagtagatttgctatatgttgcggtactgttaggcgggctagcctttatatttgcagaggtctacaaagtagttttagaagtgaaaaagatagttaaacgaggagggcaattatgagtaataaaacattagaacaaagagtaatagatgctaacaaagagataaacgataagcttaacgaatcatcaattattcgtaaacaaattgaagaattagaggaacaggaagccatcttactatcagacgtagaggacttacttgattacttagaaaatattggagtagacctataggagggacttattatgaataaaaaagtagaggaaatgacaatggaagaaaaagacaaagcactaattgcaatgggacttattgatgtaacgcaggaggcagactgggtagtattagctacttgtgaagaatgtagagaagagtacgaaggagaggagtacgaagaaggggactgtgcagagtgtgaacattgtggaggagaatactttatgattgagacagctctcgagggtactcgttgtggacgttgtgatgactactttgatatgtgggacgactactttgagtttgagaatgaaggtaacccatataaagataaacatatctgtgaacattgttatgaagaactagtatctatgggaatggaagagaaattttaagatactactaagaaggagacttaatcatgaacgaattagaagaacttaaaaatacactgattagacaaaaactttcaatgttggagagttacgaaatgagagaagcatcattttggataatgtttaatgggatattacgtgtcatcatgtcagtagctgtcatagcctttgtaaactatgctaagcatgtaagaccagataatgtagccacatggtttctagctctgatttgggttattttcctagcagaaggtattaaaggtgcttatgatgctgttgcatttggtattcaccgcaaaaaatttgctaaacatattaaaaatatgcgtgggataatcgcaatcacacaattacttattgaagaagacgaagagaaattaaaaggaggcaagctagatgagtaaagatgagaaattagttgagtggtttgaagttgccttaatggtgattatgtggttgcttatcacgttcagtatcttatacacaatagtttccttacctttcatggtacacgaaggggactggctagggattgtgcgaaacgtactactggacattgtagtattggcaattggggttgtcgctacatggttgcaattaagatttaaaaaaggaatggaggaataattaatgggatatttagagagtgcaattgaagaaattgaacgagtactactaggaaataaaagtcgtgacaccgaagaagtttatttaaacaatgcaattcggtatatcaaaaaagagttaaagaaaaaagaggtagagccaacgtggttaaatgaaccacagacattgttccttaattggtttaacgaattatacgcagtaggtggtttaactcatgtaacagaggcagtaggttttttagaatccacaggaggtagaatgaagtatccagaagcatattctgctttcagtaatttaagtgagaatgaattgcttgaggtttacagtaaattttatacagggttattcttaaaagcacaagggggtgaattagaatgaactttcatggtaaagtatttcatgataaagtatttgacattctttctcgtgattaccctgattggcagaggtatcagacagagaaacgaccacatcccaatgagcttagaaaagactttgccattgatagtacagatagtagatatgaagagtatgttatgggagagtttaatgtagaaacggctagcggagatgttaaagtatacgcagtaggaattagaagagtagttcataaaaaagctgaggaggagtaaatcaagtggagtacacagagaaagacattaaagaaggtatgaagttacgttgcacagataatagtaatgtaggttactgggaagttgataaggtttacgaggtaacacgtaataaagaccttggcttagttatcgcaggggaaggtgaaaggagtcacagaaccgtaaagtatattttaggggtgttaaatggtgacagcaaaattaaatttgaagttgtagaggaaaagcctgtacgatttgctaaggtaacttgtgtataccctcctgatagaggtcttgtagaggttgggcattgttatgaagtgcttaaagagttccctacaggaagtgtgcgtatctaccttaatagtaaactagggaaccatgagttactcccagaccagtttgtctttgtagatgaaccatcaaatgatggagaaaaagacgtagaagagctagatgtagaagctaagatactagccaagattgaacagttaacagcagaagcagaacaactgtttgctaaacgtgaccgtgtaaatgagcaagcacttaacttaaatgcaaaagctcgtaagttagaagaatctttagaggtactaagggagtacatgtagctaagtgtttttatgattacatctattaaggagatgagagaatgatttattatattaattttttagaagatttcgcatcaagttggagtgcagataagcgttatcgtgttcgtagaattatgacaactggtagctacgctattattgacaactatggtcatgtcagattcagcagtgacacagcacgaggtgtccttaagaatatagagcaggagtatgccactcataaggttgagcttacactagcagaagaagaaacaacgaataagcctaggtttaaagtaggggaacgagtgaaagtgtctaatgatttacaggcattcgggatagaatataagactcacataacctctaagatgatgggctgtgcaggtaatgaggctactattacacgtgtttgggggagtaacgtacgctactttattaacatcgatggtatacaccaagattggtgttggacggaggacatgttagataagattgaagaagaacctacactatctattagatgtgttgaggcagttcatcccttttggacaaaaggtaaagcctacgagataaaccttacatctgatggtcgctatcgggtctgggatgacgaggaagatggtagcagtggcaaatccataaaagaactactggacgttatcaatagtggcggtaacaaatttgagctactagatgaaacaccctcagaagcagaacctaggctaaaccatgctatatctgacttagagaaaatagaagctaagattaccgctttatcagaagagtcttttcagctattcaataagagtgaagagttaagtactagagcaattgaactgcaagatgagtcaatagctttagaagaagcattgtatactattaaacaatatttataggaggagatttaaatgcgtaaaaatgtaatttgtagattagaatgtgtttcaaaagacaaagacaacttaggtgaatggactgtagataatatttaccctgtgtttgaatcagaactaggtaaagtatatatcctcgatgatgaaggtaccacttgttccagagatagcgtgtctcttattatctctagtatggctagctttggggtaacatttagggtagcaaaagataaagcagaagaccctatccctagcaatccacaaagcagtacatcattagaaatagttaaagggtatgaacacttagcggagtttatagactcattaagtagcaaccaacgtgtagtgtctcactcagtagaccctaactctcaatggcactatatcatttatgaaactaagtcagctgaattgggcggagtaaccctagaggaattactagacacactagtgtataatgtacatgttgtagtgatggaacgtagtaagagaacatatgagccactagaaaatcacacgtttaagtgggaatatggaacaaagaataccaaggattgggaaaaaattgtacctttattaggttgcaaggtgtttaatactaacctcaatagtaacagagggttccatattactattttgaaataaactgttgacaactactatagtccatgctatagtaggtacatagataaaaaacaaacaatattaggaggtagcatagagtgaaagaaacagaaaagaagtatagcagagagtataaggggctagaatttgaaattattatcacttattaccctgaacaagacatgtattttgtaattgtaaggaacggacagcaccgtacactaactaaggttacagggaaagagtggggaatgagccctcatacagaggaagctgttattgaggtagcacttgatacatgctacacctatattgaaaatcaagaagcgcaaaataactagattaaggagggactatgatggtaggagacttcattttatgggttaaacaagcatggaaagaaacattctgtattcatgactacacggttaaaggtgtatataaaacattagatagtcatgggtacttaaagtgtaaaaagtgtggaagaattaaataggaggacaacaacatgaaccagagacagaagactagacaagaaaataaatggtttgaggagcatgggtatgatacacagcaaccacgagaatgtattgagtgcggggctcctttaagttggaaagatgagttacagaaaagtcatggagtgtgtagtgagtattgttatatgagaagtgttgggctgtcgttatcagattttatttaaggagatgaaacactaatgtttaaaaaagataaaaaagaagaaaagacttatagagaaggagacctccttaaggctgtagggggttactacccagatgctaggttgagtttaggaatcacatatccattgtataaaaccaccaatgagggttggtatattatcaataacgaaggtagtcgggtaaccttaatcgaaatggatgctttaggcattgactacgctgtgatggaagaacccttattagaattaaaagaaggagacccattgctagtcgtgtccgaccttaagagaggtgttcgaggcttagcaggtgcagaagtacagtgtttaaacattaccggtgaaatggcttcactagcaggtacagttgttcattatgataaagatatgagccatattgcaaaggggctgttcactgttaaagagaacgattcttattggtgtgtagcgattgctattccactaaataaagtagctgaccctgattttgcattagagcatttgcttgctacgttaaataaaaaagcctctactaaacgtctggtattgaatgagataaaatatgatttaaaccttcttcacgaagagctagacgaggtgtccaacgaagtagagaagctaacaaaaaacattgaaacaatctataataacagataggaggtacttagatgagtatgccgagtgatttagggaaaacattaaagaaacctattgcaataaataagaatcctgatttttatgaattagcggtaggtggtaaagttatctacaacgaagaagtaatggagattgctaaagctttctctaataagaagaccaagtactacctactaaacacacgaagtaacaaacaagtatgtgtaccagtgtatcatgtaagaccttatgatacccaagtagagggtcttaaactaggtgatgtcctagatgctatgcacattatgacaactgtaacgttaagggcagtgaacaagcacgggtttgttgtcgatgaggatattattgaatgtttagtagatgacatcccagaaaatgcgcttattgttactagtgaggtatcccgtattcagccagaggattttggtaaggtaactattgactattttgtttagatatgttaggatagacttaagataggataggataaacttaggatgcgcttttgtttaggataggcttaggataagataggataaacttaggatagacttaggatagacttaggatgcactttggtttaggataggatgggggatataactatgagttacgttaacgagtttgaaacaattggagattggttagatagagaaatttatgatgtgttactaagagatgagcatgatattgaagaattagataattggggaatggctttgtttgcattaagtgaaggttacgttctaacagatggacttgacaaaccattcctagagttaactagagaagacctagtagcaggctacaaccactttaaagaagagctgaatgggtggttacgaggaggtaaactgctagaagtctctgataatttatctacaattcaggggttcagttttgaccatgacgatgttttattcttagaggataacaacaaagcttatgcaatgctagtaggtattatcattgaagcaagagacacatataaaaatggtttctgtaagggtcactatgtaataccttaccaagattgagttagccttatggctagctttttcttttaccctaagtagcaggctacaaaaatcttctaagtagcaggttgcaaaatcttctaagtagcaggctacaaaaatcttctaagtagcaggttgcaaaatcttctaagtagcaggctacaaaaatcttctaagtagcaggctacaaaaatcttctaagtagcaggctacaaaaatcttctaagtagcaggctacaaaaatcttctaagtagcaggttgcaaaatccggatgcgcccggctagcggtggggagtcaagccatgcgggttcaccttaatagctaccgtccccagattgtcggtttttcttactatatatagtaagaaaaataatttaaaaaaaataaacttttctattgacaaaaaacaaaagctagtataatatagagcgtgtaaggaacaacaataataaaaaaaataaagataaaggggcgctattaaaatgaacaagtataaatttacctatgcagacattaagaatttaccagaggaagaaaaagaaaaagaattaaaaaatcggtgtggtgttttagcggtagagtgcttaagcactaaacagctacaaaagaaaaaacctcgatttatggttttcttaaataccgttatttttgatagtaccgcagaaacaggcggacaatacgcaacggcaaccgttaaaaccgaaccgataggggacggacgttttcgagtgtgtgacggttggggacagctttctaatggaattattgaactgttaaaataatttataaaaaaaatattgacaaataacaaaagataaactacaataaacttgtcagataaagaagggaagttatgaacatgaatgaattagaagcagtgaaagaatggaataataaaattgaggaacaacaagaagtgctaaacaaggttattgttgctttttataaagaaattgacttaaaggttaaaatggtaaaccgtggcttgctagggcagttaccagcttttaacgaactaaaaggaatgctatcaggtatcgagctaacagcaaaggttattgcacccgataacgtgctgcctattacaacccacaactttttagaatatttatttctaggggataacgaacaacgagcatacgcaaaagaatacctagacggctttttaaaatcagtagaataaggggaggaaaattttcctcctttacataaaaaaaagattgacaagttaaaagaaccatgataacatataaatgtagacaagggaggggctttacatgatgaacggactaaaaaaacttgtgaaagctaggcaatacaagaaagaagtaaaaaaaattatcactatgcaaaagaaagcaataaacgaactagaaacattaaacaaaaatttaaaattaattaatcaaaactattgacaaataacaaaagataaactataataggtttataagataaagagaggaagttattgacatgacagaacaacaatttaaaaaagagcatttattagaaccaacagaatggcgtagtgggggctacttagacactagtttaattgaccaatcacaatcttattatattgagtcacgtccgagagtctacggcgggtgttacgtttaccaatatgttacaatgaaagatggcacggtttacgagctttacagcatgacggcaagcactaggggaattgttgcacataactgccacgctagaaacgtattgcaaagagatgtaaaacaatacagagatagcgccattcattattaaggaggggagggctttcctcctttacatagaaaaaaaattgttttatctattgacaaataacaaactatagtgtattataaatttataagataaagagaggaagttttaaatatgaaattatctaatattattctagtggggttgcttgttagcgttgtactactttggggctaccttagcattatgatttgcttacaagtttttagagcgttaggcggttgggatattagaacgttaacggtttgcagtggtttgctatttgcctatgttttcggtttaaaaggaatttgggaacaagggacagggaaaaacaaataaaaaaagtttataaaaaactattgacaaaaaacaaaatatagagtattataggcttataaagataaagagagggagttataaacatgaaattgaacgttattcatttactattttgcttatttcaagaacaagaaagctattctattttaagttacgaatcagtagacgaattttattctaggttaggttatgacttagagagtgagtggctacttagggacttaggtattaatggaacaagtgacttggtagagttgctaacagattacaataatttattagagaatgagataacaaaagcagtcttttctgataaatggttataatttaaataaaactattgacaaaaaacaaattaaggaggaagaataggggaaacggggagggagggacttcctccctttacatagactaggagggcttaaaatgacaacagaggagaaagcactaaacattgcagagaatagaggtataacagattataaggttagggggaacgtattaagctattatactagctacccgatggaaaaatgcacataccttgtaactattgacattgaaacgctagaagaagaaagaaaagaactcaaaaaatattataaaaaaggcttgcaaaatgcttgcttatagactataatataaagaggggtggcggttgttattaataagagaataaaaaaattacaatatgaaagaatcagaaagctagaaaagagaaaaagaggtgaaccacctgaatttattttcaacggtaactattcattggaagaaatagagctatttttacattttagaaaaaaaagtgagggcaaaaaatgagcgtggtggctttgcttggtttacttgtaaaaattacatttatttttaaattgttagcagataaaaaaagttaatcaaaactattgacaaataacaaaagataaactataataagtctatcagataaagagaggaatggtaaacatgacaaaagcagaactacaatataaaaaagcaataggagttgcagtctttgcaacaagtggaaaggataaaaagcaactaggaaacgtggcaccgtttagcatttatgagattttagaaattgacttaaataaaaatcgggtatattatgctttaaattgtggggaacgacatgcagtatgctttactaaactacgcaaagaagaagaaacagggaacgattttattttaatcaataaacaaccatttttcttaaaagatatgcacaaaggtttaagttggtcaaaaagtttataaaaaaactattgacaaataacaataactaatatacaataggtttataaaataaagagaggaagtttttaacatgacaaaagaaaacaacgtatttttaaatgaaaaagagctaatgaaagaagttattgacactttagaaaatggctttgatggttattattgcgacttacatggtgagatttttaatcatggagcaaatgctgacattaaagacttggaagaatatggaatttttaacgcaattggagaaatacaagaatacgaagaagaaaattttggggaggttttgacagacctaggaaacccgacggaggttaccaatacgctttactatattaaaggtcacgagtttttatatggtagattagactttaatgatgttttagcagatgttgcagaggggctaaaattagataaagacttatggaacgaggaagccaccgaggaagtgaacaaggctattattgagtgtttaaaaaaagaagtgccttatttaatagattagaaaaacagggaggagtttcctccctttacatagaaaaaaaatataaaataagggaagtgctaaacatggaaacattagaaaaattcggttatacatggcaaggaatgaaagaagttacaaaagaagaagcagagaaaaacattaagaacggggtcggcacttttctattatatccagataacaacaattgaagcagtgaaagaaagaaagcaatgcaatattagataaagtattgagagcttgcaacttgttaccaactgaaaagaacgtgcaaacagctaaaaactttttagaagaacaaggctttaaagtagaagctagtaaagagttagcgggaaaataccttgtaaaattttcaatttaataataaagaatgaagaggggaagttataaaaatgaaactaacagaaaaggaactaaacacaattttaagagatgatgaaacagggaacgggggaacggctttcttaggtgaaacactagccgacttcttagaagaatcaggtattgactttacaaacctaactattttagaagtaaatgaattactagaaaataatggaattgaaccaattgaggtagtgccatgttaaaaaatatcaaaaaatcagataaactcactagaaaagatatacaaggtttttggggagatgaaacaaaaacattagaagaatggtataagtcaatttcaaaagaatcagacaccgaaaaagtagaaactgctaaaatgattaatacattgaaagaatatgcaaataacaacgaatttcatttcgtaaaaggagagcaaggacaatgacaaacacaaacacaaacaaccaacaatggaatcagaagtttaatgatggtactatgaaccagaacaaccaacaaaaggaagttatcactttacaagtcgcagaaagtttcgtcagtcagattttaacaaaagaatattcggtgattggtttagttattctaatgttttattttatgtttggcatgtttggcattttcgggggtgcaatctatattgctttcactcacacaaaccgtaaaatcggggcatggcaacaagtaagaagcgtatacactattaaggaggaacaagaagaatggaacaattaaaagggctaacaattagagaattgattaagaaactagaagaagtgccagaagaaaataaggacttgcctatttatacttttgaaaatgaaaactctttgcctattaaagatatttcattatatgatgaaaatgctaaacactcacaagaaaacccgttaagttttgatgtaatcagataaggaggggcaaagatgaatagttttatgaataaacaagctaaacaggtaaaaagaagtaaagaaataaaactagtagaagaagtaagaagaaaaaacgtaaagaaacgtttttcagaggaagttagaaagtacctagaaaaagggtatataatcaggttagaaaataaagtttttccatttgctttaatatctattgacctagaaaaaggggaaaaggtcataagtcttattcttgtgaacgaatatgatggaatagcaaactatacagcaatgaaaaaggttaccttaagagaaaaagggaatagagctatcctaaaaagaacgttaacggataaagatataaaagtagtgagtatgtggaaaggaatataaaagaatgagtgtatacagtttaaaattactagcaatcttagggatagtattattcttttcagttatcgggatagtgtacgataataaacaggacgaaaagaaataaacatataaagaggtaaagagataaggaactatagagctatataaatgtgtacacttataggaataagaagaaaaggaactatatacctatacactcatacactcatattcagatagacacataataagtaagggtaaaggagagaggaggagggagagaaagaggaaagaggaaaaaagttgtttacctgagattttaaagaatcgactccatcaaaaacccgacaagggggcgcataagtctatttcaaaataatctgaaataagtatagttattactgtttatagatggttatccttaaatatctgaaaataggggcgtttatctgattatatagttagctatcttatactattaaccatctagcctattactgcattcattgctattatattctatatagggggcgcttatatcgtttatagtgtaattatgaggggaacgactaggaacgcttatacgggcttatagggggctttaaatgcataggctatttatacatatattagaatacacaaggaggaggggcggaaagttagtagattagactgttaaaaacaaacgggggatagatgcacattgttattttactgattgggctaggttaactagctaaaataagaatgctattgtagcaacgtttataagaaataggggtgtacttttcccctagggaggttttaaaagggtataaaattcttttgttatttaataaaaaagtccatcttagctattgacaaataacaacaactttggtattctatatttgtaagataaagaaagggagttatagacatggaatatacattagacgaattgctagaagaggaatatagcacactagacgaattgctagacagtagagaatttaaaaaacaaatggacaaccttaatcacgtcccacaaatgcaaccgcaaagccataacagcaatacgctagcagatacgggacgttatcctgaaaaataaaattgaaaaaaggggttgacaagttcagcccctagtggtattctatatttgtaagataaagaaagggagtttttattatgaatcattataaattatatgtagatatgaaagagggaactcacgattatgtttcggcaactgtctataatatacttgatgaaaaagttttagggttgccagatattaaaaaacctgagaacgtagcttactatactgatgaatggaaaaacgggctatattcttactatgaaaaactcgcaatatcagagttaaacgactacaacgctactttttcacatttataaaaaaattaaaaaaaactattgacaaaaaacaacaactagtgtattttattaagtgtaaggaggaacaaacctccttacaccacacaacaggaaggaagtttttactatgacagaatttgctaatatgaataaagaagaggtattggagctacttaatgattggtttggtgttagtgactatgatacagtgatggaagagttaggagagatgaaacaagttacctttacaggtagcacaaaccaacctctattaggtggtaacggtaacttaattagtttacctcaattctttaaaaataacgaagcagaatcagagttcccaacttatggagagctactagaggaactagagaaagatacatggaatctcgaagcagaggacaacacttacaattatagtggctttttagaaagtgaatcagattttaaagttattcaggcagaaaattcagacacgactattgcattctttgcaatccatacgggtatagacataagagcgggctactcaaaagcaatcccagttatttttgaaacttactatgatttttatgaatttctaggtaactacttttgtagtcaaggttactatgcttttaaacacgacaacaaggaatacacaatcagtttagacgtttcggctacctcagaatatgtacgaatttatatagctgatgaaaacaacgaggaactacagcaaggctatgaacaagaaacttgtatggacttagacatagaaagcgtagaaggatacttgaaagaggaaggaattgagtttactgacttaaaacccgcattgtaaccatataaggcactagggagcttatacaatagagctacaagcctcctagtgtaattataaggtaaataactagaaacgcttatacgaaagaatagggggctttaaaatgacaacggatgaattaaaagagttttactatgaaaacgggattgacttgtggaatgataacctatattttgaacaagttgtttctagtggtggatggtactacgacaatgaacgcggtttatggtttaattatgaggattaaaaatttaaacttttctattgacaaaaaacaaaaactttggtattctatacttgtaagataaatagagaggggaactaataaaaatgaaactaaaagactttatcaaactagcagaatccaagggcgctacattagaagcatacaacgagctaggaggttatgaactaactagaggggacacagtagacccgaatccggttttgattgcttacatgcaaggggcttacagcgtagaaataccaaacaaggaactagaaaacaaggagttaacagaactagcgtttgtctataaaaatgtaagtcttatttatccaaatgaaaaagaactattgtcaggactaggactatagcacaacggcatataaagcccgtagcgaggttttagcgggctttatatataaataccttaaggaggaaacaaggtgcttacagtggaaaataagggcgttaggtggctagtgagtaaagaagcatggaaagcaggctttgctatggaggtgctaggcttgccagattgtaaaattagtacagtattaaaatcggtctataaaattattatctaactatttaaactaatctattgacaaataacaaaaactttggtattctatacatgtaagataaataaaacaaaagaaagagagtgacaagaatggaaacgaacaaagcatatgaaagactattgaaagaagtagaaaacttacagaatgatttaatggatatcgaggactattcagaagaagtatatcaagcctttcaaagattaatcgaagaactcgaagaggtaaccgaatagggctagaccagtcctataggtatataccagttgacccgcccccgtggttttttgaccgtactttgggggtggggctatttgcctaccccgaccctggggtataaatttttttgtagctagaaaatttttatatatttataaagtcaacaccccacatataaagtcaacataagggctcaccctagggctcctatataggctcacctaaatactcccatataaaaaagacccctccccgttgataaggataggtcttttttatttagccgtctgccctatgattggttattaggttcaggttccgccatagtctttgcgaagtatgtccagtatttatggaagtctgcaaagtccaagaagtactccccgacaatctctcctgcttgattgcggtaaagtggtactttcgttttctcgtctttatggactccatactctgtgccatttaatgaaatccatacaatatccggagtcacactagttactgttgccttatcacaacctagtatcgggtcacgaagttctggttttgtgaaaactgtatccccaaccttcaatttgtctagtcgctctttgtctattaatgttgtctccatttgttctccctccttatacattataaaaaatatttaacgtctaattactgccctcaaataaagaacattactacccatccaataagcataaataacaatgttgatacagtagcttttgcaaataccatcaaaatagaatcttctgtatttgtagtagtcttagctgtaataaaactaataaatacatctagcccaattgcctgcgcccatgtaagtgttaacaccccaaatgttggggcaattaacccgttccacaagaacatcgtaacataccctccaatagcaagggtcaacaccactagaactaaagtcccaaaaaatttacctaatgcatttgccaattcgtcttttgtattcttatccatcgttttcctccttaataatagctatatttacctcttatttttttgttaattctatttaggcttgcaaaagtaattatgttcaagatatatgcgccaattactgatactgcctgcattgtgcaaaacacgattgttatccagtagcttgtagtagcttccccgctagttagcccccaataaatgctatatgtcaccatgagtgtgtttagcagtatagctacccctcctaccaataatagtaggtaaccagatagtttcatttagttcccctccattgaatgattaagtaagctcttgttcagttcttttaagtaatagtcacacctaacgtgcacaagacccatacgttcccttgtaatagggttataatgtaatcgtgtaggtactgtgtactcattaggtatagataagtctaattgggtagttaaattgactactctatccggagggcacatccatagaggcttattacagtgccaacatgtcccactttgtagtacctcgtattttcgtttaagttgtttctcttcttctattgttaattagtcgtgatagcactgtgtcattgcgtatggctccctccgcttttatatttgttatagtttagtgttaaaccagtcctatatcctctcctagcgtttacaatagttgtttaaggtgataataggtagaatacctatcaccgccctaagaggcatatagggtacttataggactggtgtttagttaactgttttaagtggcataaaaaatatgcgcttaagtcaacattagttcttttactttagatgatgtcaattgcaatataatgatttgttttggatacattagcaatttcataatctaagtatggttctagtacttcgttgttacttcctatctttgttctaactgttatggtagcccctgccgtgggataagtaatgagtacgtccactccgggcttcattaacttaactaaatcttttaacttcatctttatctcctctttaatagcatatgcttaaatctattttatgtcaactgcttaatttttgtgctcgtagttgcacagatattgtatcaacaatgactgcccactgctcctccgtaaaattgaagtcaaactgtgtatagtcttcctcacctgttgtagtaattgcaatgtctccataatcatcaactgagaaatagatagttgcagtcgcattttcctccggattttgaggaagtgtaatagctaactctccttgctctactttcatctattgcccccccttagctctcttccttctcaatcatcttgatacctgtaaaggcatatacagggagttcttctgtgtaagtgtactgattagctttaaaggtaacttcgtagtaactctccatgccacagtgtaacatgtctacatatctaatttccttacaaggcatagcatttttctcactcccacagaagagccagtcttctgtacagtattctactctacctgtgtggatacttctaactgctacgtatggtttttccatctattcttcctcctgtgtaatctcttctaggtcacaagggtgtacatctagtgttcctgtccttagactataacgagagtttcctcgtactgcgtaaacaccatctgggtatactttttcaagatatacagtatccccaattgtaaacccatggtcataacgggtatccccaataaccttaaactgtctttttatcgtatacccatacatgtaagcccgtgctaatacgtattggttaccctcatcaatccattcaactagcttgtcatctggtgtttcatcgtatgggtcaaaatactcattagctaataagctcaacattgaatcgtactttttgattgctcgtgcaacaaaactaggtatctctacttttttagccatctattcttcctcctatttaatcataatacatacaaaatacataaaaaagctaacatcagcaaaacaccaccccatccagctgttacatatgacatatagaaaacgtatataaggtatgttactgctataattgttaataatacaagtatcgtgttaatgagcttttctaaatcaatcattatacaacctcctagtcctcacaagtgcgagtctggttcttattatactcttactcctacttatatccaaagaactttaagtaattttctgcttctttttctaagtgctcgtttagttcatctagggtaacaactttcccacagtcctcacaggtgtaggtctggttcttcttatcttctagcagttcaccatcacatacaaggttgatacaatgggttgtccaactccctacatcatcaggtaagtgccccattatacgtcacctacttttacggcaaatgccatgaatcgttcatccattttgcggatttctttctctgtaaaggtagggatgtcttttaggtagtttgtaaagtcaggagaccctaatcggtcgatatagctatatccccaaccatctttatcttttgcaataatgatgtagtactcgtcttcttcttcctctaccgtatgacctagtacccatgctttggcaagtttctcatggttttctgggttattagctaaccaaaagtacatcttactagggtagcttcctttgtcaatcatgttaataaacgttaagttctcttctttgcacttgtcaatatatttccctactttataaggaataacaactttttcaggttcgtctaaatcatatgctaaggagactgcttttgctatccctgtattgtagcctagagcatgggggttcaatgtaccgtcacaccctacttgagtaaaaacctcgtcacttagtctactaataaattcattcttattcatttagttccctccttaaaaatcaagactgttttcaataagttctgatagtcggagcattacctcatgaggtagctctaattttgtactctcctgtgagtctgcggagctgacttccaaagtatattttacttctgttttctcatttacacgggaagccttcttctcaacacatactttataaagtgctgagttattgactgcgataattttttcttgtgtatttacactagtattgctatcataagtaatttcatagcccattataaaaccctcctatttgtatactggtacagcaaaagcccagtatctttcatcaatttcttttatttcttgttcggtaaatttgctcttacccatgttgggtttatttgagaagtatacttcattattgtgggatgtttcaacccaaagataacaatcttctcctttattaccaagaccagtaaacacgacatggtaaagtggttctttctccacctcatatccatctttcattcgtattaaagtttcaatagggttattcttactttggtctaaccaacaatcgaactctgattcatgtgggtagctgttgccatctaacattctaatttgtgtaaaaatagctaggtctaatgcatgtttattttcctcgtaccattccgcaacaaactttggcacaattacttttttaggttcgtctagctgttttgctaaagagattgcgctaataattgatagatttgacactatacgataaggtgttttactagattcttttagttcttctaattttttaatcaattcttgtttattcatttaatttctttcctttctttcaatagcccactggctgaatgcttgtaagacttgcaactgcgcaatttctgtcatgtatctataatttttataaacagggctattccgataatctgtttttgtagaattggctctcagtctccaaaatagttctataggttcaatatctgttaacgtatatttttcttttaaccaacccaaaacaatttgttgattctcacttagttctacttggtctaccttatcatcagtgtatttgaaccagattttctcatatgttgtttgtccgcctgtgattgttacaaattcggcgcttggttgctcattttgaaatttttctagttgttcttcgtaatgtatatccccaacatcaaattctttaaatttaatcattgtactccccctgttctaaaaaccaatcagtaaatgcttgaataacttgcgcttcctccgttactgataaagagtaatatgcctcttctgttttagggtcttcataggtctccccaatacgttcgagcgcctcaaataaggaatctttactacagtaacctacttttaaccattcaaatacctgtttctgatttttattcagttctggctttttaactgcctctactgcagtcttatacgctatttttaaaaggtctccttcaaaactattagggaaattaatttcaccatttgctttcatatacatatagcaaactctatcaattatttcgttatatctttgtctactcattcactatccctcctcgtcctctacgtcaccccaaccaaagctacagtaggaagagaacacgtctctagctacttcgtctatctcctcattcgtagcattatcgggtacttctactgtctctatttcaccaatacctgcccaagttgtctcaatatatacatttatttttcgcatagtttaatacctaagactacatagtcgtctttctgtgcataatcggtgatataagtaacttctactttaataaactctcctgtatacgaaccacatgtgtactcatttaataaaagaatatctcccacatggtattgtctatcatttttacgtatttcaaatagttttctaccttccttaactgctttaaagtacgtaggtgcaatcttgaggttatgagtaacttctaatttactaactaaatcaaaaatgatagtgtttaatttgttaccctctacctgatgattcaatttttgtaaagttgttgatattacagtatgcctaccttctctatcaataactgagtttcttctgttatacttagtaagtctttccttttctgcttttgcctgtgctagtccatttattgttttagatacttttacttctccatttacaataacttgtactaggtatctgtcgtcctttgttgcaaacttattatccataattagtacctctctttcataatcttaattgaccagttatcgttgttactgaatacccgttctaggtcattcaatgagttggtatttacaatttctttttttagttttctatctgaattaatattaccaaatcgtttaaggaatctttgtttaaagtgggcataacccatatagtcgaaggtaataacgtgttctttaccaaatataccccgctctcttaacttaatctctacactctcataagagctatctactttcataaaattatttagaagagtgtgcaaatcaatacaaatagatgcccctgcactaccgcctataagtatatatttagggcactttatatcggggtaacaaggggcatctaattcataccacatattatttacgtctaccccataccatacactatttacatctactgaggctctttctgtcttaaatggttttatgcaagtatatttcattgtctctcctccaaatcgtctagtacgtcttctaatgttgtgacaaccccctgcaaataaccaagttcatgccacccataccctctcttatcttgctctaacaaattattaattctttttgttttacgtttaatttgccggttatatcttctttttagtccctcttcaaaggtcactaccttttttgcttcctctatatcttttaataattggtctagcccatctccattagtgccatagctatacactagcgctttctcgtccttataggtagttacccctaatgattggtatacatacttcttactggggacaaatacaagagtaatgggtctgtacaattgaggtaaaagacaatcttctgacagcccaccaaaatctgttttagaagataccttctctaccacatacctcatatcttccatacttaacgacttaatacataaaatatatctgttaataaccattttctttagctccccctacacccaaaatagttttcgattctctgttggtttaaaagactccaattctcgtgaagtattactttttccatctgttaaaccttctttcactttatatattaaaaaaaataaatctagctatctacaaatacattgtatcatcagctagattaaaagtcaacactttatatttaattattttatattacaatagttctttatctaaaattattttagggatagcccatattgtagtgtaacgaacccctttatggttacctgtaactaatacgaacgttgccgtgtctagcttagtaccgagtacagatgctagtagttcgtggtcttctttgctaattggtacttcaaaatcaagttctccaagctctaccacaaagttatttgctctaattcccataaagtattcatcattacgttttacatggaatatattcttcgtatgaaaactttgcataacaatatttgcaaaataactgttatccctagctacaataaatctatctacatagatagcctctttactgagtagttcttcaatgcagttactcataacatattctcctcctcttctaatagtagctctgatacgtaaatttccatcattagactttgttcaatcccgtctagtaataaatgcatagcacacaagccacacaacatttcatctaaataaaaatcaccacatgtctcctctaatggtacttgacacattaaacactctatcattgtacagccctccttaatttaagttttctctaacttctgttagcacctctcctaatagattaagtccttcccatttactcatatcacgagagcgtgggtctgattcacgtaaccctattccccatactttatcaaaaggtgatgcctctgcaaacttggttcctttagggatggatagcataaagttacgtaaactatcattttgtgtgaatttataagtatttccagctaaaacgattgatttacgatgctttacccacaagtcttcttcaaaatttttaacttgtctacctaaacgtttagcatcttttgggctctctgtttttaaaattctttttgctgtatcgacatcattaaaaagcattgctttacgtaccatcatgtagtgctctgctgtcgggaaaataatagcttcccctaaacccttaataggtgcactgaactgtgatgggtaccactgtgacaagcactcttttcctagtttattacgtttgcttggggtatgtccccaaaataaaatatatttactcatttaatgttcctcccaatattcatagtagtttcccttatgttcaaaaacaaaatgagggctaggtaactcaccattaacttctatatgctctgggttattataagaatagtagggttcgttaccagtaggactaattgctattactggtttatctttaaaaaatggtggtattttatctccatcatttaagtttaatttataggtacttaatggcacgcttctacgatgccctttcagtgttgtatactcctcaagactaattattctaaggaaacccttagcttttagaggcgctaaactgtctatcgaaacgtcttcttgcttataagtgacaagggcgctataaatggttgaggggtttttgtatgccactgaataattaattgaagtgtgcttatggtttgctaaaaatttctctaattccttagataaaccataaggtgtatcactatcaataacttttactttaatcatgtgttatcctccctatatgcttctctaactgttcctatactttggtctgggtctggtttactaaatggtaagcttgcacgctcttccttactcaatgtttttaagcaagccacatgtactgcaatgacccctgacttagcttccatactatccgggagtgtaagtatatagtcattatacagtttacttaacactagccaataacgattgctactacttttcatattagctaaaatcatcattttttcatagtaatcttgccccatacaagaaagtcctcctattgcagattggaggagctcatcttcaagagctaagatagtatttgcgtaccctttcagctccttgttaagcccctctatagcaatctcaaaacattctctttctggagagcctacagttaaatcattaagtggctcatatgctcttacttctctcccactaggggcttgtcttcgtttacctatacgataagagtctttaaactcatactcggaacgaaaaatttcttcttgactatttcttccagaccttcctccaaaatagcaatcttctactactccaccaagaccattataatgtcctctagttgtccctatgactttagaatgtctaatatgggttagctgacagagctcccctccgttatcagggtcacctacaatagctgtctcacatacaggacagatatatccaaaacacatcactttatctacctccaattaatatacattaagaaaaagttacaattttttcacaaggaatatcatagtatgcctttaaaccataatgttccaacatgtattctttagcataatctacaaggtgctcagggcatttaaatgtgtaagagccactcatcattacaccactattacttaactcttctctcgaagctttagcaaaccacttagcacactctacaggataaccaataacacaccctaaaacttcctcgtcattaaaccctagcttaattgattcattgtatacttctatactcatcttatctgatgttactaggtatatactaccatataacctcgttttatagtaagagcgttccagatggcttagctcttcttcccctaatacgattgctacacgatgacctaaattaaaatctaaaataggctttggaaaaacgtattctgctttctcaacaaactccacttagccaccccttttctcattccctaaattatcttaaatgctgtattagttagaacggtaagtcactattgtgttcttcctcttctgggatatataggatattttcaatcttttcttcaatatgtccaataatctctgtgtgctctttaattttctctttatgattttctctttgcttatttaactttgcatattgctgtaattcatctggtgttagctcttctagtctttttttcatttgttttctccttctaatgtaattttctctacgtcatcaacactaccaaaagatgggggctgtgtcaagttcttatctaaccagttagcgataatgtcatgtaactcgtctatagcctcatcgcttacttcatccgttgggtagtagtcctccgctacttctccatattcactgtatagctgttcccctacagattctaacatacctactacatctacactaataactgctttattgaactgccctactgcaaagcttgttgttcccttttcaggtaatgctccaaatatatcctctacgtgcatccctaagctatctacatatgtttttccttcattaatggacaataatgcaagttttcctgcagacactgcctcttctctcgtagagaacgtctcacacgctttccatacatctgtgtcttcctctagtgctaatacatagtctttatcttccattgtcttgccctctctatccttttaatataatcatatttgtattactgtctagttgccatccatcaaattctaagtagtggtcataagggttaattggttcacctacaactatatagtcctctagtgcgtgaccttggtcttttagctctagtaattcgtctaataaatcttgtgctgtcaaattattcatgccatatagtatcctttctctttagcttcttcccactcatctacagaaaacaaacgctcattccgagacaaagagccataacagtttactgttaagtctaccataaggaagtccttaccgtattgttttgtccaactctctgtatatggtgttactgagtgcacttctttaatatattgctctaacatattcattttatgttaccctttcttggtttaaattttcgtgtttgtgttcggttgtttctacttacttctttgtatctacggattcctaatgccttagattctgggcgagaacgacctatctgtcttacatataagtctagcgcttcttttactttatcatcatacatcttccctaattctcggaaatactcaaactcacctaaatacacataaggcatacgccagtcatctagggtagccgttaccattgttcgtttgtttaaatcataattatagatatatagaaacactatataagcacctgtcatcacagaatagcttgtcctaatttcacttagagttacgctgtctcttaatgatgttaaataaccattccacttttttttacgttcttctgctaaagtttctatgaagtagtttacctctttttcgtccctcaccacttgctacctccttgttgtttatgtctatatattatcatctactttgttatatgtcaacacctttgtaataaaaaagaacctagtaatttacttacttaggctctcttgtttatacgtgtttagtaagttacctttactatcgacaacaacagcattaagctgaccaccatatgcacaggcaccatcaatgaaaatacttctatcacctaagaagacatcgtagctgttctcttttctcaaattaattgtgggtgtgtgacccattacaattgtcttatctgttttattcttctgtaacgctagcggtctcgtccaaatcatttcatctttagtggctgttttccaatcaggctgacgataaacaggtatccctgcgtgtacacataaggtgtctccatgctcatagtatggttctaataaactaattacttcaactacatttgttttttctaataacatctttctagtggtaaacgcatcctgtaggtgttcatctaaatccaatagactacttattgttttatcaccgccattgtacatccacattgcgtacatctcacttaggtcttcgtagtctgcttctcttatcaatggaaatgttaaaaaatctaataacatttggtcatgatttcctaacaaagcagttcctccattaataatatgcttataaacgaaacccagtacttctgcggatttgctacccctatctacgtagtcacctaaaagtattaagtcctcttcatcactattccaatgtttattaagaagcattattagctcatcatagcaaccatgtatatctgatacaataaatactttatctttcaatgaataatagcccctttaactacttctgctagccaataagtagctagtactagtacagtattgacaataaatgttattactataaccagtgctaacttataatttttactcctagcattatagtttatataattttttatgttaactctaatatttttaaacaaagcactcccatatacgttcagtgctatatatagtaaaagcaatacgataaagtagccttgagctagaaacacgtcagactccctgaacgagttattaaaccatatgctaaatatcgcaatcacttggtgaattataagcattgcgccattaccaaaaagaagtatactaaacgctataccgactacgtctctgtactctgaaagtagtctatcatatactattatccctttagtaaaaataaaagcaacaactgccatctgtataagtaaaaatattgttacggctaataagttttctgtatgcatagtcataatttagccactcctttcaaaatgggtaaagaaagaataataggtatatcgttctttttctaccctaccttcatgtataaaggtaaactcaacaaacttaactcttagcggtatatctggtgctttctcccaaggaagtactcttgggaaatcatagaatactcttgtggggtaaacttctttcataagtatcctagggtatcttttctttggtataaatcttttacctattatacttgagtagtcaggtttcattgtaagtcaccatgaatagagtatgctctatttgctttgttaaagtttacttgttttttgtttactaatcttattgcatcttctaataaaagaggttttcctaatttatggttatctaattctggtgagtctacccctacattcagtaagtttggttcgggtctggctaactcatgaatgtgcccatgtagattaattaggttatctctatctcctaaaattagtgggtaatgtgtcatatgcacaaccttatgcattcgttttaaaataataccaacgtcttcccaatgaaccctatcattcagggaagtattgcgtttaatctcttttcgtagaggactattatcgtggttaccctttattagccatatagtgccatttaagcgctctaagacgttagctatactatttaccttggcacccattgcaaagtctcctaggtgatatacaatgtcctctgggcgtactgtagcattccactctctaattaagtattcgttcatctcttccacatctttaaattgtttccgtgtgtccataaaagaggcttccccacaaatgtttctatggaagaagtgcatatcagatattacatattctctccccatacttgctcctccttagtgtgttgcaaaccatacgaatacagctagttgtagatagtgtactgtttggtcgataattagttgtgtctttttattaggtactgtttttaagaaccatgcactttgtgcttttaaatagtccatgataaaatgtggaacccataagcatactacaattagcccaagttttactggtgttcctaagaacaatgtagttgcgacaataatatacgtccagatgtttacatggatgattagtagatataaatcagtctgctttccttttgcgatatagtcactttgtaaggcatagtcccctactgcatgagccattgtaaggataattacatagtataagtaattcaaattaagtcctcctctttgtatgggtaaggacaagtgtcacattcaaatccatattcgttaggtgctccctctaaaatatttccgccacattctgggcaagttgctagtttcattgttctgcctcctttacatgatttcaagatatagccctgcacttggtgttgtagaaatcagcataacttctaggtctaagtgttctccgataccttcgtattgttcaataagtggttttgtttctgataaagtgaatgttacaatttcttcatccgtcatgtgctctactaatgtgactgtgcgaccaaattcaatatgttgtaataaatgtcctagtttaatcattataatttcccccatcaattaataatagtaagataccacctatcacaagtaaccagaatactgctaagattagtaccatttagttgtcctccttgaacagctcatcgtataattcttgaattgcctcacgctttacttttaacattgcaatctgtgctgatatgatattgcttggttttcccaccaaacgtccctctaagtgcccaatatccatattgtattgaataagggtttgttgaaatttttttctaatctctgtgcgttcattaattggttgctctggttcaatctcaaacagttcaaacattgaacgccagcgcccatttacgttattcaataattcactaggtgtgcccccaatatctactgtgtcatacccattgtctttaaagaagtagcccaccgtttcgttgtgataaacaggatattctctcccttctatgaactgtggttctagtgcatctgcttttgtacatttaattccgtatgtcattttattaaacctcccattccttaatgatgtattggcttttatagtttgcatagaaatctgagtcacttgagaagtatatatctagttcttttactttttctagtactccttgaagggatgtaccaactgccatgttagtacctgtccccttatcaattccgagatagagtgtaagtttctttggttctgcaccgagcaattcaaacttagaatgccaatagttatttaattcagctaatagtagctcaggagtggctcctgattctataatgtctccctcatcatctctaaggaagtaacctctagcatcatcatagaatacatcgtactctttaccttctgtgaagatatgctctgttttaagtgtacatctaatttttactgtcattctaattttcctccaattcaatttcttttattgatacaaagccaagtatattgcggaaagtacggtcttcattccagtatataaattgtgttagaagtggtttgtggtcatctgtgtatgttgttttttgtctcgtagtagctttcttcaatttgttcatcaatattttgtaccatttcattataatatgtgactgctttatcatatgaggtgaaagccctcatttttaccgctctatactcaaatttcactaaccatgctgagcttaatttcgtcatttatttcttcctccacttctttgattgacttgattatatatctatggttctctctaaatgcgtggtaagcatcatcaagtgaatatgcgtataatcttgttgtttgcattacagttctatatccgttacgtccaaccattggttcgtcaacttctacttctaactcaaataatagttgttttctaatcattgtttttactccccttttctatgatataatattaccctactattatgattctgtcaacaggcaaaaaaaagaagtagaaaaatctactcctattcatcgtttgacaacttttccataccatatagtaactgtagtagtacatatagtacaatatcaaatccgtcaagtggctttccaagtactataactttaacaattgtcaataccgctaaaaaaataaatagccacccgattattttatttgcatgttttctaattctcataactttctagtacctcttcaatattctttctggtttcgttagctaacttaccagtccgttcaagccaacctctaaccatttctttttctactttgctatgtttattcgcatcctccttgataccttctacattttccatcaagttatctaagtcctccataacatctaataaagtgtttcttagttttaacacatcgatagacaactcatagttccgtttagacaatttttcgttacggataaagttcttttttagttcttgttgtgtttctagtagctgagtagttttaataatatcagcttctaatttactaattccgtctagttcattcatcacatgtcctcctcatattctactacttcctcaataagtttcagtacttcttctgctgtgcccactgtgctatagtccgcaaagttttctgcaggtttcataatagccactgaatagggtttgttctctacataaatatgcccgaatccttttaaagaatgaattacctctactgcccatccattagcgtactcttctcggtatactacttgctcactggttgctcttactggtttattcattgttaaaaccatagaagtttcttacaatgttttctacacgttccatgccctctaagtagctacgtttctcaggggagatatagttcttgtaatgagggacttccttctcttcctctacctcttttgtagtacgttcaatcagtttaataagttttacttcgttctctagttgagactggataatgtctaacagttcatttttcgagcagttgtttagtggtttacttccatagtcaataattgtcatagtagtcctcctattttaatgtgtactctttatatcctttatgtgtatcgtgcccgcactttgtacaaaagcctgcttgttcaatatctattgaagagtaccctgtttgtactgcatacgtctcataagtatggtcacacgtatcttcttctgattcatctattttctctaaacgaatagcctctccttctgccacttcgtggttaaagagcaatactgcagttttaataggctcatatacctctgggtggacggcttcattcatcttaaagctatttccactaaattcattgaaagcatctagccattcctgactgttctcataagatacaattctgtaattcatacgaaagctcctctcgtgttttcttaaataaccagtaccgttcatcaatttcttttatctctgcctctgttaaatagaagtcttttaatttggatagggtatcttgactcaatggctcgtttctaggtagtatacttactgctaactgcccgtccttgcgtaatagtaacccgtagtctctctcctgtttctgaggcattactacatagtacttaggtaaactagcagtgtttgctactgcttgaataaaagtatctgtattagcaaagaaccatttactaaactctgacttggggtactcacatgcgtgtctctgcccttccaagataatttgtaacttatccataagttgttctcgttgtttatcaataaactcttttacctgttttggtacttctacctcattattcatagtttgtctcctttgttatactttgtcaatagtgatatacacatacttgccctctaactgcttaacaatatctagtatgtcatgaccacctagcttaaatgtgtttgtctcaaacccttcgatagtaaaggaagaccaaccgtaccaaccttcttcaaagtccaagacccccatagatttaagtactatatttttagtgatgtcttctaatgaagtacgttctacagcagagaaaatctgaatctctgcgttatcaagatgatacttagaagaaatgcctccatcgtactcctcttctgttgtagtgtcctcagctcctaacgcatacagtgcattacaaataagcatgtttaaggctctgtgctcatggtgatactcaatttcttttactttttcttttattaagtaaggttcgtttgtttctgcaccggggctgttatcaatagttacccaaccttttaatatctgtttacccatgattgctcatccttcctttagtacagcctatcgctgtcaccagtaaatctaaattttcctttgtcagagttactgtttgttcatgtacacagtccggtctaaatacctctactgtacgatttactacagcaatatctacagtatcttccgttgtctggcttaccttgataaactgtttggaaaactccccacggctaacaccttctatcataagctccatttttttatagcctcctctctggaaagtccatgaaagttgtggaaagtacgctcttgtagttcatctactgtatttggtaatgtacgaaattcgtctacccctagtgaaatacttgaggctacctcttcataataacatttaacgtctactcccattttaccataaggtaacaccattacttctatatgaaactcatatggagcattctgtgttaatggttcgtataataaccatgtctcatgatagtttacaggaatatctaatagtaaactgtttaaatcatctagctgttcagataagtatgcaattcttgtcattttacggtcttctgctataggcattgaacaacctaacgtgtcttttatttctttaatttctttggtaagctcagccattaattcaattattttataaaacatttctattccctctcttctatatattccccttcttctaagaaaaagcaagcaggttctccctctccattttcagtatcacctaggtattcatcatctaagaatgcacagtatccagttgagtagagggttacacagtccttatggtacatcgaatcgtccgttaaccgcacaacctcgtccatctcactgaacacttcattacacgccccgcatgatactaactccttactcataggctgcctcctttatctattacgtagtctaccagttctctaataacctctgcctcctctacactagagaggtctgcccaaacttgaagtgtcgcatcgttagccttaccagatattaaattgtgtaagctatctgcaatagttagctttgtacgttcaagatagtgaattagccagactaatacaattagctgtttctcagttagctcagtattagtctttgtgtaaacctcatagttatctaaggttaatgggaatgtttcttcattattaattacttgaaacccgttatttggttcgttttcatattctccataagttactctcttacctatttttagttttacatagatgtctttaccttctttgtgtagtttatctaggtcactattataccactctcttgtttcaattttagtaagttccataaagctaaccctccttactgagttccttgatacgttgtttgatttctgcttctgttttctctagttgtcgcattttgtttttatgtcgagataattcatgttcctttgcagtttctgccattgctaataagttttctaagcttgctgtatttgccattagattgccacctcatagttaaattttccattatgtttatagtttactactttaatttctgatagtggggaatcaaagaagttcctccccttctcccatggtaagataagttctggcacttcttctgatattggtgcattcacctgttgttcaataagttctaaatgtcgttcgtaaatgtgtgcgttatcactcgtccaatataagttacctaactctaaccctacagtatttgccataaccaattgtaatgcatgatactgaataatattaaatggaagtcctaagcaaacatccgaagaccgagccttcacatgtaagtttaatttaccctctacaactgtccagtgagttgtccatacacatggctctaatgacatatcgtataaatcttccacgttccataaagtagtcataattctacgagagtttggtgtgctcttaagttgttcaataactgcctctacctgatttagctttaggtatggttgatgtgttcctgctatcccaccaccttttttaggtacgacttttggaataagtgaacctgctttgcgatttttagctaactcaacatctccactataaacaggaataaaacgttctttgttaaataatgcgtaaccatacgcttttccaatagtgccatcttcttgctcccattcgttccaaatagttacacctcgttcttttaaccacgaaacctcgttagacatttcttgccaaatccactgcaattctgttagcgcccatttaatacctacatgcttactacgtaataaaggagcccccatatctggtgtaattgtaaagtttacaccttcaataaacttagttgttgcaggagttccatcagcatatactgcacgagtaccttctggtagctctgttactccgttcttaataatatccattactaaatctttataaattttatcaaaatccatgttgtgccctcctacatttcttttccctataatagaaatatatcatatctaaatttaaaagtcaacaaaatattataaaaaaaatatgagacatattggtatgtctcatatctactaaattctatactaaactggctagcttgtctaaagcgttatagtccgcatcggttactggttctactttacctaataagtacccattacctacctgagagaagaagtcatggttactagttgttgtagagataccattcattacaatagggtttacgtctgcacttgttgttgggaataaagggttcatccctaagttagctagagctttatttaaattgtactccaaaaatgtattaacatcttttgtccaaccaatctcactatatagttcagcagtatactgtgtttcgttctcccataatttaaatgctaaatcaattacccattgttccatttctttttgttcagtttctggtaactggttaaaccctaactggtatttatagccgatataggttccatgtacagactcgtcacgaataattaatttaataatttcggctgtattaaccatttttgcctcacctaaatagcgtagtggtgtgtaaaaacctgagtaaaataggaagctctccaatagtacggatgcactctttttctgtagtggtgtaccgtttcgataaatatcgttaataatgttagctttatattgtaaacgtttatttgtagctacccattcaaagatattgtcaatctctgtaggtgtattaaatgtgctaaaaattgttgaataacttttagcgtgtactgcttccataaaggctatgttatttaaaacagcttcttcatgctgtgttcttacatcatcaagtagtgagtgtacccccgattctgattgaactgtgtctagtaatgttaacccaccaaacactttatttattaaatcttgctccatatcagagagctttgcccaatcattaacatcgttacctacagggacacgtgtgtccaaccaaaattgctcagtaagctttttccatgtggcttggtcaattacatcatcaatcttattccagttaattccttcatacttttcttgcaaattcatgtgctcatctccttaaattgtacaactttcacactctgaaacccctacttcgcttccgtcttcttcggtgaatgttctaacataataaattgtttttataccttttttccatgcataatgtcttaataaagttaagtcccgagtggatgtagcgccaccctccaccttccaaggataaagattttctggtaactctgagcgcataaacaatgttaaactcataccttggtcaatatgtttttgtgctgttgcgtacacgttgattacgtcaatcatacttgtattgtacgctgacttgtaatatggaattgtcttctcagataaccggggtgcagggtaataagttttacctgttttcccatcttgacgttcttcaatcatagagataattgggtgcaatgaagaagtagtctcattaacataagcaatactaccattcgtttataccgttactttcgtaatactttaacactgctcttagcagtcggactagactataccttatactatcccaaaatagtaccaactattatagtcgttggacgtccctcattttacagaggtttcgatgctgatttcccattgtattacccttagcacctgtaacaaggcttttatttcagcataggctatctaactaattttttctgctttcgcaacattcacgctcaccgtttccagtcacgttgtagtttagttagctttagggggttccagcaatttaagttgtttttgactcatattcacatatgagaaagcccaatattatttaggcgccacagctaaacggttttgatggtatagaccaccttcaataatactgtttcttaatgtttcccaatcttttacattaggtagtaccactccatcaaatacttccgccaccttactagagatttcctgatttagtgttggtacatattcatcaaagtaagaaccgtctgcgtatttagagttctcaaagttatggaatgttgtgccacgctctttagcaatcttattacttgccaccaaagtagcatagttaattaattcaaacagagcatccgtcatttcaatagattcaggtgagccatattctacttggttacttgcgaaccacgcatgtagccccattgcccctaaaccaattgtatgggctttatcattaccattcttgatagtaggtactgcttttatatttgacacatctgtaatatatgttagagctcttaccatcgtctcaattgatgccactacatcattagatgtttctaacaagttaaggatgttaattgaacctaaattacagctaatgtctgtacctaactcttcgtatacttgttcatcatttagcttagatggtgtctgtacctgtaatatttcactgcataaattactcataatgattttgccatcaataggattggctttatttacagtactaacattcataatatatgggtaacctgactcttgttgtaaacggctaatttcttcttctaaatctcgtgcattcattaccttacttctgatatttgggttctgaatcatgttattgtattctgaatcaatgtctacaaatgagaatggtacaccgtattctttagcaacatcatatggagaaaataagtgaattacatccccagactcagctagctcataaaatttatcgggaacaactactcccaaagaaagtgttttgatttgctttgcggattctgcattttcttttctagttgataaaaagtccataatatccgcatggaaaacatttagatagactgcgcctgcaccttgtctttgtcctaactgatttgcgtaccggaaaccatcttctagcattttcataacagggacaaccccgctacctgctccctcaattcccttaatagggtctccaagagctcttaggtttgaaagatttaacaagtagtccatgctttaacatggctcagactatatcttaactaaatttgttacgtttagttctacgcgcttccaaaacaagaatttcacttgtaatgtactctactaggttactcgctaatatcctcccgacaatagctacccgttcgatagtcgttacacttttacaatttttctcctcgaaattttctacacaacttagctttatctccaagtttatcttttcttttaaagtagccggatacgttagctaatgaagtagataggtacctactagcctctgacatatctttaaactcaaaagattcgtttgtttcgatattggttatttttacaggaatagacgtagtatggcaaggttttctccctagtaccctaaaaccatgtttagtgttctctgatatagtacaccattcaaggttctccaaacggttgtcttgtttgtccccatttttatgattcactactggatagttgttagtgttaggtaagaaagtcatagcaaccactctgtggacaagtaggtacttcctaataccttccttgttatacatagctgttttgtagtaaccgtctttatcagtagacaacttgaagtatctgtccttttttctaattctgccgagggttgaaacctcgtaggcagggaaatcagggactgccttccagtattctttttccatataaccacctccttaaataaggagaaaaattgtacttagcacggtattgccatatctttcgacttaggttccaccgttagcctacataaagtagacaccctaggtttctaggttcacgtagtttatagtgagctatattctctaacccactccaccaccaagtttagatagttgaagtgcactgttcaacgttctaccaattgaagacattgaatcttctacttgaattagaaaacagctgacatactcccctcttctaagcctacctgcatttaaaaaagtaggggttgcaggttggtatctacggttaattagctcatctgcaatcttcatagcaagctcttcgtcaccatcacccattgtgagtgcattaaacgctactctatcttcataacgctctaggtatcgttccccatcatctgttttcattgcgtattgtttgtagaaacggtaagcccccataaatgtgtcgaatctgaactttttactatagatgaacttaaataatttttttataaattccattgagtacttgtcagtaatcactgttttatcgatgtacccttctctaataaggtaactaattttctcctctaaagagtagaaaaatactgtgttcttgtttacatgttctaaaaagaatgctctaacagcttctttatctttgtctaactgaatctttccgttattagggatattcaattggttattaagctcaatatatgtgttcatatctacaccccaagttctttttctagttttttaaccaaatcaggtctaacaccattaaatgagaaaccatcatcagcttctacatatggtaatgaagacactcctttttcttttagataagctaaagcttgctcatcatgagagatatttttctcatcaaatgggatattctttccatttaacatattttttaaaaataaacattgaccacacatatcttttgaatatactgttacttttgtcatttactacattctcctaacttttttatcgtatttattaattatacactattttgcattaattgtcaaaaataaagaaccaaaaaaactagagactacaaaagttaattgtagccccttttaataagttacaccttgtcacctaagaaatcttctgattcctgcgatttattcgtaaccttatcaagtagtaaaacagaatagtttttaccagtttcaacctgcaacctattaaacactttctgatattcttctggtgtgtctgtaacttctaataagtattttgcatttaaaaatgatagtaattcaagtagttctgccttactacctgccatttgaactacaacgttaccttcatcgttcgtgtatgttccaattttatttctagtagccaaacaaatcagtccttcgtaaatttaatgtatttgttaactgtatacacatttttaactttttcccaaacgttagggtatacgttcatcaataacttagtatctgcgctagcacgtttgtactctggcattaatttaaatgtgcccccatcaatactaattttagattcccctaactcttccatatcagaaatgatactactttttagctcatcaatctcttctttaatacttttttgcaattcatataatttcttgtaagagcgtaagtccttctctagtagctcctttttttgtaaatctgttgttttcatacatatctctccctctcttatttctataataagattatagcatgtcagatatgtaaagtcaacacttttttatacaaaaagaattgcccattataaaggcaattcttgtccgttgtcttcttcaaaaagaatctctacaggtatattatataatttagcaagttttactctgtttttaacacgaggttcttttataccgttttcccaataagagattgatgaccagtgaactcctatcatattggctaactctcgtagagattcacccctagcctctctcactcttttaaggactttaggttttggtaccttttcttccatgactatccctccttattcttaaaaaataagagcctatcaggtagacaggctcagcatcaggaactatgcgaaagccccgatataagttactttaccattacatttacgtgcaaaagcctctaactctttacgagcacctaaacggtcaggttgcgaagattgaacagtaatttctttaggtaccgttacttcacgtgtacgaatttcagttttaccattttttaatttcttctcatactcctctgtacgagttgttgtcgtagaaatgattccataaaattttttcatattaatagctccttactgttttttttaataaattataatagtggtaatagggttttatgagactcctactcattgtaagccttccttaatagatacttacaactatacgtttatagacctctctcaaaaagtctccgtaacgtcttaccttcatcatttaaaacgtacacagaatttacaaaagttttatacccttctttttcagttctgtactcgtaaggtgaatttggcacacgagtgatttcttcatgtttagagttaagtaatgaaaaagcattctcttgctctaaaagaaactgtaccccatcaattaattcaataaaaggcttaacaataggttcctctgtactgtctttacaatcgtattttcgttctcctaaaatttgtagtatcatgtctatctatctcctctgtttaagtattaatttgtgagtttccactcacaatgctgattgagagagtcgaactcccattcccgggttacaaaaccggagtaatagccattatactaaatcagcgtaacccctcaatagagggagtttcttatactaaattaccatatccgtaggtatttgttttagcttgtttaaacatgatactcttgatagctaagtcattgtacttttcatcgtcttcgtcatcaaggtacacatcaacattaacgttcttacctaaaatatcgattgtttcatctttacctacttgtaagtctttactgttaaatgatacatcaaaatagatgtcgtcttcttttgtacgactaccgaatgatactctatcttcaaataaatttaaacttcgagagttaattacaacaggttgtagcccaccttcaaattgaatagtaactgtataatactgattttcaatattaagaatgttcaaatcagcaatagcttcaccaaatgagatgccaaagcttaattccaacgcaattgctcgtaagcaatcatagtttaacttaattctacggctaaacttaacaacactgtcaatttccccatagtaagctttgtctaacttatcttgcaagtaagtacgaatttcgtctgcatcagggtagtcgaaacgtaaatggtaatggaaacgtcccggacgattaagcataaagtcgtttacacgatttaagttattaacagtaagtgcataaatacgcttgcgttgtgataacccatcgaataagctcaatagtttttcttgtgattcacgaccgtcacggtcattgaatactttttcaaattcatcgaacaagataagagactcttggtcaatactgtcaataaattctgcgatacccggataagcttctgtaattaagataacaggcataccctcttcaatagctcgttgagataagatttgagtaaatagtgatttaccaatccctttatccccacttaaaataacccctaaactacgattgattgttttaaatgtgtgtagtactttctcaattttaactaaacggtcaccataaactttagattctttcaatttaaaatcgtctgtaaccgccaatgagaacccagacattgggttgaatctaactttataagtttgcgcaggcaacttatcataagttttcaggtcgtttgcataaatctcataattactaccataattgattactttcatatattctctccttaatactttttaataaattataaatggagagtgatggagtcgcaccacccgagcctaagcaacagatttacagtctgctccgctactacttacggaataactctccttgaataaccaaccagataggtacctgacacacggacagcacctgtgtctctctgttactggatgattaattgtgtatttcgcatcacctaatatagttatcaaggtaggacttgactatactagatttagctaggttctaactataatttcctatgatagctcctactactaatcatatttatatacagttaaactacacataactaaaccgattaccttggttcgcatgttaagaggcgcaggcaaccaatggacattgcaggtctcgaacctgcgaccgttcggttatgagccgaatgctctgaccaactgagctaaacgtccgtagggtagtagcaacaattacaaatgctactctcctgatgattataaacttatcaaatcggaaagacaggacttgaacctgcgacatcagactcccaaagcctgcactctaccaagctgagctactttccgtgttacctgtttaatttggtcttttaaactactacacacaggtaaagataaaccctctgccaaggggagactatcatcgaaccgtatgtaagttgcgatgggtagtagccatattatattaggttattaggaagttcacctatgcagaaggtgggagtcgaacccacatgtccattacagaccgatgtttctaagacaccgttgtctaccagttccatcacttctgcggttgtactaccaaggttacctctaaaaggctaaactcgtgtctggtagggagccataccttacatggattgcaaggaacctaacctcagtagcaccttttactattaagggtttctgatttaacgttttccctagaccgtaccttaacagtaatactggtgagaggatttgaacccctcttacctacaagcctccgacaagcgctatgggaaacaagcggtgcattaaccataactatgctaaccagtacactactgttttacgcagtcctcatactaataattcatgtggactcaaccccattcagggaagtgttagtctattttttggtgagaactggttaactccatgtacgtcaaacattccctagactactcacttacattgttatttaatgtcacatgacttatgacagccgtactcaaaagtttcaaggacttttacctcactatccaccgacagtatgctcggcaacgtctttctaataataaattacccatcactgttacagtaacagaaccattgaattaacgagcaatatcagtattactaaaagtagtctgtctgtgtggtacaagcactagcagtattacaacctatagtatgtctgtttgtcaatcgttaaattcttttacaggagtacttgttaaacttagggaggtataacaagtatgtgcacataacccgagtgctactccctaaagtagcctatacgggttaacgtagatggagggaatcgaacccccaaccgtccgcttagaaggcggatgctctatccgattgagctacacctacaaattatgggggtaatgagcccccataataactcatagtagtttcatctatcgaggattaaaatgaatatctaacttgaataaagtataacactatttacatagcatgtcaacacttttattaaaataaatttctatacctcactaatgccaatgactatacgtaaggagagaacgttgatggcactggctacttagttggcgctaagttagtgaggtatagaaagagaactacattgaccgaatcgtattatacagccttagtagttgttaacaatgtttggaacttagtagcttactgcaataagctaccccgaagcatcggggtgggactgtggtaagccccaaacccttgggtatgctccatcctgcctccggagaagtcaggctcaattctcattagttaaaggtttactagttaacggttagctgattagtcatactacgtaaactactagtaaaatatagttttccaattaaggctaacaatcggtagaggatttgaacccctattattggttttggagaccaacgtgttaccagttacactaaccgactatgtaaagaaggaaagcgaagaccttctttacagtaattaaaaaaaacaaacaaaaaaaatacaatcatggaatcaaggtgggatgtaaggagatgccatgtgtccacttacagtggaataggtaactacagatttgcactgttttacatcttgtttaatggttacctgttaatagctaacttccagtgataagtcctcttatatggtagttcatgtagtatttgtttgacaatatggtagctagctaaaatgacgacagtaacgggactcgaacccgtgtgttccacgctgacaacgtgttgggacagcctctgccctatactgccattatttatgccgtagtttttttagaaaggaaagtttttttataatatacaacaacagttgaagcgctgatgttactacggcataaatatattttttatgagcttttaataactcaaaacttaatataatagggcttttactcctgcttcatgcacactcactgcattcggtcacacacccagagaggctgaactatcgggagctacccaatagcttctctctgcttttaatgtatggtctagcacggtggctaacaacgttcacctaaacattcagcattaaatagtattgttataagttcttcttatatcatatattttgtaagctgacttaggctacttgtaccaaggtctcttgttaaacccatatttctatggttctcgtcaaagggagtcttttgaggtttctaaggtctgccaagtttctcacgcttccacctaacttagattcttttccacaggaacgtctattatatcccccaagagtcttgtaccttacaatccatgtacactccacataacgcttaactgatactagcttttactagtagttactcttatgtcaccataagacatacctgctacctaaaacactatcgcactctaggctacattcagaatcacgccacgttatcctagcaagctgttcaaactttctgcactaggttctattatattaagttttcaattatcaaaagcagtttttctttactatttaataatagcacaacctctattattttgtcaactacttttttttagagagggtgcccctaattttatataggggcaagagatattaaacatagctgagctatgtaaaagctaatgtaggaattgaacctacttaatgtaagcaacaccagtttagcttataagcattgtttgcaaagtccatgctatgcactcagtaggaatcgaacctattgccgaaggtaccaaactaccctgagtgctcctatagatatattataccacataacgagatattaattttttttggtgatatagtatatctatattttttaaaattttagaaatacctttgatacattccggttatccaacgtatgaatatataatatcatgttattctgattgtgtcaataacttttttacattttttttataattgtgtaatgtcctatttctttttttctgattccttatatttataatatatactatatagtactatatatatatattaattactattagatattatatatagataataagaatctaggaaatttaaaataggacattctaatgctgactcagttacaataaacttatggtggctacctttttacaaaaatgtcctatttcattttttctatctccttatattattatttataatatatagtattaagtattatatattattatatatatagtatataatataagaaagacaaaaatttaaaataggacattttacttaaacaaaaaaaaagagagcagttaagccctcttatcttaatgagaaatagttattaattgttcccaatctgacttcctcatcttctggtgtttcatcctctggtttcgtatacaagctagtgattctttctggaacatctactacgttctcagtagctgtctgtatctggaatgcatttacataagttaactcagaatctctatcagctagtttatgaactggaatcattggcaactctgcacctttcattgcaccatttacaattgacattgcatcattagttgttacaccgagtcttctagggaacacagaatatgtcccagatgctaatgaaacctctacaactttctctcttttagggtaattcatgatacttctcctttcaaaatatgttataataatactatatactataataacacattttacaaattacttaaacatgctgaacacgtaagtgacaactgctcctaagacaatcataaaaacgttctctacaatatccctcttgtggtcgaactctttatcgtttactccttccagtgcatctatagtttcttccaacttagtaatctggtaggttaggtgtgcatatttttcttcgtgaacagcaagtcgcttatcaagactattgacaatatctctcaactcactaaccgcactattcagttctacattgtcctgtttaatgcccttctcggttagctctccatgttggagtttatcttccagtcgttgtagtcttaaaacaaggtcatttacttggtaatcgttcatatatgctcctccctgtaagttatgttgctctatattagtcagatgtaaaccacagacagactagtatacctataatagcgcctaccgtgtagactataggtatatagtacccattaaaaaacaagtatagactacctatactaattccatagagcacgaaagtgaacttgtatgatgccaaagggctcagttctgcttgtagtttcttatactgtagtgcacgagtgacatagtaggacatcaagtaaacaaacatttgtagtaacagtacacagaccagtgctgtttcatacattat